European Patent Specification EP 4 001 436 B1, published March 13, 2024. Title: Diagnostic gene marker panel for colorectal cancer. Applicant: Clinical Genomics Pty Ltd Commonwealth Scientific and Industrial Research Organisation. Application 13788103.3. The sequence listing filed with the application follows.

SEQUENCE LISTING (78 sequences)

SEQ ID NO: 1 - DNA, 102 bp, Homo sapiens
cagtgcccgaggcggcggcgagtacacgtggcgggctggattgcagaccggccctctcgcggcggagactcgcgacctagcggattgcatcagcaggaagac

SEQ ID NO: 2 - DNA, 87 bp, Homo sapiens
agatcccaagggtcgtagcccctggccgtgtggaccgggtctgcggctgcagagcgcggtcccggctgcagcaagacctggggcagt

SEQ ID NO: 3 - DNA, 95 bp, Homo sapiens
gacgacgcaccctctccgtgtcccgctctgcgcccttctgcgcgccccgctccctgtaccggagcagcgatccgggaggcggccgagaggtgcgc

SEQ ID NO: 4 - DNA, 92 bp, Homo sapiens
ccggagttgcggctgagacgcgcgccgcgcgagccgggggactcggcgacggggcggggacgggacgacgcaccctctccgtgtcccgctct

SEQ ID NO: 5 - DNA, 110 bp, Homo sapiens
cgcctgccctccgcgctcctgcgacggggtcgccacaagctggacgggatgagctaaccggactgtcggggccccaggagtggctgaggcggggccgtccaaggcaccca

SEQ ID NO: 6 - DNA, 299 bp, Homo sapiens
caggaagctgcagcagaaggaggaggcggcggccaccccggaccccgccgcccggactcccgactcggaagtcgcgcccgccgctccggtcccgaccccgggaccccctgccgcagccgccacccctgggcccccagcggacgagctgtacgcggcgctggaggactatcaccctgccgagctgtaccgcgcgctcgccgtgtccgggggcaccctgccccgccgaaaggtgcgtcccccgcccgccttcaggatctgctcagcccctctccgactccctacagggcctgctgactccg

SEQ ID NO: 7 - DNA, 258 bp, Homo sapiens
gacagagacagccccaggcaagttgaaggtccgagagcccccggtgggagaagcgggccggtggctgcgccgcgtgcgttctcactctgaggaagtgcgtggggagccgctgactccggatagcacacccttccgaggggactccccgattcctgggctgggggcctgccgcctggccccacgtctgacgtacggggcgcgagggccactgctccctggacttctgtcggaaccggacgcagtgggaggggtcgcagg

SEQ ID NO: 8 - DNA, 206 bp, Homo sapiens
atctgtaaaaatgttgacttctgcttttcagactacgcgcacagcctctttatttcctactgcggcttcattccctcacggaacactgacgccatcgcgaaggaagcatttcgagcacgactgacgctccccttattatttgctaagccgctgcgctcgggtctggctacgatttgctttcagaataacgggaaggtgcaacaaga

SEQ ID NO: 9 - DNA, 63 bp, Homo sapiens
gaaggaagcatttcgagcacgactgacgctccccttattatttgctaagccgctgcgctcggg

SEQ ID NO: 10 - DNA, 88 bp, Homo sapiens
cggaagtcgcgcccgccgctccggtcccgaccccgggaccccctgccgcagccgccacccctgggcccccagcggacgagctgtacgc

SEQ ID NO: 11 - DNA, 92 bp, Homo sapiens
gacgacgcaccctctccgtgtcccgctctgcgcccttctgcgcgccccgctccctgtaccggagcagcgatccgggaggcggccgagaggtg

SEQ ID NO: 12 - DNA, 95 bp, Homo sapiens
gtcttcctgctgatgcaatccgctaggtcgcgagtctccgccgcgagagggccggtctgcaatccagcccgccacgtgtactcgccgccgcctcg

SEQ ID NO: 13 - DNA, 110 bp, Homo sapiens
tgggtgccttggacggccccgcctcagccactcctggggccccgacagtccggttagctcatcccgtccagcttgtggcgaccccgtcgcaggagcgcggagggcaggcg

SEQ ID NO: 14 - DNA, 27 bp, Artificial Sequence
  CAHM FWD primer
gaaggaagtatttcgagtacgattgac

SEQ ID NO: 15 - DNA, 19 bp, Artificial Sequence
  CAHM REV primer
cccgaacgcaacgacttaa

SEQ ID NO: 16 - DNA, 17 bp, Artificial Sequence
  GRASP FWD primer
cggaagtcgcgttcgtc

SEQ ID NO: 17 - DNA, 20 bp, Artificial Sequence
  GRASP REV primer
gcgtacaactcgtccgctaa

SEQ ID NO: 18 - DNA, 20 bp, Artificial Sequence
  IRF4 FWD primer
tgggtgttttggacggtttc

SEQ ID NO: 19 - DNA, 15 bp, Artificial Sequence
  IRF4 REV primer
cgcctaccctccgcg

SEQ ID NO: 20 - DNA, 29 bp, Artificial Sequence
  BCAT1 FWD primer
gtttttttgttgatgtaattcgttaggtc

SEQ ID NO: 21 - DNA, 20 bp, Artificial Sequence
  BCAT1 REV primer
caatacccgaaacgacgacg

SEQ ID NO: 22 - DNA, 24 bp, Artificial Sequence
  IKZF1 FWD primer
gacgacgtatttttttcgtgtttc

SEQ ID NO: 23 - DNA, 16 bp, Artificial Sequence
  IKZF1 REV primer
gcgcacctctcgaccg

SEQ ID NO: 24 - DNA, 28 bp, Artificial Sequence
  GRASP probe
ttcgatttcgggattttttgtcgtagtc

SEQ ID NO: 25 - DNA, 26 bp, Artificial Sequence
  IRF4 probe
tcgtttagtttgtggcgatttcgtcg

SEQ ID NO: 26 - DNA, 21 bp, Artificial Sequence
  BCAT1 probe
ttcgtcgcgagagggtcggtt

SEQ ID NO: 27 - DNA, 102 bp, Artificial Sequence
  BCAT1 resulting bisulphite converted sequence
tagtgttcgaggcggcggcgagtatacgtggcgggttggattgtagatcggttttttcgcggcggagattcgcgatttagcggattgtattagtaggaagat

SEQ ID NO: 28 - DNA, 102 bp, Homo sapiens
gtcttcctgctgatgcaatccgctaggtcgcgagtctccgccgcgagagggccggtctgcaatccagcccgccacgtgtactcgccgccgcctcgggcactg

SEQ ID NO: 29 - DNA, 102 bp, Artificial Sequence
  BCAT1 resulting bisulphite converted sequence
gtttttttgttgatgtaattcgttaggtcgcgagttttcgtcgcgagagggtcggtttgtaatttagttcgttacgtgtattcgtcgtcgtttcgggtattg

SEQ ID NO: 30 - DNA, 26 bp, Artificial Sequence
  BCAT 1 oligonucleotide for measurement of methylation levels
tttttgttgatgtaattcgttaggtc

SEQ ID NO: 31 - DNA, 20 bp, Artificial Sequence
  BCAT1 oligonucleotide for measurement of methylation levels
attacaaaccgaccctctcg

SEQ ID NO: 32 - DNA, 19 bp, Artificial Sequence
  BCAT1 oligonucleotide for measurement of methylation levels
agatcccaagggtcgtagc

SEQ ID NO: 33 - DNA, 18 bp, Artificial Sequence
  BCAT1 oligonucleotide for measurement of methylation levels
actgccccaggtcttgct

SEQ ID NO: 34 - DNA, 87 bp, Homo sapiens
actgccccaggtcttgctgcagccgggaccgcgctctgcagccgcagacccggtccacacggccaggggctacgacccttgggatct

SEQ ID NO: 35 - DNA, 95 bp, Artificial Sequence
  IKZF1 resulting bisulphite converted sequence
gacgacgtatttttttcgtgtttcgttttgcgtttttttgcgcgtttcgttttttgtatcggagtagcgattcgggaggcggtcgagaggtgcgt

SEQ ID NO: 36 - DNA, 26 bp, Artificial Sequence
  IKZF1 oligonucleotide for measurement of methylation levels
tttgtatcggagtagcgattcgggag

SEQ ID NO: 37 - DNA, 95 bp, Homo sapiens
gcgcacctctcggccgcctcccggatcgctgctccggtacagggagcggggcgcgcagaagggcgcagagcgggacacggagagggtgcgtcgtc

SEQ ID NO: 38 - DNA, 95 bp, Artificial Sequence
  IKZF1 resulting bisulphite converted sequence
gcgtatttttcggtcgtttttcggatcgttgtttcggtatagggagcggggcgcgtagaagggcgtagagcgggatacggagagggtgcgtcgtt

SEQ ID NO: 39 - DNA, 17 bp, Artificial Sequence
  IKZF1 oligonucleotide for measurement of methylation levels
ggagttgcggctgagac

SEQ ID NO: 40 - DNA, 17 bp, Artificial Sequence
  IKZF1 oligonucleotide for measurement of methylation levels
agagcgggacacggaga

SEQ ID NO: 41 - DNA, 92 bp, Homo sapiens
agagcgggacacggagagggtgcgtcgtcccgtccccgccccgtcgccgagtcccccggctcgcgcggcgcgcgtctcagccgcaactccgg

SEQ ID NO: 42 - DNA, 110 bp, Artificial Sequence
  IRF4 resulting bisulphite converted sequence
cgtttgtttttcgcgtttttgcgacggggtcgttataagttggacgggatgagttaatcggattgtcggggttttaggagtggttgaggcggggtcgtttaaggtattta

SEQ ID NO: 43 - DNA, 17 bp, Artificial Sequence
  IRF4 oligonucleotide for measurement of methylation levels
gtttttgcgacggggtc

SEQ ID NO: 44 - DNA, 18 bp, Artificial Sequence
  IRF4 oligonucleotide for measurement of methylation levels
taaaaccccgacaatccg

SEQ ID NO: 45 - DNA, 110 bp, Homo sapiens; identical to SEQ ID NO: 13

SEQ ID NO: 46 - DNA, 110 bp, Artificial Sequence
  IRF4 resulting bisulphite converted sequence
tgggtgttttggacggtttcgttttagttatttttggggtttcgatagttcggttagtttatttcgtttagtttgtggcgatttcgtcgtaggagcgcggagggtaggcg

SEQ ID NO: 47 - DNA, 27 bp, Artificial Sequence
  IRF4 oligonucleotide for measurement of methylation levels
tagttatttttggggtttcgatagttc

SEQ ID NO: 48 - DNA, 299 bp, Artificial Sequence
  GRASP resulting bisulphite converted sequence
taggaagttgtagtagaaggaggaggcggcggttatttcggatttcgtcgttcggattttcgattcggaagtcgcgttcgtcgtttcggtttcgatttcgggattttttgtcgtagtcgttatttttgggtttttagcggacgagttgtacgcggcgttggaggattattattttgtcgagttgtatcgcgcgttcgtcgtgttcgggggtattttgtttcgtcgaaaggtgcgtttttcgttcgtttttaggatttgtttagttttttttcgattttttatagggtttgttgatttcg

SEQ ID NO: 49 - DNA, 20 bp, Artificial Sequence
  GRASP oligonucleotide for measurement of methylation levels
cggattttcgattcggaagt

SEQ ID NO: 50 - DNA, 298 bp, Homo sapiens
cggagtcagcaggccctgtagggagtcggagaggggctgagcagatcctgaaggcgggcgggggacgcacctttcggcggggcagggtgcccccggacacggcgagcgcgcggtacagctcggcagggtgatagtcctccagcgccgcgtacagctcgtccgctgggggcccaggggtggcggctgcggcagggggtcccggggtcgggaccggagcggcgggcgcgactccgagtcgggagtccgggcggcggggtccggggtggccgccgcctcctccttctgctgcagcttcctg

SEQ ID NO: 51 - DNA, 298 bp, Artificial Sequence
  GRASP resulting bisulphite converted sequence
cggagttagtaggttttgtagggagtcggagaggggttgagtagattttgaaggcgggcgggggacgtatttttcggcggggtagggtgttttcggatacggcgagcgcgcggtatagttcggtagggtgatagttttttagcgtcgcgtatagttcgttcgttgggggtttaggggtggcggttgcggtagggggtttcggggtcgggatcggagcggcgggcgcgatttcgagtcgggagttcgggcggcggggttcggggtggtcgtcgttttttttttttgttgtagttttttg

SEQ ID NO: 52 - DNA, 20 bp, Artificial Sequence
  GRASP oligonucleotide for measurement of methylation levels
ggtagggtgttttcggatac

SEQ ID NO: 53 - DNA, 21 bp, Artificial Sequence
  GRASP oligonucleotide for measurement of methylation levels
aacgaacgaactatacgcgac

SEQ ID NO: 54 - DNA, 258 bp, Artificial Sequence
  GRASP resulting bisulphite converted sequence
gatagagatagttttaggtaagttgaaggttcgagagttttcggtgggagaagcgggtcggtggttgcgtcgcgtgcgtttttattttgaggaagtgcgtggggagtcgttgatttcggatagtatattttttcgaggggatttttcgatttttgggttgggggtttgtcgtttggttttacgtttgacgtacggggcgcgagggttattgttttttggatttttgtcggaatcggacgtagtgggaggggtcgtagg

SEQ ID NO: 55 - DNA, 258 bp, Homo sapiens
cctgcgacccctcccactgcgtccggttccgacagaagtccagggagcagtggccctcgcgccccgtacgtcagacgtggggccaggcggcaggcccccagcccaggaatcggggagtcccctcggaagggtgtgctatccggagtcagcggctccccacgcacttcctcagagtgagaacgcacgcggcgcagccaccggcccgcttctcccaccgggggctctcggaccttcaacttgcctggggctgtctctgtc

SEQ ID NO: 56 - DNA, 258 bp, Artificial Sequence
  GRASP resulting bisulphite converted sequence
tttgcgattttttttattgcgttcggtttcgatagaagtttagggagtagtggttttcgcgtttcgtacgttagacgtggggttaggcggtaggtttttagtttaggaatcggggagttttttcggaagggtgtgttattcggagttagcggttttttacgtatttttttagagtgagaacgtacgcggcgtagttatcggttcgttttttttatcgggggttttcggatttttaatttgtttggggttgtttttgtt

SEQ ID NO: 57 - DNA, 21 bp, Artificial Sequence
  GRASP oligonucleotide for measurement of methylation levels
cggagttagcggttttttacg

SEQ ID NO: 58 - DNA, 20 bp, Artificial Sequence
  GRASP oligonucleotide for measurement of methylation levels
cgataaaaaaaacgaaccga

SEQ ID NO: 59 - DNA, 20 bp, Artificial Sequence
  GRASP oligonucleotide for measurement of methylation levels
agagtgagaacgtacgcggc

SEQ ID NO: 60 - DNA, 20 bp, Artificial Sequence
  GRASP oligonucleotide for measurement of methylation levels
caagttgaaggtccgagagc

SEQ ID NO: 61 - DNA, 20 bp, Artificial Sequence
  GRASP oligonucleotide for measurement of methylation levels
cgcacttcctcagagtgaga

SEQ ID NO: 62 - DNA, 206 bp, Artificial Sequence
  CAHM resulting bisulphite converted sequence
atttgtaaaaatgttgatttttgttttttagattacgcgtatagtttttttattttttattgcggttttatttttttacggaatattgacgttatcgcgaaggaagtatttcgagtacgattgacgttttttttattatttgttaagtcgttgcgttcgggtttggttacgatttgtttttagaataacgggaaggtgtaataaga

SEQ ID NO: 63 - DNA, 28 bp, Artificial Sequence
  CAHM oligonucleotide for measurement of methylation levels
gcctctaaaaaaacgatcttattacacc

SEQ ID NO: 64 - DNA, 206 bp, Homo sapiens
tcttgttgcaccttcccgttattctgaaagcaaatcgtagccagacccgagcgcagcggcttagcaaataataaggggagcgtcagtcgtgctcgaaatgcttccttcgcgatggcgtcagtgttccgtgagggaatgaagccgcagtaggaaataaagaggctgtgcgcgtagtctgaaaagcagaagtcaacatttttacagat

SEQ ID NO: 65 - DNA, 206 bp, Artificial Sequence
  CAHM resulting bisulphite converted sequence
ttttgttgtattttttcgttattttgaaagtaaatcgtagttagattcgagcgtagcggtttagtaaataataaggggagcgttagtcgtgttcgaaatgtttttttcgcgatggcgttagtgtttcgtgagggaatgaagtcgtagtaggaaataaagaggttgtgcgcgtagtttgaaaagtagaagttaatatttttatagat

SEQ ID NO: 66 - DNA, 18 bp, Artificial Sequence
  CAHM oligonucleotide for measurement of methylation levels
gaaacactaacgccatcg

SEQ ID NO: 67 - DNA, 21 bp, Artificial Sequence
  CAHM oligonucleotide for measurement of methylation levels
cgtagttagattcgagcgtag

SEQ ID NO: 68 - DNA, 25 bp, Artificial Sequence
  CAHM oligonucleotide for measurement of methylation levels
aggggagcgttagtcgtgttcgaaa

SEQ ID NO: 69 - DNA, 285 bp, Homo sapiens
cacggtcggagggctggtgggctttccttggccgtcgggcccgccacggcgcgggtcttggctgcggggcggaggtggggcgggagagccgaggataagagtttgaggcttttcgaggcgcgtgccgcggcgtccgcctctgcgggactctgcgccgggcgccctcggccggcgcgcccggctcccgctttgtcgccgagggaagcacgcgcgacgcccctcccgtcgccgccgtggcttctttcggtgttcgtgatttgctgagaggctggaaagcagcacggc

SEQ ID NO: 70 - DNA, 285 bp, Artificial Sequence
  CAHM resulting bisulphite converted sequence
tggcatgatgaaaggttggagagttgtttagtgcttgtggctttttttggtgctgctgctgctttttttgcagcgcgcatgaagggagctgctgttttgcttttggcttgcgcggctggcttttgcgggctgcgttttagggcgtttttgcttgcggcgctgtgcgcggagctttttggagtttgagaataggagctgagagggcggggtggaggcggggcgttggttttgggcgcggcattgcttgggctgctggttttttttgggtggttgggaggctggcat

SEQ ID NO: 71 - DNA, 20 bp, Artificial Sequence
  CAHM oligonucleotide for measurement of methylation levels
gtttttttcggcgataaagc

SEQ ID NO: 72 - DNA, 20 bp, Artificial Sequence
  CAHM oligonucleotide for measurement of methylation levels
cgcctctacgaaactctacg

SEQ ID NO: 73 - DNA, 18 bp, Artificial Sequence
  CAHM oligonucleotide for measurement of methylation levels
cgtcggtcgagggcgttc

SEQ ID NO: 74 - DNA, 10924 bp, Homo sapiens
cccaccccccacagatgctgtctgtcaggagcaggcaacagacggtcctggggtccatctgtgctaatgcttcacaatagagtcccatgtttccccactgacaccccctcggcccctcagctgatggccacttggtggtgccaaggcgggaggtgggaggagggagaagaaggcactaagagagctacctcttagctcctggcagtcctcaatccaccccggccccccacccaacaagcatcctgccatctggacttgtgcaatcactgaggggcggaaaagcaccctcttccacccacacctcttgtaggggatgggggcctagaggactgggggtggggaggagaacacagagtcaaggagactagagaagaagactgagccaggcgcaagaactgagacaggcaggaggcagaaagtctttcctggcctcgcaggtggacgtggccattgcccctctgtgctccttatgccacgtgtctaacacagcacatgtgcaaggtaccactccctaccaggccaagagcctctgtaaccccagtgcccagccagtacctggcacacagcagggcttaaatgttggacaacatcacagagtggttagattgcaggctctggaaccaggctgcctggctttgaatctcagctctgccgctgagtgacttagggcaaattacttatcttctctgggcctcagtttcctcatctgtaagggaggataatggtgcttatttcgtagggttgttatgaagaccaagtgagttaatgcatgtatgtaaaaggacacacagaacaaacagtgtgcatagcacatgctaagtgctcaataaatgttaactgtgaaggcataacagatttgggaagactgggggaggagggaggggacagacaagggcaccgcattgccgcctctgcttcttggccgatgggtgttgggacatggagtccccagcctgtgctgctgacgccctgtggtggctagccgctctttagacaccagacgctgccttccacttcctcctctcacttcttattcgggcaccactgacgacagagacttcggctgggccattcccgcctctcctaccgcctggcagccatggtaacagcctgggggatggtccctaagatggggtcagagaacggctgagcatggccatccccccagccctgaactcccactcagcctgggctcatcccaacctcctgagtcaagtccacagtaagcgtctgtctcctgggaagggggatctgaccccggcatcaggagctgaggaaaggtgttgccagcagggatcactcaagccccttggaggggacaggccagaactaagcctactgctttcagggtttccacctcttcccttcttcctagacgtgcgaacagggggcagcctctttcagctcttctggggcagctgcgtcaagggaaaatcctgggccctctccctccctgggggcttctgcgcagtgagttcagggagtctcctccctcctccatcgggcctccacccctactcctgcgcagccccgctgccgctctccctgccctggagtctcctgcagccccttggatctccgtgactctccctacctccccgactccccaggcttcttacagtgacctcttaccgtgccccactccatgaatcgccagagctattcgtccctaaatttcaaaccttgcgcaatgtcccttcacagacccctccaggtatcacgcagccccgagccccgagccccgccccgggggcctcatcccgccccttcgcgtccgcggctcgttttcccccactgagcgcccagctcccgcagtttccccggccgtcgagcgccgtgggcggggctccagggcggcggcgcctcgcggggagggtcctccgtgctgggggcgaggccacccgaggcagctccccgcccgcccccaaccccgccccgctctcggagcctataaagggaggcgacccgcggcccgcccggctggcatcccccagccgccgccagccccgccgaggggagccagcgccgtctctgaggggcgtccggcgccggagccatgaccctccgccgactcaggaagctgcagcagaaggaggaggcggcggccaccccggaccccgccgcccggactcccgactcggaagtcgcgcccgccgctccggtcccgaccccgggaccccctgccgcagccgccacccctgggcccccagcggacgagctgtacgcggcgctggaggactatcaccctgccgagctgtaccgcgcgctcgccgtgtccgggggcaccctgccccgccgaaaggtgcgtcccccgcccgccttcaggatctgctcagcccctctccgactccctacagggcctgctgactccgcagtgccctctcctcggcgtccgcggagtcccccaccttcttccccggcccgctgggtgcctcgactccccgcgttccccgctgctgcgaaggccgtggccctcgcctgcacaccgcgcccaggctcggtggctcttaactccgcgccccatgcacgccccctctctccctccttgactcctcccagcaccccccttctcctacccgctccatctggctttctgccccccatgccccgcctccccgtggccaggtgtcctgggtccccaggagcccctcgcccgagggacagagacagccccaggcaagttgaaggtccgagagcccccggtgggagaagcgggccggtggctgcgccgcgtgcgttctcactctgaggaagtgcgtggggagccgctgactccggatagcacacccttccgaggggactccccgattcctgggctgggggcctgccgcctggccccacgtctgacgtacggggcgcgagggccactgctccctggacttctgtcggaaccggacgcagtgggaggggtcgcagggcgcccgcggggcaggaaggatgcgggccgcgcccacctctgagtcccctctgccagcctcttcctctggccccaggagacctgaggctcagaacctacacaacaccaggttaagaagaggggcctggtggcctttcctcacccagccgccctccttcgccccggcccccagctagcccccacacaatgaacagcttgttgagaatttgcattttatgaaaatcatgttgaaagacaaaggggtctctctgtgctgcccagtccttcctccctggccgtttgggaactgtccccacccctgaggccaatctggttctgaaccttctcttccttgccttgggcagctttgggggagggttagcaaaggcacagaacagaaaggccctgggctgtgcaggctccaaagaaaagggctgctctgggactggacctcctcccaggaccaaaaagttagggagggtgagagactactttagtttatcaaggaccctgaagagacaggaaccttcatctctcatccttcctccacaccccccaccaccacccctaaagaactcccagtctcggtcctttagtgagacttgctgacaagtttgacatctaagatgttttgtcccagaaagcacaaaatatatggcaatggagagagagacccaggtatagctgggcacagctggtcacctgcagctgggatccacaactggtccttgaaacggcctgtaccttaggagacctggcacctctgaccccacattctggctgggattgccagcccttcgggacagggtccctgaccccagccctcccaagccactgtctgtagctgagaaattagatggagagacccaactggcagaaggtcctcggagcaccttgataggtgagcccaggggacacctatcctctgaatcccactggggaagagcccctgcctcagctttgggagtctggatggcctgagcctctacagacatgggccctaggggtggagaccattttagaataatgatctccccacctgctgccagtgtggaaaccagcaagggcttagaggttcatggatctggaacccaggaggatggttgtgtccctgcagtcccaggtatgaaggtaaggcctgtagagaaagttgaggagtggtgccagtagtggcacttggcaaatagttccaccagcaccaaaacaggtgtggatgtggagctgggaaggggcagacaggaagtgggtcgctgtgtccagggtaacctctcagtgtctgctcaaggacagtcccgccttacctgctccttctgaccatcttactgcccagggctcaggattccgctggaagaatctcagccagagtcctgaacagcagcggtgagtcaccaacacccagcccctgccatggtccaaaggggtgaggtgctgggttggggggtgccaggacagcatctcagcctagcgagggtagtcattctcctagcctttaaacatggctcccccgctgggagtgagggcaggtgggggtgagggctgtgtgaagggggtggcagagaaaggaggtagggacttttgagtcattaggtgctcttcaacacacccccagtccctgccagttacccctccctggggagatctggatgaacggatgtgggagttgggagggggtgtaggcaaagtctatggggaacgtcctaacccaggcctcctgggctcccctgagccctcctagccttggcaaaccccacgggcccagaccttagccaggctgtgtccagctgcttggggctggctgcccctgcctccagaatgtcagtcctcttctggtcccagcctgtggcagccctcttaggagggatctgagcgtgggcagaagtaggtgctgactccaggccctgggaccccacagtttcccttctctactcatgtcccatccctgatttgggcttgactttctctaaaatggatcagcaaactgacctgctagccagattggcctgtttggcccttgagctaataatttttaaagagttgtaaaaataaaaacaaataacaatatatgacagagatcataaggggcctgcaaagaaagcctaaagtatttaccatttggccctttgcagaaaaagtttgctgacccttccaaaaaaccctagaacattggggtagacgcggaactcccagccaccctgctccctgccccaatagtacagagaggggaaaggcctgctgttcagagtgagaggggctcgagctggagtggggaggtgctgctcagcatttgggggaatctctgggtcaggctggaagcggagaagcctggtctccagggcctttccgaggctgagctacttgaaggggcctttggaggctgctttaactgtgcctctggctgggcgggaaggaagggggtgggagtgggcagaggaaactctgggctcccccagcaggcgaggatctggagcagctccagaccattgtgtccagcgggcaggccttcagtgcgggaaggggcggcctcgaggctcccctcccccagcccccacatctggtgggctggccccagcatagctgggaggagcagctgtggtcttgctgagcctcgtgactggcctctgggggtggggccagtcctctctccaaagctgtggaacagaggaggctccaggctgtggctgaatttcgggccttagctagtcagtaagtggtactgtagggctcactggaaagctgggatggggctaaaaaactcagccggctcatccttcaggggaccggcccttctctgtgcttccctcccaccactagaggctggattggttctctgtggctccatgaggctgatttcaattgggtatgggaaagacattccaataatctgtgatgagactgagctgtcactggagacagagtcctgctggaatgttctagaccagttgccaatatccagggaggcccaagctatgggacttctacaccttttaatcctaattgtcttgacccctgtgtctcttgcaggaaagtgctgacgttggagaaggaggataaccagaccttcggctttgagatccaggtgggagaagctgcacacaggggtcaggggggttggatgaccagcctgagggatgaacggacttgtcccaaccctgggctgagggtccccttgtccattacagacttatggccttcaccaccgggaggagcagcgtgtggaaatggtgacctttgtctgccgagttcatgagtctagccctgcccagctggctgggctcacaccaggtggggcctgagcccaggacacccaggtctgggaaggggatatgaccttactcccaagcaaagggggtgagcaatctctcctgaaatcaattcctcttccttttccttctttgagaaggccagaaagaagaatggatagaatctgggctttggatctaggcaaatttgccatgtactgtgtgatcttgcacagccccatctacaaaatgagggtaataatgcatccaaacatcacagtgcggcaaggggattccctgggcacactgccagggcctaattaatggtggatgatgctgctgctgctctgattcctcccagcaaccctggcagtcagcatgggcaggagccagggaagaagcaacattccattaagtctgtttgatattggggatcaggccaatcctgccccaaaatgggcccagtgctgaggaaccgatgttactcccttttaaaaaattagaaactttttttttttttaagagacagggcctcagtctgtcacccaggctagagtgcagtggcgtaatcataactcactataaccttgaactcctgggctcaagcgatcctcctcttgcctctgcctcccaaagcaatatgttacttcctctaacaaggaaattatgcttcagcaggagatccctggattgagcagatctagagtccccaggttccaggaagggcagcctgaaactgtatgaatcaatcccccctccaccatctttgcccctaagcccctacctccttcccacttaccagcagcccgtgctagctatcttagtccattttctgttaccataacagaatacctgatactgggtaattataaagaaaagaggtttatttagctcatggttctggaggctgggaagttcaagactgggtggccgcatcaggtgagggcctcatgctgcgttctgacatgatggatggcatctcatggcaggaacgcctgcaagagtggtgagtaggcacacgcaaaagagacaaaacatgggtgatcttgctttatagcaacccactcgccaggtaactaaaccagtcctaccagagcaagaactcactccccaaaaacagcatggatcccttcactgggcagatccttcatggcccaaatgccactttttttgagatggagtttcgctcttgttgcccaggctggagtgcaatggcatgatctcagctcactgcagcctctgcctcccagattcaagcaattctcctgcctcagcctcccgagtagctgggattacaggcactggccaccaagcccagctcatttttgtatttttagtagagatggggttttgccttgttggccaggctggtctcgaactcctgacctcaggtgatccacccgcctcggcctcccaaagtgctgggattacaggtgtgagccacggcgctcggccccaaatgcctcttaaaggtcctaccatctctcagcactgttacgttggggatgaagcctcaacatgagttttggggacaaacaatatttaaatggtagcagtagccaagtggtatactacaacttctcaaagtagtttcaaatccactctccctccccatcatccctgaagcatccacagcagggatccatacccctttttacagataggaatggggccctgacatggggcacactgtgcttgaggtcaggaagctctccagtggtgcagggtagcagaactatccctctgggggccagtcattccctgtgcttctctcccaccaccagaggctggactgattatctgtggatccatgaggccatgccatgcctggggccagggtcggttcccagctgggtgctgctcacctgctcttccctgaattgactgggtcttatggccagcgtggactggacagaaataaccaaatctgagggtagcccagggtcctgggtgggcttagctttgggacagaacttcttttttttttttttttttttgagacggagtctcgctctgtcgcccaggctggagtgcagtggcgcgatctcggctcactgcaagctccgcctcccgggttcacgccattctcctgcctcagcctcccgagtagctgggactacaggcgcctgctaccacgcccggctaattttttgtatttttagtagagacggggtttcaccgtgttagccaggatggtctcgatctcctgacctcgtgatccgcccgcctcggcctcccaaagtgctgggattacaggcgtgagccaccgcgcccggccggacagaacttcttgagggcagagtgagggtgttgggtgtgtgaggtccccaccctttggctggggtgctgggcgtggacaacctggtagtcactacaggcccacaagaatggctgtggttctgtgtgtttggatcgagtatgagagatgtcagaggagatctacagagaaccatgaggagttggaggagggagttcaggagtattccctggagttactacccacccttctcccctttctggctaaggtaggaggctggtattctagcatgccccatggagcaaatctaacccccttgtctgcctggcaggggacaccatcgccagcgtcaatggcctgaatgtggaaggcatccggcatcgagagattgtggacatcattaaggcgtcaggcaatgttctcaggtatgtctgggagccgaggtgcctgaattcctgagctcagcctcttggtatttcctcagcctgtggctcactcaggctttgattctccaacctcagactggaaactctatatgggacatcaattcggaaggcagaactggaggctcgtctgcagtacctgaaggtaggggaacctagataacgtccagcctccaccctcctcttcccaagcctctgccctgtggggggtcacttacagctgaatctcctgtaactgaagatttcttttgtctactccctgatccctcgtctgtacccacgtcctgctagtttcctgctagcttgtgacagtggggtggggactgtctcttgcagcaaaccctgtatgagaagtggggagagtacaggtccctaatggtgcaggagcagcggctggtgcatggtgagtagatcccggggtgtgaggggccacttgttctgctacagacaccccatctgcgcttccccctcagaactggcgggttctagtaaagaacggtttactagtaaacctccacagtaaagcaaggtttgttgagctactactactttgggtactgccgcagccacatttctggttattctcacactagccctctgcaggtaagtaacagatagtgtcatcttcactttacagaggggaacaccagggctcaaagagtttgtgtcaattatttccgaggcccgtttgtgctaagcggcccccataaggatctgagtgataattcctgatttgcgggtgagggaagtagggtctcaggtttgtgcctggccagggccacagagatggtcagcaggacggagcggggacgccccgcccatgccctccgaccctttgcagaggccaccacggtccaggcctgacccgccccctacctctcccgtctctgcgcaggcctggtggtgaaggaccccagcatctacgacacgctggagtcggtgcgctcctgcctctacggcgcgggcctgctcccgggctcgctgcccttcgggcctctgctcgccgtgcccgggcgtccccgcggaggcgcccgacgggccaggggcgacgccgacgacgccgtctaccacacgtgcttcttcggggactccgagccgccggcgctgccgcccccgccgcccccggcccgcgccttcggcccgggccccgccgagacccctgccgtggggccgggccctgggccgcgggccgcgctgagccgcagcgccagtgtgcggtgcgcgggccctggcgggggcggaggcgggggcgcgccgggcgcgctctggactgaggctcgcgagcaggccctatgcggccccggcctgcgcaaaaccaagtaccgcagcttccgccggcggctgctcaagttcatccccggactcaaccgctccctggaggaggaggagagccagctgtaggggcgggggcgggcagggaggtatttatttatttattcgcaacagccagcgctaaaagagggggaggccgagccaagaggaccccaggagcccagagcagcgggagagggtccttcctagcctcggcccgccgggtcggttcctggctggtgtctgctgagggagtggggggcccagccccttctcttctcccccgccaaaccacagtgggagctggggcagggggagagccaggcaatcgggggccaaagatgggggtgctcgcctacagtctgcatctgtagtgccttgtggggtatccaggaacaccctcccagcaggggatgggaaccctgtcccatgaagccctctcctcagctttacttgctcccccgcccttagccttggggagaaatggcccgtggtgggctgaccccccaccctccacacacacagttccatgacccagcgggcccccaggggcatcaggtgctggtcctcctccctcctggcctcgacccctaagggcttcgcccctcccaggggcctgtaactaagtcgggtcctgccaggcagggggcctgtgttctgtgccccttgggagacaggaactggcgagttcaggtggggtggggacagcacagactgttccaccgttgtgcatattgttgcttctgaaccacaaactgtataaatggatggttttttg

SEQ ID NO: 75 - DNA, 2886 bp, Homo sapiens
agcataatttcggtctcctacggaatttctttaaactaacgagccccacactgacttccacttagtattgaacagctgcaccaactccccaaccacgaaaccccgctttagtcctcacgggaggggagagctcccgaacgcggggcggtgggggtccgcgcagagcaggctcgggaggccgagcggaggagcggggcccgcgccgggcacacgcgtcctccaggccggcggcgcggcgtgggcctgctctcgggagggctcggcgaggaccaccgagtccgcgcagcccccgccgacctctcggaaatgtgaccgccgaagctagaggggccgcagggctcaccccgcagccctccgcaacgcgccaacttggacgccagcggcgcggggtcccggccgggcagggggcgtccggcaccggcgggtccaccccggcccgcccgcccgccgcaagcccggcccggcacctcctttgtgcgccctcctggcctcccagtccccccggcgctcggtcccgcccggccgtgaccttcccgccctccccaccatcccaagcggggaaaggggccgccccggcgggggtcgggccggggccggggccctggagacgctcaccttcgtccagcagccgctcgaggtggttgaagatcccgcagaagttgggcaggctgctcatgagcttcttgtcgttcatcagctgcatcaggtaatctggggtgggcttcggcttctccttcgtttccatttccccgaccatattccaggctccgcagctcactccgcccgccgccgccgccgccgccgccggagaggagggaggggcgggggcgagccccggccgcgggccgctcgggacccggcgtcccgctccgcgccggctcccgctctggctcccgcgccgagccccggggcggccggcaccgcgcgctcgcccgccccccgcaggcactttccgcccgggcccgacgcgctcccagccgccgccgctctcggccgcccggctcggcgcgtccctcacgaggccggcgggcgggcgggaggcgggtctcggctggccgagtgcgggcgcggggcgcgggctgctggcgccggacgaggaggagccggggccgccgctcgctcggctggtcgagcccgctcagcgccgccgccgcctgtgccgcgggctcggggggtctctctgggctggtccccgccgcggcgcctctgccgctgccgccgcgctccgactgcgctcctcctcttcctcctcctccttctcctcctcctcctcctcactcacttggcggcggagttcgcctcagttcaggcggcgctgccagcggcggcggcagcagcggcggcggcggggggaggggcagcggcgcggggagggccgggggcgggcggcgggcggggccgcgcagggcggccgttagcgggtcccggccggcgcgctcccgctgcctgctgcccgccgccccgcgaccggggcagccgccggcgccgcgccccctcctccctgcctccccggcggggcgggcgacgggggcaacgggagtgtgacggactgcggcgctcggcgggcctgggcgcaaggactgggtcgccgccgtgcggggcgcccggggcgggtgggtgtgggctgcggggccgacggccgcggggggggcgcggggctttccacggcacggggcgggtggggctgcgggcgcggtcggggctggcgcggcaggcgagaggaattccagcgggacgcgccagcgctgcctccgcctcgcctcccgttactatagttttttcagaacctcttatccaccccgcagaagagaaatttttttttaacgtcctgttgcttcacgggggactttcggggtgggcatcacgtggcccgacacgtagccgtggggctccagagcgcgtgcgcgcgtcgagcccggtcgccacgccccttccgagggtcgctccgcccccgtcgggccccgcgagcgcgcggtgggggaggggagggccccggagcgcgcctgcgtggggcgggggcggcagccgactaggggctgggtctggccgtttagggccgggtcttggcccgtcgcccacggtgcggagggctggtgggctttccttggccgtcgggcccgccacggcgcgggtcttggctgcggggcggaggtggggcgggagagccgaggataagagtttgaggcttttcgaggcgcgtgccgcggcgtccgcctctgcgggactctgcgccgggcgccctcggccggcgcgcccggctcccgctttgtcgccgagggaagcacgcgcgacgcccctcccgtcgccgccgtggcttctttcggtgttcgtgatttgctgagaggctggaaagcagcacggcggagaggagccttgcactcgccaggcgggaagcctgcgcggacacgcgtgcgcacccacggggcggcgggcgggcgtggggggtccgggccacgcgggcgacgcgcctctagggaagcgatcttgttgcaccttcccgttattctgaaagcaaatcgtagccagacccgagcgcagcggcttagcaaataataaggggagcgtcagtcgtgctcgaaatgcttccttcgcgatggcgtcagtgttccgtgagggaatgaagccgcagtaggaaataaagaggctgtgcgcgtagtctgaaaagcagaagtcaacatttttacagatgaagaaagaatacggaggcaagaggtctttctctgcagtttggtggatttccaacatttagacttgtttggaagaatttcctcagctgcaccaatgaagtccttgatctatagaagtcggcagtccctaaatctacgtctgcattttgttgcaaatcctttataacattccattaaaataatgcagagttatttaata

SEQ ID NO: 76 - DNA, 21705 bp, Homo sapiens
agattagcaattacatttaaaaacaaggtagtggtgtgaaggctcagagtttcacacaacgactgttgttctgaactaaaagcagaggatgtggatgagtgaggggagggtatgttgaaaatgactaaacccggtgcagaggacacgtatacgaaagtgcaaaaagctctcatttgccattttttgtcctcagcaaactcctctctggtatgtttgtgaacgtttgagggaaaggtaacactgattaaaatataatgcaacaagaaggcaacgatctttgctttgttcactgatgtgttccaagtgcctaggacggttcctgacaagtagcaggtgctcaaaatacatttgtcaagtgaataaatctgtgaaaggaaaggaagaaaaacaggttgtgaccagaactttttgtgaacaaaaccctgttgtttattacatagactttggtaatggaaaacttacttgggtgaaataaaaaatggcatcctgttaatttctgagaacgtctgttggttttaggaaaagcatacctatccatacctcactacctgttttgctctagcctaaacatagattcttctttggttaggagacattgacccaatatataagattaaaacaaaaactgagaaataagtgaaatcaaaagcttttcaaaagttgcaggttgacctacggtggtggtggtctaaaatcatatagaaaccagagatctgatggtttacctgaaaatgcgaagtaaatgcacatactcagcatctcagacgatcgaaagctcaacgggtgaaagctcagggggttaattttgcgattaaggacatcttggaaaagtatgtaaaatccctggtccacttaagtattattcctattttgggcttttatttatttattttgagatggagtcttgctctgtcgcccacctcggctcactgcaacttcagcctcccgggttcaagcgattctcgtggctcgtcctctcaagtagctggggccacgcccggctaatttttgtatttttagtagagatggggtttcaccgtgttggccaggctggtctcgaactcctgacctcaggcgatccaccgcctcggcctcccaaagtgctgggattacaggcttgagccacagcgcctggcctattttgggcttttataccccactggtaaactgctttcctccaggttgaggttaaaacgacatcattttaaggtgaactgaagtctggaagtgattaagcacttggatccttagggagcctctccccgcccccatctctttcatgctaagataattaaaacttcggggccggggcattgtctgagtcacttcaattcaccagcctaatagatgcaaaaggatgtaagcatgtcagacacgcagagacagtatttgaatcaagcttaatagctcaagggagctgggccatttcctattttctttttagtgagtgcgatgttctctaaacaccgcggagaggcagggttcccggtgatggccttgccgagggtgctcccgcaacctccacctccagttctctttggaccattcctccgtcttccgttacacgctctgcaaagcgaagtccccttcgcaccagattcccgctactacacgccccccatttcccgccctggccacatcgctgcagtttagtgattgactggcctcctgaggtcctggcgcaaaggcgagattcgcatttcgcacctcgcccttcgcgggaaacggccccagtgacagtccccgaagcggcgcgcgcccggctggaggtgcgctctccgggcgcggcgcgcggagggtcgccaagggcgcgggaaccccaccccggccgcggcagcccccagccttcacgccggccctgaggctcgcccgcccggccggccccggctctcggcttgcaaagtccctctccccagtccaacccccggcccccacaggcctcggcgccccgccccgccccaggccccgccccagagagttctataaagttcctctttcccacctcgcactctcagtttcaccgctcgatcttgggacccaccgctgccctcagctccgagtccagggcgaggtaagggctggagtcgggcaggaggaggggtgtgaggctgataccagagaggacccggagcgcgaaccagaggttcgacctccagggcagcgcagggtaccccggcttcggagcgggaagggagcgcgccccgtcctggagctccgactcccaccccatctgcgctgagccggaggcgctggtttgggctccaaggcccgcctccttggctctgcccgagcctccccgcctgccctccgcgctcctgcgacggggtcgccacaagctggacgggatgagctaaccggactgtcggggccccaggagtggctgaggcggggccgtccaaggcacccacacaagacggcacaactgcctgcgagaaacaggcccggccctgtggaccccaatccgaggctccttcccctgctcttcgttcctaaggggcccaagctcacggcggcctccggcgcggtgctcacccgctggcgcaggaggaggaggagctccacatttgggtcgctccgagccttgcgtgcggtggcctagccggcctggcgcggtccctgcctcccaggctccgcagctgtcgtcgccctctcccgcgccctccccgcctccgctctcccgggcctgctccggggtccggcggacgctctgcgcgcggaatcccccgtactggggctgcagcccccgcgtctgcgccacttgtcgtttgcagagcccacttagtgcgcgctagctgggcagggataggggtcctattcggggcgaagggtctggatgcgagcagagaaagcggagggtggaggaacccggggctgcgcccctggaacgcccggccgcaggcgaggtcctccgcgcgtggaggccgccaggggagtggaaactgacagagtcgcggggaaggggcgagaagcgggttgggagtgagcgaaggcaagcgagagctgcgagtgagtgcggaaggagggccaggaggggtggcggctgggtggggagagagggtgcaagacgagcggcgcgtgtcgggagcctttgggctgcgggtgcgttacaggagagcaggcgggtaggagccttcgcgggggccgagctcggaaggcggacggctgtgcccgcccaggggatgcgcccgggccggccgcgaaggtgccttcttccgggggcccggacgaccctgacacggcacgcgcgcgcttcgcagcctcaaagactccggggcctcgtggtcactggcgcaggggatcggggcggggtgcccggagtgcggtgcctcgtggctgaagggcagctcttctccccgcagtgcagagcagagcgggcggaggaccccgggcgcgggcgcggacggcacgcggggcatgaacctggagggcggcggccgaggcggagagttcggcatgagcgcggtgagctgcggcaacgggaagctccgccagtggctgatcgaccagatcgacagcggcaagtaccccgggctggtgtgggagaacgaggagaagagcatcttccgcatcccctggaagcacgcgggcaagcaggactacaaccgcgaggaggacgccgcgctcttcaaggtctccggcctcgggagccggcgggggcgcgccggggagggcccagagacagagcccggggtccccggcgccgcctccgaggcgagcccaggggaccgcgcggggcggacgggcgggcggcggaggcatcaggtggcgtcgccggagccgcaggaggaggaaaggaggcctcggctctcagcgggaccgcgggggccgggagccgggtcctgggcgcgtggaggctgcagggaaaccgctgaaggcccggccgggcccggggaagggcggccaaaggcttgaggggttttgcgcgttcgtccgtgcgttctcgtttccacgcaagcctcccgcccttcctccgggctcccgtctgccgcctccgtccgtgggtccccctcgccctctccgtgcgtccgcgcctgtgccggcggctgttttcgtctctcaccgcgtctctgtttctcttttcgctgcttttctctctgagtctctctctctccatgtttttcctgaggtcagcctctcttctcgctcctgctagctctctgcgggtactcccacctctgtctttctctttgtgtgtctctgtctctctctttcccccatcgcagtggaactcagggcctctgtctagagctgtctcccttgccctttgcgcgagtgcacacacgtgtgtcgttgttacgattgttctcccctaaggcagtttacccagagaactacgtgtctgggcccagcccccacctgtgggcagagcaggggaaggggacttcctccgggaatttggtctcaatttgctctcagagtgcctcagctgtgctgccatccagatgtctcctgtgggtgacagctcacaccacagctgtccttagtcctaggcaagctcactcagacactgggtgggtagagccccctcaaggaacctccgcatctcactctaccggttataaatacccagaaaatgtgtcttcaacttggcagtgatagggtccaagatggaaaatcattttcctagagcatagctggggtctttcagtttacgttctgagcaacggtgtaaatctgaaggacctatgcgccattctttcttttagaaatacaatttcaagattccttataaaatatctgtattttgggtttagcatggtggctcacacctgtaatcccagcactttgggaagatgaggtggaaggatgcctatgcaacatagtgagaccctgcctctgcaaaaaataataattaaaaaaattagccaggcatggtggtgaacacctgtaggccgagggcccagctactctagaggctgagataggaggaccctagaactcaggagttcgatgctgcggtgagctatcatcgtgccactgtactctagcctgggcagcagagcaggactctgattccaaaaagaaagctaataaaccagacatgtattttgacttttcgttctcttcattctttcccaccaggcttgggcactgtttaaaggaaagttccgagaaggcatcgacaagccggaccctcccacctggaagacgcgcctgcggtgcgctttgaacaagagcaatgactttgaggaactggttgagcggagccagctggacatctcagacccgtacaaagtgtacaggattgttcctgagggagccaaaaaaggtaggggctctcctgaatttgggtcacctaacagaggcagccagatccttgaggcaccttaacttcattctgagcatcactttctagctttccttttgtattgcctgcctgcctgccttctgcctcacagtgaagcccagcctccttgcctgagttatgtgggtcacaagttgaaattcctgtggggttcagcataggagaattaatcacactgtatgcctcaatgtatatgggggggggtgcattgaatatgtgttttccagttagtctttcaaaaaaaaaaagaaaaaagaaaactggataacttgttaaaatttacttatctaatagtctttagtgagtgactattttgcagaaaaggagtaatgagaggaatatctcatcactatgcatggtaataaaactgtcaacttttaaagtgtaacatggtcagctgaggtgtttattaaaagtcagattcctggacccctcttttcaagattctgaccagtgtgtctggaagagagctcaggaatctgcatctggaacaaatccttcaggtgacctcacttgggaaacatctggctggcggggtcctttatgtcacaaggcacattcgcatgccatctgtcatgtatttctttacctgtcctgtacaactcagaccttgtagaaaaaaatcagtttaatagcatgaaaaaataacttcccaagggagttgctgaaaaataccttatttgtcaacaccgtgttatgcattctaagaattaaatgctcaggtatttttacaagatttgacatttagttaggtcagttcctgtttttacgttgtgccatttcccttttccccaaacatgtaggagccaagcagctcaccctggaggacccgcagatgtccatgagccacccctacaccatgacaacgccttacccttcgctcccagcccaggtatggtggagggcactgggctccctgagggcgaggctgtgtgggccagctgcccacatggccagagaaccacagcagcccagacagcagaacttgccatttgctatggctgctccaacagcccagaaaaaccccaggtcactgaacgaatgtctcactttccacacggtgctgccattggtgtggattttaagttggggagggtcgggcgtgtccgcctgttggaatatgcttctcaggtcttctgggaaacagatgttttgtggaagtggaagattttggaagtagtgccttatcatgtgaaaccacagggcagctgatctcttcaggctttcttgatgtgaatgacagctttgtttcatccactttggtgggtaaaagaaggcaaattcccctgtggtacttttggtgccaggtttagccatatgacgaagctttacataaaacagtacaagtatctccattgtcctttatgatcctccatgagtgttttcacttagtctgatgaagggttcactccagtcttttcggatgataaaatgcttcggctgtcagtctaataagggattccctgaggagtttggaggctgtaagagcaccccccgtctcaatgccagtgcttcttatctcagcctctcctgcactcctttacccccgtctcgatgccagtgcttcctatctcagcctctcctgcactcctttacccccgtctcgatgccagtgcttcctatctcagcctctcctgcactcctttacccccgtctcgatgccagtgcttcttatctcagcctctcctgcactcctttacccccgtctcaatgccagtgcttcctatctcagcctctcctgcactcctttaaccccgtctcgatgccagtgcttcttatctcagcctctcctgcactcctttacccccgtctcaatgccagtgcttcctatctcagcctctcctgcactcctttacccccgtctcaatgccagtgcttcctatctcagcctctcctgcactcctttacccccgtctcgatgccagtgcttcttatctcagcctctcctgcactcctttacccccgtctcgatgccagtgcttcctatctcagcctctcctgcactcctttacccccgtctcaatgccagtgcttcttatctcagcctctcctgcactcctttagcaggttcacaactacatgatgccacccctcgaccgaagctggagggactacgtcccggatcagccacacccggaaatcccgtaccaatgtcccatgacgtttggaccccgcggccaccactggcaaggcccagcttgtgaaaatggtaaggaggataccagtgcaggaaatagaagagctaattgctaatgtggccatgggccatggcgaatcctggtctgtcctgggcagcaccaaagctctttccccttcttagaggctgcgtgtgcagctcggggagaggggggttttctcactcctgtgggatggtggcatcccacagccaagtttactctcaggatccatgctaggcactgcccttcgtgggatcttatttaaacaccacagagatcactccaggcagtggaaaacagccccccactttttatatagagaggagattgtggaagctcataaataataagtagggatgctgggagattattgagctggtatatttctctcgaatagtggtgtgttcattgttgctattgttggaattagaggtgatactaaaaaaggaacggaaaaataccatggcaaacacataaaacgtctctacaggtgcctacctaccactgggtcccagaaagacttgctgattgtggattagatgtggtcccctgccctcgggagttccccagacatcaaaatgagctccctcagcagaagctctcattagctgggtgcagggagaatctagcaatgcggtaactcaggccttcaggacttttgagttagttacttaaatggaagtcctgagacaggtcaacacactgaaccctttggatgttttaggaatatttgttcctttgcaatttggcctttttttccccagtcatgttcaggttatccttggctgcaggtagtgaagaggtgtaccactctttaatgtttgtactgagtggcatgttcacaaaaaagctcagaattcagttgcattggcttttcaagagggatttgcagcaagggctggtttccaatatggtagtggaggaattggctaacataaaactagctcctgaaattcagacttgcgtttactgctctggctctatggaattagtaaccatgggaaagaggcaatgcttagaactgtgtaaagtgatggagtaggtagagacctgtcttgaagcatcggtaacagtaaatgaagcagcagcaagatcaggtgttctgtgccacattctttttccattcatgtttcatacaacattgtcttcaggaacatggttcagtgttctcccaacccacaagagacaagcaaaataaaaatggactaaataatttgctagtttttaattgggctctttggcacagactcaagtagacctgaactctcagctctgttgtgaacccgctttgtgaacaaggacaaagcatgtcatctgtctctgagcctcagtctccctgttagtcagttacagagagagcgctccaagtttccttccaaagctgtgcactggctcgtttctccatcagctttggttttccagttggtctccagctcatctttgcctcacaagagcgtgccctgctagttgctggtgctgggagtgggtgggaaggtgattgggcgccagccccttccttcccaggcttcacacacacaccccaggaagccccgcggtgcgtcggactctctgtctagacatcatctgatttttatttgcaaatgcaggttgccaggtgacaggaaccttttatgcttgtgccccacctgagtcccaggctcccggagtccccacagagccaagcataaggtctgccgaagccttggcgttctcaggtgagtgcagggtttgctcctggaggcaccgcaggaggccagcctctgctgccagctctgtcatctttgggcagattcgatgggactttagacacttgctttgctccctctggggtctggagtagatgtagacacatcctgtgtgtgaggtgaccagggtgatttaggagcaccattagaaaacctgacatcactgcttgtggttctgctgaccgtttcagccactggcttgaatggagtcattttggcttcttcactggcacctctctgaatttctaggaatgtgcctttacctttaccgagggcccctcttcagccaacattctcacgatgtggaataattgcttggaagtgtagaagggcttctcattttgagaagctgatcatccttccaggttgagccacaaataagtcctcctcctctactccctggggacattagttctggtccctcatctctaaaacattgatgtgcctaagagtaatacacattttggtcttcctctgaactttaatatagcttgcaaacaaatatggattcaatctgatttttaaagttttatttctaaaaaaaaaaaaaaaatccctgcaccatggagatcttacctactataaagaaggcacctctaggcttggcaagcacacgtgctatatgtatatttatttttcagataatattttggattgtttttaaatgggatttgtttttatattaaaaccaaatagcttaaggtttggaattctcatcttgccctctggcatctttaaaaatcagtgatgaaaaatactaactaaattctgaaggtttcagggaggcgagagttgtggcacttttgctgctcagaggggagctggagtttgacctaccagctctttctagttgtgaatgaggcttgcacctttttttctgaggtgctcgtgagtaactgaggatgccctttgggaggaggtgcttctgagcaggaaggcttgtgtttgtttttagaaactttcaaacccttgtcttgaacacctaagacttgtgtgggtgcctgaagagtaggaaataaacagctatttatatctcggcaacctcgtgatttctgatgacattaaatgaaatgaaacctgccccgagaatcacctcgaatggccaacacccactctctttggggcgcactgtctgactcgctttcagacagtgtgttgaagcagagaattgagacagtgatgtgggttaagtctcaaaacctgctgttgaggaataagatagttttgtgggtttctttttttggtatgcatgatacagattaattatcagccatgagcacatttattagataactgtgattcccattgattttggggttccatacagttaccagtggcagctgcctcctgtctgtgccactcccctgcggtctggctgaggagcttgtgcaaacccagcttggttctttcaactcatgggcgatattttaaagaggcttctgaaatcagcaaaacgtttgtaaatggattcatcttgtttaaagtttcagagagcgcagttttagagttcttttcaaacttaaacacaaagcccagtgggaatttcagcagactttacatgaacttttagagtatttttctcattaatttctttcttttcacaagaattaattttgtgataaaaacaccacatatccagtgtggaaaactaatttaaaaatcagaaaaacaaaaatggaaaataaaaatatcacattctaccacccagaaatcaccattaaggcctcagtgcttaccctttaatgtgtgtatgtgagtgtgtttatatataaattatatagacataaataattaagcacctaattctatatataatttatatatgtacacacacacacacacacacacacatttgctttttacctaaatgatgtcatgttattattttggggacgtttcaggtatgtggaccgacttgcttctttctgaaacaccgttatattttttgctagtataaattaaacttagggttcatttcctccaaagtaaaaattgatttgcttaaagatgaattttcattcagtgacacatgacttaaatgacatcaccactatcatcatcataattcacaaataagacttagcaagttcttaatagtgatgctctataataggaattcaacttacatttccagaaaattaatgaaagatacacttgttccttaaaaaaagagtcggtggccacatacgtttgtaatatgctggtttagacagattaaatgggtttctttccacgggacttctccaagtgttgaccgagctcatgctgtctgtggatctctgggggagacaagggcacgctgtgtttcccaggcctccttgacgcgggaaccttttgttcccccacgggacatgtgggacactagagttccaccacaggtgcttggctctgtggagtcgttggcctcgaggtggtgtccttggcccccagcactgactccggagctctgtgtttgcagactgccggctgcacatctgcctgtactaccgggaaatcctcgtgaaggagctgaccacgtccagccccgagggctgccggatctcccatggacatacgtatgacgccagcaacctggaccaggtcctgttcccctacccagaggacaatggccagaggaaaaacattgagaagctgctgagccacctggagaggggcgtggtcctctggatggcccccgacgggctctatgcgaaaagactgtgccagagcaggatctactgggacgggcccctggcgctgtgcaacgaccggcccaacaaactggagagagaccagacctgcaagctctttgacacacagcagttcttgtcaggtaaggcacctcgttatctgttagaatggaggtggtgatggcctgcctgccacaggggtcagaaaccacagggtccctcccaccccaggctgaggtcttcctcctgttgacttcggcgcccactgggcttggggcttgactccagtagagatcttctgtctggctctgttgtgggcagagagtccggatcagatggtccaggtggaccatggctcaggctgttctcttgcaattctggttttcagcagtcgcctcttaaaacagttccatttcattgcactatgatctcgacaaatacgtctgctgatgtggcggctcttttcaggttcccagaaaaatcataaaggttggaagcatattgttaacattcttggttgtcaggtgtgtcaccctcatgcagatgctggcccacgagtgagacggagggtggagtggactgtactggttttgcacaggagaagttataggagagtgctataagttggctctgtgatatgaacatttctaagcatatttttcagaaccagtgagttttgtttttctaccttggatttcatgacaattcagcgaacctctggctggcttctgtgaagcccctcgccctgtcatgctgggcttcctcactggctttgtggggctgtccaggtggagggagcctcccgcgtgggagggagctgctctacccgccactcgccaccccaccgccaactcttcctctgccttttcccagtcctgtcccttcctgagccccttcagaaactcctgtgtctttgatttctcatgtgcctccccttttcttgaatgtgcttcttcattcaacttatttaaaataaaaatatgacacgtctgtgtgctctggcactgttgacatgtgctcgtacttctgggtgtaagtgacccaagtttttgtaagctcatccagattttcttttggtgcccaaagcaaatatgtccccagataactaagcttcaggccaggtgtggtggcccatgcctgtaatcccagcactttaggaggctgaggtgggcagatcacttgaggccaggagttcaagaccagcctggccaacatggcaaaaccccgtctctactaaagatacaaaaattagctgggcgtgatggtgggcgcctgtaatcccagctactcaggaggatgaggcacaagaatcgcttgaacctgtgggaggcggaggttgcagtgagctgagatcgcaccacggtgctgcagtttgcaggacagagcgagactccattgccccccgcaccacaaaaaaataactaagctcacacagaggctgaccataggaagagggagaactgtgctggttccccgaggcggcggcaagtgaggaagtcacctggggctggacacctctcattctaagggcagaaccatccccaagccctggccagggcggtcccatccttcttggggttgggcatggtgttcatgggggaccaaggaaattgaagggcaactggggggaccccccctcccctgtcagcatctcctgtgtctgccttgggatctggaagagctcacatgggccaggaaggctaaggcccactgggcctggatttctgaagactctggaccttggtgccagtggattcagaagataccacaaggtgagggctttctaatgaaagtgtcacaaggaactggcactggcttttctgagtgcctcttgctgggcgtttttagggaggtagagcccccgtggtgactaagctggaaggtgcacattgagtcacaggtgcactgcgtgagagacagcacaggcagggggtggacgcctgtgagtgtcctggggctgtagacttgcgcgactagaacttactattaatctgtgagcaagagctggtcttggctttcattccttcctctgtaaccaagggctgtgctctttgcccactgcagcctctcacctcaaagtgttcactgaggttcaaggaggatgctgtgaacgtaaaaactgcagctgtgccaaccagcttctgcataattaaggattcccaccaaacactctcatgttatctagggttggagccatgctttctcagagaattgtgccaactcgccattctgattagcctgtgtaggtgtagtctcagatcacggcagtgtgaatgtattttacagattctgactaagtcatttgggtttgatttgaattctggaaaaaaaaaaaagcaggaagtcaaatagtcctgtaagttagctagaaacttctgttcagttgaagagaacagtggagatctttgatatcttcctattcaggtctgcacagcactagggacagcccccagggcccggcccgagggtgtgtatctgataaggacgcgtctgttctgcagaagctgtagcggctcctgtgtcaactcgtttcttttgcgggcgtgacattttattgtagctacaggcagaagatttgtcttgtgtacaggggagggagcatgggctaaagtcaggggatgggcacttgtctttccaacaatgttccagtccgttttgtatcttttgggtaggtgtggtggcttcaggatgtacatgtgtatatccacaagcgggaggccaggggggctgccccactcctgttctcaagtcaagttactgttccatccctggagacaggcaagaagtctactcagagttacacagttcaggcatagtgacagtgggactcagctgccgatggctggtgctcagtcaccacgttgacgttacatattttctgtggtgcctgagttacgtggatgtccgcagtagcacagatactggattatgtgggctctgtagtgaggggatgaggttttaaaatgatcctgggatgtcgaaacattctgattttttaaatgaaaacttgtccatggcataaattggtcttttgccattgcgtgactacgtttcttgttctttatctcccgacttcactgtggtctactaccttttgaatcttcgtgggtccaatgctgcaaagcagtgttctttagctgtcgactagttcctcttgaagaatcgagggagaccgagggccctggggggaaagcacccaaaggaatgcatacatgctattttgtatctgagatgttcacatcaagagccccactcagcggagtaagagtgctcattcctcttgcagtgttcagaatcacagtaagctcttgcttcctgtttaacctggtgtgttcggtgatgagggtttctgaacatggtctctttcttgtgggcttctacagagctgcaagcgtttgctcaccacggccgctccctgccaagattccaggtgactctatgctttggagaggagtttccagaccctcagaggcaaagaaagctcatcacagctcacgtgagtcctcagttacactcctaccatagtggcttcctgttctttgtaaaggccagagtttcatttagaaaagtcccaaatgaaaagtaaatgtcaaatgacctggaaaaataagcgtaacccttaaactagtgagggaggaagcatggtccaacgagcagcacagtctgaggactcacgtgctcctcccagacttgagatctgctcatcaaagaaccagggaggacagcctcaaaggagggtgcctctttccccatcttttttatttttcaggaaagttgtcgtatttccattttatagggattgaaaaagattgatggttaaagttgccctttaaaattctccaggttaagattgctgtaagaatgctatctagctagtggatcttcattcaatggaaaagcttttcccaaatgagaaactatccattccctggaggcattttgtaggtctctgcagctgtgtcctagcacctcttttatttctggaattttagaaattatttaattattgggcatatgatatttgaaagaggctgaatctttcaaggaattcaagcaaatcagaccctctcgtaatgttctctagcatagctcaagatgggttcaactgtggcaagtaacactaaaagggtagggttaggattagggttagagttttcttttttatgagaaaaggtttccatagataacatgaagcattaatttgccatgggaaacagaatcttgaacccttaagacttttgaatttgaaaacttcacattgctacatacttgcaagcattattaacgggcttgcatgctgagcaataccaggtaaaagttacaccccctaacatcaaagttctcatcatgttctagctctgatgctatttctcattgagaactgaaatgaaacatggtttaatcttgaacatacaaccccccttcttgattttaaaaacaaagaccagccaaccaaccagtatataatcccatagactcaggagttttctcatgagttctctccagtgattgacttaataattgatatgattgttgaaataataactgatacattgttaacaacaggaattgctaaatgactaaataaacttggcattgataagcagcatttaagaagttgatgatcggccgggcacagtggctcacgcctgtaatcccggcactttgggaggctgaggcgggcagatcatgtggtcaggagttcgagaccagcctgaccaacatggtgaaaccccctctctactaaaaatacaaaaattagccgggcgtggtggtgcgcacctgtaatcccagctactcgggaggctgaagcaagggagtcacttgaacccaggagtcagagcttgcagtgagccgagattgcaccactgcactccagcctgggtgacagagtgagactctgtctcaaaaaaaaaacaaaaaaagaagttgatgatcagctcagctatcacatcaatccagttttaaagttgacatggatgcaagtcactgtcctctaagtcagggaaagatggatccccagatgaccccctcatgctgaagacgaggctgcgtggtccataaaatgaataaacacacgtgtacacctatgagttccacttttaaaaattattaatttaattcatttcaggtacttaggagtttagcttaagtcgtcatatataaaatacagtctctaatatcatgattgatggagagcattcagcttgccttagatgctgtaaattcaggaaaagctgaacattaaggcgtttttgttttttggtgagtgtgatccacgctaataaccagacagtataaatttgaggccagttagcttctctttttccacaatagtagttttgttgttgtttaactttactttttatttcttttacctctggttgagaactatacagattacctagaaatcaaatcattcaggatgagctccttgtttctttcaaactgcagttgtggaaaaacaaaatcattggcctaaattaccctgcagattccctcagacttccttttaatttgatcactttacttgatttgatgcagttttagttaaatgtacattttaagtggcagtcgatttgaaagtaacatctttaacccagaattaagtcactttggctgtttttttacatgttgatctatggaaggactaaccaaaaaattgcttctttagatggctccaaatatgaaatgttttgatgtgttctaggatgtaactttgggctttacgttactgtctccttagaatctgagtgctgtttaatagtgagccagttgcaggatatctcagtaatgtctttttaaaatctcttattaaaggtagaacctctgctagccagacaactatattattttgctcaacaaaacagtggacatttcctgaggggctacgatttaccagaacacatcagcaatccagaagattaccacagatctatccgccattcctctattcaagaatgaaaaatgtcaagatgagtggttttctttttcctttttttttttttttttttgatacggggatacggggtcttgctctgtctcccaggctggagtgcagtgacacaatctcagctcactgtgacctccgcctcctgggttcaagagactctcctgcctcagcctccctggtagctgggattacaggtgtgagccactgcacccacccaagacaagtgattttcattgtaaatatttgactttagtgaaagcgtccaattgactgccctcttactgttttgaggaattcagaagtggagatttcagttcagcggttgaggagaattgcggcgagacaagcatggaaaatcagtgacatctgattggcagatgagcttatttcaaaaggaagggtggctttgcatttcttgtgttctgtagactgccatcattgatgatcactgtgaaaattgaccaagtgatgtgtttacatttactgaaatgcgctctttaatttgttgtagattaggtcttgctggaagacagagaaaacttgcctttcagtattgacactgactagagtgatgactgcttgtaggtatgtctgtgccatttctcagggaagtaagatgtaaattgaagaagcctcacacgtaaaagaaatgtattaatgtatgtaggagctgcagttcttgtggaagacacttgctgagtgaaggaaatgaatctttgactgaagccgtgcctgtagccttggggaggcccatcccccacctgccagcggtttcctggtgtgggtccctctgccccgccctccttcccattggctttctctccttggcctttcctggaagccagttagtaaacttcctattttcttgagtcaaaaaacatgagcgctactcttggatgggacatttttgtctgtcctacaatctagtaatgtctaagtaatggttaagttttcttgtttctgcatctttttgaccctcattctttagagatgctaaaattcttcgcataaagaagaagaaattaaggaacataaatcttaatacttgaactgttgcccttctgtccaagtacttaactatctgttcccttcctctgtgccacgctcctctgtttgtttggctgtccagcgatcagccatggcgacactaaaggaggaggagccggggactcccaggctggagagcactgccaggacccaccactggaagcaggatggagctgactacggaactgcacactcagtgggctgtttctgcttatttcatctgttctatgcttcctcgtgccaattatagtttgacagggccttaaaattacttggctttttccaaatgcttctatttatagaatcccaaagacctccacttgcttaagtatacctatcacttacatttttgtggttttgagaaagtacagcagtagactggggcgtcacctccaggccgtttctcatactacaggatatttactattactcccaggatcagcagaagattgcgtagctctcaaatgtgtgttcctgcttttctaatggatattttaaattcattcaacaagcacctagtaagtgcctgctgtatccctacattacacagttcagcctttatcaagcttagtgagcagtgagcactgaaacattattttttaatgtttaaaaagtttctaatattaaagtcagaatattaatacaattaatattaatattaactacagaaaagacaaacagtagagaacagcaaaaaaataaaaaggatctccttttttcccagcccaaattctcctctctaaaagtgtccacaagaaggggtgtttattcttccaacacatttcacttttctgtaaatatacataaacttaaaaagaaaacctcatggagtcatcttgcacacactttcatgcagtgctctttgtagctaacagtgaagatttacctcgttctgctcagaggccttgctgtggagctccactgccatgtacccagtagggtttgacatttcattagccatgcaacatggatatgtattgggcagcagactgtgtttcgtgaactgcagtgatgtatacatcttatagatgcaaagtattttggggtatattatcctaagggaagataaagatgatattaagaactgctgtttcacggggcccttacctgtgaccctctttgctgaagaatatttaaccccacacagcacttcaaagaagctgtcttggaagtctgtctcaggagcaccctgtcttcttaattctccaagcggatgctccatttcaattgctttgtgacttcttcttctttgtttttttaaatattatgctgctttaacagtggagctgaattttctggaaaatgcttcttggctggggccactacctcctttcctatctttacatctatgtgtatgttgactttttaaaattctgagtgatccagggtatgacctagggaatgaactagctatgaaatactcagggttaggaatcctagcacttgtctcaggactctgaaaaggaacggcttcctcattccttgtcttgataaagtggaattggcaaactagaatttagtttgtactcagtggacagtgctgttgaagatttgaggacttgttaaagagcactgggtcatatggaaaaaatgtatgtgtctcccaggtgcatttcttggtttatgtcttgttcttgagattttgtatatttaggaaaacctcaagcagtaattaatatctcctggaacactatagagaaccaagtgaccgactcatttacaactgaaacctaggaagcccctgagtcctgagcgaaaacaggagagttagtcgccctacagaaaacccagctagactattgggtatgaactaaaaagagactgtgccatggtgagaaaaatgtaaaatcctacagtgaaatgagcagcccttacagtattgttaccaccaagggcaggtaggtattagtgtttgaaaaagctggtctttgagcgagggcataaatacagctagccccaggggtggaacaactctgggagtcttgggtactcgcacctcttggctttgttgatgctccgccaggaaggccacttgtgtgtgcgtgtcagttacttttttagtaacaattcagatccagtgtaaacttccgttcattgctctccagtcacatgcccccacttccccacaggtgaaagtttttctgaaagtgttgggattggttaaggtctttatttgtattacgtatctcccgaagtcctctgtggccagctgcatctgtctgaatggtgcgtgaaggctctcagaccttacacaccattttgtaagttatgttttacatgccccgtttttgagactgatctcgatgcaggtggatctccttgagatcctgatagcctgttacaggaatgaagtaaaggtcagtttttttttgtattgattttcacagctttgaggaacatgcataagaaatgtagctgaagtagaggggacgtgagagaagggccaggccggcaggccaaccctcctccaatggaaattcccgtgttgcttcaaactgagacagatgggacttaacaggcaatggggtccacttccccctcttcagcatcccccgtaccccactttctgctgaaagaactgccagcaggtaggaccccagaggcccccaaatgaaagcttgaatttcccctactggctctgcgttttgctgagatctgtaggaaaggatgcttcacaaactgaggtagataatgctatgctgtcgttggtatacatcatgaatttttatgtaaattgctctgcaaagcaaattgatatgtttgataaatttatgtttttaggtaaataaaaacttttaaaaatttgtta

SEQ ID NO: 77 - DNA, 139436 bp, Homo sapiens
agtagggaggtgggcaggagccagtgatgacggaatggcaatcacatttgacctctgatctgtttatttcctcctccttgacgtctccatataaatgttacacgggcatccccacactcggatacgcacccacagtggctgattcgggggtaaccgtgtcatttgcttgcaacactggcacctctgccctgcaccccgggagtgagcagtgagtgaggctcgggtctgggcgctggctccgaatcttcgggctgggagagactccaccatctgggggcggcctgggggagcagccttagtgtcttcctgctgatgcaatccgctaggtcgcgagtctccgccgcgagagggccggtctgcaatccagcccgccacgtgtactcgccgccgcctcgggcactgccccaggtcttgctgcagccgggaccgcgctctgcagccgcagacccggtccacacggccaggggctacgacccttgggatctgccctccgctcagctcgagcttccctcgtggccgacggaacaatgaaggtaactacttatggttttgtccgtgttttacaaaaatgtgtgcgtgaatcgaaccggcgatttctccaagaaacatagttggcagggaggggaggaaggcgagacaaccatggcttatatcccccgcaaacgtctcagtatcttctttatcaatcgtagtttgcggggaccgtgcattctgttcagatttcggtttaacctccactcgcaggacgtgccttctcggactttttcacattcgcttttgggaacggaggtgaaagtctgctacagctccctcccctgcttgtgaagtttggaaaggaagtgagggcttctctcagtttctcctatgcacaggaggtggggaattttggagaggaggtctggggatgtcccgggctgtaaatgcgctttcctgcagcgtgtgttcgtgatgcaggagggagcggctggaagagttgacccgggtggagaggggagggagaacgatcttttcactgttaaaagcagaaggcccctcttattttgtttcttgtggaaattaaagcttctaggagttacaaatgatagacgcctaagggcattcatttgttaaaccagtgagcaccctaatggctctgatcttgctaatcaaggataattagcctagctgcctattatttctgactatttaggtgtagggatgtacaccgttgagtgttttgttttcctagtttcacacactggaaaactgcaatcgcatataaaacccgaagagcaactttttccaaggaaagtgaaggatgggcagatattcttgccatctaacattttggaattgagatgaccataatgcaatctgaacttctggtaggaataaagcctcgtttcagagtttctaaggagggagatgaagcgtggttctcaactgctcttatctacaacccatcccagaccatagtttcacttagaagaaataatatgtaaatagcgcctttgttgccaaacaaaaactttcactacaattaaacagtaaccgagtggaaactatgcgtttttgtattcaacagagatcacacaacttttcttctatagttagaggttctatttctggcttcctcatgcttgtttcatttcagatgaaaaacacactttagttgattatagctttagtaagtaaaaggagaaaactaagaatgaacagtcttgcttttccagctttttcctgtccatgtgcagttgtggttaattacgcgtttttgtaggtccaaaaacccctgtcccttccacaagatacttttataacatggggaactaggtaagatatctacaagtagtctcttttctgtttcctgatatttcctaagattaagaaagaaatgattgtattctaggtatgatcgaagaagtatggaaggttccattaagttagttttatcacaatatttcaaacatctttccacttatctcttaaatatgtattgctatcacaagcttgattttttaaaaaaatgttatttgcacatggcatcttgattgcctttgtcctcagcaaattctccgggcttaagtcatgcatgagcttgtattttaagacagacacatgcagaatgggcaacttggataagaaacataggatatacactgagtagcatgtgtacaaaaatggtaagtgagtattatgacttaataaatttagatggggatttaaaaatgatacacatgtaaatgggattggaggcaagggaagtccgtgtgtgtgtgtgtgtgtgtgtgtgtgtgtgtgtgtgtgtgtgtggagggaagacgggaggcctagtggggagagaggttttacattccagacacaggatgtggcccctcaggctaggctcagagatgtaaagctagttaagctggcctaacaaaagggtggtggttagaaaaaggaaaaaaagaggtgggggttggggaggaaaagaatttaatgctggccaatattttcatctgataagtttcagtaatgagtaatttcactggatttcagaactacagagagaaaaggggaaaaatatttttccttttttacgcaagaatttctcttgcttttcagctcattagaaccagatctaattatttgaaatgagtttaaaaccttattatgaaaggaagttgaaaacattcgatcacaattgagttttgtactatggactaaaaccaagatgtgctttctgtcagtagctgtgcaactccctgaaaaaagaaaaatagcgcagagcgatctgagctttgtgaaggctacacaatttatcaggcccagagagataggagtgtgagacttcagtcacgtccccccgtacgcatgcgcaggagtaattatttaaagacattttgttcctgactaactgcctcactcattatgttcctggaatttgtgatacaaaaaaacaatgtttagcctatcaatagtttatatagtttatgttattttaatataaattcttctcaacttagaaactgcctcttttttcttttaaaaacccacttgtaactgctgtatatattcagggcaacttgatttggtgtttcgttggttgcagtcctcaaatttgacctcaatatactctctacttatataaattttgtctcagttttgtccgtaggctgacattccaattgttttcctaattatatattttgttccttatttctcatgtctagaaataaagctagggaagtaaacagctggaaaactgatagtggtgttattaacctaactgagagggctgggcttatgagtaaattattcctgtgcataaatgaaagattgtttctaaatggcagctatgttgagcctttgtattagttacatcttttggggtttcaggttgccagcttctttaaatggcctcttctcaactggtataggaagttggaaaataaagaactttctttatttccctttagtgttggtaaccacagtttctttaaataacagatgcccaccccagggaaacccagtggcatgatcagccttatgctcaggaaggtttggttgctatactggagagtgagaatctgggaccttccatgatagacataattgtgccagctatcctctactttctatatgatgctatcattcttttttcttttcttttttttgacagaatctcactgtgttgttcaggctggagtgccgcagagtgatctctactcactgcaacctctgcctcctaggttcaagcaattcttgtgcctcagcctcctgagaagctgggattaccaccatgcccagctaattttcgtatttttttgtaaagacggagttttgccatgttggccaggctggtctggaactcctggcctcaagcgatctgcccatctcggcctcccaaagtgctgggattacaggcatgtgctatcattctttttgagcacaggaggaaactatggctgatctgctcattttactgtcaaaaatataggcagcttttgtattgtaacattatccccttaacagctgtccaactggtctatacatttcacctaacatatggtaaatgttcctactgttggcctttcctgagcctctgtccattcaactaaggccactgcaatgggattgtatgcagttcagccaagaaataaatgtgaggtgcaactcacattttttaaatgtttcaaaattaagcatttaggtgcttttattcataaacatgactttgcaaatattggtaaacagtttcatcataagaccttgtcagtgactcacaatgtcaatggtgaacgcaaaggagaatctgtcttttctggaacaccaggttcaggtatcagtttcaactatgcttataatttgtgctctaaagtccacaaagctaaattatctttcccctaaaaattgagtactcatatccttaaaatagcttggaaattagattaccttatgaatacagcatagcatgtcacataaacgtttttctactgttatacctttttggtgggaaagactattttgcaaaacatttttcttgtgttcagtaattaatgggaaaaacaaactctaaaagaaagagacagttatgtcccaaaaatacaggaaaatggaagaatggaaacagggaagaccaataaagaaaaaaatagaggaaattacaagtaataaactgaagtcatactgaaaaacatatggctctttcttattgaaagttgtgaaatacttgcaaaactcagctagttccattaagaatagtctttaatctaaaaagaacaaattcatttgtcagttctttatttcggtgtgtagatttgaatgtttcatcaattgcatttacggtttatccctcagtgtgagaactgtttttgctgttttgactataaatggatatctgctttaggaagacttaggaagcctgggacataggattacagatcaaattctatttgactccatagaagttgagacggaaggagcacctgttgggatattctagaccaaacattccacagctgtctcttaacgtgactgacaaagagacacagttgagacgaagtttgggtatatcctgggatgaggccaagggtggatttgcacaggatggtcacagggcagttgttagcattccaccactacataaaagggtgattttgccaagtgcatttcatttcatttcagttgatttagataccaagttatattgttttgactttaggactagatgtgagttcaggaatttgaaatcataataaatgtttccttgaactttgaagataaaaggtagagttaaaagacagctgcgaagtctacatggggaagcataatacatgactcagggttccatggttttcagtgtcggtgagtgctctgtacacttataagaatagtgctggtgtttatagaagaaacacatgcaggtttgaggcaagacttccttgcttaattggtgcttttgctttccattttctaaatgccatgcaaactacttttttttttttcttttgttgagacggagtcttgctctgtcacccaggctggagtacagtggtgcgatctcggctcactgcaagctccgcctcctgggttcacgccattctcctgcctcagcttcctgagtagctgggactacaggcgcccgccaccacgcccggctaattttttgtattttttgtagagacggggtttcaccatgttagccaggaaggtcttgatctcctgacctcgtgatctgcccgcctcggccacccaaggtgctgggattacaggcgtgagccaccgctcccggcctcaaactactttaactgaaaacattcttctaaggaaagcatcagaaaacttactagaattgcttaagaataaataaataatacaaataaaagagcaaaatgagaaagtagacagactcctagtctattgtgctattgatctctccaggttctaggctttcttgggtctgacaccactttgtaaatttttttttttttttttttttttttccagatagggtctcattctgtcacctaggctggagtgcagtggtacaatcatggctcacttcagcttcaacctcctgggctcaagtgatcttcctgcctcagctccctgagtagctgggaccacaggcatgtgccaccacgcccggtgaatttttgtattttttgtagagatggggtttctccatgttgcactggctggtcttgaactcctgggctccagtgatccacccaccttggcctccaaagtgctgggattacaggcatccgtcactgcactgggccagtttgtaaatcttatgaaaagtatggccaatcttttgcaaaatgtgcaaacacatatagacacaaagttttatatctaaattattggttattaaagccaggacaatagagtgcatatagcatggaagacaggtagaaaagactgaaatggtttagttattcagagcagtggagggctattggctcttgcctttgcagtcagctgagatatgaaactatataagcagaagcttcacgctgccatttgaatattgaaaatctccacttttagttcaagagataaacaaccaatggtttgtttgttcacagcacataagttatcactttcttctctgtttcatcccatcaagatctaaggtgtatagttacagaatagaactcggttcataccatatgcaccctaatttcttcgatcttcaactagtttggaagtgtgtgtgggtgttttcttagccaaggttaatatgcaatttcttagtggagtgtaggagtttggggtgcctagccttcctacttcccacttagataacttcccctacctgttgtacctgtcaaaggagaaggccagtatggccatgttctttgcaggtgactccaccttagccacagctgattgtaacaagggtgtatatttggcccaagtccagccatcttttttttttttttttgaggcggagtcttgttctgtcacccacgctggagtgcagtggtgtgattttggctcactgcaacctctgcctcccgggttcaagcaattctcctgcctcagcctcctgagtagctgggattacagacacccacgaccacgcttggctttgtatttttgtatttttagtagagacggggtttctccatgttggccaggctggtctagaactcttgacctcaagtgatccgcccgccttggcctcccaaactactgggattacatgcccagccagccatcttttacttctttcttattctcttattccacatattcaagcaggtaccacgtcctgtggactctgtcttctctgaatctataggttctctctttcccattgccctgcatactggtttatgctctcattacttctcgcttgaattattccaaaagtctcccaactggtctgaagcttaattttcattatgtgctgttcgatgtcattccaccacgcaaaatctatggcttctccattgtctcctgagtttagtttagtgcatgagaccgtttaaaatctacctacacctcttctatgtgcatgcatttctctagtcataagagaggatttgatctatctcaaaatgtgttcttatatttgcatttactggtttttaactccctccatcctatctataatttgcaccatgttgctcaccatgcagcccactccccagacaccttgtgagaacagtgatcatgtttttgcagtggaatgaacatgggcgaaaggtgggaaggtatgcatagatttacattttgaagtcaggaaataagatactgatcaatgctttaattcgactgtgctttttaccttttcctctgttgtagcatgaaccttgccccaaaaagatattgatcatatgctgcaactcctctgcacttaccttttcttctaccatggcaggaaccttgcaccattgttggtgctttacagatattggttgagttaaatcgagagcctatttctggactttcaagattcagattaattgattctgttttatacttctctgtttttgaatggcacatacatctttccacacttggatttctttgaagttaaagctttaattgacttccaaaagacagaggattataaaaacacagagaacagtaaagtatttacacggtcttaatgcctattgccaaacacatatagctgctattaatgcctattgccagactcatatagctgcaaactcatgtagcttaatgcccattgccaaactcatatagctgctatatatgtctactggaaaactcacatagctggttgattttaaattgattgtaggaaaattcatacaaaaagatgctacataggaatataaactgaacaccacaaaaatcgtaatgaacaaactcagtaatgccagcctgttcaatcactagttttcagattaaggcagtatgcaaagggaaacatccttggaatggtcttagaatatagaacaaagtcatgtgtttgggaatcttaaccaattccaatactgttcaacatgtttttctttgttgcaaacaatgcagtttttaagcaaactaatgaatgcataccctgacaaacaaatccaacaaaagaggtacttagagcagtgttcattgaatcctagaattttgaaagaaaaaatctattaggtcattttgggcttttacttctgctgaagaaggattgttcttttgagtttatttttctagctttcagttctattccatttaaatgcctcgagaaataggacttctcaaattccctgtggagagttctggcacctactatattcacttttgaaagtctcctgataactgatttcctttttcttttggttatacacatcaactattcatggttggctctgctgatagttttccatgattctttatgcttatttaaaagaaatcatataacattaatcatataacatataaccattacttggttataaagcatgatattaactaaactggcttttaaaaattcaataacattagagcaaatattttattaatattgtcagtagttccatgaatatatagatgtaggatgtcaataaagtttatgccccttaataactgagtgtgttaatgttgtatttgctggttaactggcaccttccctccttttgatcaatgttcttagaacagtatgtacaggagtactttagtctaccacttgatattcaaggacaacacttcgaagcttgaaatgagggattgttttaaccatattaacgtaactgcatagtttgcaatagatttaatgattcaacatcattgttaatatttagtttaattaaaagtgccttatattaacttgtacacatgtgaaatgacttatcaacaagattatttattgcagcattgtttgtgattacaaagagtggaagtcatttgcatagtcattaggcgtaaaaaataatgacattaaaagaaaacaattgaggaaagaaccagtaagctctcaggtagagataaaaagaaagttaccgtgagccttttcactgtatatatttatatatttgatttttgacacgtgagtttattataatcaagattgaatgaaaaaaattgaagccttttaatgaaattagcttgacaccagagtcattatcaagaaaatctgaaatactggtacctatgcacatttgattttattatttttagttttattattttttgagacagagtcttgctctgtcgcccagactggagtgaagtggtgtgatctcagctcactgcaatctccagcctcccaggttcaagcgattctcctcagcctcccgagtagctgggattacagatgcctgccaccatgcttggctagtttttgtatttttagtagtgacggagttttgccatgctggccaggctgatctcaaactcctgacctcaggtggtccacctgcctcagcctcccaaagtgttgggattacaggcgtgagccactgcacccggccatttaagcaaattttagttaagaccagtaacatatttttgacagtatttccgaagtgttgtatttaatttaactaattgaaaattatctattaagaaagcaagttaaatgtaatgtgtatacttcatagtatacacattataatgattcatagtaaccattatatgaagagtgtctaaacttttcttcaaatctaccatttatatagtacaataatgaccagcaaacaatggctaagttttacttaattagacatttgtgtagctcctaccaaggctaccagactttgtacccagtaacaggaaaacagaaataattcaagcattattctcactcttgagaaacaattctatttagggagatatacataaaaagcaaaggtggctgggtgcagtggctcatgcctgtaatcccagcactttgggaggccaaggcaggcagatcacttgaggccaggagttcgagactagcctgaccaacatggtgaaaccctgtttctactaaacatacaaaaattagctgggtgtggtggcatgcacctgcaatcccagctactgggcaggctgaggcagataattgcttgaacctgggaggtggaggctacagtgagctgagattgcaccactgtactccagcctgggtgacagagcgagactccatctcaatgaataaataaataaataaataaatagcaaaggcaataatgtgcatatagtaggtgctacagtagaagtctgcacaaggttctgtgtatgtggaaaagacaagtcagaaaaattaggaaaggctttattgggaggtgacatttaagcagaatcacgaaagaagacctgatgaacatgggggtaagagcacttgtacacaaccccatactcctgggctcagactcacttgctcattccctaatcatagaagaccttgaggaaaagcatgctggggttcccttccagcccactggtaaatacagagaggcctaagcacccaacatcccccagggaatacaccactgggacttaaagcattggcaacccagcacccagttaaattccccttgtcactgtttccacattgtccccatcaccttcactctcttgatgctctgcattttctctcttaactcgacccacagtagaccctcccactcaaatctgcccccaataacctttgcaaccaatattaccgcactacactttatcttccctaagggtttcctgctcctcctggtcttaggtgaggtcatttctctgccagcctttaaagtggaagctgctcattttctctgtccctcatccagggctggagtgggactgatgcccttcaccctgcccagtactgtttccacatgagactccttgcatagcatctgctctctgctactcagaccaggagtctgtgctctctcttcctctaaccatcattggaagacaccccagtccctctggccccattatccactgtagattttagcacttacctcctctcttccctcccatgtgctgttttcccatttattttaaggtgcatgtggatggcccattccccttcctggcatcttaatccctttaatttctcatttccattaatttgctacattcctcatatgccagctacccctatggccatatcccagacctttgaatcacacaccaaattccatcaagtcctatgagtcatttttggtccaagacctatcttacatctatgcagtgctatctattttaacaaccatgtgcccagtttaggccactgtcttctcttcactgaatatatgtgttcctgttttttctcatccccatttgtttcccagacacaatttgttctccagagcagagtgatcacatcagtcacctgctataaaaactcctcaacccggtggggcatggtgactcacagccccagcactgtaatcccagcactttgggaggctgaggtgggaggatcacttgagcacaggaggagctgaagtgatctgtgatcacgtcactgcactccagcctgggctacagagtgacaccctatctcaaaaacaagcaaacaaacaaacaaacaaaaaccaacaaaaaattttttattaagcaaaaaacctcttcaacctcttcctgttatgttttgaataaaagctaaagtccccaccatgctccagaagttcccaagggatctggtccttctcatctttacagcctcatcttgttttgccgtttccacctccctcatcccccaaactctttttcttcagggcctttgcacttgctgatgcctctgcctggaaggtcttcttctgattccccatccaggggtgccttatcaccctgccctgccaacctcagattggatgctacttcctcaaagagacccttgggactcccatgtttcccaggctttcagtgccctcatctcaacttgtaatgattgtattggggtgattatttgtatgactttgggattgatatctgactcttccactagaccatacatttcttgagagcagagagcatatccagtttttttaccactgtgcaaccatatgtcgtccaatgcttggcccataatagggggttggtgaatgtggtaggctgagtcatagcccccaaggatgcccatagcctcatccccagaagctttcatggtaaaagggattttgcagattgtgattaagttatggatcttgagatggagagattatccttgattatctaaataggtccaatataatcagtagcgtctttataagagagaggcagagggtcaaaagcagaatcagagaaggagatgccacagtggaagcaaaggggtgtgtgtgtatgtgtgtgtgtatgtgtgtgtgtgtgtgtgagagagagagattgagatttaaagagctccattacttgatctgaggataaggatgagccaaagaatgcaggtggcttgtagaagctggagaagccaagaaaacattctcactctagagcctccagaaggaatgcagctctgctgacaccttgatttggaacttccagaaccataagataataattttgtgtagttttgaggctgggctcatgcctgtaattccagcactttgggaggccaaggtgggtggatcacttgaggtcaggagtttgagactagcctggccaacatggtgaaaccctgtatgtactaaatatacaaaaattagccaggtgtggtggtgcacgcctatagacccaactacttgggaagctggggcaggagaatcacttgaacccgggaggtagagattgcagtaagctaagattgtgccactgcactccagcctgggctacagcgtgagacttcgtcagaaaaaaagaataattttgtataatttcaggccacaaagtctgcagtcatctgttacaacagcagtagtacacgaatacagattttggtacctggaaatggtgtgctactgtaacagatacctaaacaatgtggaagtggcttttgaattgggtgttgggcagcatgtggaagaattttgagaagcatgataggaaaagcctagcttgccttagaaagactgttagtagaagtagggatgttaaaggcgctgctggtgaggacttggaagtgaagagcatggtaaagaaaatgtgtttcattttagagaatatcaaagtcattgtagaaggttggcagaagtgtaggttttcataatgtgttgttggtgagggctgagaaagaaatgaggaccatgtttagggaaactggaggaaaaagatccttgtcatacagtggaatgaaactgtggaattgtgtcttacagttatatgggaagcagaatttgtttgaacttggatatttggcttagctttccaagtaaagtattgaaggtgtagcctggttttctcttgctgttttatagtaaaatgcccgagaaaaagggataaattgaggtaggaactgttaagaaaaaggaacaaagacatgatgacttgggaaattctcaggatacctggtttgtaaaagatgctagaattagaagattcattgtcaggaaagtgtgctctggagaggaagccaagggtgagttccttgtggcgtaggttaggggctgtggcagggatgcagggaagagatgatggtgacttggactaggggtctgacggggtatgggaaaatagagaggaatgagttgattctgttgggactttgtattgagttccttgattccataagtggaaacacatgtagagctctctttcctggccacctaagctctctgaccatatccctgactctctccagaatgccttggcttcatgtccacgtgaggacaaatcatatttttctgcattttgcgtgctggattcctctctggactaaagatccaatgagaggtggtttctagctttctgctctttcccacaacactccgtcagtgagtcttctggatgtcctataggcaactcactggatccacttggtctgtggaagaatcactaccacatccatttcaccttgggcacagactagaaggtgaggcagtcatgtcctgcagtcactgggtagcttacaagtgctaatacagcaatagcttaattagagagagagagaagaagaagaatgttatggagcctgtttctagagaggaaaccacaatatcttgatcaagagaccctaaaactggaagaaccagagcagctggtatcaaaatgtggaaaaaactgagatgtggcaagtggtacaactgatagccaaggaggaaaaatttgtatccccctgtaatcccagcactttgggaggctgaaacaggtggatcacctgaggtcaggagttcgagaccagcctggccaatatggtgaaaccctgtctctactaaaaatacaaaaattagctgggcgtggtggtgtgcacctatagtcccagctacttgggaggctgaggcaggaaaattgcttgaacctgggagcagaggttgcagtgagccaagatcgcaccactgcactccagcctgggtgacaagagttaaactctgtctcaaaaaaataaaaagaaaagtttgtaccctcttcttttctcttgcctcaggataactgagattcttataatgcatttattgaacaaatatttgaggagtactcattatgtaagcatcagacactgctcaaggtcttgaggctgtgagggtgtattagtccgttttcacactgctataaagaactacctgagactgggtgatttataaagaaaagaggtttaactgaattacagttcatcatggccagaaaggcctcaggaaacttacaatcatggcagaaggtgaagaggaagcaaggcacatcttacatggtggcaggagacacagtgagaagggagaagtgccacacttttaaaccatcagatcttatgatgatataggagttaagaagaaatcacttaggtagatagtgagggtacgggagtccttggtaaggcttttcttttaaatgaaaagcagccccacacatagacaagcaagctgggagcttgcacgggtgaatgccggcagaaactaggaaccagacacgttaagatggcggctccattttcccttctctgccagccaagtgtacagtaaggagcagacaagctggtgccggccaagaggagaattcatgtgcataataagattagggtggggtgaccagccttcccagtgcgctatgtgaacatcatacctgattgaaccaatctgtgagccctatgtaaatcagacaccacctcctcaagcctgactataaaatctggtgcattcgccacccgccggtgtttcctctcagaagtcccctctctctcattagagagagggctgttttcctttctccttcttctgcctattaacctgtgctcctaaactccctgtgtgtgtctgttctgaattttcccggcatgagaggatgaacctggggtatataccccagaaaacatagccacttaagtgagaactcactcactattcacccccaagatccaatcaccttcgaccaggttcctcccctggcgtgaggggattaaaattccacatgaggtttgagtagggacacagagccaaaccaaaccatatcagagggtgaagagcaggtaaagttgcagctctcctgcaacttgcagggaaaggccatataacacatggttatgagcacaaactgggactggactgcaggtgtgtgagccccagctttgctattgagtgaccaccagcaagttattaaactgtgcctcagtttttttgtttatgaaatggtggtattagtacaacccacctctcatggatgatgtgaggattaaataaaataacatgttgccaggcacagtggtgcacacctgtaatctcggcacattgggaggctgaggcccgagggttacttgaggttagaagcctgagacctgcctggccaacatagcgaaacctcatctctgcttaaaatacaaaaaaaaaaaaaaaaaaaaaaaaaaaaaaaggccaggcgtggtggctcatgcttgtaatcccagcactttgggaggccgaggcgggtggatcacaaggtcaggagtttgagaccagcctggccaatatggtgaatccccgtctctactaaaaatacaaaaattagccaagtgtggtggtgggcacctgtagtcccagctactcgggaggctgaggcaggagaatcacttgaacctgggaggcagaagttgcagtgagccgaggttgcgccactgcactccagcctgggcgacggagcgagactccatctcaaaacaaaacaaaaaaaccaaaaaaattaaccaggcatggtggcacacacctgtaatcccagctactcaggaggctgaggcaggagaatcacttgaacccaggaggtggaggttgcagtgagttaagattgtgccactgcactccagcctgtgcgatagaaggagacagtctgcaacaaagatccaaaaacaaatataaagcacttataacagggtctggtctgaaataagtactatgtaagtactgtaagtattaactaatattattacaatttatcctcatatagtaacatatcaaatattttcagtcagtgatgcaatatgaataaaatgaaatgatgcagtagtgacagaactgagagaaagctggtacaaatttatactgactggtcagggaaagcttcacagaaaaggtgaactttcagctgacacctgagtaccatggtctggaggtaagagtgtcccatgcatatggaacagcaaatgaaacttcccagagcataatctgagaggggagatttcaggagtggagccacatcattgaagttccttagtcctggtaagtgtggattttattctaagtgtggtgaaatgcccctgagaggttttgagtagtagatggaattccatttttaaaagtcactggtgagtcaagtagtgtactatggttacatttttttccccttatacctcattttgtttttcctgcagttaattcttgcattatttccttttatttacttaccttactatatatttattatgaattctttccaattcccaacttcctgacagcctctcaatgtaattttacttaggttaaatgtatctgacagttcattttcttttttgtctctgtactctttctgctaccattctcattcttgcactaatttgtgctggtttctctctgagccagctgcacagctgcctgcctaagacttcctcttggcatcttttaccctctctctgtgttacatccccggttttctgaatcgtgtggcgttctcctttttactttacttcctcatttgtgttgcacgtatgctctagttgtttttagataaagagtgcatcagaggtagatgttttgattccttacatgcctgactttttgttctacttttgctctaggttaatacttgattttgaataatatcctaggttagaaatgatttttcgtcagaattttaagggaattgcttttctgttgtctagtttcctgtgttactgataggaagtccaaaggggctcgtatttcaggtcctttttatgtgtaacctgttttttgttccttgaggtattcagggtctctttttattgctaatttggggagctttatcataacatgggtccttagtcattcatcctagaaaattttcctttcctatatctttgatgatttcgtctcctctgctttccctcttttctcattcttaaacttctatttgtttgacattagacctccttgtttgatcttctaatttaatttttctctcctagtgtccaatttttgaggtgggagaaagatctcatcaatgttatctttcagcctttcccctgaattttaaaattttactcttcatatttcttctgattaatcctttaaaaaaatagcatcctgggccaggtgcagtggctcacacctgtaatcccagcactttggaaggctgagcggggagtggatcacctgaggtcaggagctcaagaccagtctggccaacatgatgaaaccctgtctctactaaaaatacaaaaacttagccaggcgtggtggtgggctcctgtagtcccagctacttgggaggctgagacaggagaatcaccagaacctgggaggtggaggttgtagtgagctgagattgtgtgccattgtactccaacctgggtgacagagcaagactctatctcaaaaaaaaaaaaaaaaaaaaaagggccctgttccactgaggcttcagtgcggagcatggagggatactacctccaaattccaaacacgtttgacacatctaaagaaccttctaaaggatgactaaactaattctgcaagctttagcctctaacttatctccaatttatatttaatagaaggctggaaattgaacagaaaggaaataagattatttggaaataaaaaattgtcagccaagcaaggagagcttggcatttctggaaacttctttaccctggaagaggtaaaaaagtgattctcccattcccccaacagggcattcactaaaaattaagtgagaaatgctttgcctagaggatctgtagcttgcgaacacttgacttgtgccactggtgtacggaacatagcagtgtcagctctgccctgggacagtcaaggctggctggtgctgcctgtggttagagtcaagagaggggtcttcagtgggtgcagtttgcagttccagagtttagtagagcaaagacgtcatgaactatgtgaactctgaggaaaggtgtcatagaaacacctcaaaaggacactgtctaagaaggctacttgctggggcaaggagaccccaggggtcagaggctgtgtagggaataatgccagagctggggttgaaggagaatccttagaggtgagacagaatgtgcatcattgcagtggggctgtgcaaggcagtggtctccacaggaggtgaggacaagggggaggggaggttgtgaagaatccgtaagtgaccatgatgcaatagaaagccagaatttgggcatttgccataggagagggcccccagtgccagattataatggtcacagacaaatgagatttttaaccatttcctctaattcatggtccacacttaaccccgtgggtcctggaaacagcagctggagaatggagaggaaagtgatgtgggagagagaaaactttctttacccttttcataactgagtttatgaagtaaactgacagtagaaagataaataggagaaaagacataaatttattttgtgcgtacacatgggagtcccataaaatatgagactcaaagaaaggccagatgattgaagtttatatagtattcctgagctacagaaaaggaatcagggcttggggcttattgaggggaggtggtgacaggttataagagggtgaggagaggaagtgtatagcaagcataggttgtcttgttatgcagataaaaagtctctcaggtgataaaagttgtctcagagtcccccatcagaagaataggtaatagcctgtgacaaggtctacctgtccaatcttctccctggtgataaaatcttccctggttgatgagattcttatcaaagtttttttctttatagatataaattttgtttacaaaaagacagtttttcagagctactcctgtgtctacagtgtctcagaataactaactggaaatacatcaaataagcatatcctgatgtggcatattctggtcatattttgggatggtgcgtcctgagctccaatgctgaaaaaacaggaaccccatttctgttggatgtgccaacctaaaataatcaaaagggtcagaatctagtttaaagatactttattcaagtgcaaagtttaaggacagtgctagggaaacacggatcccaaagaatggaagtcagcgttctgaactttagaagtttgggattgtttatagagagagagtttagggaagcttaacagaatttcaacatctttctgtgtaaggcttaatgcctagttacaatgatctgattagtcaaggtggtcactttcatttgagaaaggcatatttaacatttcacgggctgggagcggtggttcatgcctgtaatctcagcactttgggaggccgaggcgggcagatcatctgaggtcaggagttcgaggccagcctggccaatatggggaaaccccttctctactaaaaatacaatacaataaaataaaataaaataaaaaaaattagccgggcatggtgcacgtgcctgtaatcccagctacttgggaagctgaggcaggagaattgcttgaacctgggaggcagaggttgtggtgagctgagattgcaccattgcactccagcctgggcaacaagaatgaaactccatctcaaacaacaacaacaacaacaacaacaacaacaacaacaacaacaacaaacatttcacactgaaggtgtaacagtcatgggtttgtattttcgtttttcttggttttttttttttttttttgagactgtctcgctctgtattgcaggctggcatggcacaatcacagctcgctgcagcttcgattttgtgggctcaagtgatcctaccacctcagtctcccgactagctgggaccacagtcatgtgccaccacacccggctaatttattttttatttcttatagagaccagatcccccttttgcccaggctggtctcaaactcctggactcaaacaattctcctgcctcagcctcccaaagtgcctggattacaggcatgggctactgtgctcatcccatggggtcttttgtgccaactggtgtgagttaggtacaggacaataaaggaggcagttaatccattaatccataacaaagatcagtgaagggggaaggtctggtctctggtctctcctagtcatttacagaactagaacgatgagaagagagtgaatctataacctaagaagcagaattgcaaacatgctatgtgactcagtttccagtacttaacttctcccttggcataataaataattttagagagttttaagaattttgttttcttttacagatgttaacaacctcagcttgctgggggctggtggtggtggctgctcagacagtaaagcattgaatgcaatgtgaggtcaaagttttattacagatcataccggtcttttaagtacttgcagcaagattttcctaatacttaaaagtgactggaaactcaataggatcagtgtgatcttctccagatagggatggtagatttttgaaagtgggtgtgaagggcagtaatgagagaaaaataaaactatttctggttgtactctcccaagtcaaggtcattcaatgaatggttatatagatttgcatcaaaagtccctgttttcagcctcacctttggaaacacctggattctctattctgagactttctgagatgagggaaaggtggcttctcatcagtatctccttctttgtgcaatacagtttcagttctttctaatctacagagttagttccttctctactgtcagctttctaccttccaaaatgtgttaatgtcactcattatcatgtttcccattctctttcccttatggtttaaactttaaaagacaatggtatttgtttaagtgaatatctaaaaagatgtggagaaagattcatgtgttcagtctaccatgtttaattggagtcactggtagatttttaaggaaaaataacattctaggtttttccagtattgctatgtagcttgtctatgtagatcaccttgcattcttctgtttctctcttataacttgatttttttcttttcttttcttttctttttttttcgagacagagtctcactttgtcacccaggctggagtacagtggcacaatctcgtctcattgctgcctccatctcctgggttcaagtgattctcccacctcaccttcccaaatagccgggattacagacatcttataacttgatttttactcatttcattatcatccaagagatgaaatttaactcaaagcaaatgactattgtttcaaatacaaatcttaatcagggagaaaagattataacttatagttgaactggggtttggagattatatgtgttttttaaaattattctgtcccacatgtaacatacaagtgaggattttaaaaatttgtctgcagtttttttttttttaattgatcattcttgggtgtttctcgcagagggggatttggcagggtcataggacaatagtggagggaaggtcagcagataaacgagtgaacaaaggtctctggttttcctaggcagaggaccctgcggccttccgcagtgtttgtgtccctgggtacttgagattagggagtggtgatgactcttaaagagcatgctgccttcaagcatctgtttaacaaagcacatcttgcaccgcccttaatccatttaaccctgagtggacacagcacatgtttcagagagcaccgggttgggggtaaggtcatagatcaacagcatcccaaggcagaagaatttttcttagtacagaacaaaatggagtctcctatgtctacttctttctacacagacacagcaacaatctgatttctctatcttttccccacatttcccccttttctattccacaaaaccgccattgtcatcatggcccgttctcaatgagctgttgggtacacctcccagacggggtggcggccgggcagaggggctcctcacttcccagaaggggtggcctggcagaggcacccccaacctccctcccggacggggcggctggccaggcgggggctgcccccaacttcccagacggggtggctgctgggcggaggggctctttacttctcagatggggcggctgccgggtggaggggctcctcacttctcagacggggcggccgggcagaggcgctcctcacctcccagacggggcagcagggcagaggcgctccccacatctcagacgatgggcggccgggcagagacgctcctcacttcctagacgggatggcagccgggaagaggcgctcctcacttcccagactgggcagccaggcagaggggctcctcacatcccagacgatgggcagccaggcagagaagctcctcacttcccagatggggtggcggccgggcagaggctgcaatctcggcactttgggaggccaaggcaggcggctgggaggtggaggttgtagcgagccgagatcacgccactacactccagcttgggcaacattgagcactgagtgaacgagactccgtctgcaatcccggcacctcgggaggccgaggctggcagatcactcccggttaggagctggagaccagcccggccaacacagcgaaaccccgtctccaccaaaaaaatacgaaaaccagtcaggcatggtggcgcgcgcctgcaatcacaggcactcggcaggctgaggcaggacaatcaggcagggaggttgcagtgagcagagatggcagcagtacagtccagcttcggcttggcatcagagggagaccgtggaaagagagggagagggagaccgtggggagagggagagggggagggggagctgcaattttttatttagcaatttccaaacctattgtgttaggcagggttctccagggaaacagaaccaatagggcatatctatatctatatttatatctttatctatatctatatctataatctttctatctatctatcaagagatcgagagagagagatttattttaaggaattggttcatgtgattgtgggagctggcaagtctgaaatccatagggcaagttggtcagctggaaattctggtaagagttgatgttgcagtcgtgagtctgaaatttgcagggcaggtcaggtacagtatctattgcaattgcagtcctgaggccaaattccttcttcaggaaacctccgtcttttttgctgttaaggccttcaactaattggatgaagccctcccacattgagggcaatctgctttactcaaagtctgctgatttaaatggtaatcacatctaaaaaatactttcacagcaacatttgaacttgtgttgtctaagcaattgggcactatagcttagccaagcagacacatgaaattaaccatcactctgtagagatgaaagaactactgtttcaaaaaacaactgtttttgaatccgtcatttatcaacggattcacccaatggttaacctttctatatgctttctctttctcccaagtactgaatcatatgaaaataaattatggttgtgatatttcctatctaaatacttcatatgggacattctcctacatagcacacctaagaagattagtattaattcagagagatcatgtcatatctggttcatatataattttccctagctgacctcaaaatgtgtttgttttgtttacatattactctttatagttatgtttcttttaatacggatcaatatttgtgtgtttttgctgctattttttttaatgacattgttttgaataattcaggctcattggctatttcacatcctgaatttctctaattttatctttatgattagagccaggctctaattcttggcaagaataacactgaagtgaggttgtgtactcctaattgccctgcatcaaagacacatgatatgcattggttcctgcattagtcatgttaagtttgattagctggtgaaggtggtcgccaccatttctcactcttgtaaagggacattttctccttttaaattaatatgtaatttgtggcacaagactttgagactgtgtaaatatcccattctctgacaacctttcttctgatgactttagcattaactgatctaattatatcattcttggcattgagtagcattcttgtgtaaagaaggggttctctttctctccctcctctcattataatttgttactgttattttcttacaagttactaagaattactcaaaggcagtatttttcaataaatcattggtaatttatggtcttctcactctagaaaagggaggatgggtcagaaagctgaggggaaaaaaagggaggaaacgagaatgtatattatcgacataatcggttgaaaatgtctagtgctgtaattatgccatcatgcagattaaaaagccacctgtgaaaaatcaacttgtattgttttgttttgtttgatttttaataaatccttatagtgtatgaataaaaattaaattaattgatcagtatcttcactaatggcagagaaggggatggactgagcagattctgcttttcactctgatatttgttaattgccctgtgtggtctgaagacctgggttctagtaccagctctccctctgcagacaggtgtgttactttggtcaaggcaatcaatcttcttgatactcagtttggttctctctgatttgagcataagaaatatacttgaaggccgggcatggtggcttatgcctgtaattccagcactatgggaagccgaggtgggaggatcgcttgggctcaggagtttgagaccaggctgggcaacatggcaaaacctcaactctacaaaaaacaaacaaaaaattagccaggcatggtggtgcacgcctgtagtcccagctactcaggaggttgaggcaggagaatcctgggaggcagaggttgcagtgatctgagattgtgccactgcactccagcctgggagcctgggtgacagagagagaccctgtctaaaatatatatatacacacacttgaatgcttcatgtcccttgctcagtgacagccccgtcctctgcttctgcacagttgaccaaggcttctcagtctactcctgtgtagaaaagaattaaagcaggcctgaggctgctagtcttagaaaggcttgcaaagttggcccttgtctggtgtctgggaacttgaatttctggagggttctcaccattccctgaaaagaatggctcacgatgcctaaaatatttgtacaaacaatgaagtttctgctgaacatctgcttccttctgggagtctggaattttaggatgtgctaggtaggggtgtttacatgacagccccacataaaaaccttgggcactgagtgtctaatgagattccctagtaagtaatattttacacatattatcacaactcattgctggaggagttaagtgcatcctgtgtgactccactgggagaggactctgggaagcacatgtctgatttcctttgtcccatgtgccttttccttttgctgatttttgccttgtaaatttttttttttttttttgagagacagagtcttactctgttgcccagactggagttcagtggccccatgtcggctcactgcagcctctgcctcctggattcaagcaattctcctgcctcagcctcccgagtagctgggactacaggcgcgcgctgccacaccggctaatttttgtatttttagtagagacggggtttcaccatgttggccaggatggtcttgatctcctgacctcgtgatccgcctgcctcggcctcccaaagtgctggaattataggcctgggccactgtgcctggccataatttttatcctgtaataaattatagtcgaaagtattgagtcctgtgaatcaacttagagaatcaccaaactgcttccaattttctcatatgtaaaatgggttgctataataatgatgatatctaccttatagggttgttttaagtatgaaaaatatggtgaaatatgtgtgaaactaggggccggatgtaggatgagtcatacagtgggtggttattattacggatcatattaactcttcaggtaaaaaccatcttgtagctgggcaaggtggcacatgcctgtagtcccagctacttgggggactgaggcaggtggatcgcttgagcctaggagttcaaggctgtagtacgctatgatcacgtctatcaatagccactggactccagcctggacaatgtaatgagagtctgtctcaaaaaaaaggaacaatcttgtgtttgcgtgtgtgctcatgtctttgttggaataatactgacacagtcactcaaattaactctcaaatctttgattattcatttgatgggaacaacaggtttatgtgccagcttatcaggacccctagttctttcattaaagtgtgtatgtgtgtgtgtatgtgtgtatgtgtgcacatgtgtgctagttttcttatctaacgacgaagtcctttgggaggtttactttttcattactatttttttcatgctttcctttgatgtgcacctggcaatttatagagccaatgtgtactacatattctgctgcagaaaatgacagaggtgaggaaggagcaggaagcagatttagaaaggaatgttacagtttatcaagttgtgactaatggaagctattaaaacaaaaggtaccaacccatcttaaatattcactgcctctacaactatttttctataactgttgttccttgtcagctctggggtggagggaatattcctgaatgttttattaagtaattcaaagatcttcctaggtatgtgtatcaaagatcctatgatgtatctgtcttgtaaattgagactggcatatattgggcttacattactgggaaaaatgtatgtcatcatcattggtgaaaaagagtttccatagcagttttttctaagtagagagataaatgaatcagacttttggaggaggtatgttttaactcactggaggatcacaccaagtctgaacatctaaggaaccctagtggaaaactggttttcctgtatgctgctctagcgatctgaggaaaggcctaaaaaaagccagtgtccctgtgatattgtgaaatacatatatgtggtctttgttcctgtttcctggcatacaagtactaaaaatccttggaatctccaaagtgctgtctttttgtatattagtgttgactgatagcttcagagtggggctggtcaagttgatcaccaatggccagtggtttaatcagtcatgcctatgtaatgaagcctccatgaaaatccaaagggaatggactggggagcttctaagaagtgttttttaccttcccgtgagcctcctgtgctgaacacgtggagggtcacgggaaggtaagcaaaaattcattcacatgctgggagggtggcacatcccaactccacgaggacaaaagctcctgtgctcagaacccttccagacttggaccttgtatctcttcattggcttttatttgtattttaaaaaatatcctgagtgataaactggtagatgtaagtgtcttcctcagttctgtgaaccacgctagcaaattaatcaaaccggaagagggggtcatggcaaccccaacttgaaacctgttggtcagcagttccagagacctgaacttatgactggttggaaggacggggtgctcttgtgggactgagccctcaacttgtggatctgatgctatctctgggtagacagtgttggagctgaattggaggacacctagcttgtgtccactgcagaactgattgcttgcttcctgctggggagaaatccctatatattttggggtccagaagtcttccgtgttgattgtttttgtgtgagagcagaggaaaaatggtttgagagtttttcgggaaacagcccctcttagtatagtggtagaaacactccaaaaataaaatatgctaccccaaaaataaaaaatgaaaataaaaataaaaatctggagtggtcagtttgccaagaggatttatggagcatctaaggtcaagcattacttctcagccctgcagcaggcctctaattaagccatgccacagagtgcggtttgcagagaggtggagttcctgtggattcattcttctctctaaaattataaataacgcagcttccaaacatgccatattacctcacaaggtctaaagactcaatatgaatcttcaacttaacaattataactgacacagattgagatcttcctggatgctgaaataggctttacatgatttatctcatttagttctcataaaactctattattaatattattttacagatagagaaatggaagcacagagagggtaagtgtattagtccatttttatgctgctaataaagacatacccaagacagggtaatttatacagaaaaagaggtttaatggactcacatttccacatggctgggaggcctcacaatcatggcagaaggcaaaaggcacttcttacctggtggtggcaagacagaaaatgagaaccaagcgaaaggggtttccccttataaaaccatcaggtaacatgagacaattattcactaccacagaaactatatgggggaaaccgcccccatgattcagttatcttccattgggtccctcccacaacacgtggagctacaattcaagatgagatttgtgtggagacatagctaacccatatcagtaagtaattagacaaaccttgcaaagctagtaagtggtattgctggaattaaatctgccaatgtcactccagagtctatgtgatttactggtatattatagggtctacctataagcttgataaccttatgttagaacaaataaccatgacatattctgttcagtagtttgcatttccttttgactcctacaggggaggaggccgaggttcagggacattaaagtggggtttagagacattaggtggtttacccaagctttatctactagatactagataattgtctatctgacaataaagctagaacttacacccagctggacaatggagctacagcttaaaacaaaatcttctaatgagctcagaactcatggcttaataagatttgggaaaagtcctgcggacatttcactgtctatccagaaatgcgaggaagttaggagaaaaggcaaagtatctcatagacagataaaggcagttcagtaagtagcctgaataaatagccatatttaaaatctaatttggttcttttgtgcctaacacaattgactttatgctggtatctattttctgctctgtctctctttctgtctctacttatgtgtgtatgcatgtgttataaaatatatcagcccattgatcaatttttaatttaagcaaaaacatggtagattaatatattcaatcaatttattgagtagatatttatcgaggctcacacatttatctgactgtgtactaagcactggaaacccaaagagaatgaagtcactgcctagacagttggaggctgacacataaacaagcagggtaataatcaagtgtcataactagtctattacatgcaatgttaaactagcatctctaccatgcaaaacttgtgctcttggggatacaggaagactttccagagaagtacacaggacaggaatgtgttaggaaaccagtcagttcccaggtcctcgatcaggtcacagtgacttgcgattctattttgaacataggtcttaaatctttattttgatagcaagggttttaaacttttgatatatgatatacttctgaaaatcaaatttcatattctaaaattaagtatttttgcccttaactaacttgaacataatactataatacattaacatatattattaataataaataggacccctggaagtccaagagagacatgaggcttatttggtatgttaaaatcatacaggaagtgttgttaaataagaaatggtgttacactttctttgagttatatttatatggatatgttgttaatatgtgttccaacattgtatgagattcctaaaaatctgatatggacatccagtgtggttgttgggtcctctatgagcctagggagcactggccggttaccttgcatccattcatgtcagcgttggtagtgtcaggcacccgatggttcttagaagagtacttagctctactctgcagtgtctgaagttgctggatatatacctgctgtataaactgctgactagggcgctgcagtttacttactgtcttctcatggggaccttccccttcaactctttcctcttgggtttcacatcttgggtggggagtttcatcctagtagtttgcctgagaatacaggtgaacccacagaacaaagtggacttcgaaagcatctccttggagtgagactttgcttctttctctttgctagcaccatcttgtaccttatcgtcatgaactttgttggctgaatcattcccatttacttaattgaagagtaagagactggaacaatgctcactttgattttcctggataagagttaagagttcttgagatggcagcttgtttgacacatgaattttcttcaaatttgtgcttactaccaactgatttggtgtggaggagagcccagagaagttccctctctctgtcagaacaactttgtaacatttattaacctgacttctgccttcaattaactgtaaccttttgccttccaaattaaaaagttccacattactccaaaaataaaaagtgaaaataaaaataaaaggctgatatgtcatggtatatgcagtaaattgctttattctgatttttttttctaaaagccttttgcaaatcctgaagtgctgtgtattcaaggaaattcatgaaagggaccttgacaagtagtcttaaatacaggtttctgataactttggagatcacacctttggactaggtaaaaacatccaaaactcgtctgggcgcagtggctcacgcctgtaatcccagcactttgggaggccaaggcaggcggatcacgaggtcaggagatcgagaccatcctggctaacacggtgaaaccccatctctactaaaaacacaaaaacaaaattagccgggcgtggtggcgggcgcctgtagttccagctacccggcaggctgaggcggaagaatggcgcgaagcggcaagacggagcttgcagtgagccgagatcgcgccactgcactccagcctcaaaaaaaaaaaaaaaaaaaaaaaaagtccaaagctctaatgaaaaactgatgcattcatgcagattgctaacccaacatcaaggagaacgagaattacatgggactgagtgaatgaaggattgaaattactattttaaagggtttttgtttgaaacattactgattttttttatgttttgttttccagactcaagaaaatattttttttcttttgagctatttatagcttacagcattggggtaaagtatacttctgtgagcaaaatggaaacatttacctttctttctacctgaattcttcagaatttggaaactattcattagtgttcttattttctggcaatatagttatttgcataagttcaataagaacctattttcggctgtgcatggtggctcatgcctgtaatcccagcaccttgggagggcgaggccggtggatcacaaggtcaggagtttgagaacagcctggccaagatggtgaaaccccgtctctactaaaactacaaagattaaccaggcgcggtggcaggcgcctgtaatcccagctactcgggaggctgaggcaggagaatagcttgaaccttgggtggcagaggttgcagtgagccgagatcgcaccactgcgctccagcctaggggacaagagcgagactctatctcaaaacaaacaaacaaaaaaacaaaaagcaaacaaacaaaaaaagagcttattttcttttgtaactggacacatggaaacagtggttattttaccaaggctttgactggaatgtcttttttttgagtgcaaccggactgcttcgagggattgaggttgactttatacagccagtagacttggaaaaagacacacctggtaccttgcccacacaattcctttatagcgtttctaactttgcaataagtaaagaatgtcactttctgacaggcccagggacctcaagatattttggagacgttgaaaagagagcaattcacccaattcatacaggttttacaggcacagtctgatggcgaatctttggcttggcttcattgcttcaagagtttgtttttttgacacggaatctcactctgtcacccattctggagtgcagtggtgagatcttggctcactgaaacctctgcttcctggattcaagtgattctcctgcttcagcctcccgagtagctgggattacaggcatgtgttgctactcccagctaattttttgtatttttggtagagatgaggtttcaccatgttgcccagggtggtcttgaactcctgacctcaggtgatccacccacctcagcctcccaaagtgctgggattacaggcgtgagccactgtgcccagcccttgagaggtttcaaaagtcttaatctgagattccttatgaaaaaattccaacaaagccaacttaagagccatccctgtagaaaatatatctatttaaatatcgtctgttttatgccacaatgtttgttttgcgttgcaagccgttatctcctaggcatgggtaatccactttgagaggaaaatccagacatcattgtgcctaatttgctgccacctgtgtctgtgctggatcttaccagggttagctttattttctttcaactggcaaaattctgataaagcatgtagcttcacggtagagcaaaaagtgtaacttaattgaaagtcatgactttcaggagtctaatgatgctaatatattttcttctagagaggtgtctttattgtatgtaattccctgaagaaatgtaaagatttatctaattcctattgctctgacaggcgtgctcaatagaagcattgaagtaaaataaaaataacctttttaatctgtgtatttctcttgcccaccaagatatttaatttttttcttgatctttgcttttgtttatgtgaagatatttatgtctatatcatttctgtatatatcacagaaaagttttcacttgcttgacattttattctacaatgatttttagtttaagtttaaagaatggctacattcagatttattttcacaactatagtcctgctaaactgcctttgttgaaaactcagtttttataataaataaaaaatatcaaagcaaaaaaaaaagagccttcatgataaatcaccattcttactgcactttaagcagataatcatgccagagactaaactgactttgcaaataaattagttttattattattatctttgtgggtaaaagttgggatgactgtagaagagaaaattatatttcagaagaaaattataccatacttgttattagattctagtcttgataattgtttttttgagtttttgttatttgcctacaatttgggctgaatcctgaattccttcctgggtacaagtctccaaactaatgtttcctaatttttctaccatttttctgtcttggaatcaccaagccctgcaggctttagctagacaacttgatataaactttggaagaaataatgacagcaacttaatatatgagcagtgttcatgtcagctgatgtatggattactcagaaggtttacttgaacacctgattcaaactataatccagaaatatctgtaagattgccactgcaatctgaagctacttcagagactctaggaaaattagtttatagacaactccagatgttaatctttgtttttcttttgttttcatggaaatgccttttattaaacatctgattgcttgattcatagaggcctgactttggtggaagcaacaccactgcctgaaatgagatataactgttaaccgtttaattggagcggcctgttctcacgactgcaagactagttcaatggcttataaaataatccacccgctgggcacagtagttcacacctgtaatctcagcactttgggaggctgaggtgggcaaattgcttgagctcaggagttcgagaccagccagagcaacatggtgaaaccctgtctctaccaaaaatataaaaaattagccgggcatagtagcatgtgcctgtggtcccagctcctcgggaggtggatgtgggaggattgcctgagcctgggaggcagagcttgcagtgagctgagattatgacactgcactctagcctgggcaatacagtgagaccccatctcaaaaaaaaaaaaaaaagataatctaccaacccaatttctcaactggggaatgttgggctcctgctctcctgtctctgacctttcattctcccttgaggctagccatcaagactacaacccctcttccccaaagtgggccatagaaacaaaaccccttttccccaaagccaaccataaaacctaaaaatagtactctaacttccaccacccccagcctgtctgtgtaaggccataaagaaattatctgactcactttgtttgactgaaggttataagacccccattccagagagggtccagcaccacacccagaaggaagaaatgcatgctcagagaggcaagaagggtccagacagacaggctgtgctggatttccctgctcagtctattagcattagaccataccttttttgtccaatcatatttctacgtggctctccatactttgtttaacctaacctaagggggctcagggttttggcctgggcattgtctgttggggaatagagtgagtcatccccagctcatgggtttgcatccagttcttgttgtaaaaggcccaaagcctgttggatggcaaccctgagccatcgtggaaggggggttccagtttcacaaatagatactcagacagccaaactaccatctacttggtgccaacgtttgcactgtggtcaaagacttacctagcacagactgaacaaatcttcccatctgtcacataaatgtccccaagcaatgttgaagcacatgccaggatcggccttgctaggtcctgcttggtagataagcaaatggcttccttgtggtgtttttattctattttgtctcattaacactacaactttgtgttatctacttgataatctgtaattgtaaatacatacaggattatgtaatttgtgtaaatacataatgacagacttctgaaaactggtattttttacttggtgtccatttgaagctgttttaggttctgtggcacatgaaccaatggcatttaaaaagcatactctccttgctcttaaaaaaacaaacaaaacaaaacaaaaactgtccattaaaatttttgtatttttgtaaagacagggtttcaccataaaaatggacagtttcccttatatctttgggtcttcgttctgtaggctctcgtgtcacataaaattatgatcaaataaatttgtatgacttttctcctattaatctgccccttgtcaatgattttgagcaaccttctgaagaaagtgatggggaagtattccctttgctgccacaaggtatatatcagataagtcagtctattttcttgaacatatatcacattcataggaaaaacactttttccaaaagattactgtcttcccaaatacccacgttctccattttttttttttttttttagagatggggtctcactgtgttgtccaggctagtctcaagcttctggactcaagcaatcctctcacctcagcttcccaaagtgctgtgattacagacataagccatcacgcccggccccattttctcctttgggtgtatgtatattgctcattgtcaggcatcaaccatttctcttctctgagatggagtctcactctgtcacccaggctggagtgcagtggcgcaatcttggctcactgcaagctctgcctccctggttcacgccattctcctgcctcagcctcccgagtagctgggactacaggtgcccaccactacgcccggctaatttttttgtatttcttttttggtagagacggggtttcaccgtgttagacaggatggtctcaatctcctgacctcgtgatccgcccgcctcggcctcccaaagtgctgggattacaggtgtgagccactgcgcccagccctcttctaattttttatatttatcatgtatttactagaactggtttattttcgtgagcatatgttgtggattctactataaataatgcacttaataatcattaataaaacttaaatcctttccgtcttgattgtggccttttctttttgctattaatttcctcagcataggttaacctgaactcttaaaagctatttaggtactggtataaaacaaaattttctccaaagcaatccagtatataatatctggattttaaaaaagcagcctcatttaattaggattaatttctcctttcagaagttaagtgattctgtttctgtaaaacgcaaaattataagcttaattgttttccacacaggaaatgaaattcctaatctttttatccagaatcttcatgtgtttgtctctctgtccatctgtcactcctttttaaggtacctggagatgacctagaggcttgccacgcttagggtttcctccctgtgcagaagaagatgggaagtgcaaatgaggacgaggggtggggagggaagagggagtcaggtgattcagcaagtgcaggagcccacagactaagctcaggaatttgcactttgtctgctcgcagagtgagtttcatcgtggtgtgtatatattgagatatgcaacagactccactggaatgtcagaagaacttatgtttatttttcctctaacatgtgggaaagattaaactgtatttgtatttaactcacatagattggcacgtgctcattctgtgtgtcaccctgccacgctgtcacaaacttcgagcagggtcctgaggggagaggagggcatagctcctgctcccagggggttgcctgtgtagccctgcgcattcattctcttccagagggttgtgatttgtggcggtctgtgtgagcctggttaaggagagttacagattatgtcatctggtgttaactgataatctttgcaaaagggacattggctttaagagatgtctgcaaaaaaaactctaaacaaacataaataaaaatttaaaaggataaagccagaataataatgaaaatattagtaatgtaaaacaaggaaatgtgtcatgtttttcatgataactaatattttttcaatttttttttttttttaagacagtctcactctgtcaccaggctggagtcagtagtgcgatcttggctcactgcaacctccacctcccaggttcacacaattctcatgtctcagcctcctgagtagctgggtttacaggcactcgccaccatgcccagctaatttttgtatttttagtaaagacagggttttaccatgttggccaggctggtctcaaactcctgacctcaggtgatcggccgccttggcctcccaaagtgctgggattacaggcgtgtgccactgtgcctggccccagttcttattataagttctccattaaccatatcatgagattaaaaaaacaacaatgatttcatcggaactgacaaatagtgggtgacacaattttgatcatcaagaagactttaaaagaaggatttgtatcactgtcattactgattacttggcccttgtgtatactgggcctttagctagggctggtacaataaaataaccatagttagaaagatattttaaaggattacttatttcatgtttatctcacccttttatccctatttttgggcatgatttattattattaggtttttaaataaataatgaaataagcatgttaggtttgcatgctgctttggttaacattgctatataaccaaccaccccaaactttgtggccttaaaacaataatttatttatttatttatttatttatttatttatttatttatttatttttgagacagagtctcgctatgtcacccaggctggagtgcagcggcatgatctcggctcactgcaacctccacctcctgggttcaagtgatcctcctgcctcagcctcccgtagagctgggattacaggcacccgccatcaagcccagctaatttttcctttatttttagtagagacggggtttcaccatgttggccaggttggtctcgaactcctgatctcaggtgatatgcctgctttggcctcccaaagtgctgggattacaggtgtgagccactgtgcatggccaacaataatttatttttatctctcatggtctctagattgcctgggcccggctgagcagtctgagtcagccttatggtctctcatgtgtttttaatcagtcatgaggggccggcatcatctgaaggcttgactgggctggatgtttaagacagccactcacagggctgacagtgatgctggatgttgcactgttgactaatgagcctgcacgtggctcctccatgtgatttgggctatttatagctggggtgactgggttctaggtggggtagttccaagatccttccaagaggaagaaagcagaaactgcctggccagttagtgtatatgcttagtcttagaacagtgtcacttccatatttctccatagtccattaatcaaagcagttacaggaagcagacagacaggaagggaaaacacaatgcaacagaaggagagattgaagtgttggcagctgcaagccaagaaacacctgggttaccagaagctagaagaagaaaggtaggattctcccctacaggttccaaaggaagctgggcctgtccacacctcacctctggaactatgagacaatcactttctgtgggtttaagctacccagtttgtggcactttgttactaccgtcctaggcaaatgatacagtaactacatacacagtacatagaattgctcattttacttcgttgaatgggacttggcattgaataagcccaaatgagaattcttttgtcaagatttttttatggctcacttttccagagacgtgacatggcaggagtaaggggagggtttggcaggtaggaattatactcatctgtcattgtcttcccaataccaaccaggaagcatgtaaataatagctgtgcagtttgttttctgaaccaaactgggccttattttttttaaagaaactttattaaacaaacaaaaacctagaaacactagatgtatatttttaaggtttctctcacataatatcctaatcatcagtataccgtaatccaagggctacatataactgaaaaataaatgggtcttaaaaaaattaaaacatggtatataacactagctaacatgtactgagcagttactaagtgctaagtactgctaagtcctttatagatatcttcatgttgagtgtcgtcactgcccattacttactctgagtttaaatatgagactcaaaagaggttagtaatttgccaaaagtcatagggcttataagtgatagaaccaggataacgaatctcaaccaagggacttcaatgcccaaaccggtgctcagactgtagccccatgtagttagctatttacatttgaaaaaatttttaatgtttattattttttttaagacagggtcttgctctgtcacctaggctggagtggagtggtgtgatcttggctcactgcaacctccacctcctgggctcaagtgatcctctcatctcagcctcccaagtagctgggaccacaggtgtatggcaccacgcccaactaatttgttgtgttcttggtagaggtgagtttcaccatgttgcccaggctggtcttgaactcctgagctcaagtgacctgcccacttgcctcaccctcctaaagtggggggattacaggtgtgagccaccatgcccggcccagctatttacatttaaatataaattaaaatgaaacaagattaaaaattcggtttctcaatcacactaaccacacttgaagtgctcagtagctacatgtggcttagtggctacctggcagatatagaacgtttccatcagcacagaaagttctactggaaagcattgatccaatctctttgaacagtcacaatgcatataaagtccttattatgactgtacaagggaagacaacgagtagaggaaggcagaaaataggaaaaaaggaagaagaaagatttagggtgagggagagcagttctatgaagaaaagaagctcatatctaggagtggagtggaccctgagaacatgttagtctattatattctaaactttggcagttaaaattccaaagtatattaagtacatgctttctaaaatattagagagctgcagttcaacagatttttaactctccacagcatgtccggcactgggtgaggtgggatggctaggtgaataatataggcattgtcatgtgtgttcgtgtgaagagaccaccaaacaggctttgtgtgagcaataaagctttttaatcacctgggtacaggcgggccgagtctgaaaagagagtcagcaaagggtggtgggattataattagttcttagaggtttgggataggcggtggagtaggaacaattttttgtgggcaggggatggatcttacaaagtacattctcaagggcgaggagaatattacaaagtaccttaagggcagggaaggatattacaaagtaccttctcaagggtggggagggtgtatcatacaaagtgcattcacaagggtggggaaatatcacaaagtacattatcgcaagggcagggagggtgtattgtcacaaagtcaattgatcggttagggtggggcaggaacaaatcacaacagtggaatgtcatcagttaaggcaggaacctgctattttcacttttgttgatcttcagttgcttcaggccatctggatgtatacgtgcaggtcacaggggatatgatggattagcttgggctcagaggcctgacagacatgaacttcccatcataaaattagaagagcattaatcaaatgattagaataaaatattaccattattttgaaatggcaagcattgtatgtaaataaacagcagaggaacccactgtagcctagacagggttcagagacgttcctgccaaggacatggcacagggactgaacaaggaaggatgacagtgcctggcaaaggcagggaatgttacaggtatttgggcacctgtgagaaggcctgatgtccgaaaggactgaaataaattaaatgtgtggggggagagagaaagaaagagcctagcaaaaggtgagctggagagtcagaggcagaaggcagaatctgggatgggctgggagcttgccaatcattttgtcaaatgggtgatgtgaagccttgaaggttttttgaccaagaggagatgtcttcagatttgcgtttgagacattttcactggttgtcatgctaagaatggcttaaagagaagcaaggctggggtcagaggagctgcttggaagctgtttggtactaggatgcggataacatggttggagaaatggcaactgtcagggtatttggagcaagaatggatagacattggtgatcatcacttggatgcatttgagggacaactgctatgtttctactagagcaactacatagagcaggagtaagcaacttacagtccacagaccacatttgctctgtcccgtttttcaaatacagtttaatggaaacagagccatgcccgttctttcacctattctgcatggctgacatcaggcatggttctaagtaatatacataagtttcatatattaatgctcatctatcccagttgacaaacatgaagtgttgctattgtctcattttacagcggagaaaactgacatagagattctctttcgcacccatagcttcagttaccacctctatgccaatgattcaataatacctctaatccagacctcttctctgagcttcagacaggcagatctctcacagccagtcttggagacacttcagaaatcataggtcccaaaccagactcctcctcatcccctcaaacacattctttttcaacattccttttttcttagtgaacatcaccaaatagataagcaagtcagatccaaggaggcctccttggcacttctctcatccttgtcccaccttatatcatctatttttctttttctttttttttgagatggtgtctcactgtgtcacccaggcaagtgcagtggtgtgatcctggcccactgcagcctcaacctcaccaagttcaggtaatcctctcaccttaatcccgtgagtagctgggactacaggcacatgccaccgagcccggctaatttttgtatttttaccagagacagggttttgccatgttgcccaggctgccaccttatctccattcttgctgaaatctggctgtttctctccacttctattaccaaccaccagccaaatctgacttattaaaaggatcatctcgtatgtgggttctgtaatagcttcttcaaaatccattcctctccacccagaccctcttccaatctccaaactgcagccaataccttcaattctgtcaccgctcctgcatactccacctaatccttaacctttcaatggtttctcttgcccctaggttaagctaaattgaaaactgctaaagctacagcttcttagtgtaactagtaagtacagtgactactatgtctggtttacttcagctgttgctgactaatagcacttcttgaatgaagaaattatattaccgtactgtagggaaaaatttgtacttcaatggaaaactgaattatttagagcaaacctttaaggttatctgattctgattccatgggccctttcattgggtcttacattgtttcattgtttttgagttattttacagatgactgatagaaatgcaaaataattattgcatgcagtcatgcaagtaaaatctgaaggtcagggttcaattaacttctctcccctactgtggaagaagccaatttcatttgcatattcatttcaatatttctgacctataaacatgcctgttctttgaaccagtttttatatctgcctggtaacttcattaaatgatttaaataaactctataatttagtttattttatacctgtatgacagtcaggcttttaccttatttttgctttttaaaattattctttagctctccctaaggcactacttggctggccctttggctactcactagcccaagctccatcctcttctgtctaccgcagccccaggctctcttttggccctttgttccagccctcctcagagaagttcttttgtcctggaactcactttcataccaggtgctcttcatcccttcttcctttagtaaatttctttaatctttcagatttctgctcaaggatcacttgctgaaagcctttccaggcctttctgagtcaatacaatccattattagaggctcttagagcacaggcagcacttgttataattttacatctgtctgtgggattccttaacactttctaacacaattaacacttttctctctggctgggggcaatgcatgataacaggatgatggtatgctctcaaccctcccccagcaactagcccagtgcttcgaacatggtggatagatacaccgtttttattttagacagatttttgagtagcaagtacctactgctcaggagacagatggactgaaaaaatatatttgggagtcatcagcacataggtgcagccatgaaaatgcacgagaagcaaaaccattggcaggaacaaaatgaaggctattagagaccttatttaggtggaataattggacagaagcccttaatggggaggaaatagaagcagttaatacagatggaggccgggcgccgtggctcacgcctgtaatcctagcactttgggaggctgagataggtgggtggcttgagtccaggagtttgagagcagcctgggcaacatagcaaaacccggtctctacaaaaaatacaaaaattagcccggcgtggtggcgcaggcctgtagtcccggctactggggaggctgagatgggagaattgcttgaaccggggaggcggatgttgcaattagacgagatcgcgccactgcactccagcctgggcgacagagcgagactccgtctcaaaacaacaaggacaaaacttatcttataagcgaccctggacttccagggacactcgccgctctatggtggtacgtgacctgcctggactctgtggtctttggagcttgggaccccaccccagcgtaagaggcctttctgtgccttgtataaaggagaggaaaagtgtaggttttctgagttgataagattagagctacagtatattatcagtagcgttgtatgaaaccatttaaaaaaccaaaccggatttaaccgctttcacccagaataaactgccctccccctctttccaagatcaagtcagccccagttaccacttcctattaatttaaaaaccaggaaggctcataatttaggctgacgttgccccaggcgaacactgcatataagacaatagctattccaatcctcctttccctttctaaaccgaatagtacttctaacatcacttttccagtcctctttctaaatattgcgatcacgagcctacatcggaaaactatgaaaacagtatgattggagctcttgatggtctgctttgcctgaaaacgatgaaaggcattgagatctttgggcagaaatggcccttagggaatgcgagcctggtagccccataacaccccgagttacaaattcggtttgggtaggtggcgcagggaaatctaaaagctggattcacgttctcccccttcagtttgcacatagcggtcagtggcagacaagagcagacgcacaaatgtcaatccccgcccgcaaactctcgagggcagaaactgctttttgtcagttggatttggagtcggtggaaaagctgccctaatgtagtttctccgaggtttccttagccttgaccgaggggcgcttcccggccattcacctagaggttgtttaataaacaaggatgctcgcgaaatatctgcgcttggaaaggcgctcgttcgtggcgcgcattctcgggcctccgcaagcgaccccggtgacagggacaaccgcttcggttttagcgactgcagacagactgggacgagacggttggaggctcctccccaagggatgctggaggggttgcgtcgtaccctgcgcctggccctggcgcgcggccccaggtcgtggtacccagcgccctatgggccgtgcgccggggcttggccacaccgcctgctttcgcttccagccgcgcgctccgtgccactgccgctctctgcagccccgcgtccccgcagcctccccatggccagcccgcttcgctccgctgcggcccttgcccgccaggtacctcgaacccgggcgtttgcggaaggggggaggattggaacccgggtctcggtagctcgcgggcctggccgggcgccttgtcgccgtttcctgcaccatcctccttcgccttgccctccattccgcctccagcgaggcgtcttcccttccccgcatccctgcccgaaatctggagtcccagcctgcaatctccacctcttcgaggttcccgctgcccaggtctagcaccctcatgggtaacccgctccggagcgtggcgaggaccgccacgggggacgtgagggtagctatggactcgctctgagggaggaggcgggagctgaatctctgggctgccagaacccacagccacatcctacgtgactctgccaccccaaaatattttgaccgcagccttctgcctccttggatctcttccttccccacccccacccccgtagttatttagcagattacgcattaaaacaaatgtctgcaggttttcccaattagtcccgcttccctgtgtctttatcttttaaattgcccactaataccatgaggtttaaggtgtggggtggatgctgcggcatcggaggaccctgctggtggaggaaatggttcacgcccgtccccgttccctttgcaggcttgctattgtgcgtctgtgattgacaagaccacgaggctgagcgcgccctggagatttttctataaatggcttaacaccccagtctagactatttgctcggatataagggagacaattgtttttttgttctttgccggcgaaccctggctctgtagggctgacctggaatttaaccagtcttccctgagccggcggaggaggacaaaaaccgccgcgaccccggcagggtgggaagtgcagggcagcgctcccaagacacgcttgttggaggttcgggcctgggtgcttggttgtctgagcctccttttttgtgtttgcctgggtcctggagaggagcgcacggtatcatggtgagcgtcacgtaggttaccccgggtcccgcttacccacctgcatttacttaatggtggtttaattcttctttaaggattgcagtaacggatgctccgcagagtgtaccggagaaggaggatcaaaagaggtggtggggacttttaaggtaagttgcttgccagaggcttagtgtctaaagcaacgttcaactgaataaatccatttcttgttgagattcggggaaattttcactgtgtgggttacccagttcctaggttgtgttgccagacttttaaaattccactcttagaggaaaaaaagccatttagagagtgacagtacattcatcacaacaaaaattatctagcagctaattgctgattttattttgagtcatatatttttcttgaaaaatagtcaatgcgtaaatattaaactagttgtttatcagattccataatacgtacaaaccttcagtctacttgtagaaaaagttaaactgtgatttttctctttcagtagcacataacactctacagtgaaagtgttgcattttcttcttttctatctgaattgcggggtttatatagtaaatagctcatacttcaaacagtgagaaacaaagcacgttgaaaactgtacaaatacaaatgtaagatgtaatattattttttctataagtctatctcctaccctccctcctcgtggaggttttagcttcttctttttatgcctagtgctgctcttctgcctgtttgagtcactgtcaattgtcatcagacaattgacacagagtgtcctaatgatctcacatcctggcggttcagagagggaaggaaacttgactcatcagtttctcacacattgagctctctcacagtgtgctggagactgtgccatgcattggacatccaaaggtgaattcaagattaggtctctacttgcaaggaatttttattttatttttctttttccttctcttgctgtcatcttagcaaggattttttaaaaagcaaaattagaatattgcaatttcttttctgttttttgagacagggtctcgctctgtcacccaggctggagtgcagtggcacgatctcagctcactgcaatctctgcctcccaggttcaagtgattctcctgcctcagcctcctgagtagctgagattacaggcatgtgccatcacgcccagctaattttgtatttttagtagagatggggttatcaccatgttagccaggctggtctcgaactcctggcctcatgcaatccacctcccaaagtgctgggattgcaggcgtgagccaccaagcctagcctgaagaattctttgcaaagaaaaatatcaactcaaatttaaataatcttttcctttctttttcttttttttgagacagagtcttgttctgttgcccagactgaagtgcagtggcaccatcaattaggtatcactttcagccttgatctctcagactcaagtgatcctcttagcctctcaagtacctgagactatcggcttgcatgccatcaggcccaactaatttcgtcattttttgtagagatgggatctccctgtgttgcccagactgatctccaactcctgggcttgtgcaaccctcccacctcggcctcccaaaatgctgggtcacaggcataagccacaatgcctggccataaataatcttttttatttgttaatttagatttctgtatattaggttttatttaggggaattgcctgtttacactcatgtatttacacatcaaaacatgagttatggtggatgtattcacagcacatatgtaataaggcatgtgtaaaaatgatattgataatttagggaataaaaatggtagattttatagaccatctttgtttttgatatacttttctctgtctcaaaaaacaaaaacaaaaacaaacaaacaaacaaaatatatatatatagcctacattgttgttaactataatcaccctactctgctatgaacagtagactttatcgcttctatctaactgtatgtttgtactcattaaccaacctctcttcctccacctacacccttcccaccccctgccatcttctgatatctatcattctatgagtactctcttcctccatgagatcaacttttttttttagctctcacgtatgagtgagaacatgcaatatttgtttttctgggtttttttttttttctgtgtttggcttatttcgcttaccataatgacttccagttccatccatgttgctacaaatgacacgattttactcttttttaatggctgagtagtattccattgtgtatatgcaccacattttatttgttcattgatggacacttaggtgattccatgtcttgactattgtgaatagtgctgtaataaacatgggactgcagatatccctttgatatactgatttcctttcctttggaaaatacccagtagtaggattgttggtttatatggtcattctacttttagttttttttttggaaagcttcataccattttccacagtagataaactaatttacattcttaccaacagtgtataagcgttctcttttctctgtatcctcatcagcatctgttattttttgtctttctaataataaccattctaactgtggttgcttttgacatatttctctacctttttgttaatctacatcatttataacatttcatatggccttttgggtctctcttgggtagttttcgtatttcttctcccctccccatttatgatgcagtcatattacatgaggatgcagttttgcagcagggcctagcaatgagatacgttgttacacatcctggcgaatctttctgtggactctaggatcctcttcatttgcaagaggtcagccatctatttcttccaattcctccagcttcacatatctccacagaatgcaacactgcaaatctgcagttctcttcatgatcctctttattagattttaaaagagtatctccaaaagatgaacatagtgcctaaggctttccaaatggagtaagaataatgcacaagaacctagaataaagttattaaatgtctgatacagttgtaatacagacttgatttttgaaaaatgtggccaatgaagagaagagcaaatgtgctatacgatggtgagcaaaaggtgttgacaggcctggcatggtgactcacccctgtaatcccagcactttgggaggctgaggtgggtggatcatttgaggtcaggagtttgagactagcctggccaacatggtgaaaccctgtttgtattaaaaatacaaaaattagccaggtgcgatgacacatgcctgtaatcccagctacctgggaggctgaggcttgagacttgcttgaaccggggaggcggaggttgcagcgagccgagattgtgccactgcactccagcctgggcaacagagcaaaaaaaaaaaaaaaaaaaaaaaaaagtgttgactgaaccctggctgaaacagttttcaggtgctttcaacaaatttacacttccctgccctgagcctccctatttcagaacaaatgattacccaactgcaaactttgaattaggaagttgtttttaatatgccctgtttttctcaatatttcttgccatttcacaatcagttattgtggcattccaattcttccacaaacatatgatgtgaaacatcctgacttcgatgtcatcagggaatgtggagcattggaaagagacagattaattatgcagaagaaagtatcatttgacaaaatattatttttatttatctttggaaaggaaatctagaaaaagaaaatactttttaaagaacactgataaaaattgtttataaaatttgtttcctttaggaaacaaatcgttcccttaaaactacatttcatatctgccccaaacgagtcacatgtcttcagctaatattgcttgtttacgtttgaactttattcaattctatcacctagtaatttagtattcttaggtaatttctctttgagctcaggttaaaagttgttatttttagttttcagagttgcagaatttttttttcaagtagagaaaagttcatgatgagattctgaagccacctaatcgtatattactttgaaaaactggatatatgccgggcgcggtagctcacacctgtaatcccagcactttcagaggccgaggtgggtgggtcacctgaggtcaggagttcgagaccagcctggtcaacatggtgaaaccccatctctaccaaaaatacaaaacttagccgggtgttgtggcacatgcctgtagtcccagctactcaggaggctgaagcaggagaatcacttgaacctgggaggcggaggttgcagtgagcccagatcacatcactgctcttccgcctgggtgacagagtgagactccatctaaaagaaaaagcaaaacaaaacaaaactggatacagggcagtgcttaggtacaaatcagaaagttagaggttgctattcatatcattaagaaataatgtgtcttacgaaagaatgtagcagtttactgaaatagaagtcatacctagaaatgtaataatttatctttaattgtcagaaatttaactgatattatgaagttctaattataagaacacttatttgaggttaaaaattaccttattctatccctgctttgccgctaatttgatctctctggattagtgggttattgtgggtcctatgggtattttaaggagaggtctcagaaaactaaaaattatatatactggatcataatcattcttgtcacccactctcatctttctgtttttgttttgtgttttactacccttccccttttactaagtagtcttagtagaagaaaatttgcattaagtttgtcgtactgtattgatatggctccaaatgtttcttagcccagggtcctccccattcactgataaaagctaactaaggtaaatcacaggtgtttattgtgcaagaatactgtgaaactattcatgtaataaaaagtttgtgttagaatttcactctctttaaatcctggacatcttctgtgagtgtatctgaaagcagccagacatcttcagtatttaagaaaccctttactattctgtgtgctaggcactgtgttagctttggaattcaactgtgaatactctagccagacttcttgtctaaatagtccagaataggggttgctaaactttctttctttttttttgagatggagttccactcttattgcccaggctggagtgcactggtgtgtctctgctgactgcaacctctgcctcccaggttcaagcagttctcctgcctcagcctcccaagtagctgggattacaggcgcccaccactacactcagttaatttttgtatttttagtagagacagggttgtgctgtttgccaggttgatctcaaactcctgacctttggtgatccacccgcctcggcctcccaaagtgttgggattcagggtgtgccactgtgcccggcctgctaaactttcttaaatggctagatgataaatattttaggcttgagggccatcaggtttctgttacaactagttggctgtgctgccactgaagatacaagaatggcgtgactatgttccaataacattttaatttcaaaacaggccagctggctgcatttggtctgcaagtaaagtctgcctgaccccctacctagtccagaggacaacgggagagaaaagggattcaaagataaaaataatttagctggaatatatttctttaaataaacttattatacttagtaaaaagtcttaaattaacgtttttacttgaattaaatagtggtaaaacaggctgggcacagtggctcatgcctgtaatcttagaactttgggaggtcgaggcaggcagattgcttaagcccaggagttcgagaccagcctgggcaacatagtgagtccctatctctaaaaaaaatacaaaataataataataatggtagaacaaagtcaattttttattgaaacttggcattttattggcatattacaaagtagcattactagactagcctgaacattacagtaatattctgtccttaatgccttttgtgtcactgtaatatgagctttctgtttgttttggaatatgttttcagcctgaatattattctaaaaatacaatttactatcattcataatatatcaaatgactcacgtagctgcaaggcagtgaattaaacagaattagatcattttaaaaataatgataagagctgatgatgtaaagtgaaggtctgtatttaatttgggagggaaaagactttttttgtatattcaaagagatggagtttgacatcccttcacaacctgttacaggttgaacttgcccctgtttttttaactgatcaaaaagttccttctcttgtgtttctttttttcttctcttttctcttcttttcttttcttttttttttttctgagacagagtcttgctctgtctcccaggctggagtgcagtggtgcgatcttgactctctgcaacctccgcctcccgggttcaagtgattttcctgcctcagcctcctgagtagctgcgactacaggtgcatgccaccacgcctggctaatttttagtatttttagtagagacggggtttcaccatgttagctaggatggtctcaatctccaaaccttgtgatctgcatgcctcggcttcccaaagtgctggtctcctgtgtttttgtcagcattccacagatgctataaagttagtggtggtatcgcatgcaatttgtacgcttaatgtttggccatttgcagtgggcaaactggctatgtcgggagctggtgagatgctgcttgtggggagttgtttcctattactctgatttatctttgtttaaataagagttcctttgttcactgtttcctccacacagaacagaggatttatatcttagtgttcattctcaactttcctgttttcaaagaggaaaacatttgcttcactttgctcatttcttctccagtgcacccagaggattttgaaggcttatgccaacaattctttggggcagttggagtgtaaccattgctaaatagcagttcagtacttaatgacattcattttagtttaacaaatcattgtgagtgttgccattttttattagggaaaacatctctttcatctttcccaaatactcaacatgagtcctatggtgagagtgaaaaagggttgtattctttttttgcatcatcttaccccatctgctattttgtccctcttctatatatcactgaaatttggttctgatattctattaggcagtgtacattgcagagattatgaataactggccgaattctgaatgcaggcatgatttgttcagctcagagtgttaaatttctgtgttagctgctaacctttaaaagtcaattgatttcctttttttttttcccctctgtataatctagccagcgaatgctcagtagcttttctgtaaatagtgatgatttttcttccccaggctaaagacctaatagtcacaccagctaccattttaaaggaaaaaccagaccccaataatctggtttttggaactgtgttcacggatcatatgctgacggtggagtggtcctcagagtttggatgggagaaacctcatatcaagcctcttcagaacctgtcattgcaccctggctcatcagctttgcactatgcagtggaagtaagtacatgggaattaaagagagtgacatgcttgcacttcactgtgggtactaagtagcttctcctgctaaaatagctcttgggcagtatgggctttatcatatttaccagaggaagccgaaaatgtctttaaaagttttcctatagacagttggattgaagataaatcttagcagctaatttttcagataatcttgcattttctgtgacgtcaataaaaaaattatttaaagcaaatagaaaggacagctggtgggaaaattggcaattaaaaagccagcactgttgataatttaataagtcacctttcttcttagatcttctaataattgagaaagggtcattgagaacaatattatgatttgattttaatgctaactccacatttttatgaccagtaataatgtctagttatgcatgttaagggacatgtaattaaatgtcctccttcagccatgagttgaaataattttaagcataaaatgtttaaagaattctttctctggtccttttcagggtgcacaattaaccagatgcacagtatacttcccattgtcttgattctcattgtattttacttttgaatgatttggacatctttcccagaataataggggtgctggaaataataatagtcttcctattaagtgctaaaatatggtaatagtaaaatattaatagattaatgataaaataacaacttttgtttactgaattcctgcaatacgttctgtattatgttccatatatgaatcatctcatttaattaccttaagtgagaaggcatgtgattaagcattcaggctttgaagtcagacatcctgggctcaaattcggtctcatttgctccataggaacctttatgacttgaggaatttaatcatttgtgctttaatttctttatctataaaattggggtagttataatatctatcttacagtgatctcataagtataaaataaagtaatttatctaagcatatagagtcatatctggtgcatagcgagagcccagttgttagcaataataattaactcttgaagcagtggtctcatccattataaaaggaggctcagaagagttgtttcttgactaatattacacagcagtaagggtggagctaaggttccaatgagaagcttctttctgttatatagcccctacatgtatacaccaaaattactaggatgcttttgcaattaactccttcaaaattataaattcatataattttggaaagatattcactgtccatatgtatccacaaaatgttgaatttaggaatctaagtttctgttcccagctcttcctgttatgtcaatttgaatgagttctttcattatttgccacaagccctcaccatgtcataaggtataataaagaacaggtgaaatgaagtgcttttatttatttatttttcagacagattcttgctctgtcacccaggctggagtgcagtggcacgatcgtggctcactgcagcctcaaactcctgggctcaagcaaacctcgtacctcagcctcctgagtagctgggaccacagacacatgtcaccatgtctggctaatttttacatattttgttgagactgggttttgccatgttgcccaggctggtctcaaactcctgggctcaagcaatcctcttgccttggcttcttcaagtgctgggatgacagccatgagccactgctcctggctatgtgcttttaaatttgaaaggaataatatgcccaagcccaggtcactggttctcaaacttaatgtgcatcagaatcagctggctacatctccagagtttctcatttctaacaagtgtccagatcatgttaattttgtcgctccagggaccacattttgggaattgctggcctatgggaagtaaatgagaaatgatttaatgtcatttttggaagttaaaaaagattttggtggtcactggtttttgaaaactctttgaaggctgggtggggtggttcacatctgtaatttcagcagtttcggggagatggggttcttgggaaatgagccctccacccatgggatctgatgctatttccacgtagataatgtcagagtcgttcaaaccagagtgactccatcctgaataggggctgggtaaaataaggctgagacctactgggctgcaacatgatgagaccctgactctattgaaacaaaacaaaacaaaacaaaacaaaacaaaacaaaaaacggccaggcgaggtggctcacgcctgtaataccagcactttgggaggccaaggcgggcggatcacgaggtcaggagatcgagaccatcctggctaacatggtgaaaccccatctctactaaaaatagaaaaaaaaaaaaaaattagccgggcgtggtggcaggcgcctgtagtccaagctacttaggaggctgaggcaggaaaatgacgtgaacccaggaggcggagtttgcagtgagccgagatcacgccgctgcactccacactgggtgacagagcaagactccatctcaaaaaaaaaaaacaaaaacctctttggccatctatttagatgagttggaatgctactttgattggttttgccaatttagatttttgtaattagggtagtttaaaaaaactctcaaattactgttatcctttgttaaaaaccaaaatcttttattattagtcttctgcttacaatataagtaaaataaatgttttgtattaataactggattgtatattgcatggttaccactatgtaacaaaattaatagcttaaaattacaagcgtcattttaaaattatttttcatgtttctggggttgactaggatggctaagtggtttttgcttggggtccgtcacacggttgctgtcagtggctggggttagagtcagctcacaggcttcctaactcatatggtgctggagggagtgtctcttagcatgctaatgcttcataatttgtgtataatgaacagtgaggatgaccagaggtcactttcattgccatctgggctgcaaaactcaaggagttgaaggctcttccggcattacttgttctccatgtggtctcctcaggatggcagtcacagagtaggcagccttcttatgtgctgacctagggcccaaaatctgtatgtgtcagttgactgagcccagatggaagctctattgctgtttacgccctagcctcaaaactactctttcaagaaaaattctccaaccgagtttttcctctactctcacaccaccacaacaatagtcaacataggagacttctatgatcaaaggtgtagggatttctccccaccaccaagcagtgaaccccagctgggtgtcctccaattcaattctcacactgttattacgggaaaggtgtcccaatccagtccccaagaggttcttggatgttgcacaagaaagaatttggggagagtccacaaagtaaaataaaatttattaagaaagtaaaggaaaaaaagaatggctactccgtagacagaggagctccgagggctgctggttggctattttaatggttatttcttgatcatttgctaaagaaggggtagattattcataaattttccagaaaagggatgggcaattcctggaactgagggttcctcccctttttagaccttgtaggttaacttcccaccattgccatggcctctgtaaattgtcgtgacactggtaggagtgtctgttagcatgctaatgcattataattagcttataatgagcagcgaggacggccagacatccctttcattgccatatgggatttggcaggttttggctggcttctttaccacatcttgttttatcagtggggtctttgtaacctgtatgttgtgccgacctcctatctcatcctgtgacctagaatactaacctcctgagaatgcagcccagtaggtttcagccttattttacccagcccctaatcaggatggagtcgctctggtccaaacacctctgacattatccacctggaaatagtgtcagatcccatgggttaagggctcattccccaagaccctaaccaccctcacctggcccagacacaagtcacaagtcctgtcctctggaatgtctgactgagaggcatcaagttggagttcccatgaccccctcttctggtttgattaatttactggagcagctcacaaaactcagggaaacacttaggtttagtggtttattataaaggatactgcaaagtgtatagatgaagcgatgtgtagggtgaggtatcgggggatagagtgcagggcttccatgccctcccggggtgtgccaccctttaggaaccttcatgtgttctgctatccggaagctcactgaactcattcttttgggtttttatggaagcttcacgtcaatattccttcccctggggtatgaggcaggaccttcaccggagagggtcttttattttatttcattatttttaaaatataagatggggtcttgctatgtagcctagggtggtattgaattcctgggcccaagtaagcctcccgcctctgcctccgaaagtgctgggactacaggcatgagccacccagcccctttggagaggatcttaagactcacagttagaaaggagggcaggagaaggtcagagagattctgcttcctgcccctgaggcctaacacacccagcattataacaaaagactgtaacaagggctatgggagttaccagccaggaactgtaaatcacacagtattatttctgccttactcttatcagtcatgatggttacaaaggcctgtccaagttcaaaaggaggaaaaaagcactccacttcttgatgaggaaggtcagggttctggaagagcatgggggactggaaatattgttcggccatttcatggaaaatacagtctgtaatagacatcagtgataaatggggagatatggtggatgtattgttttcctctgagtgccaaattgggttctaagatttcacaggccagatattattgaagtggctacgttgtctggggtatataccttggggttcgtcattttgtgccaggaaaatttaggacaaggactcacacgaggagtttaggagtggaggtttaataggcagaagagaaacagaaacagttctttctgtagggagagagggatcttcgagggaaaagaccatccagcagcagatgagctggattttatagtcaggtttgaggaggaagtgtctgatttacttagggctaacaggttggtttgatcaggtatgacgtttacatagcacaccgggaagtctggttgccccaccctaatccttttatgcaaatggactttcctagttgattggagctatcttgtctgctccttactgtacaggtggctgacaaagagaagggaagatggagccgccatcttgaacatgattgacgcagctgtggatatctatgtctgcagcttgattttacaggctgctcttctttagaaaggggctgcttttcattaaaacaaaaaccttactgaggactcttgtaccctcactatctgcaggtgatttcttaactcctgtatcattattatagtgtcataggaatctaggaagtgtgattgccttctggagagaacttcagggtccctggattttctcactaatcatattcatttcattccctgtttacctgtttaataaatgttgagtggctactatgtgcccagggctgtgcaaggtgcctggaataggatggcaagcaaaccaaccatgaccttgctctcaaagaattgttttctttctttcttttttttctgagacaaggtcttgctctgtcgcccaggctggagtgcagtggcctgatctcagctcactgcaacttccacctcctggcttcaacagattctcctccctcagcctcccaggtagctgggattataggtgcccaccaccatgcccggctaatttttgtatttttagtagagacagggtttcatcatgttggccaggctagtctcaaactcctgacctcaagtgatccgcctgcctcagtgccgagattacaggcatgagccactgcacctggcctgttttctgtcttttttttttaacccccacatggaaagttaggcagggatttaatttcaaagagtttcttcccaaatattgtggtgaaacatctagtccatttatgtttcaggctttttcatagatattactgtttctcttagactgacagacttaggacatcacatgattgaatgtcaacctgacttttaagttcaataatagtttcattttttaaatgcaaaattaaataggagtaatatccttgaacatgtttctccttcactcatcggacctattgagtctagaatccattttattttgagagctccaactacatgtggtttctgttaatatctgaaagtaatttttaatatctgaaagtttcaaatagtgataatatttgaaggtttcaaatagtggaggagagacgcaaactgcgagtagggaacgcggattgaaggaaatgaaaagttgataataggcacttcattttcagattataacaaatatttagtgaaataaagcataattttaaaaaatggataagacatgtatgtactatttaatgtgtactaataaatgaatgctcatatttgccatccagataaagaaatagaacagttgaacatcacagaagccctcgcgtgtcccattcagatcacaaactctatctttctactggtaaccattattcttacttttgtgataacctttctttgctttcctttatggagtgtgtagattcttaacactatagttttgcctctttttgaacttcatgtaaatgaaaaaatgtatatattttgtgtttgtgtgcatgtgtgtgtgtgtgcttgcacacgtgtgaataccccttattgtttgagcttagtattatgtaagatctaaccaggaaggaccaacctaacatttgtggggcctgggacctaagtatagacagagatgacatggtccactccatatctgttcccatcccagttctgccctgtgctacaaggggtcttccagacactgcataggtacccataccacctgcaggcagatgacctttgcctgtcctttggagttaggcctgggtaccctactagtggtgtctgctcttgggatgataaacccgaggggcttatcagctttatatatatatatatatatatatatatatattttttttttttttttttttagctagcatctctctcgttcttccaggctggagagcagtggtgtgatcttggctcactgtaatctccacctcctgggttcaagcgattctcctgcctcagcctcccaagtagctgagattacaggcacgtgccactatgcctggctaatttttgtatttttagtagagactgggtttcaccatgttggcatgtgagccactatgcccggcctcttttttttttttttttaagagacagggtcttactatgttgcccaggctggtgttgaactcctggcctcaatagatcctctgtccttggtctcccaaagtgctggctcagtcattatgttctttactgccatccattgcagtataaaaagaataacagttttccctcagaatattcttggtgaaacagtaacaattattaattttattaaatcttggctcttgagcaaatgtcattttaatattctgtgtgataaaatagcaatgtcacataaagtgcttttacatacttaagtactatggttgtctgaagaaaaaggagttgtgtgattgtcttgagtttgtaagtggaactacttttttcatcgagcaccgtttttacttgaaataacaaagtatgaatatgaatgcagatttggccatttggcagatttttatttatttatttgagacaaggtcttgctgtgtcacccagactggggtgcagctcactgcagcctttacctcctgggctcaagtgatcctcctgcctcagcctccttagttgctgggaccacaggtgtgcagcaccatgctcagctaatttttaaattttttgtggagacaaggtctgaccatgttgcccaggctggtctcgaactcctgggctccagcaatcctctcgcttcagcttctcaaagtgctggaattacaggcgtgagccacggttcccagctcgccttttcatatgtttattgggttgctaaatatgttcttatttgaagtgcccacttgttcaagttttttgttcacttttttattgctgtctttataattttttgatgacaagaaatatgtttaaattaaaggcagttttgtcaatctgccttatgtttggaatttgttgtgtctttaaagactcttttcctgcccttatattataaagatatcttatagtattgatattgtcattcacagttaggtctttaatcctagaagttgatttttgtatgaagtaagggcccaatttatttttttccacctatgtatacccagttttcccagcaccatttaaacgggcggtactttcccctctgatatgtcatgatgacacctttgtcatgtacacatgagtttgcttctggatctctatttgtgttcagttgttttacttgtctgcataaatgccacagtcttggtttctcagtcattataatgagccttgcctgctaggaagggtccttctactttgttctccaagagtgccttggatattcttggtcattttctttccatataatttttagatttggtttatcaagtcgataaacttttgtcatgcagttttttaaaagaaaataaagtgccctaatgtgattttttttaatttggattacattgaatacataaatcagtttggggaaaatcaacatctttataatattgaggctttttatccatgagcatgaaattgctttctacattaataacttggtaaagttttatattttccttatggatctttcacttcttttgttagatttttctccacctaagtactgtatcttttaattctactgtaaatagtgtttttattttttaactgctgctattacataggaatataattttgcatctggccagcttgcctaaacagatgatttcaaaatattatctgtcagattttctgtgttctctatctctgtaatcatatcatctatgttttatgatctatgacagttatattttttcatctccaagctgatattttaaatttcattattcttgctttatactggttgtacatattcagttagagtgattgcagtaggcaatttgcgatgttcccaatttgataaggaaagcttttacattttaccattaagtataacgtttgcgagcttattatagctatcctttgtcacttagggaagttatctttgttttttagttatctaggaaactaaaaaatcagaaaagttagtttgattttatcagatacatctgctacatctaatgagatgatcatatagtttttttcctcccataaactgtgaatataatgaatcacattaattgatttttttaaatgttaaaccaatctccatttctgggataaattcaacttagtcatgttgtattagccttttgtatatcttatatctataatactgaatgagattatcatactctttacatgtatttgaagccatgtcattaagtgcatacaatttttattaaatttttaattgacaaataattgtatttatttatggggtacgatgtagtgttttgatatatgtttacattgtagagtgactaaatcaagctaattagcatactcatcactgaacatatttatcatttcttgtggtgagaacatttgaaatttaatctcttagcaattttgaaatatatgatacattattattaactacagtcaccatgctgtgcgataggtctcaaaaacttattcctcctaattgaaattttgttccctttgaccaacatcttccaattccccaacccctagcctcctctggtaaccaccattctactctctacttccattagtttgactttttcagtccacatatgagtgaaatcgtgcagtatttgtctttctgtacttgtcttgtttcacttagcataatgtccaacgggttccccatgtcattgtaaatgatggaattttcttttttatagctaaataacattccatcatgtatacataccacattttctttatcgattcatctgttgatggacagttaggttgcttctgtatcctggctattgtgaataatgctacaataaacatgagagcacagatacctcatgctgatttcaattcctttggataagggtccccaaaccccaggctatggaacagcagtggtatgtgtggcctgttaggtactggatcgcactgtaggaggtgagcagctgcgagtgagcattaccacctgagctccatctcatctcagatcagtggcagcattaggttctcataggagtgtgaaccctattgtgaactgtgcattgcaggaatctaggtggtgcactttttatgagaatctaatgcttgatgatctgaggtagaatgattgcactctgcaagactccccacgctcatccctgtggaaaaattatcttccacaaaactggtccctggtgccaaaaaggttggggactgctgcttttggatatatacccagaagtgggattgctgaagcatatggtagtttaattttaattttaatttaatttagtttaattaatttatttttagcacctaggctggaatgcagcagtgcaatcatagctcactgcagcttccaattcctgacctcaagccatcctcccaactcagcctcccaaatttctggaactacaggaatgagccatctcactcagccctatttttagtgttgggaagaatctcaaaaagtaatgactgtactaatttacaccgctaccctcagtatacaagggttccatatcctcactaatacttatcttttatctttttgatagtagccattctaagtatgtatagttttaaaattatgaagtttaaattgaaccttaggaagttgctactctgtcaccaggctggagtgcagcagcgtgatcttggttcaccacaatctccgcctcctgggtttaagcaattctcctggctcagcctcccaagtagctgggactacaggcacatgctaccatgcctggctcatttttatatttttggtagagatgggtttcaccatgttgtccaggctggtctcgaactcctgacctcaagtgatccaacagccttggcctcccaacgtgttgggattacagacgtgagccatcacacccagccttgaagttgccttttttatcttcagtagtgcttcttggcttaaattcttttgttttataaatagtaatggaagcttgccagttttattttagaaagtatttgcaggccaggtgcagtggctcatgcctgtaatcccagcactttgggaggccgaggcaggcacatcacttgagcccaggagttcgagaccagcctaggcaacatggcaaaacctcgtctctacaaaaaatacaaaaaattaacttgggcgtggtggtgcgcgcctgtagtcccagctactctggaggctgaggtgggaggattgcttgaacccagggggtagaggttgcagtgagccaagatcttgccactgaacttcattcagcctgggtgacagagaaaaacaactctgtctcaaaaaaaaaaaataaataataaaaaataaagtatttgcatgatatatctttttctgtctttttgattcagatattgtcagctgagtccaatctaacaaacttatattttaaccgaagctttagtactgttatatttaataaactaataatatatttgcacttaaatacaacatctaattttatgctttttaattatacatgatttgtatttctttttttcccatgtaagtttttagggtatacatctttaaaggccttacttttcattatcgttcagtttaacttattttctaatttccatttttcttctgtgacctatggtttagttagtggtggatttattttccaaaatatggatggtgtccagtcaaacttttggtattgatttctggcttatcttgtgtttggaaaatatgtgaattctacagctggtctgtgtaagagttctctgtatcagttagggaagtttgttcttcctgttgttcatatcttgcatatctttactaaggtttagcctgtttgttctataaattacttagagaagctgtgttaaattttcccactaaaattattgatttttgtctttctctgtatttatcagtatgtatctactgaagtcttttcaaatccctgatcagtggtttgttcaggacagcactttgattgagggaggtgacgtggcttaacatagtatggtcttgagctgcctggtttctgtgatttagggactgaaccagctctggtcacatctggattatctactatccagcattcaaatgaaccagattacatgaaaggatatgggggtactctttgggggccacggtgccacaaggcctttggtttcgatctccattgcctagggaattaacctgtgctgtgtgattctagatgttttcttcctgctcccttaaataacacctaaatgtgttattcagcagtgtggctcctgctaagcagaggagaactcggaattcctaccaaattctgataataaaataactttcctccacctcaaccattgtttttaccagtcctgtcaactgttagctttcctggatttaatgatctcaagttgaggtcaatgtcaacagctttatgggatgaataagatgaacgcccataggaaagtcagtctcttgaacacgggttgttttcttttggttaccctctaagattttttctctttgatctccagttatttgaaggattgaaggcatttcgaggagtagataataaaattcgactgtttcagccaaacctcaacatggatagaatgtatcgctctgctgtgagggcaactctgccggtatgtaagtgtaggagtttcttttgtgtttcttttaatgtaacgggtcacggtgttgaccaccaaataaataatttctgaatagttagataaatattcagtacaaaccatatgaacattaacattatttctgatctactttagttaggtaaaaatacaagaaaatggccgggcacggtggttcactcctataatcccagcactctgggagactgaggtgggtggatcacttgaaaccaggaattggagacaagcctggccaacatggtgaaacaccatctctgcaaaaaatacaaaaattagccgggtttggtggcacatgcctgtggtcccatcggtgtggctgaggcatgagaattgcttgaacctggcaggtggaggctgcagtgagccaagataatcacatcactgccctccagcctaagccgcaaagtgagactctgtaaaaaaaaaaaacaaaaaacaaaaaacccaagaaaataatatcatttggcaattccacaattttttaaaatcagtgtctgtgggggattcatatgcaagtgagagatgaaagagtaaggaagaaaaatgtatctcaacctaaaataatatttgaagaccacatgaaattaatattgaaaatggaaaatatggtgtgcagcacaggtattttgcggatattttgcctaattgctttagatgctagcaagatatagtaacttaattattttgatattttatcttaagtaatgttttgagataaaaagatatcaaaatggtttctcatggccattgaatcgtggctgtcacaatgtttcttatggagcagaaatcattgtaagatgggttagattttttttttgagagagagtctcactctgtcacccaagctatagtgcagtggcacaatcttggctcactacaacctccacctccggggttcaagtgattcttgtgcctcagcctccttagtatctgggattacaagtgcacgcagccatgcccagcttaatttttttaaaaattatttttagtggagacatgatttcaccatgttagccaggctggacttgaacttctggcctcaagtgatctgcctgcctcagcctcccaaagttctgggattacaggcatgagccaccgtgcccagcttcagggatttagcccaacctatgcattcaggaagcctgaggacggctaaatccaagtgttcttcattcctctgcctatttttgtaacccgcatttcacccatctcctttggaggccataatatagtagcagaggggaaattaaggtaaattctttggactagggcatagtttcgctcttcttctcattacagctagatcactggggaaaagtctttaaaatggggctggaaggaaagggaagtaatatttgttagacatcaattttgctaccaaactgtgttatgtagtttcacattccttatctgtgtaatcacagcagtaaggcgttgctaagaagattatttgttgtacagtttattagtgcctttgtacagagaagaaaacttgagtccagagagattaaatgacttgtctgaagtcacaaagagcaaaaggacagggcaagaaattagatccaggtgtttttattcctggtcaagttctcttctcactgaattctgtctctagacagcaataccaggggctgaggcaggtgctacagggttcacctatatgattggcagtcccaatttctataacattactacattattattgctgttacaggtcaatatttaaatagacaaattctgacttcatgagctttactcagatgcttatgactgactcatttctaccttaggtgacccatcacatctctgaaagtatgtttctctactttgcaagtgagcagagactaaattattttatgaagtatcacccatctagtagatgtaatttttttttctttagaaataaagtgctctttgcttttgcccattttcctattgggttatctatctcttcattgactttggggatatccaaatatatataccagttaaaattctttgttgatcatgctaccaataacttcacccagtttgttgctttacatcttttgaagaacggaagtctttaagtttcaaatagtcacattttatccatttttttccttcatgatttgtgttttacatctcctacttaagaatcctttcctaccttaaggtcacagagatattttgtactttttaaataaagtcttagtattttgtcacatttaagtatatcatctaattagaattgattggggggtatggtaagatgtagggatctaatcttatctttcacatgtggatagctcgtcatcccatcacaatttttggggggaaaatcagaaaaaattgtttggttttattattactttaaaattttttttattggtaccataaattatacatatttatgaggtacactgatgttttcatgcatgcatataatgtgtaatgattaggacaaataagaaagaaataaataaaaattaggataattaggatatccatcacctcaaacatttcttatttttttgtgttgggattattaattttttaacagtttaaatgcttcagtgaggatcatttattattgccacattgtgagaaaattctgtcatttattatgtttttcattctttcaggtatttgacaaagaagagctcttagagtgtattcaacagcttgtgaaattggatcaagaatgggtcccatattcaacatctgctagtctgtatattcgtcctacattcattggaactgaggtgcaaactgactctttattttggggtactttgctgggcaagttattattgtttattgttgtttgaaacttctagcatatagtttgcagtagccccccagtagcatcattaatgacttcttccttctgattgtcaagattagaggtagcaaacattttctgtgaagcgccaatcagtaaatattttttggctttgtggccatatagtttctaataagaaattagatccctacctcttaccataccccaaaatcaattataattcgattatatacttaaatgtgacaaaatactaagacgtttattaagaaatacaaaatatctctgtgaccttaggtaggaaatgattttttttttttgaggtctctctctggttttttttttttgcccacgttgtcgcttaggctggggtgcagtgatgcaatcacggctgactgcagctttgacctcctgggctcaagtgatcctcctgcctcagcttcccaagtagctagtactacaggcatgtgctaccatgcctagctaatttttaaattttttgtagagatgatgtctcactctgttgtcctggctggtctcaaactcctggcctctagcaatcctcccaccttggcctcccaaagtcctgggattacaggcatgagccacttcacctgaccggagaggattcttaaactctgccattttagtactaaagcagccatagacagcacataaatgagtaaatgcagtgctgtttgccttgcccaattaagactagtcattattttctaagtttacaagtgcagtgcctcccattgtggcagtacttctctgaggtagaaatggttttaaaatttaggggagggagagctgctaattttcattttcatgaggtcttgggattacttggcatggagtgagaatggaggttccccttcccacatagaaaaatggtgaaaataaagttcacagtgggagttaaggaaggaaattgaagagctgggatggtaggtttaaataacatgaccttatgatttcctggtgggtcacagtctcttggttgggtgcccttgtgaataaaggcatggattgggcatgcctggaggggccaaggccttttgagcggacgagtatgtttatatgaagaccctgtcacctgtctctggtatctgctaggcagctgtggcttgagagtgtgatattgagggataattgatggaaggagattgaatgtggctggcaggtaaagagatagggaacatatggagatatttagaataagagagtgtgagatagagcgcttttgctatagcctagccattctgttctctactaagtgttgcggggttaccaggttttctactaggctgtatgaatgcaaaaggtagagagatatatagggccatggaataaataccgaagtgttttctttggtatccttgatacctttcgaaagccgtgtaaggatctagataatgaatttcgtgaattgcagtctctctgacaagttttaaagaataggaacaattttaaaaagtcatctacttccataagttttttgacattttaagataattgaatttttttttttcagcttttaagttccagggtacatgtgcaggtaggtgtgttatataggtaaatgtaagccatggtggtttgctgtacaaatcaacccatcacctaggtattaagcccagcatccattagctattcttcctgatgctcttcctcctcccgccccttccgacagaccctagtatgtgctgctccctgcatgtgcccatgtgttctcattgttcagctcccacttataagagaacatgcagtgtttggttttcttttaatattatttttaactttatgataggaaggagtactttttaaagttggttgaaacattgttactgatctcaaagcactaccttccagttattctgagatactttttcagtctaagatctgatactcctattcctggtttgttgagagtttttgtcatgaatggatgttggattttgtcaattgctttttttgaatctcttgacatgattatgtggttttgtactttattacattattaatgaatgaattatatcaatttatttttggatgttaaatcaaccttattttcctaagctaaatcctacttggtcattgtgaataatccatttttttatcttgctatattcagtttgctaatattttaagaatttttgtttcactgttcatgaaatatattgatctagttttcatttttcttttctttcttttttttttttttttttacatctccctcctcttcctcttgatctagttttctaatacagctgcactccaacttacgatggtcctacttaggagtttttgactgtatgatgtttgaaaacaatatgagtttagtagaaacttactttgagtacacataccattctgtttttttgcttttagtacagtattcaataaattatgtgagataaccaatactttattataaaataatacacttttagatgattctgccctaccataggctaatgtaattgttctgagcacatttaagataggataagctaagatacgatggatgtttggtaggttaggtatattaaatgcattttcaccttaaggatattttcaacttaggatgagtttattgagttgtaaccccatcacaagttgaggaacatctatgtatctaattccatgattcagtaaattctttagactgccaaaatcctgtaatctagagttagacaagatcttaaatcaggttttgtggtccatcttgtagtcatgatcattctcactattagggaattcttaactttttgcatttgaatcaccgaggtgttatttaaaatacacatatggaatccaagctccagagactctgagtagatctggtgagtgattgtgatgcctgcccacattcaagaaccttagtacaaaagccctgctgaatggttctctttcactatacactctatcaacttatgtacttgatcacactttggacctcaaaatcaataatttttaaaaatctacttcctaagttgtgaggtacgaattgaaggaaataatgaatactatttggggagtcaacattatttattaacgaataccatttggggagccgacattatttatatttggttggtatatttgtatcaactatcattttctaattaatggtataggcagaataaaccatcacttgtgattcagaaaggaacatgatacaaataacatccaataatgtatatggatttaaatagatctgccccctacagatgttacgcaattcatgttggtaatgatcattcattaggttttcgtggtggctacatttgatatgtgaagtactggctggaagactggtgccagtagcttcaggtttgctgggattctttcatcagagatgactagctttacttatctttttatgttgcatgtttctatgatgggcctatcctgtcattgtcttcatagtataattgcaagctcaactctgtcagttatgtgattttttttttttttttggtcctgtcttgcttttggctgacttctatatgtttttatttcatgtccttttcatagttagattaactgggtcttatgtccaagagatattttgatttctttgaatgaataaatctatgttaggctactgtattaggttttatagacacctagttgatcacttgtgtccagtctctattccctggtatggtagttgctgtgtttatagaacattgaggattctacaatggacacattggtgttgggccccagcccagacccaaatcgaaatttctagagccaggatcagagactctgcattcaacaaactctccagagatttcataaccacttttaaaggactcaccatcccaaaccttgttaaggaatgaaatatatgtctgccagtaatttcagtgctttaagtcattgaaagctgaacttttaatggcaccaaagtggaaatatttatataattgaaagctaaacttcatcctaatggcagtgttgagttcacttccataggccctgatataacagtctaatattattgtttttcacataaaataagattcagtcactgccatataattagggagtggctctgctattggatggacttaaaatatttcattatgtttgccaagctctgtctctttacatgttttataattaactgatccttcatttttattttgttttattttatttttgagatagagtctcgcttggttgcccaggctggagtgcaatggtgcaatcttggctcattgcaacctctgcttcccaggttcaagtgattctcctgcctcagcctcctgattagcggggactacaggtgcgtgccaccatgcccagctaatttttgtacttttagtagagacggggtttcaccatgttggccaggctggtcccaaactcctgacctcaggtgttctgcccacctcggcctcccaaagtgctggattacaggcatgagccaccatgcccggcctccttcatttttaataatcttcatagatacatacttgttgtactaatgtttttgtgcagttcctcatgataaataattaaatcaattactaaaatccttatagatttatgatgataataaatggaagtgtgtattattgaaacatgtttaattaactgttcatatataaccagtgagtagggattggcaattaaaaataccaggctaccagtgcatggaaatttgaagaaaacaacaacctgaaattcagaatactccaaaatctgaaactttttgagcactgacatgactaaaaatgctcattggagcatttcagatttcattttttcagattagggatgctgaattggtaagcataatgcagattaatccaaaatctgaaaaaaatcctaaatcaaaaacagttttggtcagaagctttgtggataagggatagtccaagctttttggactgaagctttttggataaggtatagcctataatacataaatacataatacaggataatcactgacctgaatgtatagcatcagtatggtacacaaatatttaaatccatgtactttgttggatattatgttatataaacttcttgtaaaaagtttagagagtaaaatcattcacattaccaaaagatttctcatatttataaaaaggattatagcagcattttaatcagtatctcctaaagtatttatttatgggttgttaaatctaaaagagaaactacagtctggagggctctaaactactgctgattacatatcagttgggaattaagagaaaatctcagatcataatatttaaataaaaacatttacatgaatgatttctaagttttcactttactagacaagaaactaaaattatatgactgtcatgttcaatattggatacttaacaacactacatccaaggaagccaggttttgctgattttaacctcgtcctgttgagtaactccatgcaggtacagtggtacaaacacatgtggacacacagacccagacctttatttcctcggggattctggtaagtgtagaggtgtcttgaccatagtcaatagcagaaatatgcacaaccacaagctctgaaattccatttgattgttgctcttagccttccactttttaggcatatgtcagtcccatttcatcccacccactctctccatttgggaggtggtagagtgagacaatactgaactataccagggctgagaataagtgtctttgaaaagggtcgaatctgtgatgctagagacagccctggaaactgtcaggagttagcccaaccaggactgtgaccagatcccaggctgtccaccacagatttgcaggctacctgcagatgtgactttttcaaatgtactcaaagacaagctgactttggctaatgcagaaattaattaattcctctttttcagtaaactttatcctcctacacttagattgtctgtaagtacatctctggagttgagctcaactagaaagaagctgtctgcatttagttaataccagcattggatgcacacaatataatttgaataatgtagagcaacattttaatcatctctcataagcagtttccccatttgcaacttcctgggaaatcttacattatgaaatgttcattagaactcccattttaaaaccctgctgccattttgtgagtgggcagaagaaaggctggagatgagatttgtctgtctcaaatgattcactccttcatttctggttcactccacagggagcttaaggacatgtgcgtttcatagacatgcctttcttttccttttatcaccttgttaaatcttaagattgaacatacaattcagcctgtaatcatatcaattcccatgaaaaatattttccttattcactgcctctatttgtgcttatacatctgatcatctttttcctttactttacaattagtttctatgaacagaagaatctgaaagatttaaagactagttagcacagcagcaatttataaatcattaatttgggtactgtctatacatttaatgtgttctttttcatagtcctatgtgaaatacatatacatatatatatattccactgtttataaacaatattcagttttatttgcataactcaatatattttatattaacagctccgtttttagtgtcttaagacatcgagtctgtttttagagatacagtctatttgccttgattttagcctgttataatcagcttattattatctggccactcttaccagtgagtatcatcttgaggctgttcttgctcatttcaacttgtcacaggggatgttttttactctttggagtttaggtacaccaggttattaattatgctcctgattcatggtacttccatcatggggcatataaggtccctgtctttgttttattcccttctatcttcattcaccactctcatttcctctctctccactagaaataattctcaggaatcaaattaatattattctggcttatatgtgtttttaaaaatctcatcgctttttatacatgtaattttaatttatgtaagagactttgtcctacagatttcattgtgtttcttctctttttcgcccagcactgtgtgttccatttctatccagtctactatgtgtacatcaagtccatcatttctaactgttgcatagttcatgatgcgaggcatcttccacattgtatcccaattccctaactggaatcccagttccctgctacctcacacaatgctccagtgaacagctggaaaatcatacaacccaaggaattattgaaagtgattatatcccagcaaaaggcccaggcccatcttacacttccaccccaagaaggtactgctacttttcgggaatggcctggtctccttggcgaaattggcatttgatctgttctcatcactgtcgtctggcatcagaagtgaccccacttgtcaggcactgtactcagtgctttccatgcactaactctgataacaatcttttttttttctttttttgagacagagtcttgctctgttgcccaggctggagtgcagttgtgtgatctcagctcactgcaacctccacctcccaaattcaagcgattctcctgcctcagcctccccagtagctgggactacaggcgtgcaccactacacctggctaatttttgtatttttagtagagatggggtttcaccatgttggccaggctggtcttgaaatcctgacctcaggtgatccacttgacctcccaaagtgctggaattgcaggcaagagccactgagcttggcctgataacaatcttgtgagcaggtgcttatgcagtattttagggatgtgaaagtaaggtccaaagcggtgaaataagagcctgtattctcttaacctccatcccgcaacatcttttatgtgtcagtccctgcactaagtctagggatactgtgctgagcaaaaactatcttcttgctttcacagagctcagtgtctggcagggggtcagactttcataatataaacccactaaatgagtgcatattgatggcggtcactgctgtgaagaagtgggaatggttagcatggaaacatagccccaatgggggcgactaagttctttcccatctcattctactatgtctactttcatctctacttttttcttttctgagctatcagctttcttgctctcaactatatttgatgtatttaaccagattttatatattgtattatgtattttataacatgtatatatatcatataacatacacatatacatacatacacacagccaattaagtctcaagttcaattacaatgcttctaagtttaggactattcattttcattttggcagagaaattatctggtaaaaaattcaagtagaaccaaaggtatacaatagatgggaagtttccttttcactctcacactctcatttccatccagggttctacaattcatctccttccaagcaattcctattgccagcttttcttataccctttcagaaatacacacacacacacacacacatatatacacacacacacacacacccttacatgtgtttgtacattatctctctttttacaaaattggcagtgattctttgtcctgtttctgccactactcaaaaattttaaaacaaattacacacctataaacatacaatttaaagaaaagagtgaaagtgaaaatctaaggacccagcacatggttaagatgagagcatgatgggttcaatggaaagcctttgtgtacctttctcctttgcctccgttccctctccaatagagtcaaccacgttggaggttatagcacttccttctttatgtccccccatctcccatctggtatggtattctcttttactgcagatggacattttggcagacatatgtagttgcttctctttggtatttacctaggagttgaagtgctgggtcacagggtgtatgtatatttcactttagtagatactgctgttgtaggactttctccttagtttagctaaagatggggtccttgtcccaaggccatgaaaaattaggctcgcagacaatttgaaaggtgagaataatggaacttattgggaaaaaagggaaacagggactccccacaaagccagggtcctgctagcatgcttcctgccttgcagattgaatcccaggtaccacccaggaagaggaggggccaggctcctccccactgtgaatggtgtgaccgtctgtggctccccagtgtgcactcctcccagtgtgcaggccggttggagtttctctggggtcttcttcccacttggctgtctcactgccaaactcccaaagtgcttataccagtttactctcccatcagtggtgtatgtatttgcttcatttctttgccaatactgatactgtcttattaactttcctcattctaatgtatacagtcttgtgttatttgtggtttaatttccctgagaaccaattatgttgagtaccttttcataggtttaccagctacagaagtcctcttgtgaagtgcctttgcaagtcttttgtctttttaattttttgcatctttgtatattctaggtataaatcctttgatacatatatcacaaataacttcctagtctatggcaaatcctatgttggataaacgtactgcaaatagtttcccagtctgtggctagcttctgtgtctgtgtcttgctttgtcactttcttactgatatcttttgatgaacagaagtacttagttttaaagtagttaaagttttctttatgttttatactttttatgcattttaaagaaattttttgttactccaaggtcatacaggttaaataaattcttactccaagaacattcttttaaagttttgctttttttcatttaaatgaaatccatatgaaagtgaactttgttatcaagtaacatatacaatttcttttatttttctgcacggagaccaagttgtcccatcaccatttattgagtggtctatcctttcctcactgattacagtgccagttttgatatgtcatgtttccatagatgaagaatattttggggctctctatctgtaccttcctttttaaaaaatataaatagtggtgatactatgaacaattttgtttgtattattgttttttgcacttaaaatttgtcttggagatcttttcattttggcacatacggatacacccctatttttttttccattttcctagatgtggggtatccattggacatatgtaccgtactgaatttaatatagaatgtcataaattacaagatgtaacattattttatacactgagatggagaatcaaactgcaacgcagtacttccctgatcatcctgagtgattcatgagttagttatactagcctcttatttctttgaggtgtacgttttctgagggaatctgccatttctcctgccatgagttgcattgcttggctcgtgataggcatttttatttttgcatgtaattttgtaacaaatgctaacactgctttatcttctttttgtttttgtttattgagacggagtcttgctctgtttcccaggctggagtgcagtggtgcaatctcggctcactgcaacctctgtctcccaggttcaagcgattctcctgcctcagcctcctgagtagctgggattacaggcatgtgccaccatgctcggctactttttgtattttttgtagagatggggtttcaccatgttggtcaggcttgtcttgaactcctgacctcaggtgatctgccccactcagcctcccaaagtgctgggattacaggtgtgagccaccagccagctttatctttttaaaggtttcttcctattgtgggtttcattagagggcttggttgttgctttgcaagaaaacattgacttgcttttgtttaatagtcttataaatatttgtttcactaacatcaaatacatgccatgctcctgcttttgagcttttctgtgcagtaacttttcttctcagtgctaaatcataagtttttaaagacatttaacatggcacactcaacatgtgtcaccaatgcccatagccactggaagtatcatcagtgtcaacagctatgacgtttggcaatgacagctttgccataactgctgcttagccaataacaattgtggaatgctgagtccagatctcaaacatgttaaaggtaaaaaaaaaaaaaaaaaaaagatattttcgagtctgtaaaacatggtagcgtatccggaattggtgggttcttggtctcactgacttcaagaatgaagccatggaccctcgcggtaagtgttacagttcttaaaggtgtcgtgtctggagtttgttccttctgatgttcagatgtgttcggagtttcttccttctggtaggttcgtggtctcgttggctcaggagtgaagctgcggacctttgcggtgagtgttgcagctcttaaggcggcatgtctggagttgttcgttccttgcggtgggttcgtggtctcgctggcttcaggagtgaagctgcagaccttcccagtgagtgttacagctcataaaggcagtgtggacccaaagagtgagcagcagcaagatttactgcaaagagcgagagaacaaagcttccacagtatggaaggggaccccagcaggttgccactgctggctcaggcagcctgcttttattctcttatctggccccacccacatcctgctgattggtccattttacagagagctgattggtctgttttgtcagggtgctgattggtgcatttacaatccctgagctagacacaaaagttctccacctccccactggattagctagataaagagtgttgattgatgtatttacaaaccctgagctagacacagagtgctgactggtgcatttacaaaccttgagctagatacagagcgccgattggtgtatttacaatctcttagccagacgtaaagattctccaagtccccactagactcaggagcccagctggcttcacccagtgtatcttgcaccagggctgcaggtggagctgcctgccagtcccgcgccgtgcacccgcactcctcagccctcgggctgttgatgggaccaggcactgtggagtgggggtggcactcgtcagggagactcaggccgcacaggatcccacagcggtggcggggggcgggaggctcaggcatggcaggctgcaggtcccgagccctgccctgcagggaggcagctaaggcctggcgagaaatctggcccggcgagaaatctagcgcggcgccggtgggccagcactgctgggggacccggtgcaccctccgcagctgctggcctgggtgctaagcccctcactgcccggggctggcagggccagccggtcgctccgaatgtggggcctgccaagcccactcccacccggaactccagctggcccacaagcaccatgcgcagcccgggttcccgcccatgcctctccctccacacctccctgcaaactgagggagccagctccggccttggccagcccagagaatggctcccacagtgcagcggcaggctgaagggctcctcaagcgcggtcagaatgggcgccgaggccgaggaggcaccgagagcgagtgagggctgggagggctgccagcactgtcatctctcagtagcataatttatataaccagtctcttgttgattaaccattatattattgatacaacaaatataagaactgttactagtaaattgagtaaagcaggaaaattaaatttggtctcttactgatcaaccattattagattgttgataacaacggttataatgttgatcaaccgttatattgttgatacaattatatttgatgtatttaaccagattttatatattatattctatattttataacatgtatatgtatcatataacatacacatatacatacacacacacagccaatataatttcactctcagtttcttgttaatcaactattatattgttgatacaacaaatataagaactgttactagtaaattgaataaagcaggaaaattacatttgggagccttaaagatgtaggttttcttcaagaaatttatgttatagttatatcccctgttgcatgtgaagacatacattcaaggatacttactgcagctcacacaatttgctgataggttggatgtgggtgtgagagaagagatgctgttttccttttgggcgatggcaactggatagtaatcagttactaagatggagaagaatgagaaagaagtctttttttgtttgtttgttggagtgatatgggtagaataaagagttaaaacagtcatgcatgtaggtactatagatgtgaaagtctattattcaggggagagtttggaatttaagggatagattcttgtctttaagcataaaaatgcctttgaaggtgagaaactagattacatctttaaggggagaactgtagatagagatgaaaagaaggcaaggactaacccctggggcaggtcagcatttagaagaaagggagtttgtaaaatgctaagctgtctgagaagtagcagcctgcaaggtagaaagaaaaacaagagaggtttagtggactggaaaccaagtgaacctggaaaccacaagcagctgtggcaaatcctgccacagtgagatgaggcctgagaactgagtattggatttgtcaatgtggaaggccttggtgatcttgataagcatgtgttagtagggtggtggggttgcagtgtttgggatttgagagagaatgagagaatgggtagctgtgatgctgaatatgtata[450 bp omitted]gcctagtcaactgagccaaactggatataaccacaaggtcaaaggcaggagccagtgaggagatcttggttttgaggtcattcctggtgcgataataaccatcctgtagcattttcttgtcacttagagaaggcattagcaaactttttttgtaatggtcttaatagtaaatatttttgactttgtaggctatatagctactcacctctgcttttatagtacaaaagcagccatagacaattcataaataaatgaacatgttccaataaaagcaataaaaacaggcagcagtctgaagtttgtcgactcctgatttggaatcattccagaaagtgaaataaaagcatggcttcttttttttttttgagacaaggtcctgctctgtcacccaggctggagtacagtggtgtcatcatagctcactacagctttgacctgctgggctcaagtaatcctcccacctcagcctcctgagtgtctaggattacaggcatgtgacatcacacctggctgatttttaaattttttgtattgatggggtcttgctatgttgccaaggctcacctcaaactcctggtctcaagtgattctcctgccccaggattcccaaagtgctggaattaaaggtgggggccactgtgcccagccaaagcatggcctttctaagggtgactcactgtagcacctcctgagtactttcctatcaagtatcctggaccactttttaaataattcattctaaaatccatatttaggattgattccaaatttgccaacctgtatttcccaaataactggcatgataattcttgtctttttcccaaatgctcattttccactcttcaaacgttgagtgttgactgaagttctgtggtcatgtttacagtcatttttatgctctttgtattgtacatatggaatgtatttaccatttctgttagcaatgatttcttgcaaaaacaataacacttgctagttttgcgtgcttaaaaatatcgagccctggcgctctctacatattatctaatgtaatccttatattaaccctgtgagtagtcattatcacttcttttacacaggaggaagttagagaagagtgttaagtgttcttttagtcttttccactttgtctttagttttctcttagctgttcttttaaattctaaggtcattcttatctaaaaacttaaaagagttgatcagcctttttatcaagtgttaaatttataccatcttttttctttgaacagggctggcaaataaacctggatttatcccttagccctgttacagcaagtctcagaaaatttggacttcagcttccccagtgatacattttcaaatgcctatgtatggattgcccattagtttattggctagaactaaaggaaatcaggcaagagacaaaggacattttctctagggtgtcagtcaatgcaaaatgttaggactagcatcagatttttttttttttacaaatgaaaataattgaagtgtggtagaagttcctctagttctggcagtcctaaatattgttaactgaagaatgatggggctcataaatttggaaaggagagagaggggaaaagagaacgggaatttatgctgagcagggtggctaagtatatatattcaacaggctataggaggagctattagtattcacgaaggggtggcacacacatacatagtaggctaacgtgtatgcagcatgcatcacaagtcactttggggtggagccttaacatttaatgtattacagttagggcctatacatcaaaaggtgaagcagaggacacgaaagccctctgtgttcagcctctgtagactggccagaaccactctgtggtcagaggtctcttatcaggaaagaattcttgttgttgtgttgaaactgcaaaagggaggggcagtgtcaggcaggtggttgataccagtctttcagaagcactggtttctgtttaacttttagagaagaaagcttaattggagtgttactggaaagggataccagtctagaccacaagagaggattcttggatctcacacaagaaagaattcagggtgagtccacagagtaagatcaaatcaagtttattagagaagtagagaaagaaaagaatggctgctccataagcagagcagcactgaaggcttctggttggctatttttatggttatttcttgattatatgctaagcaaggggtggattattcatgaattttcctggaaaggggtggggaattcccagaactgagggtttctctttcttttagaccatatagggtaagttctggatgttgccatggcatttgtaaactgccatggcactggtgggaatgtcttttagcatgctaatgcattataaatagcctaagataagctgtgaggatgaccagaggtcaatttcctcaccatcttagttttggctggcttctttactgcttcctgttttttcagtgggttctttgtgacctgtatctgtcttgtaatgtcctatctcatcctgtaactaagaatgcctgacctcttaggaatggagcacaggtggtctcagctcattttatctatcccctattcaagatggagttgctctggtttaaatagttctgacatattttccccaatacccccaaagggacccttaatcccaaaatttgcagacagatgaagatccatcttctgtagcttcttctggctgaatacaggtgatgatatttttgcgtaactattcagggtagagaggagctcagtgagaaagcatcagtatggtgaaggccattcctaactcccgagttctcacaaaaggtgatatctggaagattaataagtgttcaatttaagaaaacgttgagtagtcttatcctgcattgctacacaaagagtaccacagcaatatattctacaacagtaaagcaaaataagtataattatcccaactaaactaaataacaagcctttccatgaactaggcagttgttggaaccaagcttatatggggttgctagccaattccaacacatgttcagaattaaaatactgatccagatatttatgttacccttctgtttcttctgagcagcagctagagatcactggttggttcataggaacaaacagggtcaatctaaatggcagaaaaaactcgaaacaatgaatgggactagagttgaataacaagtataccatagtttctgaaacataatttttctctctccagtctcccatttctattgaaaacaaatcatggtaggactgatttgtttgcacagtaagctttagtcttattatgcttggcctggttatttgtataaagcatagcaataataattatttgccacgtaggctttttaaaaattgactttgatgtaactttgttccataagaaatctcagattagactttctaaagccttgagctgagacacagatttatctgtgcctgcaaatacttgtatgagttgtgtgaattctccttttgagatcccaagataactggagctcctaggcctgtcagaaagtgacattctttacttaccacaggtcaggaaccctgtaaaggaattgaatagacaaggtatgaggccagcttttcccagaggctttcatcagttctgtaagtcaactttgattccttaaagcaatctgtttatatttgaaagaatgccattccagtcaaagccctggtaaaacaggcagtgtctctaattgtgtcctgttacaaaggaaaacagatttttattgcacatatgcaaattactatgctgccataagttaagaatactcacaaatagttttcaaattcttgagaaatcaggtagaaagaaatatgctccaaagttttctcataggagtataatttactcaatttttaacaactgtaaatagctcaaaaaaaaaggtttcttgactctgaaaaatgaaacaaaggatcagcaacattttaagcaaaaagtcactagaaggttattttgttcttttattagtttagtccatgctgttaattcctgtttgctcaatatttatgaacatattggtttcccaagggagactcttgaaagtttttttcctctctatcttaatggcacactttacaaaatttttcagaaacctgcatttaagagccctctatctgattataaaccatcttttaaagaggatcaaaacaagacaacaattttctgtggataacataaagtcttaggaaagccgtggttaaagacacaattgactagaaattttggttacttctgtggcatacaacaattttacataacagttataattattactgataacataaactaagtcatatcagaatttaggagtttcccataattttggagcacataccaataacatatttatacaaatacaactcaaagaaagctaaacaccatttcatatttgacagtgcttcctgtatgattttaatataccaagtaagccaaatatgtcatttttggacttaaggggacctcatatctaaagtattgaccagatcaggaaaaggcataatatagaatttgattttggaaagtttgtcaaatatcaaagatttaaaacacttgatattataaaatcgaatcccaggtcactgtaaagtcatttatttagccaaaatgataatacaaagattttccaaaagcaaaatcctttttttttttttttttttttgagacgagtctggctctgtcgcccagctggagttcagtggcgccatctcggctcactgcaagctccgtctcccgggttcacaccattctcctgcctcagcctccggggtagctgggactacaggcacccgccactacgcttggctaatttttttgtgtttttagtagagacggggtttcaccatgttagccaggatggtctccatcttctgacctcgtgatccacccgcctcagcctcccaaagtgctggtattacaggcgtgagccactgcgcccagcaagcaaaatcctttactcattgatagagggaagacagctttccaaacaatgtctcactttttcttctttattttgttgtttattcaaaaggcaaacaaaaatcttccatgatcttttaatattacatgaaaattttgttcaagagagaaagccaaatttcatctttgcattaatgaatgtcaaatccaattcttaagaaaaccttgtagacaaattattcaatcttaatcaattttaccatgagataagattctcataaaccttttgtagtcctttacaatttttttttgttgttgttaaagagcagattaatgctctaagaaaaccctgttgtgcttttattccaatgttctatttatggaaaaactgaataataccctttaactttagctaatattttaacacacagaatttcttttacaagattaattttcactgacctcccacaacttactcaaacctttagctttatcctatgtaacttaaaacagtcttttaactctgtaaactaggcaataagaccacattcccatgccttcttataatcttttaccaaaaacacattctattttccttacacgccttgcaggtaacactgtttctctggtagcctcaattacatgtgctacaatgttaactcttagcaacttttatatttggtgaaaagtctgataaataagtggttttaattatgtaccaggtgtggagcctaggacgccagacagaagtgcagataaggtctgagtctttccagcatagctagggggcatggccaactccacatgtccccaggccctacctagaatctaatggctccaaagcaggtgagttgaacaattatcaagttaaagaagcagtttatggcattgaagcattcagcaaatctaatttaatctgacctaatttagaccagatgtctaaattttgaagacatttttattttaccaatatatttgattctctttatttcccaaagattattaaagtcccatgaattaaaaggtgttaaagtttttatttttctgacaaaatattcaatttaagtgcttatttttcaagccaattaattagagctcttttctatgcatatcacacatacaacacacaaaaatacacagacagaagacccagtagctgttaattttttcatttgccagcttttaagaatcttaattggattactggcttcagggtggagcaacgtgtggggacagagccgggaaaacatgcagtttctggggcctaataaacaggtgcagttagaaggcaaaacagattccccaaaattacagatctcatttttatattggattctggatcccaaaaagagggaatcagcccatcccctctgggagttttggaaggtgtagaagaatgtttccataccttctaggtggccaagagcatgcttctctgatccaaacgtgcacagagtggggtattcccctataactgctattagccttcccttaaagcatatttcctgcctagttattacacaccaaggttaaaagctctcccataatgcaaagtaatttctgatacccctacaagtaaaaaacattaggtaacacaatgcaaatcagagcaatgccttggattttgagagggatttgcttgccttcaattcctggggttccatgaggaaaacagatttttcccaaaatggagcctgtggtgctccctcagttttttctaaggaagcccaggctgttagaaatgatcttaggtcctctcaatgtgggcatcaagagtggcaagaaaacaaaatgagaaaaacaattcagttgactgagaagaaaaaacttttatctagaaaaaaatcaatataaaacctgccagatagatagatagatagataatcttggacatcacttttaattaagctgacttttaaccaaatctcttattatcagactctagccaggacaaacagctaatatttctggcttttgaactttaccaaaagtaacctcccaggtgaaaccaataagccttaactaaggttatgatttaaccacaggtgtgggaggtattttcaaagaggtggtaagcagtttttacaagatctggaacctccaaacatagctcagagaaaggaagattcaagacagggagtcagaagttgttcatgaggggaagataattaataaatggcaaaggtcacatagatatcaaaccagaaaggactcattcccgaagctaggaattgaatccaggccaccactgtgaaatagcaaagccttagttactgagctgcagtactgcacagtctccattgctcctccgagaaggagcctagagcagccaattttgagcttgcaaaggcttttaactgctcaagataatttttaggactaattgacaggaaccccaaaattcacaccctctggatggcagagatcaggagaaagtacccccacgtggttacaaggtcaagctttcaaggacataaaacaagacgagagggaaacttcatccagtttttgtttcagggacctgcagaaaagtttgtaactgaccagtttgcgggccagcttgaagaccagatttgtaggattcctaggcctgcattctatcctgtggctagctagggctgccataatagaatattacagactaggcagcttcaaccacaggtgtttattttctcactgctccaaagtctagaagtccaagatgagggtgcctgtaaagctgatttctggtaagagctctcctggcttgtagatggccaccttctccctatgtcctctctgggcctttcctctatctggccaagggagctatctctggtgtcttttcctcttcttataaggacagcaggcctatggattaaggcctcactttcatgtcttcatttaagtttaattacctctttaaaggcccgatgtccaaatacagtcacaccgtgggttaggatttcaacataggaattttagggacacaattcaacccataataggagggcattggaaggagagtgttccaggcagaggaagtagtgcagtagagcatatggaagtaggaaagtgaggagcaatggaaggggttcagtatggtttgagcgtggggtgtgtagagggtgaaggctatttcacccagtgcagtaagctctatcatccacaccggggttttacagtgggagaaaggagggtgtttatttgcaggtcaagaagcaaacagaatcagggagctcatgcttaagacctgaactccacagtggcttacatgtaaggtgcagaggttacaggcaaaggcatcaatcaacacatggaagccatatattggtttggcctaaaaaggtgggatatcctgaagtaggggcttacaggttacaggtaaatccaaatattttctgatttgcacattgtttaaggaaggggatatttgtctaaagatgggatcagcaggccaggtgtggtggctcatgcttgtaacctcagcactttgaaaggctgaagaaggagggtaacttgaggccaggatttcaagaccagcctagtcaacatggcaagactctgtctctaaaaaaaataaaaaagaaaaaaagaaaaagaaaaaaaataaagatggaatcagcagaaaggaatgttaggtctggcccatgggcggacttcctccagacttctcagaaagaaatttaagacaaagaatggtgccaggcgtggtagttcacgcctgtaatcccagcactttgggaggctgaggagggtggatcacttgaggtcagggatttgagaccagcctggccaacatggtgaaaccccatctctactaaaaatacaaaaactagccgggtgtggtggtgcacgcctgtaatcccagctcctcaggaggctgaggcaggagaatcgcttgaacctgggaggtggaggttgcagtgagccaagattgcgccactgcactccaccctgggcaagagagcgagacttgagactccatctaaaaaaacaaaatggaaaacaaagaatggtgataattcagtcctcaattccttttcttttttttttctttctttttttttttttttaactgctcctgcggagcagggctacctcatagccagtatgtccagagttgtctcagttccctcgttatctgtggtctggaggatccatatgatggtgatccaggttctgaaaaacaactctggaacatctgttaagatgttatctttagtttctataggaaaccaaacatcttctgactctgacctccttggtgattattttaagctactgtttccctttttgcttatcgagttgctcatttacttctcaaggctagcaggatgactggactttctcttgaaggaactcaagctgttcctttatttttatgctcaggggcggggggcactcagcaggtccctaagaggtatccccgctgtgtctcactatgggtgaaggctcagcgggaagaaagctagataccagttggaactctcttaaagtaaggagatcttgggtactttattaatatttttttcaagctttggtaaagtatgaaataactctggattaagaggagaagaactagaacttaataaccatgacatttgggcaaattgtttgaagcctcagtttcctcaacctaaaaataggaattataactttttgaattgttctgttgtatgagataatgacagtgaaatattttggagccaaaaagcaatgcatactattgggggttattattattttttgatctttcagcaagccagctatagtagcttttcctatataaacacagtatgaattcagtgccctcgctttcctgaccctcacagcattcaagccctgtatggaccgctgagctctcccttgaagcaccccttagtccagtattctttactattttcccctttaacaatttaaacttctttcaaaacaactggcagtagttttttaaaaaagaaaacaggctactcttcaaattaaaaaaaaaattgtcttgctttaggaaaaatgttcttctgtcttttccaattatcttatttcttctgcctctcatctgccttgcctaggcagaattattctcaagcctgcacatgctgctgtgcctctctggcttctaggccaaaacataggctaatagtactcttctcagctcactgagctctttcctgccgtcattcaaatcacctctgaaatcctgccttttgataaagtaatttctgactgatcagaggaaagtgatgattttctctgtgacatgtctttttattttccatcacactcagtgtcttgtccttctatgcaacatatccatgtatttaaaaacccttgtatatgtatttgccatgtatttgtgaggtatagctcgtgaagtaaaaaaagtctttatttttttaaacacatcatcatttcagcttcaaagtcaatgtggtctcttgagaagttaaatatgctgcatttgaaattttatgtttctcatttttcatgtttttttttaaagccccttttaattcctcatgtatttgaatattccaggaagctagtagagtaaaaagccaaagtgttaaagtgtttataaggaatgtgactcatcgaaattgactcacacaattcatcagctattgtcatccatatgttctcattatttatgtggcttttgctttatttaatcagatgactgaacttatcatcgtgggattttgcttgtagttgtttaatattatataataaaatactcttgtgtgaaacaagttaattgactttttttaattaaaaaaaatttatgtgagagtcaggagttacatgtgcaagtttgttacatgggtatatgttgtgatacaaagattttagcttctaaggatctcattgcccaagtagtgaacgtagtacactataggtagtatttctaaacacttttcccctccccctcttttggaatccctagtgtttattgttcccatctttgtgtctatatgtacctaatgcttagctctcacttataagtgcggacgtgtgatattttggttttctgtttctgtgttaattcatttaggatagagagactccagctgcagctgtgttgctacaaatgacatgagttcattcttttttatggctgcatagtattccatggtttatatgtatcacattttctttattcagtccaccattgatggtcacctgggttgattccatgtctttgttgttgtggacagggctgtgataaacatatgagtgcagttacctttttttgtataacagttcataataaaatactcttaacagtagcacagaatttagattgcttttcaggctagaagggataattgaaacatagaaaaaaataatgactcctaagcatagaaacagacccaatcataaagctctcttcctctctttctgcctagtgttagatcttattcattgtcttaaagcactgtgaccattttcagtgaaatcacagttttattcatgaaaagacaatgaattggtgtaagtaatcatttgaggatgaaggtgactagtctgtgatcaacaccagtacttgaagtacttgtaaaacatgaattgaccttggttaaattgcagaaaataaagtattagtatacataaacacattttctctcagcattgaaaagttatagtctataatttacctgcttgctaagaataaaaatattacttagaggtttatcaagaccttttttctacaaatggatttaatgtacagaattattccattttctatctgtgctctgtatactaccacctagtggaataaaatgcaaatttacctgtcaaaatcaggagaagaaaatgaaccaggggaaatttatttcaggaaaaaattttcataacacgttattgttacttcttttagtataatgtagtttgcataaaatacattagtttggagtgaaaaaagtcccagccatttttgtgatagctattaaaatgctattagtttgtccacaaataagctattctattcagaaacttagaagctaggtaaattattgagatgatgccagcatattatatctctaaattatgttaagaagcttctctaaattcctcatcactagggtgtattagtccattttcacactgctataaagaactacctgagactgggtaatttatgaagaaaagaggtttaattgactcacagttctgcaggcttaacaggaagcatgactgggagacctcaggaaacatacagtggaagaaggtgaaagggaagcaaggaccttctcatggcagcaggagagggagagcacaggggaagtgccacacacttttaaaccatcagatctcaggagaactcactcactctcacaagcacagcagggaggaaattcacccccacgatcctatcatctcacactgggcccctcctccaatttgacatgagatatgggcagggacacaaatccaaaccgtatcataggatttgttaaaaaaatctaacatgttctgcttcaaggcacccatgaaatgaaggtgtcatttcttaactgagaggttaaataaaagtgcagagataagatggttaagttttatcgtagctgggaagaaaagcgggtgtgtgtattatgcttaggtttttcctcccaaacaatgaaacccaaaaaggcaaatgaagctttaaggcgctttatcctttactggtaggatggtcctcctttaatcttcagtctctgttaaagaacaaacacaagctaacaatcaaaacctgttgttgcttgctgacggatttctctaacatagtcttccatcaaccatcataggtttgttgtggccacccaggccctttggtcgtcatgttcccatggaatgctaatgaaattaccttcccatttcctaaggtgacatgcctttcagatggcattggtgtgtgcttgtgtaaacacatttttttgtgctcatgaatattttacctgcctgattttggtgatctgagtgttgagcagtgggtgagggatggtggggcaatgggtagtaaggggaagtttaattgaagttcagataaaaatatccctccagaaacattacaaagccacaaaatcagctgaagttgagtcttctattgtaaagattctctttcttctcctgacagatccccattcctatccaggtagaccaggctctagtgaagattggacacaagtggtttatatcccgaagctcttaacctaagagtcctgccttgtttttttacttcatgtggtcttatattgctgaggatagcccagtgatcatttctaccttaatatgtagccttcaaaacgttgggtctctcagttttcttccttaataaacaatgaaccctaattatttataactgctcttgtgatggaggaattggcatgattttgcattgtgggcttctggctttacagtgtttgtgggaaagatggtcttctatctttgttatttataagtcattcattccctgtttttttgaagatattgttaaataaaaaaacttcagctgaattaaatttaaaagtttttaattgagcaaagaaccattctcaattcgggcagccttcccatccagagtagtccctgtgacttcagtgcagccacatggtggaagaggatttatggacagaggaaggaaagtgacatacaggaaacagaaaagagattcagaaacagctgaattggttataactcagcgtttgccttatttgaacatggtttgaacagttggccacgtttgattggccaaaactcagtaattggcacaagagtaggctaccatctgtttataatgtccacttaggttatagttcatgatgtgcaaagaaacctttaagctgagcttaaaatgtaatgaggcagctgtaggctaaacttgatttaacagtacttatccctctgttgaaattgcactcttgctacctgctagttgatgtgggcaggtgtgctaatgacacattcgcctgcacctaccacctgctgaagaccctgccatgtcctgaagcagtcacttaggctatgaaacagaaggatgagttagagaagtaaatattatattttaccccccaaagcctaaaaccatgtctaggttctcccctttctcaattcccaatcatgcaaccttgaaaggtgttatatagatagttgttagaaatatgtctgtcctccaaaaccctactaacacgcaaaaatggacaaatctagcttttttgctaaaatcctaacaactcagaaagcaaagcaaaatgaaatgtatgtactccattctcaggatttccttcttaaaaaccactaggctttgtgtaactcaattttaaaagtatggtaatagctcctgtaattcgatggcttcttctgggagacagatataaatctattctagactttaagactggtgtccacattttaagttacagttgtatgtacttctactttgttgcagccttctcttggagtcaagaagcctaccaaagccctgctctttgtactcttgagcccagtgggaccttatttttcaagtggaacctttaatccagtgtccctgtgggccaatcccaagtatgtaagagcctggaaaggtggaactggggactgcaagatgggagggtaagtaaatctgtgtctctgtctaaaggaaagacaccttcatgaccatttagttagtgccatttcacttcagtatgaacacatataatacttttcaaactttaatgctcattgtgtttcatggttaattttcagtttaatctttcagcaagccagctgtagtagcttttcctatataaacgcagtatgaattcagtgccctcgcttttagatgtgctagtttaaaggatagcccatggccctttgtaagggagaaacactggatatgatatctagggaagaactgaagtaagaaactacaacaagcatcacatcggtgctttggataaacttcccctgggcgctggtctctggctgcaggctgacggctggcattaaaaagcatctggtcctgggacccaggctctcagttggctccagggagtcatgtctggggaaggtgcccgcttcactgaagtgctgtcttcattgccacagattgtggccacacctgctgccaactggctgcgggacagccctgctttggctctgtcaggccagtctcataggccatatgtagctggcaggaaataaaagagcatttgaaaagtgttggacgatttcaggggtggacttggccatgagttgggaatgcccctatgggtgaacgagaataactggtttaagcagcatgggttcttgctttgcatgtatcaaatggtgctgtttgcatactcagggcagcagctgtcctagaaggtgactccatggcagtcttgtgggccctggtaggacatttaggtccaggaggcaggggagagtcacatgacgtgctgctggggtattagaggcaatgaccactggctttgacccctctgtagtcttgctgtatttcctttttcttttctctcctcacctacccaaattaaaaaagaacggttataaaagtcatccccactggcaactttagcaactgcattccctcaatgggtagagaaatccaaatggagtgcattaaaactaggaagtctattctccttctggcttagagcacaccttcctgtgtcctaggctagccaggttgaaaactcctttttttgactcttgatttctttttttactggttcaaacttcttcgcagagcatgtgcctatgtaccactgcataccatatatataccatatatagagagtaaataaacagtcttgatgaaaagtaataaggaaaaagtttccctgtttaaaatattgctttctagctccccgacctgtttaggaaaaagataacctggggacacagaaattgcagggcaatctttattaaccggtatttgggcaggttgtaatttattttgtaaacaatgatttaatgcactattgcagaatacatgatcactgtaggccagttaaaaattaatgttttcagtaccacacagagtgaaccctaatgtaaactgtggacttgtggaccacactaatgcaagatgataataagaagaaaaactgagagggtgttcgggaaggggtataataggggaattctgttaccttttgctcaatttctctgtgaatctaaaagtactctaaaataataaaatctattataaaaatatttgattcattaggctcaggtggactatgatccatggaaattgacttgaaatctcttaggaaaggaagagaccggagaagaaagtattgaactcataaattaaaaatggcaagagggaaggtggtaaccaaaaggatgggcatttaacctatatgcctatcacttccaaaaagttctagggccgtctcctcctatgcttctgacctggagaggtacaaggggaacaaaatattccgcatttaatattatcctgttgagttggcaaagacatttggagtcaactttagttttgtgtattattacatctgtaaacctaattaagtcaacagttacccttgacacctgtagtcaactggtattattaaataactattgagtctcataaagtcaagaactttctgctttctatctaagtgaatctagggcagagactgagcatcaggattctttagcatgcagccaagcttgagaagcactgagctagagaaaggtcttgcactgtagaaacagctttagttccaggtgattccttggttaatttgggaggaataaggctttctgtcactctctctctctttctctctttttctctctctcttgcacatgcacacgtgcacacacacacacaaattatctctcttagttttttcttttttccttgcattctgattctgcatttaagagtacaagctttgaagtcagaaagacctggcttaaaaacctaactgtcataatggtgcgtaaatgtcgttatagatttgtccaaacccatagaatgtacaccaggaatgaacactaatgaaaactctagacttcaggtgataatggtatgtcaatgtggttcattaatttcagcaaatgtaccactctggtgtgaggcattggtaatggtagaaactattcatttggatggggagaaagggatatgggaaatctttgtacttgcctttcagttttggtgggaacctaaaactgctctgaaaaaaacctgaagtctttaaaaacaaaccaacctaattgccttgggcatgttacttaactgctctatgtatcagtttcctcatttttaaagttgaggcaataataccttgcacagattaagtgagataatagaaagtgcctaggatagtacttggcatatagaaagctctcagcaaatgcagtatgataacctaatggttaaaagcttgggtttaggagtcaaatgtctgggagttacacacttaactatctgtgagatcttctacaactgaatcctctctccaagtcttccaatgaacaataaagtctagggttgtttttagatgactcaatgaaataatgtagttaagtacttagcacccagtctggcaggtatgggttgcatatctcttatctgaaatgcttgggaccagatgtgttttggatttcaaattttggagtatttctctttgggcatccctaatccaaaaaattcgaaatccaaattgagcatcatgttggcaccgaaaaagttttagattttagagcatttcaaagttttaaattagggatcctcaacctgtagtaaactctcacagtcactgatgttgtgaggttttctcactttctcatttcatttcctggactctctttatcttagaagaaatcagttaaattttacataatagaatttattcttttggagggatgtatttaatatgtctattctcccagataacctatttaaaaccatattgaaatgtttctatgtcaacagctttcttactttttcatttttctgtttcctccaagaacatgtttctcttatgaatattggcagcacatgggcgggaacccaactatattaccatggtatcagttatcctgtggacattaataatacagcttacacctgtgagagaactctgggaaaattaaaacttgtttgggggaataaagaccatctacagaatataataatacatcaatcaatcaattaaaacttaaacataaaaaacccttttcttttcagtgcattgaaatagtcactgtctttaatcctctttccttgctcagtgcttcatgaagctgaggagccatggttttaattcagctacactttcagaaatgtgtatgcatttgtatttagaagcttctttgaaaggctaaatattcatcctgtaagaattctctatgtgttttttaatacagtctaaagggcattttgtatatgaaaaaataatttattttcaggtagggtaaaacttcactgcttcactacttcgtagttgtgtctacgaatgagaaaaaattcaaataaaatagttattattattagtttttagagatgcagtcttgctgtgttgcccaggctggtctgggacttctggcctcaagccatcctcctgcctcggtgtcctgagtcactgggattacaggcatgagccaccacaccccactgaaatagttattttttaaaaaacttaatttcattaggatgtaacagtctcatgtaactcatcctttggcttttattgttattatttattttttccaagcaacccaatgagatatataaagcagatatttttatctgccagataattaaatgagggaaaaataaggactaacttgcttaagttcacatataccaaatagtggaaatgcaagagctgtcctcaggtctgttaacaacaaacctgtggtctttctaccagacgtcccctgcaatctggtttatactcattattaaaaagcatttgtaatttaactcagttatctatttactatcagttatgaataaggattatttgactttttatggtcattaaacaatagcttcctatctgttgtctttgtctttttaatttttatttattttattgtttttttaatagcttcctatctgtataccagacttgcttcatctccacattgaccaagaatttatattttgtcatctgtatttagaagcatatgttttaagcgtcttttaatggctctttttttttttttgctgggaggggacagtctcgctctgtctcctaggctggagtgcagtggcaccatctcagctcactgcaacctccgcctccctggtgtgagtggtgctcctgcctcagcctcccgagtaggtgggattacaggcgtggtccaccaaacccagctagttttttatatttttggtagagacagggtttcaccatgttagccaggctggtctggaactcctgacctcaagtaacttgcccacctcagcctcccaaagtgctgagattacaggtatgagccactgtgcctggcccttttaaggactctttttttttttttttttttttttgagacagtctcactctgtcgctcagactggagtgcagtggcgcgatctcggctcactgcaagctccacctcccgggttcacgccattctcctgcctcagcctcccgagtagctgggactacaggcgccagccaccacgcccggataatttttagtatttttagtagagacgaggtttcaccgtgttagccaggatggtctcaatctcctgacctcatgatccggccgtctcgcctcccaaagtgctgggattacaggcgtgagccaccgcgcctggcccttttaaggactcttaacattaccttggtgtgagtcaacctcatcgtgctccaatggcaatcaccatagtatgatgtctattttccacagcttactggaatatttcagctattagtcaatattctttcagttgcaagtcagaaaaccaacttgaaattattatttatttatttatttatttttttgagacggaattttgctcttgttgcccaggctggagtgccatggcacaatctcggctcactgcaacctccgcctcccgagttcaagcaattctcctgcctcagcctccagagtagctgggattacaggcatgggccaccactcccggctaatttttttgttatttttagtagagacggggtttctccatgttggtcaggatggtctcaaactcccaacctcaggtgatctgcccacctcagcctcccaaagtgctgggattacaggcatgagccaccgtgcccggcctggaaatgatcttaagcagacaagggcttatgaaactaggatgctaggggctaaagcaattatttccaagtttcttgtgtcctttgcacatccccctttttcttcccttcttcctctgcctctggtcagagcttctggctccatgttggcctagggctctcccacttcagccgctttcttctgtgaagtgtggtgatcatggacacagccgaccccagttttacagcataccaagtaagcaaccccagaagggagaaaatgcctgtatttcaggttatagacattaaaatgagtgaatgcacccaaaaaaggaatcatgtgactgtcttaggttatatgcccaccctttaactcagctgcagcagggcaagatgctatattgtcatcagttgtggtagggcaagatgctatattatcagtccaagcagaatgacatagctctatagaaagactatgtttttataagagtatggaatatagtgcagatgaaaacagtagatatacactaacatgtggctctaatgtttaatttttattttttttgagacagagtctcactgtgtcacccaggctggagtgcagtggtgctatcttggctcactgcaacttttgcctcccgagttaagatgattctcctccctcagcctccctagcagctgagattataggcacccgccaccacgcccagctaattcttgtattttcagtagagacatggtttcaccatgttggccgggctggtctcgaactcctgacctcagtgatccgcccatcttaggctcctaaagtgctaggattacagacataagccaccgcgcctggcctcatgctcaacttttatttagacaacagtacaaattgtaattttacccagatgtaaaagagtctaagagacctaaatagatattttgtggtagattacattaatgtaatgtaatgtaatgtaggagttttacattactacatttgtagttgttttagttgtttttcattgtttgtttctgtgtatttctggggatttcatggtgcaacaggaggactagagtttattcccgatccctgactgtcttacggcagtacttctcagacctactgagttatacaaccaggggtgtagggaggcaagcagtcatcacatttatttgaggactctcatgttttgtctaaaatattcatccttattttataatatactccataattttcccatataagtttagataaaagatgataccttaaaagtattataacactaaattgtcattccgggaaaatgtgctgtgttcctttcattttaaataatctgagatgaatggtgcaggctgagaaaaataggcttttgaaatactttttggtcaacatcgagacttttaacatttgtcctatcttttaggggaatttagacattgggcattatgtattccttggatacattaaaaggtgttagataagagcgctcacacttgctgctcttctattgcaacttgacagaagttacttctctaaaccttagtttctcatctgaacaatggaaataatgatagtgtctatctcatagtattggtgtgagatttaaatgaaataattcatgtaaaattgcttggtgtgtggaaacatagtaacttttaactgttctcattaacttggctatttacctgtgttcttctatcattacatttcaagttaaaatttcaaggtttcacgttgttctctctccaatgaatgcagttaaatcacttagattttctaatgagttttcctttaatgttatgcagttgactagagagtgtatatatattaagaacataataccttcactatgtccacatgtgaattaagagcttgaggctatcagagggtagaagatgagggagtggggatgaagtatgtttgtaacctgtgtattttctctttcttaaaggaattacggctcatctctttttgcccaatgtgaagcagtagataatgggtgtcagcaggtcctgtggctctatggagaggaccatcagatcactgaagtgggaactatgaatctttttctttactggataaatgaagatggaggtaatccactcagatttcactgtgtgcatttctcagtcattttcaacaggaccagaaagacaagagctagaaacttagtacaagggagtaagtagcacagttccaaaggctaagtaaggactactgtgcttttgctgcccaaatagacacaagtttcttttttttctttctttcttttttaaagaggtggagtctcactatgtcacccaggctgcagtgcaatggtgtgatctcagctcactgcaccctggttcaagcaattctcctgcctcagcctcccgagtagctgggattgcaggagcctgccaccatgcccagctaatttttgtatttttttttttagtagagatagggtttcaccatgttggtcaggctggtcttgaactcctgacctcaggtgatccaccggccttggcctcccaaagtgctgggattacaggtgtgagccactgcacccggccgagtttcgatttaaagaagctctagaggttttttgtttttcgttttttgtttttctggctctagatgtactgattattgagatactgagatgtcacattaagggatttaagttaccatgattggaagatttgcttccttatcccttctgcagttccccaacaattttcctatctgaacaccttgcattgagacacaggtctcagatcaggtcaatggtcattcaccatataccgtatataaaatgctagagtaataaatgcagtgtactgattctactggaaggattttgtgtactctctggctgtaattgttttaacaattgttgccttttctacatattttgaaaatgtatcacaatctctccaaatttactctagaactcaatctgattaaagagcaccattttaaaagataaatcaatgtatcttgggattgtaactagatcctggttcattcaagacaatttcatatatccactatagatatcaatatttctctattatctttaatatcctgagtactcattacttttctttgctgtttttttttattagttggcagagaccataggggttcagtgaagtgttggcaacgtgtatgatattgaattaaatggccaacggtgggagaaaaacaggcatttatttctattagaattttgataatcataccaaatttagaagcgtatttttagacttgtttacattcttaggttgttcatttcacagtagtaattatagagactagaaatataaatgatgtttccaaatacttatgaagtctcagtgttagtagtttcaattaaattttttaaaatgcagtttatatttgaaagtagctacagtagcctctcttgctctaatgttatttggctacaaaaagaggaaaatggtaatttagatgtggctgaattcagagctaagtactaattttagtgttagttgcagagactaacaagatgagtcttatactgcagtcagaggtagaataaacagaagatatggtgagtaagccttgtcctgggcttggccattggtagtccttggcatatgaaaaaccagatacagatcattctcatccttccattcctgctgtttgtacttggcactgtttgaaaataaaatttatacaggaatatttatgatttataaatttgagttactgtatgtgacatataacaaaagctacacttggaagattgtagccagtgttgacctctgcacttagaagataataggccgattcaacccttcttcccatctgcccactcttacccccaccccaaactccaccaaaaaaccacacagctcaaaacaaaaacagttacatcattcagaggtggtaccatcattatttttatggatgggagatgtcagaatttaagtacactctgaatcagagctacatgatttaaccagaaacaccagaaactgtcctggtggaaaattgttctttatccaaacaataatcatgaaacatttccaccatggcttttaaaggtcagaatagaaatgagtgagtttgtcttctgcctcttgcaaaatatacaagaccttaagactgttagttactattcagattatggttgcctgggataactttagttttaatatactccttcactttggggatgttcatctaacagaacaaataaaattcagaataaggagaaaggaaatagaatatatatttgaagtaaatagaatgttaggaaaaacctttgggctaaaaaaaaagacatgcaattctgaagtaactttgatttatatcatatgattttaagaaaatacaatgaacaaacgagttgaaaatcagcacaatactgattttcacaaacgttaccgataggaggtataaacagagttctttcggtaatagcctgccgtcttttcatgagcgcccacacacactgctcctgttggttgagatggctggtgcaggaaggtggatggggtggtggatagtgtgtgttcaaagcacagtgctgtgcacagtcactatgtgtggcactcagcttgtaactcatgggagttttgatttcagtaacagcacccatggtggcaagatcacacatcatcactctgttgatgagtaatttaacccatacgcttgctattcaccatttgaacaaagcattgtatcatatcctggaccctggagataccctgaaaaataagacccaggccttgtggttgagttcacagtcactttgggaaaacaaccacagcagtgaatctcggtattgctcaggccacatcatgagtcttctcggacacgtcaggcgtgtatacggactcgacttggagcactcttcctcagatgtctgtaccgcttgctctttgacatcctccaaatctttgcttacaaatcccattctcagtctggctttccttgagctcttaatcaaaatcataaactccatttcccatttctcctcagcattccagcattctccattgcttttccttctttgtttccccctgtgtagtctaacatactatcaacacaataaatgtttacctgtgtctattagaaagtaagcagggagatatgtcagttttgttcactgctgtattcatagagcttaaaacggtaaacagcactcaatatgtatttgtagaataaatggctaattgtgctgatggtgtttagggcacttatgcagacctacattcctggtttccattagtgtttgactttgggaagtcacagatgaatcctgctgttattgcttctaaattcctcatctcctaaaaatgacttctttgtcaaaaacaagctgcatttgtaggttctgttttcctcatgttgggcaatctggagtgatttctggctcttgtaagtatgtttgtggttgcagaggaaaatgaatatttctcacccaaatgttgtcatgtcatcatctctgtctggcaaccagagaagcagatgttctgttccttgacctcaggctagtggttacagttctgggtgttaaacatgtttcacaaaacagcacttgcacatgcggggctgctgttttcatttaacttcatgtagtctcagggctcagcaagctttaggaaaggtccggtttgggggcactggaagtgtgtgtgtgtgtgtacatatatatacacacacaaatagatccatacatttatgtatctagttggctagctattgcaaaacacatgtttattttgagatcatcaacacttctaaacatgacaaagagtagccctaagaacattgccaagaacaaattttctcctttccagaaagcaattttcagcagatgattttcagaaacaaaattcaaaaaagccatactgctgtatcctagcaaagataacttattcgtttattttttactcaaaaacatttattatatacactctgggctaggcacaatgcccagttttgaggatagaaggatgaagatagagtttggtattccagatagagcttgattgttgggcatgtctgatgtaaccccagtggagtgggcgagcctagaaccaccatgtattgagggagagggtggtggcctcagtgtcaggactcactagattcagactcctgggtgtcagaagtggggaggaaagggagatgctgagtgccagagggtactgtaaggagagcttgtgcagctgatggatcatgcatgatgcctgtgaacaattgtcctactagacctcacagtagttagggatgtctgcagtcatctcacagtagagcagtagctcagctttggagttttgtttcttgaatgtcttcttttttaaccgtacacgtgcttgagctcactctgataagcccattacatttgaatctcagagagcaaaggcagcatctccatacttgttgctgatgctccaccaggtttgaaaatcactaaagatagactcttaggctgggtgcggtggctcacatctgtaatctcagcactttgggaggccgaagtgggcagatcatctgagctcaggagttcgagaccagcctgaccaacatggtgaaaccccgtctctactaaaaatacaaaaattagccaggcgtggtggcgcgtacctgtaatcccagctactcaggaggctgaggcaggagaatcacttgaccctgggaggcagagggtgcagtgagctgagatggtgccactgcactccagcctgggtaacctaaaaaaaaaaaaaaaaaaaaaaaattagactttccaagggcagcgtggaagcagtgaccagcctgagtaggcacgcacacttcttggggatagcctcctccatagcattcttagaaggtttggtaatgaccagtttttctgagtaagaccctatctacattattctaattagtaaccacctttcatctgctaaggtaaattttcacttcagaatattcctcttaagaccatgcaataactcttactgtttgttggtggaaaaccatctcattattttactggttaagggtaaactgaagatgattagataactttccttccttccctccccccttcctcccttccttctctttcttccttcctttctccctccctccctccctctctctttctttccttctctctttcttttcttttcttttttctttctttctttcttttttctttcttccttccttcgttccttcctccctccctccctctctctctttctttctttctcttttctttctttctttctttctttctttctttctttctttctttctttctctctttcttttctttctttctttctttctctttctctttccttccttccttcctttctttctctctctctccttccttccttccttctttccttccttccttctttccttccttccttctttcttctttttttaaataagggtctacctgaagtgtgaactgatttgggaaatttgatcatgcagaacagtaaaattttctttatgtttgttgctagcaaaattgtgatggttttttaaaaaaatggctattgataataaggcatgcctaatgtagtgaaagtttgaaaatgtcccaatttctgattgacagaagaagaactggcaactcctccactagatggcatcattcttccaggagtgacaaggcggtgcattctggacctggcacatcagtgggtgggtgcctttgatatgaacaacttttgtaagcctgaaataaaaaataatcaaaataagcccagcctagtgttgaaataatatcctgtggttccaaccaatgttatctaatctttaaattctaacgtgaatgaaaagtattcttctagaagggctttcttggcaagactattaaaataagtattgttgatagcaagggcagagagaaaccagtttagcaagatgtcatagtggagaagtattctagtagtagtctcagtctaccaggtatctcccaccaacttttgtctggttcatacctgatgtgcttccatccagacattccttaacttcccaagtctgtgttgcttccaaatggcaatgatacttcttcctttcctttatttataccagtgtaaccatgcttgccgtagaaatgaaataatttcactgacatataaatgtttactaatataacattattggtttgactgccttctttttctctctgtcctacccccatcctccaaaattcatatacatgcctattttaaaatcagaacatgcaagcaaatgtaaagttgttttcagtagactttcaaattcgtgtgacacaggcaagcatattaaacaatttggtggaccgggtgcagtggttcatgcctataattctagcattttgggaggccaaggcaggaggatcacttaagcccaggaattcgagaccagcctgggcaacatagtgagaccccgaatctacaaaaaaatcaaaaacattagctgaacatggtggtacatgcctgtagtcccagctacttggaggggctgaggtgggaggatggcataagatctggaggtcaaggtcgcagtgagctatgatcaagccactgcactacagcctgaatacagggtgagaccatgtctctaaaagtaaattaaataaataaataaataaataaataaataaataaataaataaaataaaatttaaaaaggtttggttttggaaatgacgtaatgtattcaagacaaattattgaatgaattgggtgtctggtaaaggttcttggatggaacttttgacccaggtgttaaaatggtctccaaagaacatgaaaaggctttgagcttactgtggtcaaagagtactagtagtaataggacaaatgtttagaaacacacacgttatctaggagcataccagcatggtttctctggaaaagactttcaaaatagatgaaatgtgctataaataattctacaaaaccctgaagtagacaagacccaactgctacatgctggctggcgcattgggcatgacatttacaaaccgttggtataattttcaaacagcttgccctgtcctaaatatgtttgcaattggaaagatatttttgaagctcagtaatttttgttttattaaagaaaaatatcaaccaagtacagaaggttcgacgacaagttgcaagtggaaatactttcccacactaatgatttgctagcatgaaaaataggttattatggaggaaattttttcttgacttcatagctgtaatttattttaaaagctattttaaaacatgagacgtgaaatgccaagaggcatgtagggggtcaccactatttgccagataggggaaattgtccaaagataagtaagggtgagcagagcaaaaacaattctgcttatttacaaaagagttttcttttcttttctttttcaggacacagaactcagcttgttttcaattaatttgcctgattttctgcagttcatttacttttgaacaacataattgcaattgtagactgagagaaattgaaactttcaaagagccatatttctattgcagatatattttcctgctcttccaaatctacttacagcatgagttcttcttttaaatattcaaatattttgaatattgccaagagctttgatttccatttttatctcttgtgggtttataaattaagaaaaaatactcatcttatttttttaaacctctctatttttattgccctttattcaaataacttgttgacaaactttgaacttgaaccactgaggtaaaagaacaagaattaaacagatagtttaaacacatagcttaaaaggatctttttcccatttcctatccttgagcaaagaatatattcaaacactttggcagaagtcaatgaggttataccactaattccatgatgaaaatcaactgaatgtgatactgaaagagaaggaagagaattgtcactgtaaagtcaactgttagtcatattaggaaaaaaaatacatacaatacaatttctcaaataaagtccaaatatacattcaacgtttaaaaataatgagtatttcagatatttgaactcagtctgttctttattccataaaagatataggtaagccgtgcacagtggctcacaactataatcccagcactttggcactttgggaggctgaggtgggaggatcacatgagcccagcctgggcaacatagggagacccctatctttacaaaataaaatataaaatataaaacctagttgggcatggcagcatacacctgtagtcccaggtgctcaggagactgagacaggaggatcacttgggcctgggaggtcgaggctgcaatgagccaagattatgccactgcattccagcctgggtgacagggcaagaccctgtcttaaaaaaaaaaaaaaaagaaagagacaaacgtagaaagagtaccaaatttggagccaatcagatcagacctgggttcaaattgagtttctgtcacttacttcctttgtggccctggagatgcccttcaacctccttgaaccttagtttcctcatctgtaaaatggggatgatagtactcacccttaaaattacagaacttggcataatagcgggtgcttgataaatggtagctataattattaatattatataatacattgttctcctttatggtaaagtaggttttaagacactgatttttttgttttgttttgtttttggagacagagtctcactccgtcacccaggctggactgcagtgacgtgatcttggttcactgcaacctctgcctcctgagttcaagcgattctcctgcctcagcctcctgagtagctgggattacaggcacccgccaccatgcctggctaatttttgtatttttagtagagacagggttttaccaggttggccaggctggtctcaaactcctgacctcaagtaatctgcctgcctcagcctccccaaatgcagagattacaggcatgagccaccgtgcccggcctaagacactgttaacacggagcatgcatcaagcagcatttgggatgcatcaattttgtgagactttatacaagttaacaaataagaaggcaaaaaagaaggcatatgttaaagtataccatgtgtcttgtggtgataatcttatattttatattctgataatctcatatataaatctgtgaccttgaagtaggttacttaacacctcgatgtgttcaccagtaagatggtgtgccacttccagctttcccttaaaggatgattgtgaccttgtctaagtgcaatcagaatgttaagcagaacagtaagtattgcaattgttttgcatgccttttcctttaaaatatacttgttattttttatattccatgcagggtgaatttaaggtgtcagagagatacctcaccatggatgacttgacaacagccctggaggggaacagagtgagagagatgtttggctctggtacagcctgtgttgtttgcccagtttctgatatactgtacaaaggcgaggtacgacaagtatttcctcatttcctatcatttccaatcacattaaattacatttaatttaagtgtatgaataaaattgtatctggacccagacccaagatgcaaaagttttgtcgttgttgttgtttttctttattttaaagagatggagtctcgctgtgttgcccaggctggagtgcagtggctattcactggtgtgatcatagctcactgcagcctcaaactcctgggctcacgcaatccttctgcttcagcctcctgagttgctgggattacaggagtgcgccaccgcaccatgctaggtcttttttgttgttgtttttgttttttaacttggcactacaaaaaaaataactgggacagtttatccagatgaaactgtattagcatatatctactatgtttccagtgatttcatgtaagcttaaacatggtgggaagttagttttgtccttggacacgtgtaagatctgtcttacctacatgtcgggattggagctatgccgacagtcttctactcttctctcttccttcctaccagctcactagggaaggctctataggtagttacatttcagtttctggttaaccaaaagtacttccaaaccactggattaggaatggcaaatagttatggaaaatgcattcgagtggtcaatcccttgatttttttttactattaatgctgttatcattaatagtaagtagaccactttacaagaattattcattggcaaacctggtgcatttactaaaatcttacaaaaggaatttgaggatttggttggaagaaatgttctcctcttagtaaattagtctgattttatatgtgccatacttttgttttcttgtcaaattgttttgcttttcactttataacaaagctccaatacttatgattaacattggcatctaactttataacttaaaggcatgtaagtattagtcttataatgtgaactggcttaagttattcatattatagcagatccttgaacaacacagggattaggggtgtcaacccccatgcagttgaaaaatccacatacaactttttttgtttgtttgtttttttaaacggggtctttctctgtcacctgtactggagtgcaggggcacaatctcggctcactgcaacctccgcctcccaagctcaagcgatcctctcacctcagtctcccaagtagctgggaccacaggtgtgcaccaccacacccagctaattttagtattttttgtagagacggggtttcaagatgtttcacaggctggtctcaaactcttgagttcaagtgattcacctgccttgacctcccaaagtgctggtattacaggcgtgagtcaccatgcccggcccacatataacttttgacttcccaaaaacttaactactagtagcctgctgttcaccggaagccttatcaacaacaaaaacagtcgattggcacatattttgtatgttatgtatgttatatatgtattcttacaataaagtaagttacgaaaatcatggggaagggaaaatatatttactattcattacatggaagtggatcatcataaaggtcttcatcctcattgtccatcatgttgagtaggctgaggaggaggaggaggaggagggattggtcttgctgttttaggagtggcagaggcagaagaaagtccacgtataagtgaacttgtgtagttcaaacccgtgttgttcaagtgtcaaccgtaaatgcaaactccactggttttcaaattttactttagagttattttccctcagctgattggagttttgctcaactcctctgactttaataatggctgcttcatttgttgaggttttagaacttgcttttaagggattgctcttgacataattgcatcaacagatagactgtttcatgggagaagaattgttctgtttcatgtcaatacttacattgataagaatgcatcaaggtaatgtgatccatccactgaagttgtcattaggccagattttttttaagttgaattattatttcacttctagaaataagaagtttataaagtttagcataattttaatgatccaggcttaggaagcatttacagccaaaaagtaagtatatataattatcatattatactaaagggtataatatgaaaagtgtttgagagcacagactatctcctaaaatcaaactatcaaaacctgcaagccagcaaggcatgagtaggcatgactcagatacaaattagaagcatgaaatctctttcagccatgcatttaatcatgctatccaatattgtggaggtagtggcccctggaagtttaccttgggccagagataggtatagaagccccttttatgaagtcatagacttgctttaatttatgctcccagaatgacttgcattaaactgtggcaaaatatctttgagttctcatattagccagagggttaatatgtagaagacaatcattcatccttacagattctcagaatcttggaagaggtagggttctttaagtttagccactattttaggtaactgtagctcctccttggttcttcaaatgatcctgaaggctggtatacaaaccagttatgccctaaaattaattggtaggtaggcaatgtataacctgtcattggctagtttttattcaaattttggatatgaaagtctttggcataaggtgctagcactcagagtcagtaggttttagtgctattccttaacttcagtggaattgccttagtatagcagaattgcttgagtgtcttatctgttatcaccatatacatgagtaccctcaaattatctcatttccctttcttttgtagacaatacacattccaactatggagaatggtcctaagctggcaagccgcatcttgagcaaattaactgatatccaggtaaagcttttcttttcttttcttttctttccttttcttttcttttttttatgtcaccttatttctgtcagagcttacaactaaattatatttcaatgaagaggattaaataatacaatttgagatcaataagttaaatttaaggaagatattcccaacacaatgtgtgggcatgagcaaagcagaaatgggaaagaagatgtatgttttaaaaaaagaaagaaaatattgttcaggactccacattacttaacattaaaaaatagatgtaatttttggtaacatttaaaaatctcattaagaaggataacataacttttgttaaaaaaaggaagaaaaaatttgaaagtagaagcaacttcaggaagaaaattacagtgcatgtgattccaacactgagatataatcactgttaattttttatgtctttttatttttgagctggagtttcactcttgttgcccaggctggagtacgatggcacgatcttggctcactgcaacctctgcctcccgggttcaagcaattttcctacctcagcctcccgagtagctgggattataggtgtgcgccaccatgcccagctaatttttgtgtttttagtagagatgggatttcaccatgttggccaggctggtcttgaactcctgacctaaggtaatccacctgccttggcctcctaaattgttgggattacaggcatgaaccactgtgccctgccattttttgatgtcttaaccttcaatattttgtaagcatttatatactttatttatttatttatttatttatttatttatttacttatttatttttgagactaagtctcgctgtgtcacccaggctggagaacagtggcatgatctcagctcactacaacctccacctcctgggttcaagcgattcttctgcctcagcctcccgagtagctgggattacaggtctcatgccaccgttcccggctaatttttgtatttttagtagagatgaggttttgccctgttggccaggctggtcttgaactcttgacctcaggtgatccacccgccttggcttcccaaagtgctgggattacagccgtgagccaccatgcccagccagtatacttttagatagttattttttcctaacaaaatgggatcatattgtacataattttgttacatgttttttcactgaataaatgctttgcttttttatatcaataagtagttttctccaacaccatttataaagtttaattgaattccattatattgatgtaccataatttttttaaaaaattatattattgaacatttatgttgttggcaatttttttttcactagtatggacagtacatcctcgattacttcctaaggataaatctgggatcaaagagtatacacgtctattttttcatactgctaactttgttttgcctattttttttctgagcaataatctacagtaatgcctcatcaggcagttaagcaggcatgctaaataccagataacactgggctactcagaaaagagattatcctgtaatttgcaagcatttcacaagttagaagactttgttgaagccagttactatccttgtcaattagtaaaaatatccaagagggcctgagacttacattgaaaagtaaaataaagtttgatcatttgagtgatgtcggatggcattaagtcatgaaactaagtgaaacttaaaggtggctgagaatgcaacaggcctccagagagcaatggaggtccttgggtagtgataaaaatggcatttctggctgggtgcagtggctcacacctataatcccaacactatgggaggccaagacaggaggatcgcttgaggccaggtgttcaagactagcctaggcaacatagtgagaaccttcctctaaaaaaagggaaataaaataaaaataaaagtttaaaagagagtttaaaaggcagttttaaaagagacttactcagcaagttttctgccaaatttacagtattaaaaagaaagaaagtgtgtttttgtttctgtttgtttttttgagacagagtcttactctgttgctcaggctggggtgcagtggtgcaatctcagctcactgcaacccctgcctcctgggttcaagtgattcttgtgcctcagcctcccacacagcagggattatgggcatgcaccatcatgcctggctaatttttgtatttttagtagagtcgaggtttcgccatgttggccaggctggtctcaaactcctagcctcaagtgatttgcccaccttagcctcccaaagtgctgagattacaggcatgagccaccgcaccctggccttgattgtggttttttaatcaatgagctgccatacttctgctctccagcaaaggttttctatgagaattttctgtaagctaagtaaaggaatatcttaatattggaagaaataaaatttagtcagagttgttttctacctttgtacacagcaacacttacaagtaatttgaagagtagctaataaaaatttctgcatggatggcttaggcattttaatttttttaaggttgcctgagtaaatctgaaaataataaattattacagttttgctcaaataaagaacacaaatagaacaaaaaatacataactggctagattacatgaaagcctttttccaaaacagaggtttagaggccagggcaaataggcaggaaaaataaataaagggcatccaaattggaaaagaagaagttaaattagctttcttagcagatgacattatcttacacctagaaaaacctaaagactccctcaaaaaacctgtagaactgataaatgaattcagtaaagttgcaggatataaaatcaacatataaaaatcagtagaatttatatatgctaacagtgaacaatctgaaaaagaaatcaagaaagcaatcccatttataatagccacaaaaagtataaaatacctaggaatcaatctaaccaaagacatgagagatctatacaaggaaaagtataaaactatgatttaaaaaattgaagaaaacacacaaaggtggaaagatattccatattcatggattggaagaattaattttgttaaaatgactatactacacaaagcaatttacagattcaatgcaatccctattaaaatactgatgactttcttcacagaaatagaaaaaacaatcctaaaatgtatatggagctaaaaagaccccaaatagccaaagcaatcttgagcaaaaagaacaaagttagaatcaccacactaccttacttcaaaatttattataaaactataataaccaaaacagcatagtactgatataaaaacagacatagtagaccagtgggacagaatagagaacccagatacctaagtccacatgtttacaaccaactcatctttgacaaaggtgccaagaactgtaacggggaagacagtcttttcaataaatggtgctgggaaaattggataattatatgcagaagaatgaaactagattcgcttctcttaccatacacagaaatcaaatgaaagtatattaatgacttgaatcttagacctgaaactatgaaattacttgaagaaaacattaaggaaatgcttcaggacattggtctaagcaaagatctcattctgtcactcaggctggagtgtagtggcatgaacctggctcattgtggcattgacctcctgggctcaagcaattctcccaccttggctttccatgtagctagaaccacaggtgcatgccaccacattccactaatttttaaattttttgtagagatggagtctcaccatcttgcccaggctggtctcgaactcctgaactcaagggatcctcctgtctcagcctcccaaagtgctgagattactagcataagccactgtccctggccagcgaagatttcttatgtaagacctgaaaaagcataggctatcaaagcaaaaataggcaattgggattatgtcaagctggaaagcttctccacagcaaagaaaacaatccacaaagggaatagattacccaaagaatggatgaaaatatttgcaaactatcaatctgacaagggattaataaccagagtctataaggagctcaaacaactgtataggaaaaatctagtaatctggttttaaaatgggcatgagacctgattagaaaactcaacagaaaaaaaaatttgattaaaaatggataaaagatctgaatggacatttctcaaaagaagacagacaaatggccaggaggtacatgaaaaaatgcgcaacatcactaattatcagagaaatgcaaaacaaaaccacaatgtaaaatccacttgccctagttaaaatggcttgtattaaaaaaaaaaaaaaaaacaggcaataacagatgctgggaggatgtggagaaagggaaccatcatatattgttggttgaaatataaatagtacagccactatggagaacagtatggagggtcctccaaaaataaaagtagaactagaacttccgtgtgatccagcaattctaccaccgggtatatatccaaaagaaaaaaattagtatatcaaagagatatctgcactcccatgtttattgcaatagtattcacaatagccaagatatggaattaacctaaatgtctgtcaacagataaatggataaagagaatgtggcataaagatatatatatatatatatatacacacacacacacacacacacacaatgtggtactattcagccataaaaaagaatgaaatcctgtcatttgcagcaacatgtatggaactggaggccattttgttaagtgaaataagcgagggaccgaaagacaaacatcacatgttctcatgcaggtgctaaaaaagtagatcctatgaagacagagagtagattagaggttaccagaggccgagaaggggagtgggaagtagaggataaaggaaaaaaacaagaatataaatgtatttattaccattaaactgaacatttaaaaattgtaaagatggtaaattatatatgtgtattttatcttaattaaaattttaaaaatcaggagtttagaaatttttaagagaagtgtgcccatagtgataagaaagaaagacccttttggaaaattttcttgaacaaattatacagtattttcttaaacaaattgtacattctgtagcagttaatacaccaaataagatttcagggttacctcttggagattgtatgaaataaaaacatttaggtgggcatgatggctcattcctgtaatcctaaaactttgggaggctgatgcaggaacaatacttgaggctagtacttcaagacgagcctaggcaacatagtaagacccagtctccacaaaacaaccaaaaaaaatagcaagtgtggtggcacacacctgtagttccagctactcaggaggctgaggcaggaggaacacttgaggccaggaatgtgagactgcagtgggctatgattgtgccacagcactccactccagccttcactgtagaaagagaccctgtctcgaaaggaaggagggagggagggagggagggagggagggagggaatgaaggaaggaaggaaggaaggaaggaaggaaggaaatgtaaactcatttgatttggctgtaaaggattaatagaaaaggaaaacgtagtcactaggctgagaaaaattgaactctattgaattggtataaagatctaagtggaggtgtttggcagacatgatcatgaagctttcactgaggaaggaaactctaggaggcaaaagcagaaatgcaactcatcaaaattgaaatggtgacaaaatatgtgcattcaaacctgaaagtgactgaaagagaagcccaaacacacaattttggggtaagatgggaaaccattaccaaagttctcagaaagagcatttttaaaagtaagattatagaagccaaaaggatatgtagtagtctgttctcacactgctgtaacgaactacctgagactgggtagtttgtaaagaaaagaggttttattgacgctcagttctgcaggccatacaggagacatggctggggaggcctcaggaaacttacagtcatggcggaaggcaaaggggaagccagtacatattacatggtgggaacaggaggaggagagggagggtgggaggtgccactcactttttaaaacaaacagatctccttagaactcactcactatcatgagaacagcaagggggaggtttgctcccatgatgcaattacctgacaccaggcccttcctccaacatgggggattacaattccacatgagatttgggtggggacacaaattcaaaccatatcagaatgttagtgactaaagtaaatgttcttgtttaactctttaatgtgtatattgagtgcaagccatatgcaggggctattctaggtactggtggtttactcaagaaaaagggggcaaaaaaatgaagaaggtggccaggcatggtggcttacgcctgtaatcccaacactttgggagactgagacgtgagaattgcttgagcccaggagtttgagatcagcctggtaacatggcaaatccctgtctctacaaaaaaatgcaaacaaacaaacaaacaaacaaacaaattaatcgggcatggtgtcacatgtctgtagtcccagctacaggttgaggtgggaagatgccttaagcctagggaggttgaggctgcagtcagccatgatagcaccactgcactccagcctgggcaacagagtgagaccccatctgaaaaaaaaagaagtcaaaacaaatgaaaaaaaaaaaaaagtcaaaacaaatattcagtgtaaatgtgagaccatgtaaaaaagtttaaaagtaaaatatatagtttaagcagaggatgggagacggggaaaaaaccttttctccctaactttatatactccctctataaattagtgcttatggccaataagaaatgaataatttcttttttcaccgttggtagtaaagtataatggtagttaacacaaaaaactaaatgatatattcagaacctcatactaaacaaagaaacaaaggcatgcaatcacaggacaggtggaaacagtggttctgaactaaccacaaaccagaactaccaaatgtgctacaaattgtttagtaacaaaggaccatcccttcagaattgaagagcacgtctcagttatctcatgcctatgtgcatggaacttaaagtctcaaaattactcttacaagatggcaaattgaggctgtcagctaagctcctagattgtctgtttctccaagaaaaataaatttcagtaattattaaggaaaaagcatagaattgcatcatgttttacatttcattacttttggcatgacatgggagcatggatgttttctacaaagtgctctgataaattgaagaagaggccaacaacagccaccgaaaaaaccttcaagattcttgccagtatggctcaggggaaaaattccctcataaccacagatttgacttttcaacttctgtacttctgcatatgagtaataatctctgaggttaagtattcatcccatttagctaattgtccacataactccctgggtcttagattgctctataaatacctcctaagagaagaatttttcaaatgacagtttcgtttttcctttttcttcttttaaagcaacaaagaaaagcacgtctgtgtttatatttaaccaaacttaaacttggagagcattggccgtgttgtcgacgtgtttcttttctctactgttaaattccttactgttccagttactcaccatcatactcacctttgcctctgccacttggggtcctctgttctgcagttgtgttctgctctctgatgcctccaggttttgctgcaccttctagaaattgctcacctggataaggccttggctgtcctttatgactcatctcgttcagaagccttttgaatctctcttgaagaatattccctttgctcagtccaaatacacattcactcacttgaatgctgcttcttcctccagtttcacagtgctggggatgatcccgtaaggcctttaaattacattataattagtcatgcacttctctctgctctggggctgtttgaatcgttcactctctttatacctccagtgttcagcacagagcctagggtataatgcgtatgcagtaatgtttcttgaaggagtgaatgggcaagtgaaacaccaaacaaatactaaagagcaaaacatgtattgctcttgtatattaacacattccgagaagagatgggaggaaggtcttgaataatatcaaattatttcttaagagatcttgatttagatttttttcaaaatgagatacatgttgacactgctgtcaacaaataatcacataaaagctagagcctggcttttaagtatcagggggagcatgtgtgaataatcagcattgctgctgttgaagctccataaagtgggaagcagcgactgcaaagatccagagatggacatctgaagcataggaaaggggcagcttgaatgagataggagcaggatctgtattgattgcaggtcaccagatagaattaaaaaaatctatgttctcactagtggctacagttttcaaggacaaatgactattagtggttattgtatttttcttgttttcaatggagcagctccatgacttagttacataagaagttaaaggctccacccccttccctaccaatgtcttaagctgtcctccgtgtgcatacaaactttgtttccagactgccctcgtgtgactcagtccctggaccagcttcccagccccttctgtttccagcacatcctcctccacgtgttacaggattacaaagctttgcacagcctttcaatagggtttagagcaagaatgacagattgctacctggtaggcagcactgactatagttttattggcgttgcgtagagtgactgcatgacatgcaggttgtgcttttgttttgccaggaatttaaaggcatttagcaaagccgtatgaaattatctgccttatgtacctcgaatgtgaggtaatgaacttgtcattagtcgtgttttagtttagtgttctcgctggaatttgcaaaagattaaaattctgcacatttcattaagtcttccacatgggctcaaaataccatcccgcaggctcgacctgacttgccacgttgctttgacaccatctctgattccagtgaacaaaactaagtaagtgtgacttacagccgccctaccaaacattgaaggtgtgagcctgcactgttgttttgtaatgacaatgacaagagtataatgacaagagtataatgacatcctagtccatgaagacatgttttctcttttccctccctctatgtatacttacttactcttaaggaaataatataatttctatttctgcttaaatctgccatctctacttagaattattttcccttgaaaaattaaattgcattatccatcagccaaatggaaaatctgattactaaatgcctacttctagacattatgaattacctgtaatatcacatttcttgggcacttctcagaatgctatgattttacataaaagcataaattacagaatgagaagagtaaagcttagtgcatattatgcaggttcgcagagtgatatgtggcctacgactgtcattgtaatcaaaattgatttttgatcatttataaaactaaaacaactaattgaaagcaaatttactttaactgatgaaattcaagatgaagtgacagtagtcatgaatcacagttctgtagatctgctaaaatgccaatgaactgttattaatggtgaaagtgtttaatatattaatgggaatccaagtaaggaaaataaaacacatattttgcccttaccttaagtcatgttgacatcatacataaatcaggtagaatttgaagatgtttcatccagcattcatcatgaagcaacagagtcaatagcgggcagttacagtctgtaggcaatgctttctggtgtggattatgcaagaaacttacagtcatttggcttcctttattcccctttgcatgtaaactaccaggtggtaggtagacccattcttggctgccagtatttttaccacttggatagattctgctctctgaggtctttaagacaaacacagcacatgtacattgtgatataggagaaagaacatcagacagaggcagagaactgggcttgtcaaaattaagggtgacctagagccttagtgtccttatatgtaagatgagaagcttggattaaaattcattgctccttacacttgatttttatgcagcagaactttcttcaaaagagatcactcctggaatcccaatatacaaaatggataaaagtaggattgttctgaagtaaagaagtaaaatccagagccccacttatttgagtcatctcctaccttttagatggttattaacattgtttctagttcagaaattctgatgttttatattaatttaaactaaagttaaattaggactagaagagccatttcgtgtgaaaatagacatagtctgagtgatttaggcaaacccatagtgacagatttagtggcctgatacactggcttggaaagatctgttccaagtcagtctcaatacacaaggctcggtgaacacatggcgagcagtcttggtggtggtcaagaacatggaatttgctgtgagagagagcttggttagggtctgggctcttccatctgttaactgcaaacttgagcaagttattcaatctccctaatattcagttttctcattcataaaatggattgataatggtaccttctatgtacagttactgtgggtattaaatgaggtaataagcctgtaaaactcctggcatgatgacattggcctacattaattgctcacagagtgagaacttattataaacacaggcatttttgttgaatgactgactgattgaatgaatgaatatagaactagctttctatttgtgatgtatggaatatctctatttcatttaatttcattttgaatattaaaattcaggcttgcttttaaaccaaagtatttgctgatgcaaagaatgaaattctgactatgatacagttacataacttttgaagaaataagaaaaatgctaacacagcatgaacaactttgatttagagaacagagtctctgttaaaatccatgggacttgtcaacttcatatttttgtttatgagcataaaacactctttagtgcatgtcggaatcatttgatgcttgctgaatcacaggttgctggaacccatccccagattctgattcagtctgagatgaggtctgggaatttgcatttttaacttgttgtctggtgatgctgatgctagtggtctgagaatacactttgaggatcactttttcacagtaaaagtcacagtcattaagcaagttaactcaatgagaaatgataatgaaaaggcatgtacctaaatagataaaggacctataccagctatgaatttgagttcagcaataattgtaaaatttgtaattcttttcaggtatttggtttttaaaaaactccctatgtatgcttttatcttatgttttatatggtgtccctcttttcctctctttctctctaatccagtttttaatgtgaacatgtttaatgtgaaaatgttgttcaaagcagaagcgaaccttttgtgtaaccttggcggtattaagtttgtttgtaagctatttctgccctgttagcttctgtactgaaacacgttttcttgcttttgttgcagtatggaagagaagagagcgactggacaattgtgctatcctgaatggaaaatagaggatacaatggaaaatagaggataccaactgtatgctactgggacagactgttgcatttgaattgtgatagatttctttggctacctgtgcataatgtagtttgtagtatcaatgtgttacaagagtgattgtttcttcatgccagagaaaatgaattgcaatcatcaaatggtgtttcataacttggtagtagtaacttaccttaccttacctagaaaaacattaatgtaagccatataacatgggattttcctcaatgattttagtgcctccttttgtacttcactcagatactaaatagtagtttattctttaatataagttacattctgctcctcaaacaaatgcaattttttgtgtgtgtttgaaagctaatttgagaaaatttcataggttacatttcctgcagcctatctttatccacagaaagtgttttcttttttttaaatcaagacttttaaaactggatttcctcccatcactgttttttgaaggtcctccaagtccgtgttaaggtaaatatctgttttcttcctgatgtcacagcctgagcatactctgtgcattaggaagacctgagtgcatttcccaccattgtcctttccacattatgttgtagctggctggctgtcaggcgactacaagactgagggtcttgtgccttatagatctttgtatcccccatggctgacatatagtaggtactcagtaaatggttttataatgaatcagtgaacattttgcttctatagaagtgtaccttctttgtttctatattatgaaacctctttattagaatttgtgattgattctgacagtgtatagatttaccttatattgtctttattttccatgagctactaagtcattagagatactctgaagcatagttagtttaggaaatcacttcatattgattgtattagaattatcttggaattgaagatatatccctagagcaggggaccccaacccccaggccatgggccacacagcaggaagaggtgagtggtgggccattgaggagcttcatctgtatttatggctacttcccatcactcgaattaccacctgaactccacctcttgtcagctcagtggcagcattagattctcataggagcacaaatcctattgtgaactctgcatgcaagggatctaggctatgcgctccttatgagaatctaatgcttgatgacctgaggtgtaacagtttcatcctgaaaccacccttcaccctgcagtctgtggaaaaattgtcttccacaaaactggtccctggtgccaaaaatgttggggaccactgctctagagagaggtcatgatatcataccaaccaaatggaaatgacaaatgttttatgtcaagtgttaattgcagaaataaatcttttttttttttttttggtagaaaacaaagaggcatactctgatttttatactctgtttttgcaggtgctcttttctttgaatggagatttgatgagcaagtggttaggatgcagggagagctactatgggtgatattttccttgtttaggagctgtgagttaaaattgtatcctttgtggtttatctaaggaaagtcaaatcttgacagaaaacatttttccttggaaggtcaactctcagacattgtattttggtttccctcagtcctcataacttccttcttgctgaacatattttattctcttttcagagaaggaaaataaaaaggattctaaaagtttgatgcattggaaaaatttccttgaggcatttagcaacacatagaaaatgggctttgattcttttccaaaacttttagccatagggtcttttatagacagggatagtaaaatgaaaattgagaaatataagatgaaaaggaatgataaaaatatcttttagggggcttttaattggtgatctgaaatcttgggagaagctgttcttttcaggcctgaggtgctcttgactgtcgcctgcgcactgtgtaccccgagcaacattctaagggtgtgctttcgccttggctaactcctttgacctcattcttcatatagtagtctaggaaaaagttgcaggtaatttaaactgtctagtggtacatagtaactaaatttctattcctatgagaaatgagaattatttatttgccatcaacacattttatactttgcatctccaaatttattgtggcgagacttgtccattgtgaaagttagagaacattatgtttgtatcatttctttcataaaacctcaagagcatttttaagcccttttcatcagacccagtgaaaactaaggatagatgtttaaaaactggaggtctcctgataaggagaacacaatccaccattgtcatttaagtaataagacaggaaattgaccttgacgctttcttgttaaatagatttaacaggaacatctgcacatcttttttccttgtgcactatttgtttaattgcagtggattaatacagcaagagtgccacattataactaggcaattatccattcttcaagacttagttattgtcacactaattgatcgtttaaggcataagatggtctagcattaggaacatgtgaagctaatctgctcaaaaagatcaacaaattaatattgttgctgatatttgcataattggctgcaattatttaatgtttaattgggttgatcaaatgagattcagcaattcacaagtgcattaatataaacagaactggtggcacttaaaatgataatgattaacttatattgcatgttctcttcctttcacttttttcagtttctacatttcagaccgagcttgtcagcttttttgaaaacacatcagtagaaaccaagattttaaaatgaagtgtcaagacaaaggcaaaacctgagcagttcctaaaaagatttgctgttagaaattttctttgtggcagtcatttattaaggattcaactcgtgatacaccaaaagaagagttgacttcagagatgtgttccatgctctctagcacaggaatgaataaatttataacacctgctttagcctttgttttcaaaagcacaaaggaaaagtgaaagggaaagagaaacaagtgactgagaagtcttgttaaggaatcaggttttttctacctggtaaacattctctattcttttctcaaaagattgctgtaagaaaaaatgtaagacaaaaaaaaaaaaaaaaaacaaacagaggcagaggcaggcagtagcaagaaagcagagcgtaacatcagctagatggtaacatgcaatgtcagctctcttgaagacatgggaaacctaagttacaccttgggttaaaattcttcaccatattagttttgttgcttcataaaatttacctaagcaagtggtcttgcttgcctcaaatccaagcagtcttgaacacttggaggcaattaatgagtatatcttagtcaaaagaattgttggagctttttattaaagctacagtttcagttctgcttttggggaattgtgctatgaaagcagctgccaaaataagctcatttattttcttcaatcccactcagtgctcagtcactatattctgtttcctttttttttttcaagttgcatatttggtttccccttatgattgggaaagatgaattttcagcagaaaacattgtttgttcactttcaaagagtgatagtttctaaaacatttagagcaataaatattcatcagaggtaccaagtaagccggcagaagagttaagggttagagaaatcccttatttcatgtcttgactctaaaattatcaaagtacttttccttgtaatgtggatttcttcttatgcggatatgcaaaaacttcagttatacgtagtaatgctagcaggtaattttagtagacattttataacaactgtcactttgtttcgccacatgtagagtttgttcagctattttccagatatctccccacaaaaggaggcaaagggtaccagcttttcaatgagcattacctattacttggcaaagatgatgaagactctattaatagttcatttgataaatgttgacataaccaacaatagagattaggaagttagttttaagaaatcaatggcatatagacattaccctcatggagtttgtattctactacttgaactgattgtagctataaaagcatagttagatagctgaatagttagatcataagcaaagaaggccagaacacatctcttatcaagaaatcaatgaatagtttatctcatttttaaagcaactttatccttctttaattccttcctttcttctagtgcaaaactacttaataaggttggtgtttaggttagtgttcacaccattcctcatctggtgtgaattaccttctctttctttactatttactaccaacctagtacatgtgttgactgaattcttttcaaacaatgttgagttatcatggtgcacctaataaattaacaccacagattacagcatccttgctgattttctcagcaaagccagattagatggaaataaacaaagaaaatgatcctagagtgaatttttctagaaaatatctattatgaaccatgctgtttaaagtattagcttgaaggtgatggatccagctattcagaaaataactttcatataaccatgattttgcacagtatgaggtcttaaatgtgtggaaagagataaattttttatcattaccacaaaccccttttaaagattcaaaggtggaagaaagtgatttattttttctcttcagcatacatatataaaagacttgtcagatgtttaatttggggaggttgataatgaaacatatcaacagagtatagtagttatagtagtgtttgtgggtaaataatttcctggggtcagacatatataaacatatttgcttcaaaatgataaaggcatgaaatcagtcttaaaaattgaaatgggggtgatgggggagaaaaagaagaacaaatttgaagtgccctttcaaatctgctggatacaagtattgaagttttaagtcatcttattctgtctgaaagtgtatttttcattctacaatagacccaatcaacaagacgtataacttgagttgcatgatgttcagtttatgtaatctactgttgggatggtaagaattgatgtaggctgtggtgtaagaatgaattaaaatatagtttcactggcttttctctacatatccactatcacaatggctaggtttcctgttgctcactattggattctggagaaaaatttaatgaaagatgatatcagaggaagaataagtggaggtagagaagaaaggaatgatagaggaggggaaaaaaacaaaacatatttttgtgttatccaaaggagctttttccttattctgtcaagcattgagatcttcttcagctttcaatgtagttgctaaatacaaataatgctactaggtagtgactaaatatagcaaacacttcatcagatattagaattaggtcacactattgaggttataatctgaaggttgtgttacatagaaaccactttagattattatcaacttggactaggctttattttataatagcatagtaagtaatatctattgtgtcatttcttcaaccattttattctaagatccatgaagcttcttgaggccaaataaaataataagtttagacaagaagtagattgtgacttttttcccttagagatactatttactatctcctatcctgataggtggaaggtttactgaattggaaattggttgactattagtttttaactaaaatgtgcaataacacattgcagtttcctcaaactagtttcctatgatcattaaactcattctcagggttaagaaaggaatgtaaatttctgcctcaatttgtacttcatcaataagtttttgaagagtgcagatttttagtcaggtcttaaaaataaactcacaaatctggatgcatttctaaattctgcaaatgtttcctggggtgacttaacaaggaataatcccacaatatacctagctacctaatacatggagctggggctcaacccactgtttttaaggatttgcgcttacttgtggctgaggaaaaataagtagttcgaggaagtagtttttaaatgtgagcttatagatagaaacagaatatcaacttaattatgaaattgttagaacctgttctcttgtatctgaatctgattgcaattactattgtactgatagactccagccattgcaagtctcagatatcttagctgtgtagtgattcttgaaattctttttaagaaaaattgagtagaaagaaataaaccctttgtaaatgaggcttggcttttgtgaaagatcatccgcaggctatgttaaaaggattttagctcactaaaagtgtaataatggaaatgtggaaaatatcgtaggtaaaggaaactacctcatgctctgaaggttttgtagaagcacaattaaacatctaaaatggctttgttacaccagagccatctggtgtgaagaactctatatttgtatgttgagagggcatggaataattgtattttgctggcaatagacacattctttattatttgcagattcctcatcaaatctgtaattatgcacagtttctgttatcaataaaacaaaagaatcctgtttgtgtggtttcatgaaatcagcattgttgaatgcatgaagtaataatgctaaattaacatttttatgatgtctcaaggtttctggtcaagggaagtaaatgtaggatagtatttttacaccaaaatgacacagagagaattgagcacaccagaaagaccagaaaccacaccactggatagagattcaatatgtttctttttcaaacatttggacaagaaaaaaatgggcatttaaaaattcttccttcccctggttatggatttatctgtagtaaaacttagctttgtcgtttgagatttgcacagaatggggggagtagattacctcttcccattcattgtcataatggatctacatcactgataaacaccatacttctatatgtggttaactagctttagaataaaagacactttaaaaagtaaaaggcctagagatcttcaatgaagtgtcccttttagccaaaccaggccttgcagaaattgtcctcaaaagcaccaagggagaacaaagccaagtgcagaattacccaagggtcacacattttgtattcattttcttataatttgcccaaatgatttgaagtacagcaaaacctgaagttttgcaaagagttactgtaaactgaacttaaaaatgtcagagtgctcggtgacccacttctccagaccctgtcaacctgtgaaaatattggcctttattcagatctctcaagaagttacgcgcagagtttggaaggtctaggcaaaggttattagtcaagtgttcttacagtgtcaacgctcaattcccacaagcgtgagaaagagagacctgtcattcctgagggtgatgacatacatttactggagcttatataatttatcagataagacagcagtttccttcagggtagaaagtgtgttttctacattgatttagtacaaaacaaaaagaaaaggggatatttcaaattttataattatttttctgctaagctgattcagtgtgatttaagcatatttttcaaatcatgaatctgattccatatacatatgtgccttatattgtgataatttatttttaagtgaaatatgctatcatagcctgactttatgtatagtggtgacaacttgcaggatcgcatttctgtaaccaaacggccgacagctgaggtgtagatgcttcctatggtctgtagaataatcactgggcttgttctctagctatgtctgtatgcaatcgcgacagtgttgatcaaaacccatgatcattctctccaaaggtctttgtcactaagccactagggattctgaaaagttcgtgagctgaaacaaataaattgagttggaagatt

SEQ ID NO: 78 - DNA, 130421 bp, Homo sapiens
  misc_feature (28315)..(68314): n is a, c, g, or t
cctgtctctggtgtgccctggcccccgacttggaggcctcctgggccaggccaagaccttccccggcagcgatggtctccagccacactcaactgccctgaagggacatttcctgcttattcccttgcccggctgtgtcctccacccggaaggcctgtgccttcttcgcctgcatgtcctaccctgaggaggctcccttggtctttcatcgctctccctatgggtcttcacgccttcccgaaccaccgcgcccaagcaggagcacgttctcggccctcttcacagggcgctcctcctcacaggggtgcccgggatttttattctgtgccttcctggtggctcctacaagtctggaagggcaggaggcgcatctcactcctctgggtcccctcccctagcgcctggcgggagcccaggctgcatttgtggaattcatgactttttctctcctgctcaagctgaacacattgctggctcctgctcgggtggagcccggctaattagagtgaggggctccccgtagggcgaaggggtgcgctgtcagatgtggcattcccgttttacggagacacacggtgtcttacacgccagggagaggtctgagacgcaaagagccgtcgagcgggctgcgggattgcttcgctgtcacctccgcctgcagccacccttccgcacgcacttgtgtgtgcacccaggccaacatggaaggcgccatcctaacttctgccgtgagcaggtgggagggaagagagacgagaggtattccattggttgtctgggaaaatgaattgcaccttcccctcccttgcggaggatcaacttttcccaccccctcgggtgggcactcgcatcctggggccggagcctgaacccgggagccaaggggccccagttccagggacgtgaagctgagcgtacagcgggcgctcccagacactggggaaagtgctttacgatgtcccgagtccctccagtctcgccagcggggcgagcgtgagggtgccccgaccgaccagcggccccgggtgcagggtggcgggcccggcggcgcgcgtccccctccccctcctggcggcccgcacgtgtcgcccgcgccgcgcccccacgggttacgcgcgggtcccgcagcgccgcggccgagccgggctgcccggcccgcggacacagcgccggccgccgcatcccgtgcggggccgcggcgcgatgctgcgctggaatgaggaagcgcggcggcgaggggagggcccgggcgcggtgcgcgcgggggtggcggcggcgcgccgagcgggcccggcgcgggcgagcgggctgcagccggcggcggcgccagcaggtacggcccgcacccgccgccgccccggcggcctttgggggctgagccggagcccggcgcgattgcaaagttttcgtgcgcggcccctctggcccggagttgcggctgagacgcgcgccgcgcgagccgggggactcggcgacggggcggggacgggacgacgcaccctctccgtgtcccgctctgcgcccttctgcgcgccccgctccctgtaccggagcagcgatccgggaggcggccgagaggtgcgcgcggggccgagccggctgcggggcaggtcgagcagggaccgccagcgtgcgtcaccccaaagtttgcggggtggcagggcgcgcgctctggccacccgccgctctgggcggcagctggtggcaacgcaagggcgcggcgggggcggccggcgcggagggggccaggtacggggcccgcgggcggcgctgtgcgcgcggggcagccggtcggccgggagcgcgaaagcctggtctgagccggctgggggcggggagtgtggcggagaaatggggaacaatgcgagtgagcaacttcaggaagtcattgtgaaagaaagctgggaagagctccgcggccaagttagcaggacactctaacaagtgactgcgcggcccgcgcccggggcggtgactgcggcaagccccctgggtccccgcgcggcgcatcccagcctgggcgggacgctcggccgcggcgaggcgggcaagcctggcagggcagagggagccccggctccgaggttgctcttcgcacccgaggatcagtcttggccccaaagcgcgacgcacaaatccacgtgagtgttttcaaattgaatttcaataggaaaacttggggtaactggtgaatttaaaaaaaaaaaaacacagtaaagaaaagcggtaaggttggtagaccctggtgtcgctcaggtccgcctctcttttctgaggacagtgagagagttcacttctgtcaagcgtctgttgctctgcactgtgccagcaggtgcaggaccaggccgacatgggacacttctgagcagccccgctgtcaccaggagaggagttctagctcccaaccatatttaaatttatgtagacctacatatacccacggaagtcagcctttataaagtcgtgtgtaaagagttttccttatatttgagccgggagctttctttttatactataaatatgatgagatcgagtctgaacttaatttctgcaagagaggaattatcccggctttgaaaagttagtccttttgctgaccgcaggtttgacgctcaagtcaccaaaccttctcaggaaaacccttagtaatattaaggcatcaggttacttgcggttatatttgaaatgtattttaaatatttgtcaagcatcgctgctgatgcctaaggaacctcgtgagggcttgtttttccttctaatttggaggcatctaatgaccgaaaaccgtagcgattccatagggtctgaccaggcacagctttcaaatgcagcttccctctctctagggactgcagcccacccagactgaatttcaatgcggtgcgctttgcttaggttacccactcacaatttcccactgcgccgcaggcagtatatttcagctttgagataccttgttttaaaattccagacaaaatggtgttgaggaaatgtctccttactagtcccatcaacttctgttaaaagaggaaaatttatggaatttgaaaatactgcgtatgatatttaaactttcatagacattcaaatgcttttaaggccaggttcaatttggttatgagtcgaggggtgggggggacccacatagaaatgtcctgggtcctcttgagtttatttctttgtttgaagatgtttgttcaatgagttttattgtactcatcttttatatggaattttaaaaagtaacaatttcagtattatttatattagaatgtgtcagaattatttccgtgacaaatcagatcatttgggctatggcttaaaatgtacacgaggcaaatattcatgacaagaagattcaccttcttacgctggcatcttgtaaaatgcagaacaagttaaagaaataatgtgtacacatacaaataatgatgtcacattaaaaatactacactattcttgcttgatggaatgtatctgatttccaatttcaccatgaacatatttcatacattttttacatgaaaaaaaacgtgactcttaagtctcacagtcaatcagagctggtgaccagaacattttattgaactaaatggtcatgttttcttccccttttgtttcacggtgagagttgaaggaaggagtttagaaactctccagtacttgtttaattcatcagtgttctaattagagtggtacctcttggaaaactacacacccccctaatgcagaaacatcatagcaataatcacccaccctcagggtctccaggagaccacaagggctgcagataaaagtctggatgtgttaggtttgaccctttcgaagagttttacacaggctcctaaagagaagatcagctgtggccgtttgtagccatttcctttgtcgaaaaactaagatcgcagtgaatgtattagccaagaggtctaaagccctgttgtactgcaggccactgtcttccttgtttgactagagacttggagtttgagaacagtggttctttggtttggatacattttttgttcttgatttggatgtgtgtgtttcatgcgtggttaatatagcatattttcaatataaatgtcaaaaattttgaaataggaaagaactctctatatattaatgtacttatacacacacttcaagattatgcatttattaacagatacatgaaataaattccatgtgcatatgcacatatgcacacagagcgtgcacacacacagcatgcacacagcgtggagtgagaggcatggggcagtgtggaagagttttaacatcaaacagacctgaaatgagtattaaaggccccctttatttttaaacttttactaaaacaagatggatttccctatgttatataatggtgaattttaggcataaataacgttttttgagtgttgcataattgtacgtattaatgtaatgtaactgtggttaacgaagaattcatcaaggatatcactgttttgtggcattttttttttcctcctctaatctttggacttgtgaaataatttcactatgaaataaatgttggttcttgtcatattctaagggagattgatgtaagtggctccactccagcttacagaaggtaaaccacgacctttttgcgttctctgaaaacgcttgtcttccgatgcctctgtttctaagactgacaagcactctgggggcactgtgacgcctgcttctagcggcagagttgctgcagctcctgtcctggctgtgaacattgttctctctctggtgtctctatgttcataactacagagacttcagctctattccatttcatatttgtgctgaataatcattccattttatgggagaaaacacaagatgtaaaagcaacaagtgacccatcctttgaagcttacaagaagagaaacattaatctatttcacgtcttgaaaacagatcagttttattttgctcaaaaagggcacatgtacatttttgatctaggtcttagaaacgtagagtttcagaggatcagcattatacacactgtcacacacacacacacttaaaattcagatgaggaacaagataggaatgaggttttgttagggacgcagagcacctaaaaccaaaggatatcgacagtaacaaagctgtttttactgtagtgctgactgaacactcatgctggtgtcttcatgtggaccatggctttcttgtatttctttgcagtttaataaatgacttcatatctcaggttacctttccacatctcctggaatatatgtttatgtccttaaagtttcagtgtcgtcactttagtagctttagtttgagtttttaaatgtttggtaatattccaacaaatattttttaagacattatgaaaccttatgaagtgccatatattacaagtgagataaaacagcaagcaaaagaaggtttgcagaaggtttttaagtggcgaagtgcgggcctgcccattttggtgtctccttggtggttactcctgagaagggcctggaggaagagcaactgaggcctaatctacaggcaactgccaaattgtttcagttgacgtttttccctctcatgtttgactataataaataggtagttgccagtggagccttcagccaaccacctggtaataaactgttaaaaatggtgcaaaccctaggtcacaggtgtgggggccatttgtcttgcctgttaacaggcctggccttaattcttttctcccatggccatttctgcctttggggaactcacaattcctgttgactaaaagagcacccttttccaccacaagcctgacaaatcagacgtccacataatttctgaactcgttttggttaggacaggaagcacaggctcccttcctgtctgtgttttcctaagagaaaacggtcttccctccttttttgcatatttggcaagtggttccacctttctctgcaccctggtggagtgtgaaggcagcagaggaaccttttggaggaggaagaggacacagaggccctgtagccaggcaccaagatccctcccaggtggctgggtctgaggggaactccgagcagccctaggtcctcaaagtctggatttgtgtggaaaaggcagctctcacttggccttggcgaggcctcggttggttggtgagtgccacacggtttctttgtgtgcttgcatggattggaatagccattgtgttcttccgtcttccctgctggtgtttccacagtgggtggcctgagcccagagcagctccccatatccctgtgcaggccacctgtctcgggtgatggagagcatcattatgctccgtctgaacgctctgctttcggatggccccatgctccacctcctgatagctcgtggcgcggggccacggcttaacaaatggctgaaaatgggtcctaattagtggaaaagtgctttcttcatattttctcactcgagtgtgcagtgattcatttttcttctgcaatcagctcactgctaaagtaaatctgactctcttcccgccattgcacaccaaaagttaactctaatgggtaggaggttaggtttgttgagagagcaatgcagtaaaaagaggggatccaatgtggtcttgtctgtctggtcttcctttcttcgttttttcctcccttgtcttctctgtcattcccttccctccatttgccttgcctttcctgtccttcccttcccttccttcccctctttctttctataattggtggggggtttgcacagactgccaaaacactaagaactgtgtaaagtgtttttgaatggccttacacatattgaagtagatttttatgctccatttttgagatcacacactaaaatctatacctttaaagcattttctgttagtttgaaactatttgaaaatgaacaatgtggtttagattagagtcctgttctgaagctaggagttccactatgaatattgatttatcagtttttgacaaatttttgttgttataccagattttcactggcaaacctagagcaaataaaattccacataagatacttccctagacctaatgggaaaaatgtttaatttagagtctttaggagaaatgagaatgaggaattgaccttttgtaagcttacttctgaggcactctgaagtgtgttccagtgcttttaatggaaactagagagagccagcaaccccctagtgtgagccccacttttaaccggaaaaagtgaccttttcctcctcctttgtgctgagttttgcgtagggcagaaaattaagctgatattcaaagagattcactgcaaaaacatattgataaatcgtatattctatttcattaaattaaaaccatactgctaattatctcaggttgttaaacataaggcaattaattatcattttaaaagttggtaggaagttgtgagtacttttgcagtatgagtgttttcccgctttagtatgaggttgtgtatgtttgcttgaatttacagaattttcactttaagagcagacaatgttttgttaaagaaatgaaatttgctaaaaaggagcatgtaaagtgaaacattaaaaataaataatttcaacttacttaagagctgcagaaaaatctgattgctgtgtttaaaatgaattttcccacatttcgctctcttatggacaggagcattttctgtcaggttataaataaagacatgcccattttttgtacccccacaaatgaggaagttgtaagctctctgaggttttactgatgagccccctccccctgggtttgcatgaagagatcataggccacaaataaaggactacaaaatggggtctaaactatcctggtggggcctgatacccacgtttcgcatggaccttacgatgtgatgaatggttttggcatgagtgtcttaagaatgcttccagattcgggttacaggacagccagcgctgagctccctattgcagaacaaagtaggaatctagaactttcttgctaacaggatccagctaaaacaccaagttagattcttaaatgatgttcttttctgtcattatttgattgttgtcagtagcagtaattgttaccaagccattgatgcttctattcttccctttgcccttctgagacacagctcattttgacttcagtggaacccctcgaaggtggggtgatgagcaaggtgaattttcaaagtaaagctactaagagaccaaactacaatttaaggaacctgatttttgaatcaaattccatatactgtgggtatagttcaacatagattaatttcttatagttattatgaaaaaaatctcatcttgatgatagctgataattttgtgggtgtcgtaaacaaaacagaggtcagaattcagtcccttggggaaaatttccaattagtaggaaaccaagtggcctaccttagtttgaagacacccataccccttttaaaggttaatcatcctttggttcaccggatggaatcaaacttctgtgggtacaggatgtctgcaccttttcatcctctctggaggaaagactaaatacccattattgtatataggtcaggccaaagcagccttttatattgcaaggaataagaggtaaatagatatatgtgcaacaatgaatcccctaatgtgtttactctagaacacatgttctttctgtatttatatgtagattttgtagatcttgtcttaccacctgctaatggtagatactgtatctaaataagttgaggaaaatttatagtacctaggaatgtgtcctcagtgggccaatcaatcaatcatgacttcaggttatttttaataaatatacacgtatgggttcataaacaatgggatgttcttgtgaagatctaaataattttacttctttgggactaaataaaatatagcttttgccaaataaactcacacaagcacttattttaatagaagtcaaatggctttgcagaaacttcagttttacaggtgcattgtttgaaatgttacgggtatacaagtggatttctctattatgtacagtgttaagtttgagtttcaaaatgtccacctgaaatgatttacttgtacgttaagataatttaactgctaagaaggcaagataaagcattctttgtgacaccatatggccttgctgagggaaaaacttactgttataagtttgtgtttatctctctttttaaaaaaaaatgaagaaaaaaacgtttaaaataatgggaacacagcagttcctggggtcctctgtctctttatcttattatagtaaattaccaaaaaaataatgacctggggcatgtctgtgtggacccttcttttagaggcagtttctgtgttttgtaaagctgtaggttctattttcattgcacttcatattgctgcacagctcctgaccatgcatgaaggtcctctgaaatcggtaagagggcagaagaaaatgattctaaacttagatttttttaacttaagtgatgaagtgtgaaacgccatttatatttgaggaagctacctaggaagtggctcatgtcgatggcccaaatcagaagagggcctgtaaaagcttctatcaattttgactgtgtatgcttctaccatggcggctcaataaacagcagtattagtttaagagtggatggtacagtagtatagacgggaagcctctcctctccgtgtgaaccgtgcacccctatgagagggtagagacaatacaatatgcctgtaacgtcaggacagacagtcatggccagcttgaactccagccctgggcttcttgcagcaacaaacgtgaacacagaggactgtctccaactccactttctctatttttaaaacaactttttgaatacagtatctgccatcttttcttatacctcactttgaaacaggtggctccactgtggcatttaaaatgttctgtttcttttccctctgtatcaaatacctctttaccaagaaaacattcaaacagcatagtttttaactgtattttgaaaggtttccttagttccctttgacccttcctcttttgcatatcagttcctggccataaaaataaaaaatgctaggacagaattgcacatctgagctgatttgccctcaaaaagtttcacagtggaacaaaccgcaggaggagttttctgtggctcagttaaatgtcgggggagggtggtgtgaaagccaaattggattcctgctttcctgtttaaatcttgtttttcattgttatttgcaccagcaatactctgtggaataatcatgaaaatgtgtagattggcagctaatttttgaaaaatgaaaagaatcagaaatgaaataagagtgctcggaagtttttatgttctctcaacctgttttgtcaaattgttacgaaaacctataaggtctctttgactagatacaaagactttgcacattgccttagctttctcttgaagcatttccttttttaaaatacagtgtaattcacagtgatatgatagatttgcaaaagtaaaatctaccagtctgaagatgaaaggacttgtctcttagcaggaataatgggttttattaaagaggtctgtgacctaaggcattttaaataaattacaggcttggtccctgtctcccccatgtatctactcccttcaatataagcatcattgagtatttaaggaaataaccccaaatgtaactctagtgtagcttcacttgtcagggaggaaaaagtaaatagcatacatttggccaaataaccagaactttactgtagaagttttatgatgaaatttgcctttagtgcagagtattacaaagatcatgtttagtttctagcagtatataagtagcatccatccttatctgtcatgcatttggagtgtgcgacccctgcactgggctgcaacattctgatgggcaagagtgctagggagaaagaggcatcaccatcagactgcacgggttcaagtgtcagctctgtggttgattagctgtgtgacctggggaaagctatttctcttagccttggttctctcatctataaaatggagataatgatgcagatgccttgggtttaattgggagagttaaagacacatttacatatttagcaagtaggtgttgaattctagctctacattggacactatgccaggtgctcaaataaacaagtggacaagacagacaacacccatggtcttatgaggcttaaccatttgcctcttcaatgccagaaacttagtaggttgattagataaagccagtgagtaccagtatccttttctttgcagccttttcctggcacactaaaaatactcagtacatatgaaatatcactggacaaagaatcccccttagagtaccagtggagaaggaaggcatttgcttaaaagcaaaccaacagaaagacattgtaaggcagttgtttaagtctcagagacctataatttttttcttttttcttttttttcatctcgctctgtcgcccaggctggagtgcagtggcacaatctcagctcactgcaagctccaccttccgggttcatgccattcttctgcctcagcctcccaagtagcagagactacaggcgcccgccaccacacctggctaattttttgtatttttagtggagacggggtttcgccgtgttagccaggatggtcttgatctcctgacctcatgatccgcctgcctcggcctcccaaagtgctgggattactggcatgagccaccacgcccggcaactacaattgttcttaaagcttgtagaattactgtgtgctaccaacagacaggctaattttgagtgaccctcagtactttgtacagttaatttggcacgctgtgtacttagtggctttttaacagctataaatttgggctgctagaaaagtagtaaagttgtgattcttgacaggcatctatctgcattttcatttttacttcatttgtctagactcagcttgtcagaattatggaagagactccttgtgtcagggcaagcactgtgaagagaggtattcactgtcagaaaagagaggggagctggaggcagctcagaggcctgagacccgcctccacaggagccccagcaggttcggtggagctctggccacactctcctttgggatgctgaagtcagaatgagttcacttcccagccagtcttgccaaggctcctcacctggaagcagcaactgcccagggctgttggatgtttctccccaggggacagccaggtcccagtcccgcctcggtgtggaaggaggaaaggcagggtccaggaagctgtttcaggacaggcccaaggtcccccagggatgcctttcagggtcagcggaggctgtaaatcagcagggcccacacggcctggaagaggcccctgtgctgtcggcttgcccggcttgcccggctcctagtccggcttctgctcctcctttgtaaagttatggatatgctaatagtttccaactgagactaggaaagtaagtcctacttgacactgtttggtcagaaagagggagagaaaggagaaggacagagagagactgagagagagacagtctcagacaaagggagacggagggagggagggagagacagagaaagagatgggaggtaggtgtgggaggagggagagatgcagaaggcagaggaaagacagacagagatttagacctcccaagtcagtgagcagtccagagttggagtggagggtgcctggtggcttgtgactgcagactccactccccgctcctagaggcacagccatggacagcttctgtcacgttggccctgcacttatctctgcatctatttccccttgtgcaagattcagaactgcatgctccaaaaaaacaataaaagcattcatgttcataagaattgcacaggtaaaaggtagtttgctgatattgttgtattttttactatcgcttcttttaggtcttgcctgaaattgtttgggtttcccaggcaaagtagaaaactgcggtacgtttctgtgaaataattattccttctggcatctccctttacagacctactgatcttgatttttcatttaggtgaaagtttgtgaaaacatgccattagcttgctttgtgattaactccttttactgaatgtgagctccttttaaattgaggccatatcaagcttaaattccatattttacccggcactctgcatttcttccatgtgggagaggaggggctcagtaagtgctttgtaaaatacacagccgaagtgatgcacgtgctaacaaaggagtgtgacaggacttaagtgcccttctagacacttcaggctcccctttgtaagctgtcttggaagaggccacatttcctttccctcaaacagtttctcattgtttgattattcttttagcctttctctggaagcaaagccacttttacgagaaagtcactgctttttcatctcaagagatgcaagtttggagtttggggaagttttcaggtgcccgtcaagtcatcctttatgatgtcagacgagtcaggccacagaattcacagggctcagtgcagaccgaaaacttgaggcctcttgttcagaaattattaaaaattttggtgaacatcaccccaagcaaagagatcccctaagcaccagcccccaagcaactgcactcataagcccatgaagccccctgctgtcagaaacaatgtggttgaaattgtgtatgcacttggaagtgagatggattgcaaaacacaggtctccatgctggggcaggagtggtgatagggcatggagtggaaatgtccagcaggcccacgtgcgaaaatgcagagctctctggctcttgcagacttggctgctgacaatagacgcgctccaggaaggtgctcgctgtggtgtgatctgctgcccacccctagctccctccaggagactggtgcggggactgtttgcaaatgactgcaaaagtaagaaggttcccacagagcagagcttgatttggggaccagccgagggcagtttgtcaggattccggcttgaaactgttctcacatctcaccgcctgaaaggacgagtgtgtccagaggacttagcattgatcacctctgtctccatgcagcaaactcagaggctcagcccgcattccactggaagggcgtttgccagtggtgttggttggaagagccttgactttgccttaggaaacatctttttttaagaattgaaaataacttgagtatgcaacagtagggcatttgttatataaattagttgactagtgtgtagccagtaaaatgatgatggtggtgtgtatttgttaaataaaaagatatgtgtggtattaaattaaaaaatattttaaaacaacatatttgtaatctgtttagtgtcctctttttgtaaaaagtacagaaataaatatacagaaaaaatagtagtcctaagtggtagaaattatgagcattttcttgcctttaaaaaaagttgtaaaagattgtatcatttatgtagcaaaaagttttaagtcagcattctaaaaatttcgtgttgttatagttgctgtgacaagatttaacttctgtatgcttcaccaatcaatacagaggtatttaagacccggtgtgtgataggccgcgctaaaatactatacacatcttcagaaaactagagaactaacttctaacttcctatattagtgtggcacggctgttacaaagatttttctcatttgagtctatcttgcttctttatcattgttttgacagtttcagaagaatcgtggcttttccccttttttacagtaaaggtacctgagactcttgacgtattgctttttggaaatgcttgtgctggtcacatgcttgcatctgggctagtgtgtctggcttccgtgtgctggtggatgcttactctgttttctgaaatactttttctgtacagtggccactagctgtactcctaagccacacacctaccttgaaaattcatgtcacttttagaaatagataaaagcccctcccatccagaaaaagtgactatcatgtatatcctcatcatgactaatactgatattcctgaaattgaaaatacatattccatatgtaccataaaaggtattaaagatatatggagtgatagatatattatatataacacttctaccctcacagttttcagcctaattgagagggtaagatccctgaatcatccatcagtttttcaggtctctgctgaaagcaggccacagctcagatccacacatctgaaccagagacagaggtggccaaaaataaaaagggggacagggggacaacctggtttagagtcaacaaatagactgcattttctggttagtgaaggagctctcctgaaagtcatataccagagcataaatgagcagatttccttgaggtcaccttctgctggccatagctttcttatctgtggagctgccagctgtcatccactttggggcacctgagactgccgagcggcaggccaggacccaagtgcgaaaacacagaacacctttttgtttctactccactgatgctggggttctctccctggtgtttgtggctcgtagtacactctgtggaacattcactatggtcatcgaagggcagcatcttcccagttgtttctttcttttcttttttttttttaatttaaaccgatctgagaagccagccatctgtcagcaaaacaggaaggctcgggctgtctcctgggctcgttttgctgccgtagtgagcgtcacttctccccgtgtaagagtgctggtgaaggctgaggcaagggcccagaaagattgagggacaaagacaggagcgcccgcattgcccatctgccaggctggaggtgtattcattattgatggaggtagtgcagttgctgctcagatatgcagccctgcctgggtaaatgagacattcttcagcaaattgcttcgttttttgattgctgattgtacgcgtgtcaccaagctgactcaaggttcatcgatgcatgctcagtaaattagaaagaacataactatggatcagccaagagaatgaattctgtgcctacaatgacccagggccatttaattttctgcttaattttgttgcagtcagtttgcattttgggttattatgcagtaggaaattaacaataaataacaaatttggtcctcctgtgcttgtaatgatatttttataaatctttgtaatgctgtttttaaaaggatcaaggtctgtgccagtctgatactccagcaagtatgtgaggaggaaaatgcattattcttgctagataaccttgttgttaaatagcataggggttctttatctctctctctttctcatatcttattagtatttttgctttaaactaaaatcccttcctctctttctcagataacctgaggaccatggatgctgatgagggtcaagacatgtcccaagtttcaggtgagaccttatgagatagctgtgtgggaagttcatgagaaaagcttccctggggccggaagtcacagtgcttggtatgctcatgggggaggaataggggctattctgcaaaagaaaagaccatgatggaatttgcctgagtgtttccttcacctgttacaaattatctcactttgagctgaacagaaagcctccaagatgaaattagttttactgttaaacttcaggaaaaaaaaacgggaagagttaaatacatttttgtactgttggaaggaaaaatggctgattggtttaaaacccaaacacatgccaatgatggtacttaaagagagagagagagagaagcttgaaaaacataattgttgggcacagtcatgactgtttgttcattaagcatggacacaacattgctcccctttgccatatatcttttcaagccgtattggatatagctcttctcatccaggagacccaggaagtggagaagtctgtagtaggaaaagcctaagggtaggtcacagactgtgaccatttggcagcactgagggtggacggcgagccagtccaacaaaaccgcacagttccccagtgcatggacataggaagacagctttctatctggccctgtatccagaggcgtcagccccagtagcagctttcatggactttggggttttcggtatttcatatttttgagcctcacagactcacagccagccccagaggctgacttatatttgagaaagttctcagtggcaccttgccttggctgagcgccctcgtgttttgaagtttctatgggattctacaagttggtgctcctgatgaagaccaggacctatgtgtggctgctcccctgcttggtggtttccctggggaaggtgcaggagaggatcttctgagttccatggaactggagatagatctgccaatcacaggcttccttctccaccactcctcagccgctctattcatgtttcagattttggacttaaactctcccaggtgcaaagaacaaacaaaaggctagcttatttttcttttagagtgaggcttcgtatttattacaatataattgccacattctttgtgtaattctcacatttatatcttaaatataattctcatgaatgagaattatataattctctttttgtatatcattgaatattttcacttaatttttaatttttttaatcgtcacaaaataattgtgtacatagacacaaaataattgggtacatagtgatgttgtgatatatacaatgtatagtaatcggatcaggtaaatcagcatattcatcatctcaaacatttatcgtttctttgtattaggaacattcgacatcttccttctagctatttgaaactatatattattgttgactacagtcatcctgcaatggtgtagaacactagaacttattcttcctacctagctgtaattttgtctcctttaacaaatctctccctatcttccactcccccgacctttccagcctctattagcctctgtcctactttctacttataatgatgacagcagcatttgttagtttccacatgtgagtgagaacatgtggctttttaacttttagaatgtggtattcaggcacttcatggtacagttggtaaaagtgaaaatgtgtccaaaagtttgtgattatctatataaacaaaaatggtataaatacaaatatcaattttgcattgaagaacttaccttagaggtatattctcacaagtgcacagagcatttaagcatttgttcactgcagcattgttatcagtattttaaaactatggtacatccatgtacttccacatacagctcttaaaaataaggaggatatgaatgaactagtatgaaaagaagtccaaatacatgtgaaagtgagaatagcatggttctggatggtatgcaaagtatgatctcgttcttttaaaagaaaataaattacatacacatacatattttctatatgcttgcccataacgtttaggaaaattcttgggtgatatttattaacctggacttcctcttggaagactgatggtagaaggaaggggacgagttagggaagaggaggagaaggaaaactttgcttttcatcttctaccttttagcattatttgaatttattttccttaagcgtttactttgtttcgtaaacaaaaaagcacaaaaacaaaaaacgagttaaatgggaaaaaaagcagtttagctctttatagcctctcatttggcttcgccagcctctcactgcagcctcagagagctggtctgggaaacactggtagatgaggactgtaatcctcactcatggaagaggatctcattcactgggtttgctgactgtgactagaagtgattagggtgtcaaaaaacccaagcatgttaaaaatttccagaggccaaaaagatgctttcattgttctgctcttcttttccttgtcgctttcactttgggtagcttctaaattggtattttgcatggtgcatttaaagaaaatgagacccctttggccaatgcaggagtctacactctgatattctagagtcaaagctgaatgctgacacctaggaattcatctctagaatgtttatataaggaatagcccctcagtattccgatctcgtatcttagtaacgaaactaacaaaagcctgattctcctctggtagttttcttgtctttaccataatacaaaataagtaatttgttctgcaccctgactgttcaaaggatagggtagctgggggcggggacaagaatggagaccttattacataagacttcctgaaaaaggaaactctgtttttgtttgaaatgatttggtctgaaatttagtttgtgtacacttaccaaagggattcctatttctaaaacactcatactgcttttgattcctgttaacctttgagcactctacgtaatgatgagagcacttaaagagtcatgtcacttttagtaaagaatcaaaggatactttttctacttcttcgagtttgatctctgcttctccagttaaaaccagtatttgtttttttcatttctaaagttggaagaaatgacagttagttatggcataaggatgtacatttaaccaaataggagttgacattcttggtaagaaatcttaccaagattatgttatagattataagaaatcttaacaagaatatgttcctaaatcatcctcttttcccataaaatattaaagtatcagcaatttcataggattcaacctaatgtatgcgaaatgctagataaacagataaatacttaatatctggctttttttcaaagcactgggttatttgttccttgagatttatcctaaatgtgggctataccctggtttacagtgtctcacagatgtgtagtagtagacactccataagtgtttactgacttgaatccacagggtactgagaaaatgctactgatagacttggaggagagcatatctaaagcaagctaccctttcctttagggcacgtctcactaattctttgggtaaagcgtatttttcttccttttgtgtttttggcagtctttccaaaaatacgtgttatacctatgcattattttttggtttggtttctaaagaaagagtcagccggtgggaaagtgaaggatgtgggaactgagagatctgcatcagcatcccacctctacctcccacgatgggacctgagacagttatttttgcctcctggaccactatagtatcatctgtaacaggagggacttgagccagttgatctctaaggttcctctggcacctgtgaccctaaatagatattggatattggtttaatgctatttgtagtgtgtttttttggggatatggaaaccagaagtttgtttccataaacataaacataaactgtatatatctaaaggatatggaaacctttagatatatataatctgcttacgtaaagaaggtttgtatatattgcagtgtcaatgggaatattttatcaagttaagcatagtaaatcacattgattaaatgctttgtatttaccaaacattacccaaagtgttttctcctttcaacctcacaaggacccacagaagaaaatacagttatcatttccaacctgcagggagctgagacacagagaatttaagcaactgaccggaagtccaacagggagtcagagattgctctggggtgtgatccccacttggaccctagagtggaagcttctccactactttatagagttgagattctatattttgagcttgtatttacccagagaattatatcctcttgggcaattgtgtataataaaacctcatgcatttaggagaggcgggatgacagaactttgttgagtgaattataatctacttgagaaattatttgcttacattttataagctaattataccatatctcatccagttttcccagaacacttctcataggtaatgctttatttgaaacataggccataggtaagttaagtgtaaatgtgtatttttataatttaaccagaagtttatttcatttttctaaataagtgaaattgtattgcatcttctaaattattctatttaaacacttgatgtcttgctgtctccgtctctgtgtgtttgcatgtcattgtacatgttcttaggaaaagtgtgggagcttgacgcaatatataccttatgtttctatgtgcatatagtttaccaaataataccataagtttacttagcatattagaatccatgcacattatttttattttatcttcaccgcaaccctgtgggatagaccaaaatcatgcttttcagcctcctttttccacttgaggaaaggagtcttaaaaaagggaccagtctcatgttcccattcgtcttacaactaattggtcaagccagaaagccagaactatgtcctgggtcactaactcctagtcactgtgtgttagtatttgagatgcctgttggcttgatttagtcatttattttttagtgttttataatccttgcatacttttacattttaaatggttaaccaggcaaattggtttaaaatcagtgcataaaaatactgtgcctatcatgatgggtttcatgaagtgataacttttcatcatggagatcctcagctgtcacagaagatgaggggccctgggtacagaggctcacgtgagggatgaaagtctcagcagcccggacttacactttggggcttttaggcaaatcagacaacctcttaagaactatcactgagttcaggcaaggcgagcttgaattaacacagggcccttggtgggcatgtgaatatatctcacttcactaccatccagttctgactctttactagatgcccctgtacataccaagactgattttttattctcccttctccccatgtggtttcttctgcatagagagttcctattgatcagtctgacccatggtattttagaattgcgatccctactgtttcattattcctttttctcccccatgttgaaaaaaataaatgtcctgagatgcaagatcagggacactggagcactgacatttagttcagtgcaggaactgaaggcagatgtaattcttaagaagcgtacctgttattatgaaccatcctcaacaaattgtagtggatcttgttttctcatagatacagcagttaaattttttaataaaagtaactaagagttatttggatgtattttagcatgcactgagcggaaagtacgacatttcttcattgggtaagtcctgattctttatgatcctcacttggttccagggccccatgcatctaagggtgtctcagagcatcctgcagtgctccagcatgatcgcagggaaaagctataggaggaaaagagtcaataaagtttagtttctcaacctcccacctccaccccataataatgacagctggttaatcatgagacgcgtgcacaccccacacgccctgtacatgtttactcattgggatagcatgtcaggccagaaggctccatggtcatttctatgaaggtactttagcaggtcttcaagaaggcaagtggcctgggtccctgcctccccaaattgcaagctccctgctttatgtaggagacctatgtgtatattacagttctgtgtaagattattttgttattcttacccccacacccaccccccaaccccccgctgccaccaaaaaaaaaaaaaaaaaattcctctgacaaccttcataaagtcctgggagtttgaacaccattgctctaggaagtcatcttatacaaaaataagagttgtgaggtggttcatatacctcctgcgttctcctatttggagtttttccccatttatgaaagaggtgaaaacgctaagatatttagcaattattactttaaacattttctatttataggccgggcgcagtggctcatgcctgtaatcccagcgcttgggaggccaaggcaggcagatcacgaggtcaggagatcgagaccatcttggctaacacggtgaaaccctgtctctactaaaaaaatacaaaaatttagttgggcatggtgggggatacctgtggtcccagctactcgggaggctgagacaggagaatggcttgaacctgggaggccgagcttgcagtgagccaagatcgcgccactgcactccagcctgggtgacagagcaagactctgtctcgaaaaaaaaaaaaaattctatttacagcagtgaaaatagtagtgacttaatgcacattgccaaggctttagcataacatgaacactttcactcaatgtctctctggccttttgtttttccttgggaaattcttataatcctgctccgtctttaactattcattttgtattggctatccaaatatacccaataatgctctttctgaaaatatgccaattgtggtaattacagctaagctggaatattaaattgtgatgtctgttttccagagaatgaagtagtattccccagagcataggcttggtgcctgtgcaggttctattttaaatattccaggaagggttgttttatatactgaggatgattttactggtcttgccagtcgtctgaaatgctggtattactcttgtggaaggtttattcaaacaaacaaggacatttcacacaatacctagtcatgtttttcagacattttaatgtttggttcatcatttgcacacactctcaaaaatctaggtttgtctatgtgttcatatcattttgcctgttgccagctcagtcagcaggcacactctcccaggctgttgctgttttgttagacttcttcaggaccttcatctaaaatggtcttccacacgtagctatactgcataagttcacatcatctgtttcttgcatgtgggttgtgtctcaactcaagtttaagttagatttggaagggcggaaactataggagttgcagcttcagtggagaaaagagcatttcctactagttatggcttcccaaggaaggttagattcctcagagtaggagtgattccccaatgctagaacctttggtcaaatataattctaatccagtcaaaataaatacaggtattctgtaaaacccgatttcattttgtaaatcctactttgtatagtataagcaatttttgtatttgtgtggattatattttattttcctatttcaaagagaagaatttgtattagcagactccctttgcatgcggagaggggatcattttcccagtaggcatggggttcccttccattccttgtccagtcttcttttccccactaagttaagtcaaactaagcagctggtaagatattccctggttcttgcaaagaaagtgagcagatggcagaatgtatagctctaagcagaatacctggtgtggtatcctcaaacacaaattgacaggagggtgtggtgtggcaagctcattgtgggggtaaattggaataagcttacagggggaagagttgacaaaagataggaagaaccttaaaaatatagatgccttttatgcagtgataaaatgtctagatatttatactgtggtgattattaggaatatgtgcaaagattggctattaggatgttcattacagtgttgtttaataattataaaaggacagaaagcaatgtggactcaaaaataggaaaagaatttaaataaatcctagtgtacccgttatacatgaaattatggaaatatgaccctgagcatggaaatatgtacatgagaatgtctaaaagctagttcattttgaaaaacaaaataatgtcacctcatattatttatagtatataaagatgattttaagagtggcagtgtctgggattataggtgattgtatttcttcccttttgcacatctatgttctctcatttgtattgtgtggggagaagtgactttttttataaaaagaaaaaggtatatgcatcccagcagagaagcactggctccacccagtacctgcctcctcatgccaccctctcaagccaaaagccgggggaagcccaggcaccttgaccatgaccgcccgagactcacacttcttctttctcatcagggaaggaaagcccccctgtaagcgatactccagatgagggcgatgagcccatgccgatccccgaggacctctccaccacctcgggaggacagcaaagctccaagagtgacagagtcgtgggtaagtgggtcaccagcggcctctgtgcctgtgaaacctttatctctttgtatttttccaagacagtgatgaagggatgcaagtcattttatccattgtgttccctcaactggcatattaaagaaatatggcacaaagatcagcaggatgggggtcctctggtgtgtgggaggatggacactcacaggccagcatggccgtgagagccacacaccccgcaaaatgtccaagttgaggagcaatcctgcccagggacgcgtctctgtcactgtcctctgtcctcactgcacttgcaggaatatcaaatgttatggattgtagatcgtgaaaattacacacttacgtgttttggcaacagtgcttttcagtgtttggggttagaacaagccacatctggccattttatgttatccctctaatctctagttcttaaatttcagatttaactgaaaatagaaagtttcataaatggtaatttttaaatgttagaaaaaaatcaaagcacacatttacataccttttccataaaaaagtgtgtgtgaaaccatctgcaactccactggttaacttacacatgcgacagtttgtgtttggaaaacttcacccaccctctttatttcaagaaaccaaagacggagagaagttcagtgaattaaccaaggtgaaatgacagagtcagaattgaactgaatttctgactgaaaaactagttctcgctccattataccatgttctaatgagctaatgagtcaacagttccctggaatacctgttttcttctttaaaaagagaaagagctgtgatactgagagctacctattggcataaaagaatatgaaggacatacaggtaaaatgaggtagactggatcaatgtgggtcagctacataagcccccatagccaaggagggaacatgtatgtaaaattctcaggcttatgagaatcacaactgtatgtctataggacatcctaatgcaataatgggaaaatgtgataactgaattttatctacatgtatagaaaacatattttgggccgggcatggtggctcaagcttgtaatcccagcactttgggaggccgaggctggcggatcacaaggtcaggaaatcgagaccatcctggctaacacggtgaaaccctgtctctactaaaaatacaaaaaattagccgggcgtagtggtgggcgcctgtagtcccagctactcgggaggctgaggcaggagaatggcgtgaacccggcaggcggagcttgcagtgagccgagattgcgccactgcactccagcctggatgacagagccagactccatctcaaaaaaaaaaaaaaaaaagaaaaagtaaagaaaacatattttgtatgttttttatgtgtcttagaaaccaagtggactaggtataatggttctttttttttttaactcagcagcacagttaatggcacaaacagataaagatggtggctaaagccatttggtgtagatgaatccagaaaacaagtacatttatgaattattttaccctattggaaaatggctactatatgtggaaagtagaggggaagagaaatgaacttgtgaattatctactctattctaccaaagaaagatacatatatcatttcagggttttccaaagttgggatgcaaaggatcatgtttcattttaatttatgtatttatttttgagattgtcttctatgtattgcaagtgatactggttttaccatgcactgtaccactacgagggttcctttcaaaacacattcatataaattaaaaaatcagtttaaataaaaacatcaagtcaatagtagtacatagatatgataaaagtttgcaaaagtggcacaggaatagtcattgggtggtgatgttccctgatttttttagtccctgaagcacccagcgccaagggtactgttcttcctgcttaacacaggagcaaacagatgctcacaccctgcccaagaacacagaggctcagggactgaaccagaagaaatgatccattaaccatgtaaatgaacagagagcctggatgtcagagtgaggaggccagctcgggtcgctgtggagaaagagatgggctctccctggaatccctgcagctgcccttagaggctgtgagccatcgtggctagggcatctttagagaactgaaagtcaggccgattcctggagagtgaagaatagcacacgtgccttcaaaacagtgtcagtatcctgtcccttacggacgtcatattgttggtgggttttcctgggtgggagatcacccagtatctggttggcattactgatgggttcccagagctgtcttttggttcaaagtcctgccctcggtcccagctgcccccagcacaggtgtcaccttggagtcaggggcgggtttgtcatagcccatgggtcctggccctgccctttatcatgtttgacatgattttcagtctacttttccttcaggatgtaatttagaaaatatgatttcagaattgtgaaatttaaaaaccctagaaaacctctttgctttgcttgtaaatagcagttgatgcagccctgtggacaggcgggaacagccatgtgacgtgggcactgagatgatttgggagattgaatgctcctcagtggggctagaggccacaggagtgataggttactgtaaagaaagcaaaaaagatgcaaaagcctacatgacaaaccaggcacgacacaaaggagaggcttgagaagaggaagtgaaggagggagaggattccacaagaccgaagtgcccaaggagacatggagggaagagagggctcttcacagagctgagtttagagaccaccctccatggttctggaaggaaaccagccagctttcatatgtggtgacaggctgttcattaatttgtagtgtacagcattaaataaatgaagtatgtagagaacattaggaaacaatataaaaaggtaggggaattcgtggataaagggaataacctgggtaccatatttcatcacattattccatgggaataagtcatcagtgcaaaggactgtaaggagtgcacagcaggaaatgaaaagacagaagcagtggggccgagaggaggaaatggagttgctgaaatgcagggtgagcagcaggggcggagagtgccctgtgggtaaggcacacctcagaagggacaggtccaggccctctcctccctggcctggagcttctggcaaggcttttcttctctgagcctcactttcctcttttgaaggtggcaatagtaactgaacctgcatcannnnnnnnnnnnnnnnnnnnnnnnnnnnnnnnnnnnnnnnnnnnnnnnnnnnnnnnnnnnnnnnnnnnnnnnnnnnnnnnnnnnnnnnnnnnnnnnnnnnnnnnnnnnnnnnnnnnnnnnnnnnnnnnnnnnnnnnnnnnnnnnnnnnnnnnnnnnnnnnnnnnnnnnnnnnnnnnnnnnnnnnnnnnnnnnnnnnnnnnnnnnnnnnnnnnnnnnnnnnnnnnnnnnnnnnnnnnnnnnnnnnnnnnnnnnnnnnnnnnnnnnnnnnnnnnnnnnnnnnnnnnnnnnnnnnnnnnnnnnnnnnnnnnnnnnnnnnnnnnnnnnnnnnnnnnnnnnnnnnnnnnnnnnnnnnnnnnnnnnnnnnnnnnnnnnnnnnnnnnnnnnnnnnnnnnnnnnnnnnnnnnnnnnnnnnnnnnnnnnnnnnnnnnnnnnnnnnnnnnnnnnnnnnnnnnnnnnnnnnnnnnnnnnnnnnnnnnnnnnnnnnnnnnnnnnnnnnnnnnnnnnnnnnnnnnnnnnnnnnnnnnnnnnnnnnnnnnnnnnnnnnnnnnnnnnnnnnnnnnnnnnnnnnnnnnnnnnnnnnnnnnnnnnnnnnnnnnnnnnnnnnnnnnnnnnnnnnnnnnnnnnnnnnnnnnnnnnnnnnnnnnnnnnnnnnnnnnnnnnnnnnnnnnnnnnnnnnnnnnnnnnnnnnnnnnnnnnnnnnnnnnnnnnnnnnnnnnnnnnnnnnnnnnnnnnnnnnnnnnnnnnnnnnnnnnnnnnnnnnnnnnnnnnnnnnnnnnnnnnnnnnnnnnnnnnnnnnnnnnnnnnnnnnnnnnnnnnnnnnnnnnnnnnnnnnnnnnnnnnnnnnnnnnnnnnnnnnnnnnnnnnnnnnnnnnnnnnnnnnnnnnnnnnnnnnnnnnnnnnnnnnnnnnnnnnnnnnnnnnnnnnnnnnnnnnnnnnnnnnnnnnnnnnnnnnnnnnnnnnnnnnnnnnnnnnnnnnnnnnnnnnnnnnnnnnnnnnnnnnnnnnnnnnnnnnnnnnnnnnnnnnnnnnnnnnnnnnnnnnnnnnnnnnnnnnnnnnnnnnnnnnnnnnnnnnnnnnnnnnnnnnnnnnnnnnnnnnnnnnnnnnnnnnnnnnnnnnnnnnnnnnnnnnnnnnnnnnnnnnnnnnnnnnnnnnnnnnnnnnnnnnnnnnnnnnnnnnnnnnnnnnnnnnnnnnnnnnnnnnnnnnnnnnnnnnnnnnnnnnnnnnnnnnnnnnnnnnnnnnnnnnnnnnnnnnnnnnnnnnnnnnnnnnnnnnnnnnnnnnnnnnnnnnnnnnnnnnnnnnnnnnnnnnnnnnnnnnnnnnnnnnnnnnnnnnnnnnnnnnnnnnnnnnnnnnnnnnnnnnnnnnnnnnnnnnnnnnnnnnnnnnnnnnnnnnnnnnnnnnnnnnnnnnnnnnnnnnnnnnnnnnnnnnnnnnnnnnnnnnnnnnnnnnnnnnnnnnnnnnnnnnnnnnnnnnnnnnnnnnnnnnnnnnnnnnnnnnnnnnnnnnnnnnnnnnnnnnnnnnnnnnnnnnnnnnnnnnnnnnnnnnnnnnnnnnnnnnnnnnnnnnnnnnnnnnnnnnnnnnnnnnnnnnnnnnnnnnnnnnnnnnnnnnnnnnnnnnnnnnnnnnnnnnnnnnnnnnnnnnnnnnnnnnnnnnnnnnnnnnnnnnnnnnnnnnnnnnnnnnnnnnnnnnnnnnnnnnnnnnnnnnnnnnnnnnnnnnnnnnnnnnnnnnnnnnnnnnnnnnnnnnnnnnnnnnnnnnnnnnnnnnnnnnnnnnnnnnnnnnnnnnnnnnnnnnnnnnnnnnnnnnnnnnnnnnnnnnnnnnnnnnnnnnnnnnnnnnnnnnnnnnnnnnnnnnnnnnnnnnnnnnnnnnnnnnnnnnnnnnnnnnnnnnnnnnnnnnnnnnnnnnnnnnnnnnnnnnnnnnnnnnnnnnnnnnnnnnnnnnnnnnnnnnnnnnnnnnnnnnnnnnnnnnnnnnnnnnnnnnnnnnnnnnnnnnnnnnnnnnnnnnnnnnnnnnnnnnnnnnnnnnnnnnnnnnnnnnnnnnnnnnnnnnnnnnnnnnnnnnnnnnnnnnnnnnnnnnnnnnnnnnnnnnnnnnnnnnnnnnnnnnnnnnnnnnnnnnnnnnnnnnnnnnnnnnnnnnnnnnnnnnnnnnnnnnnnnnnnnnnnnnnnnnnnnnnnnnnnnnnnnnnnnnnnnnnnnnnnnnnnnnnnnnnnnnnnnnnnnnnnnnnnnnnnnnnnnnnnnnnnnnnnnnnnnnnnnnnnnnnnnnnnnnnnnnnnnnnnnnnnnnnnnnnnnnnnnnnnnnnnnnnnnnnnnnnnnnnnnnnnnnnnnnnnnnnnnnnnnnnnnnnnnnnnnnnnnnnnnnnnnnnnnnnnnnnnnnnnnnnnnnnnnnnnnnnnnnnnnnnnnnnnnnnnnnnnnnnnnnnnnnnnnnnnnnnnnnnnnnnnnnnnnnnnnnnnnnnnnnnnnnnnnnnnnnnnnnnnnnnnnnnnnnnnnnnnnnnnnnnnnnnnnnnnnnnnnnnnnnnnnnnnnnnnnnnnnnnnnnnnnnnnnnnnnnnnnnnnnnnnnnnnnnnnnnnnnnnnnnnnnnnnnnnnnnnnnnnnnnnnnnnnnnnnnnnnnnnnnnnnnnnnnnnnnnnnnnnnnnnnnnnnnnnnnnnnnnnnnnnnnnnnnnnnnnnnnnnnnnnnnnnnnnnnnnnnnnnnnnnnnnnnnnnnnnnnnnnnnnnnnnnnnnnnnnnnnnnnnnnnnnnnnnnnnnnnnnnnnnnnnnnnnnnnnnnnnnnnnnnnnnnnnnnnnnnnnnnnnnnnnnnnnnnnnnnnnnnnnnnnnnnnnnnnnnnnnnnnnnnnnnnnnnnnnnnnnnnnnnnnnnnnnnnnnnnnnnnnnnnnnnnnnnnnnnnnnnnnnnnnnnnnnnnnnnnnnnnnnnnnnnnnnnnnnnnnnnnnnnnnnnnnnnnnnnnnnnnnnnnnnnnnnnnnnnnnnnnnnnnnnnnnnnnnnnnnnnnnnnnnnnnnnnnnnnnnnnnnnnnnnnnnnnnnnnnnnnnnnnnnnnnnnnnnnnnnnnnnnnnnnnnnnnnnnnnnnnnnnnnnnnnnnnnnnnnnnnnnnnnnnnnnnnnnnnnnnnnnnnnnnnnnnnnnnnnnnnnnnnnnnnnnnnnnnnnnnnnnnnnnnnnnnnnnnnnnnnnnnnnnnnnnnnnnnnnnnnnnnnnnnnnnnnnnnnnnnnnnnnnnnnnnnnnnnnnnnnnnnnnnnnnnnnnnnnnnnnnnnnnnnnnnnnnnnnnnnnnnnnnnnnnnnnnnnnnnnnnnnnnnnnnnnnnnnnnnnnnnnnnnnnnnnnnnnnnnnnnnnnnnnnnnnnnnnnnnnnnnnnnnnnnnnnnnnnnnnnnnnnnnnnnnnnnnnnnnnnnnnnnnnnnnnnnnnnnnnnnnnnnnnnnnnnnnnnnnnnnnnnnnnnnnnnnnnnnnnnnnnnnnnnnnnnnnnnnnnnnnnnnnnnnnnnnnnnnnnnnnnnnnnnnnnnnnnnnnnnnnnnnnnnnnnnnnnnnnnnnnnnnnnnnnnnnnnnnnnnnnnnnnnnnnnnnnnnnnnnnnnnnnnnnnnnnnnnnnnnnnnnnnnnnnnnnnnnnnnnnnnnnnnnnnnnnnnnnnnnnnnnnnnnnnnnnnnnnnnnnnnnnnnnnnnnnnnnnnnnnnnnnnnnnnnnnnnnnnnnnnnnnnnnnnnnnnnnnnnnnnnnnnnnnnnnnnnnnnnnnnnnnnnnnnnnnnnnnnnnnnnnnnnnnnnnnnnnnnnnnnnnnnnnnnnnnnnnnnnnnnnnnnnnnnnnnnnnnnnnnnnnnnnnnnnnnnnnnnnnnnnnnnnnnnnnnnnnnnnnnnnnnnnnnnnnnnnnnnnnnnnnnnnnnnnnnnnnnnnnnnnnnnnnnnnnnnnnnnnnnnnnnnnnnnnnnnnnnnnnnnnnnnnnnnnnnnnnnnnnnnnnnnnnnnnnnnnnnnnnnnnnnnnnnnnnnnnnnnnnnnnnnnnnnnnnnnnnnnnnnnnnnnnnnnnnnnnnnnnnnnnnnnnnnnnnnnnnnnnnnnnnnnnnnnnnnnnnnnnnnnnnnnnnnnnnnnnnnnnnnnnnnnnnnnnnnnnnnnnnnnnnnnnnnnnnnnnnnnnnnnnnnnnnnnnnnnnnnnnnnnnnnnnnnnnnnnnnnnnnnnnnnnnnnnnnnnnnnnnnnnnnnnnnnnnnnnnnnnnnnnnnnnnnnnnnnnnnnnnnnnnnnnnnnnnnnnnnnnnnnnnnnnnnnnnnnnnnnnnnnnnnnnnnnnnnnnnnnnnnnnnnnnnnnnnnnnnnnnnnnnnnnnnnnnnnnnnnnnnnnnnnnnnnnnnnnnnnnnnnnnnnnnnnnnnnnnnnnnnnnnnnnnnnnnnnnnnnnnnnnnnnnnnnnnnnnnnnnnnnnnnnnnnnnnnnnnnnnnnnnnnnnnnnnnnnnnnnnnnnnnnnnnnnnnnnnnnnnnnnnnnnnnnnnnnnnnnnnnnnnnnnnnnnnnnnnnnnnnnnnnnnnnnnnnnnnnnnnnnnnnnnnnnnnnnnnnnnnnnnnnnnnnnnnnnnnnnnnnnnnnnnnnnnnnnnnnnnnnnnnnnnnnnnnnnnnnnnnnnnnnnnnnnnnnnnnnnnnnnnnnnnnnnnnnnnnnnnnnnnnnnnnnnnnnnnnnnnnnnnnnnnnnnnnnnnnnnnnnnnnnnnnnnnnnnnnnnnnnnnnnnnnnnnnnnnnnnnnnnnnnnnnnnnnnnnnnnnnnnnnnnnnnnnnnnnnnnnnnnnnnnnnnnnnnnnnnnnnnnnnnnnnnnnnnnnnnnnnnnnnnnnnnnnnnnnnnnnnnnnnnnnnnnnnnnnnnnnnnnnnnnnnnnnnnnnnnnnnnnnnnnnnnnnnnnnnnnnnnnnnnnnnnnnnnnnnnnnnnnnnnnnnnnnnnnnnnnnnnnnnnnnnnnnnnnnnnnnnnnnnnnnnnnnnnnnnnnnnnnnnnnnnnnnnnnnnnnnnnnnnnnnnnnnnnnnnnnnnnnnnnnnnnnnnnnnnnnnnnnnnnnnnnnnnnnnnnnnnnnnnnnnnnnnnnnnnnnnnnnnnnnnnnnnnnnnnnnnnnnnnnnnnnnnnnnnnnnnnnnnnnnnnnnnnnnnnnnnnnnnnnnnnnnnnnnnnnnnnnnnnnnnnnnnnnnnnnnnnnnnnnnnnnnnnnnnnnnnnnnnnnnnnnnnnnnnnnnnnnnnnnnnnnnnnnnnnnnnnnnnnnnnnnnnnnnnnnnnnnnnnnnnnnnnnnnnnnnnnnnnnnnnnnnnnnnnnnnnnnnnnnnnnnnnnnnnnnnnnnnnnnnnnnnnnnnnnnnnnnnnnnnnnnnnnnnnnnnnnnnnnnnnnnnnnnnnnnnnnnnnnnnnnnnnnnnnnnnnnnnnnnnnnnnnnnnnnnnnnnnnnnnnnnnnnnnnnnnnnnnnnnnnnnnnnnnnnnnnnnnnnnnnnnnnnnnnnnnnnnnnnnnnnnnnnnnnnnnnnnnnnnnnnnnnnnnnnnnnnnnnnnnnnnnnnnnnnnnnnnnnnnnnnnnnnnnnnnnnnnnnnnnnnnnnnnnnnnnnnnnnnnnnnnnnnnnnnnnnnnnnnnnnnnnnnnnnnnnnnnnnnnnnnnnnnnnnnnnnnnnnnnnnnnnnnnnnnnnnnnnnnnnnnnnnnnnnnnnnnnnnnnnnnnnnnnnnnnnnnnnnnnnnnnnnnnnnnnnnnnnnnnnnnnnnnnnnnnnnnnnnnnnnnnnnnnnnnnnnnnnnnnnnnnnnnnnnnnnnnnnnnnnnnnnnnnnnnnnnnnnnnnnnnnnnnnnnnnnnnnnnnnnnnnnnnnnnnnnnnnnnnnnnnnnnnnnnnnnnnnnnnnnnnnnnnnnnnnnnnnnnnnnnnnnnnnnnnnnnnnnnnnnnnnnnnnnnnnnnnnnnnnnnnnnnnnnnnnnnnnnnnnnnnnnnnnnnnnnnnnnnnnnnnnnnnnnnnnnnnnnnnnnnnnnnnnnnnnnnnnnnnnnnnnnnnnnnnnnnnnnnnnnnnnnnnnnnnnnnnnnnnnnnnnnnnnnnnnnnnnnnnnnnnnnnnnnnnnnnnnnnnnnnnnnnnnnnnnnnnnnnnnnnnnnnnnnnnnnnnnnnnnnnnnnnnnnnnnnnnnnnnnnnnnnnnnnnnnnnnnnnnnnnnnnnnnnnnnnnnnnnnnnnnnnnnnnnnnnnnnnnnnnnnnnnnnnnnnnnnnnnnnnnnnnnnnnnnnnnnnnnnnnnnnnnnnnnnnnnnnnnnnnnnnnnnnnnnnnnnnnnnnnnnnnnnnnnnnnnnnnnnnnnnnnnnnnnnnnnnnnnnnnnnnnnnnnnnnnnnnnnnnnnnnnnnnnnnnnnnnnnnnnnnnnnnnnnnnnnnnnnnnnnnnnnnnnnnnnnnnnnnnnnnnnnnnnnnnnnnnnnnnnnnnnnnnnnnnnnnnnnnnnnnnnnnnnnnnnnnnnnnnnnnnnnnnnnnnnnnnnnnnnnnnnnnnnnnnnnnnnnnnnnnnnnnnnnnnnnnnnnnnnnnnnnnnnnnnnnnnnnnnnnnnnnnnnnnnnnnnnnnnnnnnnnnnnnnnnnnnnnnnnnnnnnnnnnnnnnnnnnnnnnnnnnnnnnnnnnnnnnnnnnnnnnnnnnnnnnnnnnnnnnnnnnnnnnnnnnnnnnnnnnnnnnnnnnnnnnnnnnnnnnnnnnnnnnnnnnnnnnnnnnnnnnnnnnnnnnnnnnnnnnnnnnnnnnnnnnnnnnnnnnnnnnnnnnnnnnnnnnnnnnnnnnnnnnnnnnnnnnnnnnnnnnnnnnnnnnnnnnnnnnnnnnnnnnnnnnnnnnnnnnnnnnnnnnnnnnnnnnnnnnnnnnnnnnnnnnnnnnnnnnnnnnnnnnnnnnnnnnnnnnnnnnnnnnnnnnnnnnnnnnnnnnnnnnnnnnnnnnnnnnnnnnnnnnnnnnnnnnnnnnnnnnnnnnnnnnnnnnnnnnnnnnnnnnnnnnnnnnnnnnnnnnnnnnnnnnnnnnnnnnnnnnnnnnnnnnnnnnnnnnnnnnnnnnnnnnnnnnnnnnnnnnnnnnnnnnnnnnnnnnnnnnnnnnnnnnnnnnnnnnnnnnnnnnnnnnnnnnnnnnnnnnnnnnnnnnnnnnnnnnnnnnnnnnnnnnnnnnnnnnnnnnnnnnnnnnnnnnnnnnnnnnnnnnnnnnnnnnnnnnnnnnnnnnnnnnnnnnnnnnnnnnnnnnnnnnnnnnnnnnnnnnnnnnnnnnnnnnnnnnnnnnnnnnnnnnnnnnnnnnnnnnnnnnnnnnnnnnnnnnnnnnnnnnnnnnnnnnnnnnnnnnnnnnnnnnnnnnnnnnnnnnnnnnnnnnnnnnnnnnnnnnnnnnnnnnnnnnnnnnnnnnnnnnnnnnnnnnnnnnnnnnnnnnnnnnnnnnnnnnnnnnnnnnnnnnnnnnnnnnnnnnnnnnnnnnnnnnnnnnnnnnnnnnnnnnnnnnnnnnnnnnnnnnnnnnnnnnnnnnnnnnnnnnnnnnnnnnnnnnnnnnnnnnnnnnnnnnnnnnnnnnnnnnnnnnnnnnnnnnnnnnnnnnnnnnnnnnnnnnnnnnnnnnnnnnnnnnnnnnnnnnnnnnnnnnnnnnnnnnnnnnnnnnnnnnnnnnnnnnnnnnnnnnnnnnnnnnnnnnnnnnnnnnnnnnnnnnnnnnnnnnnnnnnnnnnnnnnnnnnnnnnnnnnnnnnnnnnnnnnnnnnnnnnnnnnnnnnnnnnnnnnnnnnnnnnnnnnnnnnnnnnnnnnnnnnnnnnnnnnnnnnnnnnnnnnnnnnnnnnnnnnnnnnnnnnnnnnnnnnnnnnnnnnnnnnnnnnnnnnnnnnnnnnnnnnnnnnnnnnnnnnnnnnnnnnnnnnnnnnnnnnnnnnnnnnnnnnnnnnnnnnnnnnnnnnnnnnnnnnnnnnnnnnnnnnnnnnnnnnnnnnnnnnnnnnnnnnnnnnnnnnnnnnnnnnnnnnnnnnnnnnnnnnnnnnnnnnnnnnnnnnnnnnnnnnnnnnnnnnnnnnnnnnnnnnnnnnnnnnnnnnnnnnnnnnnnnnnnnnnnnnnnnnnnnnnnnnnnnnnnnnnnnnnnnnnnnnnnnnnnnnnnnnnnnnnnnnnnnnnnnnnnnnnnnnnnnnnnnnnnnnnnnnnnnnnnnnnnnnnnnnnnnnnnnnnnnnnnnnnnnnnnnnnnnnnnnnnnnnnnnnnnnnnnnnnnnnnnnnnnnnnnnnnnnnnnnnnnnnnnnnnnnnnnnnnnnnnnnnnnnnnnnnnnnnnnnnnnnnnnnnnnnnnnnnnnnnnnnnnnnnnnnnnnnnnnnnnnnnnnnnnnnnnnnnnnnnnnnnnnnnnnnnnnnnnnnnnnnnnnnnnnnnnnnnnnnnnnnnnnnnnnnnnnnnnnnnnnnnnnnnnnnnnnnnnnnnnnnnnnnnnnnnnnnnnnnnnnnnnnnnnnnnnnnnnnnnnnnnnnnnnnnnnnnnnnnnnnnnnnnnnnnnnnnnnnnnnnnnnnnnnnnnnnnnnnnnnnnnnnnnnnnnnnnnnnnnnnnnnnnnnnnnnnnnnnnnnnnnnnnnnnnnnnnnnnnnnnnnnnnnnnnnnnnnnnnnnnnnnnnnnnnnnnnnnnnnnnnnnnnnnnnnnnnnnnnnnnnnnnnnnnnnnnnnnnnnnnnnnnnnnnnnnnnnnnnnnnnnnnnnnnnnnnnnnnnnnnnnnnnnnnnnnnnnnnnnnnnnnnnnnnnnnnnnnnnnnnnnnnnnnnnnnnnnnnnnnnnnnnnnnnnnnnnnnnnnnnnnnnnnnnnnnnnnnnnnnnnnnnnnnnnnnnnnnnnnnnnnnnnnnnnnnnnnnnnnnnnnnnnnnnnnnnnnnnnnnnnnnnnnnnnnnnnnnnnnnnnnnnnnnnnnnnnnnnnnnnnnnnnnnnnnnnnnnnnnnnnnnnnnnnnnnnnnnnnnnnnnnnnnnnnnnnnnnnnnnnnnnnnnnnnnnnnnnnnnnnnnnnnnnnnnnnnnnnnnnnnnnnnnnnnnnnnnnnnnnnnnnnnnnnnnnnnnnnnnnnnnnnnnnnnnnnnnnnnnnnnnnnnnnnnnnnnnnnnnnnnnnnnnnnnnnnnnnnnnnnnnnnnnnnnnnnnnnnnnnnnnnnnnnnnnnnnnnnnnnnnnnnnnnnnnnnnnnnnnnnnnnnnnnnnnnnnnnnnnnnnnnnnnnnnnnnnnnnnnnnnnnnnnnnnnnnnnnnnnnnnnnnnnnnnnnnnnnnnnnnnnnnnnnnnnnnnnnnnnnnnnnnnnnnnnnnnnnnnnnnnnnnnnnnnnnnnnnnnnnnnnnnnnnnnnnnnnnnnnnnnnnnnnnnnnnnnnnnnnnnnnnnnnnnnnnnnnnnnnnnnnnnnnnnnnnnnnnnnnnnnnnnnnnnnnnnnnnnnnnnnnnnnnnnnnnnnnnnnnnnnnnnnnnnnnnnnnnnnnnnnnnnnnnnnnnnnnnnnnnnnnnnnnnnnnnnnnnnnnnnnnnnnnnnnnnnnnnnnnnnnnnnnnnnnnnnnnnnnnnnnnnnnnnnnnnnnnnnnnnnnnnnnnnnnnnnnnnnnnnnnnnnnnnnnnnnnnnnnnnnnnnnnnnnnnnnnnnnnnnnnnnnnnnnnnnnnnnnnnnnnnnnnnnnnnnnnnnnnnnnnnnnnnnnnnnnnnnnnnnnnnnnnnnnnnnnnnnnnnnnnnnnnnnnnnnnnnnnnnnnnnnnnnnnnnnnnnnnnnnnnnnnnnnnnnnnnnnnnnnnnnnnnnnnnnnnnnnnnnnnnnnnnnnnnnnnnnnnnnnnnnnnnnnnnnnnnnnnnnnnnnnnnnnnnnnnnnnnnnnnnnnnnnnnnnnnnnnnnnnnnnnnnnnnnnnnnnnnnnnnnnnnnnnnnnnnnnnnnnnnnnnnnnnnnnnnnnnnnnnnnnnnnnnnnnnnnnnnnnnnnnnnnnnnnnnnnnnnnnnnnnnnnnnnnnnnnnnnnnnnnnnnnnnnnnnnnnnnnnnnnnnnnnnnnnnnnnnnnnnnnnnnnnnnnnnnnnnnnnnnnnnnnnnnnnnnnnnnnnnnnnnnnnnnnnnnnnnnnnnnnnnnnnnnnnnnnnnnnnnnnnnnnnnnnnnnnnnnnnnnnnnnnnnnnnnnnnnnnnnnnnnnnnnnnnnnnnnnnnnnnnnnnnnnnnnnnnnnnnnnnnnnnnnnnnnnnnnnnnnnnnnnnnnnnnnnnnnnnnnnnnnnnnnnnnnnnnnnnnnnnnnnnnnnnnnnnnnnnnnnnnnnnnnnnnnnnnnnnnnnnnnnnnnnnnnnnnnnnnnnnnnnnnnnnnnnnnnnnnnnnnnnnnnnnnnnnnnnnnnnnnnnnnnnnnnnnnnnnnnnnnnnnnnnnnnnnnnnnnnnnnnnnnnnnnnnnnnnnnnnnnnnnnnnnnnnnnnnnnnnnnnnnnnnnnnnnnnnnnnnnnnnnnnnnnnnnnnnnnnnnnnnnnnnnnnnnnnnnnnnnnnnnnnnnnnnnnnnnnnnnnnnnnnnnnnnnnnnnnnnnnnnnnnnnnnnnnnnnnnnnnnnnnnnnnnnnnnnnnnnnnnnnnnnnnnnnnnnnnnnnnnnnnnnnnnnnnnnnnnnnnnnnnnnnnnnnnnnnnnnnnnnnnnnnnnnnnnnnnnnnnnnnnnnnnnnnnnnnnnnnnnnnnnnnnnnnnnnnnnnnnnnnnnnnnnnnnnnnnnnnnnnnnnnnnnnnnnnnnnnnnnnnnnnnnnnnnnnnnnnnnnnnnnnnnnnnnnnnnnnnnnnnnnnnnnnnnnnnnnnnnnnnnnnnnnnnnnnnnnnnnnnnnnnnnnnnnnnnnnnnnnnnnnnnnnnnnnnnnnnnnnnnnnnnnnnnnnnnnnnnnnnnnnnnnnnnnnnnnnnnnnnnnnnnnnnnnnnnnnnnnnnnnnnnnnnnnnnnnnnnnnnnnnnnnnnnnnnnnnnnnnnnnnnnnnnnnnnnnnnnnnnnnnnnnnnnnnnnnnnnnnnnnnnnnnnnnnnnnnnnnnnnnnnnnnnnnnnnnnnnnnnnnnnnnnnnnnnnnnnnnnnnnnnnnnnnnnnnnnnnnnnnnnnnnnnnnnnnnnnnnnnnnnnnnnnnnnnnnnnnnnnnnnnnnnnnnnnnnnnnnnnnnnnnnnnnnnnnnnnnnnnnnnnnnnnnnnnnnnnnnnnnnnnnnnnnnnnnnnnnnnnnnnnnnnnnnnnnnnnnnnnnnnnnnnnnnnnnnnnnnnnnnnnnnnnnnnnnnnnnnnnnnnnnnnnnnnnnnnnnnnnnnnnnnnnnnnnnnnnnnnnnnnnnnnnnnnnnnnnnnnnnnnnnnnnnnnnnnnnnnnnnnnnnnnnnnnnnnnnnnnnnnnnnnnnnnnnnnnnnnnnnnnnnnnnnnnnnnnnnnnnnnnnnnnnnnnnnnnnnnnnnnnnnnnnnnnnnnnnnnnnnnnnnnnnnnnnnnnnnnnnnnnnnnnnnnnnnnnnnnnnnnnnnnnnnnnnnnnnnnnnnnnnnnnnnnnnnnnnnnnnnnnnnnnnnnnnnnnnnnnnnnnnnnnnnnnnnnnnnnnnnnnnnnnnnnnnnnnnnnnnnnnnnnnnnnnnnnnnnnnnnnnnnnnnnnnnnnnnnnnnnnnnnnnnnnnnnnnnnnnnnnnnnnnnnnnnnnnnnnnnnnnnnnnnnnnnnnnnnnnnnnnnnnnnnnnnnnnnnnnnnnnnnnnnnnnnnnnnnnnnnnnnnnnnnnnnnnnnnnnnnnnnnnnnnnnnnnnnnnnnnnnnnnnnnnnnnnnnnnnnnnnnnnnnnnnnnnnnnnnnnnnnnnnnnnnnnnnnnnnnnnnnnnnnnnnnnnnnnnnnnnnnnnnnnnnnnnnnnnnnnnnnnnnnnnnnnnnnnnnnnnnnnnnnnnnnnnnnnnnnnnnnnnnnnnnnnnnnnnnnnnnnnnnnnnnnnnnnnnnnnnnnnnnnnnnnnnnnnnnnnnnnnnnnnnnnnnnnnnnnnnnnnnnnnnnnnnnnnnnnnnnnnnnnnnnnnnnnnnnnnnnnnnnnnnnnnnnnnnnnnnnnnnnnnnnnnnnnnnnnnnnnnnnnnnnnnnnnnnnnnnnnnnnnnnnnnnnnnnnnnnnnnnnnnnnnnnnnnnnnnnnnnnnnnnnnnnnnnnnnnnnnnnnnnnnnnnnnnnnnnnnnnnnnnnnnnnnnnnnnnnnnnnnnnnnnnnnnnnnnnnnnnnnnnnnnnnnnnnnnnnnnnnnnnnnnnnnnnnnnnnnnnnnnnnnnnnnnnnnnnnnnnnnnnnnnnnnnnnnnnnnnnnnnnnnnnnnnnnnnnnnnnnnnnnnnnnnnnnnnnnnnnnnnnnnnnnnnnnnnnnnnnnnnnnnnnnnnnnnnnnnnnnnnnnnnnnnnnnnnnnnnnnnnnnnnnnnnnnnnnnnnnnnnnnnnnnnnnnnnnnnnnnnnnnnnnnnnnnnnnnnnnnnnnnnnnnnnnnnnnnnnnnnnnnnnnnnnnnnnnnnnnnnnnnnnnnnnnnnnnnnnnnnnnnnnnnnnnnnnnnnnnnnnnnnnnnnnnnnnnnnnnnnnnnnnnnnnnnnnnnnnnnnnnnnnnnnnnnnnnnnnnnnnnnnnnnnnnnnnnnnnnnnnnnnnnnnnnnnnnnnnnnnnnnnnnnnnnnnnnnnnnnnnnnnnnnnnnnnnnnnnnnnnnnnnnnnnnnnnnnnnnnnnnnnnnnnnnnnnnnnnnnnnnnnnnnnnnnnnnnnnnnnnnnnnnnnnnnnnnnnnnnnnnnnnnnnnnnnnnnnnnnnnnnnnnnnnnnnnnnnnnnnnnnnnnnnnnnnnnnnnnnnnnnnnnnnnnnnnnnnnnnnnnnnnnnnnnnnnnnnnnnnnnnnnnnnnnnnnnnnnnnnnnnnnnnnnnnnnnnnnnnnnnnnnnnnnnnnnnnnnnnnnnnnnnnnnnnnnnnnnnnnnnnnnnnnnnnnnnnnnnnnnnnnnnnnnnnnnnnnnnnnnnnnnnnnnnnnnnnnnnnnnnnnnnnnnnnnnnnnnnnnnnnnnnnnnnnnnnnnnnnnnnnnnnnnnnnnnnnnnnnnnnnnnnnnnnnnnnnnnnnnnnnnnnnnnnnnnnnnnnnnnnnnnnnnnnnnnnnnnnnnnnnnnnnnnnnnnnnnnnnnnnnnnnnnnnnnnnnnnnnnnnnnnnnnnnnnnnnnnnnnnnnnnnnnnnnnnnnnnnnnnnnnnnnnnnnnnnnnnnnnnnnnnnnnnnnnnnnnnnnnnnnnnnnnnnnnnnnnnnnnnnnnnnnnnnnnnnnnnnnnnnnnnnnnnnnnnnnnnnnnnnnnnnnnnnnnnnnnnnnnnnnnnnnnnnnnnnnnnnnnnnnnnnnnnnnnnnnnnnnnnnnnnnnnnnnnnnnnnnnnnnnnnnnnnnnnnnnnnnnnnnnnnnnnnnnnnnnnnnnnnnnnnnnnnnnnnnnnnnnnnnnnnnnnnnnnnnnnnnnnnnnnnnnnnnnnnnnnnnnnnnnnnnnnnnnnnnnnnnnnnnnnnnnnnnnnnnnnnnnnnnnnnnnnnnnnnnnnnnnnnnnnnnnnnnnnnnnnnnnnnnnnnnnnnnnnnnnnnnnnnnnnnnnnnnnnnnnnnnnnnnnnnnnnnnnnnnnnnnnnnnnnnnnnnnnnnnnnnnnnnnnnnnnnnnnnnnnnnnnnnnnnnnnnnnnnnnnnnnnnnnnnnnnnnnnnnnnnnnnnnnnnnnnnnnnnnnnnnnnnnnnnnnnnnnnnnnnnnnnnnnnnnnnnnnnnnnnnnnnnnnnnnnnnnnnnnnnnnnnnnnnnnnnnnnnnnnnnnnnnnnnnnnnnnnnnnnnnnnnnnnnnnnnnnnnnnnnnnnnnnnnnnnnnnnnnnnnnnnnnnnnnnnnnnnnnnnnnnnnnnnnnnnnnnnnnnnnnnnnnnnnnnnnnnnnnnnnnnnnnnnnnnnnnnnnnnnnnnnnnnnnnnnnnnnnnnnnnnnnnnnnnnnnnnnnnnnnnnnnnnnnnnnnnnnnnnnnnnnnnnnnnnnnnnnnnnnnnnnnnnnnnnnnnnnnnnnnnnnnnnnnnnnnnnnnnnnnnnnnnnnnnnnnnnnnnnnnnnnnnnnnnnnnnnnnnnnnnnnnnnnnnnnnnnnnnnnnnnnnnnnnnnnnnnnnnnnnnnnnnnnnnnnnnnnnnnnnnnnnnnnnnnnnnnnnnnnnnnnnnnnnnnnnnnnnnnnnnnnnnnnnnnnnnnnnnnnnnnnnnnnnnnnnnnnnnnnnnnnnnnnnnnnnnnnnnnnnnnnnnnnnnnnnnnnnnnnnnnnnnnnnnnnnnnnnnnnnnnnnnnnnnnnnnnnnnnnnnnnnnnnnnnnnnnnnnnnnnnnnnnnnnnnnnnnnnnnnnnnnnnnnnnnnnnnnnnnnnnnnnnnnnnnnnnnnnnnnnnnnnnnnnnnnnnnnnnnnnnnnnnnnnnnnnnnnnnnnnnnnnnnnnnnnnnnnnnnnnnnnnnnnnnnnnnnnnnnnnnnnnnnnnnnnnnnnnnnnnnnnnnnnnnnnnnnnnnnnnnnnnnnnnnnnnnnnnnnnnnnnnnnnnnnnnnnnnnnnnnnnnnnnnnnnnnnnnnnnnnnnnnnnnnnnnnnnnnnnnnnnnnnnnnnnnnnnnnnnnnnnnnnnnnnnnnnnnnnnnnnnnnnnnnnnnnnnnnnnnnnnnnnnnnnnnnnnnnnnnnnnnnnnnnnnnnnnnnnnnnnnnnnnnnnnnnnnnnnnnnnnnnnnnnnnnnnnnnnnnnnnnnnnnnnnnnnnnnnnnnnnnnnnnnnnnnnnnnnnnnnnnnnnnnnnnnnnnnnnnnnnnnnnnnnnnnnnnnnnnnnnnnnnnnnnnnnnnnnnnnnnnnnnnnnnnnnnnnnnnnnnnnnnnnnnnnnnnnnnnnnnnnnnnnnnnnnnnnnnnnnnnnnnnnnnnnnnnnnnnnnnnnnnnnnnnnnnnnnnnnnnnnnnnnnnnnnnnnnnnnnnnnnnnnnnnnnnnnnnnnnnnnnnnnnnnnnnnnnnnnnnnnnnnnnnnnnnnnnnnnnnnnnnnnnnnnnnnnnnnnnnnnnnnnnnnnnnnnnnnnnnnnnnnnnnnnnnnnnnnnnnnnnnnnnnnnnnnnnnnnnnnnnnnnnnnnnnnnnnnnnnnnnnnnnnnnnnnnnnnnnnnnnnnnnnnnnnnnnnnnnnnnnnnnnnnnnnnnnnnnnnnnnnnnnnnnnnnnnnnnnnnnnnnnnnnnnnnnnnnnnnnnnnnnnnnnnnnnnnnnnnnnnnnnnnnnnnnnnnnnnnnnnnnnnnnnnnnnnnnnnnnnnnnnnnnnnnnnnnnnnnnnnnnnnnnnnnnnnnnnnnnnnnnnnnnnnnnnnnnnnnnnnnnnnnnnnnnnnnnnnnnnnnnnnnnnnnnnnnnnnnnnnnnnnnnnnnnnnnnnnnnnnnnnnnnnnnnnnnnnnnnnnnnnnnnnnnnnnnnnnnnnnnnnnnnnnnnnnnnnnnnnnnnnnnnnnnnnnnnnnnnnnnnnnnnnnnnnnnnnnnnnnnnnnnnnnnnnnnnnnnnnnnnnnnnnnnnnnnnnnnnnnnnnnnnnnnnnnnnnnnnnnnnnnnnnnnnnnnnnnnnnnnnnnnnnnnnnnnnnnnnnnnnnnnnnnnnnnnnnnnnnnnnnnnnnnnnnnnnnnnnnnnnnnnnnnnnnnnnnnnnnnnnnnnnnnnnnnnnnnnnnnnnnnnnnnnnnnnnnnnnnnnnnnnnnnnnnnnnnnnnnnnnnnnnnnnnnnnnnnnnnnnnnnnnnnnnnnnnnnnnnnnnnnnnnnnnnnnnnnnnnnnnnnnnnnnnnnnnnnnnnnnnnnnnnnnnnnnnnnnnnnnnnnnnnnnnnnnnnnnnnnnnnnnnnnnnnnnnnnnnnnnnnnnnnnnnnnnnnnnnnnnnnnnnnnnnnnnnnnnnnnnnnnnnnnnnnnnnnnnnnnnnnnnnnnnnnnnnnnnnnnnnnnnnnnnnnnnnnnnnnnnnnnnnnnnnnnnnnnnnnnnnnnnnnnnnnnnnnnnnnnnnnnnnnnnnnnnnnnnnnnnnnnnnnnnnnnnnnnnnnnnnnnnnnnnnnnnnnnnnnnnnnnnnnnnnnnnnnnnnnnnnnnnnnnnnnnnnnnnnnnnnnnnnnnnnnnnnnnnnnnnnnnnnnnnnnnnnnnnnnnnnnnnnnnnnnnnnnnnnnnnnnnnnnnnnnnnnnnnnnnnnnnnnnnnnnnnnnnnnnnnnnnnnnnnnnnnnnnnnnnnnnnnnnnnnnnnnnnnnnnnnnnnnnnnnnnnnnnnnnnnnnnnnnnnnnnnnnnnnnnnnnnnnnnnnnnnnnnnnnnnnnnnnnnnnnnnnnnnnnnnnnnnnnnnnnnnnnnnnnnnnnnnnnnnnnnnnnnnnnnnnnnnnnnnnnnnnnnnnnnnnnnnnnnnnnnnnnnnnnnnnnnnnnnnnnnnnnnnnnnnnnnnnnnnnnnnnnnnnnnnnnnnnnnnnnnnnnnnnnnnnnnnnnnnnnnnnnnnnnnnnnnnnnnnnnnnnnnnnnnnnnnnnnnnnnnnnnnnnnnnnnnnnnnnnnnnnnnnnnnnnnnnnnnnnnnnnnnnnnnnnnnnnnnnnnnnnnnnnnnnnnnnnnnnnnnnnnnnnnnnnnnnnnnnnnnnnnnnnnnnnnnnnnnnnnnnnnnnnnnnnnnnnnnnnnnnnnnnnnnnnnnnnnnnnnnnnnnnnnnnnnnnnnnnnnnnnnnnnnnnnnnnnnnnnnnnnnnnnnnnnnnnnnnnnnnnnnnnnnnnnnnnnnnnnnnnnnnnnnnnnnnnnnnnnnnnnnnnnnnnnnnnnnnnnnnnnnnnnnnnnnnnnnnnnnnnnnnnnnnnnnnnnnnnnnnnnnnnnnnnnnnnnnnnnnnnnnnnnnnnnnnnnnnnnnnnnnnnnnnnnnnnnnnnnnnnnnnnnnnnnnnnnnnnnnnnnnnnnnnnnnnnnnnnnnnnnnnnnnnnnnnnnnnnnnnnnnnnnnnnnnnnnnnnnnnnnnnnnnnnnnnnnnnnnnnnnnnnnnnnnnnnnnnnnnnnnnnnnnnnnnnnnnnnnnnnnnnnnnnnnnnnnnnnnnnnnnnnnnnnnnnnnnnnnnnnnnnnnnnnnnnnnnnnnnnnnnnnnnnnnnnnnnnnnnnnnnnnnnnnnnnnnnnnnnnnnnnnnnnnnnnnnnnnnnnnnnnnnnnnnnnnnnnnnnnnnnnnnnnnnnnnnnnnnnnnnnnnnnnnnnnnnnnnnnnnnnnnnnnnnnnnnnnnnnnnnnnnnnnnnnnnnnnnnnnnnnnnnnnnnnnnnnnnnnnnnnnnnnnnnnnnnnnnnnnnnnnnnnnnnnnnnnnnnnnnnnnnnnnnnnnnnnnnnnnnnnnnnnnnnnnnnnnnnnnnnnnnnnnnnnnnnnnnnnnnnnnnnnnnnnnnnnnnnnnnnnnnnnnnnnnnnnnnnnnnnnnnnnnnnnnnnnnnnnnnnnnnnnnnnnnnnnnnnnnnnnnnnnnnnnnnnnnnnnnnnnnnnnnnnnnnnnnnnnnnnnnnnnnnnnnnnnnnnnnnnnnnnnnnnnnnnnnnnnnnnnnnnnnnnnnnnnnnnnnnnnnnnnnnnnnnnnnnnnnnnnnnnnnnnnnnnnnnnnnnnnnnnnnnnnnnnnnnnnnnnnnnnnnnnnnnnnnnnnnnnnnnnnnnnnnnnnnnnnnnnnnnnnnnnnnnnnnnnnnnnnnnnnnnnnnnnnnnnnnnnnnnnnnnnnnnnnnnnnnnnnnnnnnnnnnnnnnnnnnnnnnnnnnnnnnnnnnnnnnnnnnnnnnnnnnnnnnnnnnnnnnnnnnnnnnnnnnnnnnnnnnnnnnnnnnnnnnnnnnnnnnnnnnnnnnnnnnnnnnnnnnnnnnnnnnnnnnnnnnnnnnnnnnnnnnnnnnnnnnnnnnnnnnnnnnnnnnnnnnnnnnnnnnnnnnnnnnnnnnnnnnnnnnnnnnnnnnnnnnnnnnnnnnnnnnnnnnnnnnnnnnnnnnnnnnnnnnnnnnnnnnnnnnnnnnnnnnnnnnnnnnnnnnnnnnnnnnnnnnnnnnnnnnnnnnnnnnnnnnnnnnnnnnnnnnnnnnnnnnnnnnnnnnnnnnnnnnnnnnnnnnnnnnnnnnnnnnnnnnnnnnnnnnnnnnnnnnnnnnnnnnnnnnnnnnnnnnnnnnnnnnnnnnnnnnnnnnnnnnnnnnnnnnnnnnnnnnnnnnnnnnnnnnnnnnnnnnnnnnnnnnnnnnnnnnnnnnnnnnnnnnnnnnnnnnnnnnnnnnnnnnnnnnnnnnnnnnnnnnnnnnnnnnnnnnnnnnnnnnnnnnnnnnnnnnnnnnnnnnnnnnnnnnnnnnnnnnnnnnnnnnnnnnnnnnnnnnnnnnnnnnnnnnnnnnnnnnnnnnnnnnnnnnnnnnnnnnnnnnnnnnnnnnnnnnnnnnnnnnnnnnnnnnnnnnnnnnnnnnnnnnnnnnnnnnnnnnnnnnnnnnnnnnnnnnnnnnnnnnnnnnnnnnnnnnnnnnnnnnnnnnnnnnnnnnnnnnnnnnnnnnnnnnnnnnnnnnnnnnnnnnnnnnnnnnnnnnnnnnnnnnnnnnnnnnnnnnnnnnnnnnnnnnnnnnnnnnnnnnnnnnnnnnnnnnnnnnnnnnnnnnnnnnnnnnnnnnnnnnnnnnnnnnnnnnnnnnnnnnnnnnnnnnnnnnnnnnnnnnnnnnnnnnnnnnnnnnnnnnnnnnnnnnnnnnnnnnnnnnnnnnnnnnnnnnnnnnnnnnnnnnnnnnnnnnnnnnnnnnnnnnnnnnnnnnnnnnnnnnnnnnnnnnnnnnnnnnnnnnnnnnnnnnnnnnnnnnnnnnnnnnnnnnnnnnnnnnnnnnnnnnnnnnnnnnnnnnnnnnnnnnnnnnnnnnnnnnnnnnnnnnnnnnnnnnnnnnnnnnnnnnnnnnnnnnnnnnnnnnnnnnnnnnnnnnnnnnnnnnnnnnnnnnnnnnnnnnnnnnnnnnnnnnnnnnnnnnnnnnnnnnnnnnnnnnnnnnnnnnnnnnnnnnnnnnnnnnnnnnnnnnnnnnnnnnnnnnnnnnnnnnnnnnnnnnnnnnnnnnnnnnnnnnnnnnnnnnnnnnnnnnnnnnnnnnnnnnnnnnnnnnnnnnnnnnnnnnnnnnnnnnnnnnnnnnnnnnnnnnnnnnnnnnnnnnnnnnnnnnnnnnnnnnnnnnnnnnnnnnnnnnnnnnnnnnnnnnnnnnnnnnnnnnnnnnnnnnnnnnnnnnnnnnnnnnnnnnnnnnnnnnnnnnnnnnnnnnnnnnnnnnnnnnnnnnnnnnnnnnnnnnnnnnnnnnnnnnnnnnnnnnnnnnnnnnnnnnnnnnnnnnnnnnnnnnnnnnnnnnnnnnnnnnnnnnnnnnnnnnnnnnnnnnnnnnnnnnnnnnnnnnnnnnnnnnnnnnnnnnnnnnnnnnnnnnnnnnnnnnnnnnnnnnnnnnnnnnnnnnnnnnnnnnnnnnnnnnnnnnnnnnnnnnnnnnnnnnnnnnnnnnnnnnnnnnnnnnnnnnnnnnnnnnnnnnnnnnnnnnnnnnnnnnnnnnnnnnnnnnnnnnnnnnnnnnnnnnnnnnnnnnnnnnnnnnnnnnnnnnnnnnnnnnnnnnnnnnnnnnnnnnnnnnnnnnnnnnnnnnnnnnnnnnnnnnnnnnnnnnnnnnnnnnnnnnnnnnnnnnnnnnnnnnnnnnnnnnnnnnnnnnnnnnnnnnnnnnnnnnnnnnnnnnnnnnnnnnnnnnnnnnnnnnnnnnnnnnnnnnnnnnnnnnnnnnnnnnnnnnnnnnnnnnnnnnnnnnnnnnnnnnnnnnnnnnnnnnnnnnnnnnnnnnnnnnnnnnnnnnnnnnnnnnnnnnnnnnnnnnnnnnnnnnnnnnnnnnnnnnnnnnnnnnnnnnnnnnnnnnnnnnnnnnnnnnnnnnnnnnnnnnnnnnnnnnnnnnnnnnnnnnnnnnnnnnnnnnnnnnnnnnnnnnnnnnnnnnnnnnnnnnnnnnnnnnnnnnnnnnnnnnnnnnnnnnnnnnnnnnnnnnnnnnnnnnnnnnnnnnnnnnnnnnnnnnnnnnnnnnnnnnnnnnnnnnnnnnnnnnnnnnnnnnnnnnnnnnnnnnnnnnnnnnnnnnnnnnnnnnnnnnnnnnnnnnnnnnnnnnnnnnnnnnnnnnnnnnnnnnnnnnnnnnnnnnnnnnnnnnnnnnnnnnnnnnnnnnnnnnnnnnnnnnnnnnnnnnnnnnnnnnnnnnnnnnnnnnnnnnnnnnnnnnnnnnnnnnnnnnnnnnnnnnnnnnnnnnnnnnnnnnnnnnnnnnnnnnnnnnnnnnnnnnnnnnnnnnnnnnnnnnnnnnnnnnnnnnnnnnnnnnnnnnnnnnnnnnnnnnnnnnnnnnnnnnnnnnnnnnnnnnnnnnnnnnnnnnnnnnnnnnnnnnnnnnnnnnnnnnnnnnnnnnnnnnnnnnnnnnnnnnnnnnnnnnnnnnnnnnnnnnnnnnnnnnnnnnnnnnnnnnnnnnnnnnnnnnnnnnnnnnnnnnnnnnnnnnnnnnnnnnnnnnnnnnnnnnnnnnnnnnnnnnnnnnnnnnnnnnnnnnnnnnnnnnnnnnnnnnnnnnnnnnnnnnnnnnnnnnnnnnnnnnnnnnnnnnnnnnnnnnnnnnnnnnnnnnnnnnnnnnnnnnnnnnnnnnnnnnnnnnnnnnnnnnnnnnnnnnnnnnnnnnnnnnnnnnnnnnnnnnnnnnnnnnnnnnnnnnnnnnnnnnnnnnnnnnnnnnnnnnnnnnnnnnnnnnnnnnnnnnnnnnnnnnnnnnnnnnnnnnnnnnnnnnnnnnnnnnnnnnnnnnnnnnnnnnnnnnnnnnnnnnnnnnnnnnnnnnnnnnnnnnnnnnnnnnnnnnnnnnnnnnnnnnnnnnnnnnnnnnnnnnnnnnnnnnnnnnnnnnnnnnnnnnnnnnnnnnnnnnnnnnnnnnnnnnnnnnnnnnnnnnnnnnnnnnnnnnnnnnnnnnnnnnnnnnnnnnnnnnnnnnnnnnnnnnnnnnnnnnnnnnnnnnnnnnnnnnnnnnnnnnnnnnnnnnnnnnnnnnnnnnnnnnnnnnnnnnnnnnnnnnnnnnnnnnnnnnnnnnnnnnnnnnnnnnnnnnnnnnnnnnnnnnnnnnnnnnnnnnnnnnnnnnnnnnnnnnnnnnnnnnnnnnnnnnnnnnnnnnnnnnnnnnnnnnnnnnnnnnnnnnnnnnnnnnnnnnnnnnnnnnnnnnnnnnnnnnnnnnnnnnnnnnnnnnnnnnnnnnnnnnnnnnnnnnnnnnnnnnnnnnnnnnnnnnnnnnnnnnnnnnnnnnnnnnnnnnnnnnnnnnnnnnnnnnnnnnnnnnnnnnnnnnnnnnnnnnnnnnnnnnnnnnnnnnnnnnnnnnnnnnnnnnnnnnnnnnnnnnnnnnnnnnnnnnnnnnnnnnnnnnnnnnnnnnnnnnnnnnnnnnnnnnnnnnnnnnnnnnnnnnnnnnnnnnnnnnnnnnnnnnnnnnnnnnnnnnnnnnnnnnnnnnnnnnnnnnnnnnnnnnnnnnnnnnnnnnnnnnnnnnnnnnnnnnnnnnnnnnnnnnnnnnnnnnnnnnnnnnnnnnnnnnnnnnnnnnnnnnnnnnnnnnnnnnnnnnnnnnnnnnnnnnnnnnnnnnnnnnnnnnnnnnnnnnnnnnnnnnnnnnnnnnnnnnnnnnnnnnnnnnnnnnnnnnnnnnnnnnnnnnnnnnnnnnnnnnnnnnnnnnnnnnnnnnnnnnnnnnnnnnnnnnnnnnnnnnnnnnnnnnnnnnnnnnnnnnnnnnnnnnnnnnnnnnnnnnnnnnnnnnnnnnnnnnnnnnnnnnnnnnnnnnnnnnnnnnnnnnnnnnnnnnnnnnnnnnnnnnnnnnnnnnnnnnnnnnnnnnnnnnnnnnnnnnnnnnnnnnnnnnnnnnnnnnnnnnnnnnnnnnnnnnnnnnnnnnnnnnnnnnnnnnnnnnnnnnnnnnnnnnnnnnnnnnnnnnnnnnnnnnnnnnnnnnnnnnnnnnnnnnnnnnnnnnnnnnnnnnnnnnnnnnnnnnnnnnnnnnnnnnnnnnnnnnnnnnnnnnnnnnnnnnnnnnnnnnnnnnnnnnnnnnnnnnnnnnnnnnnnnnnnnnnnnnnnnnnnnnnnnnnnnnnnnnnnnnnnnnnnnnnnnnnnnnnnnnnnnnnnnnnnnnnnnnnnnnnnnnnnnnnnnnnnnnnnnnnnnnnnnnnnnnnnnnnnnnnnnnnnnnnnnnnnnnnnnnnnnnnnnnnnnnnnnnnnnnnnnnnnnnnnnnnnnnnnnnnnnnnnnnnnnnnnnnnnnnnnnnnnnnnnnnnnnnnnnnnnnnnnnnnnnnnnnnnnnnnnnnnnnnnnnnnnnnnnnnnnnnnnnnnnnnnnnnnnnnnnnnnnnnnnnnnnnnnnnnnnnnnnnnnnnnnnnnnnnnnnnnnnnnnnnnnnnnnnnnnnnnnnnnnnnnnnnnnnnnnnnnnnnnnnnnnnnnnnnnnnnnnnnnnnnnnnnnnnnnnnnnnnnnnnnnnnnnnnnnnnnnnnnnnnnnnnnnnnnnnnnnnnnnnnnnnnnnnnnnnnnnnnnnnnnnnnnnnnnnnnnnnnnnnnnnnnnnnnnnnnnnnnnnnnnnnnnnnnnnnnnnnnnnnnnnnnnnnnnnnnnnnnnnnnnnnnnnnnnnnnnnnnnnnnnnnnnnnnnnnnnnnnnnnnnnnnnnnnnnnnnnnnnnnnnnnnnnnnnnnnnnnnnnnnnnnnnnnnnnnnnnnnnnnnnnnnnnnnnnnnnnnnnnnnnnnnnnnnnnnnnnnnnnnnnnnnnnnnnnnnnnnnnnnnnnnnnnnnnnnnnnnnnnnnnnnnnnnnnnnnnnnnnnnnnnnnnnnnnnnnnnnnnnnnnnnnnnnnnnnnnnnnnnnnnnnnnnnnnnnnnnnnnnnnnnnnnnnnnnnnnnnnnnnnnnnnnnnnnnnnnnnnnnnnnnnnnnnnnnnnnnnnnnnnnnnnnnnnnnnnnnnnnnnnnnnnnnnnnnnnnnnnnnnnnnnnnnnnnnnnnnnnnnnnnnnnnnnnnnnnnnnnnnnnnnnnnnnnnnnnnnnnnnnnnnnnnnnnnnnnnnnnnnnnnnnnnnnnnnnnnnnnnnnnnnnnnnnnnnnnnnnnnnnnnnnnnnnnnnnnnnnnnnnnnnnnnnnnnnnnnnnnnnnnnnnnnnnnnnnnnnnnnnnnnnnnnnnnnnnnnnnnnnnnnnnnnnnnnnnnnnnnnnnnnnnnnnnnnnnnnnnnnnnnnnnnnnnnnnnnnnnnnnnnnnnnnnnnnnnnnnnnnnnnnnnnnnnnnnnnnnnnnnnnnnnnnnnnnnnnnnnnnnnnnnnnnnnnnnnnnnnnnnnnnnnnnnnnnnnnnnnnnnnnnnnnnnnnnnnnnnnnnnnnnnnnnnnnnnnnnnnnnnnnnnnnnnnnnnnnnnnnnnnnnnnnnnnnnnnnnnnnnnnnnnnnnnnnnnnnnnnnnnnnnnnnnnnnnnnnnnnnnnnnnnnnnnnnnnnnnnnnnnnnnnnnnnnnnnnnnnnnnnnnnnnnnnnnnnnnnnnnnnnnnnnnnnnnnnnnnnnnnnnnnnnnnnnnnnnnnnnnnnnnnnnnnnnnnnnnnnnnnnnnnnnnnnnnnnnnnnnnnnnnnnnnnnnnnnnnnnnnnnnnnnnnnnnnnnnnnnnnnnnnnnnnnnnnnnnnnnnnnnnnnnnnnnnnnnnnnnnnnnnnnnnnnnnnnnnnnnnnnnnnnnnnnnnnnnnnnnnnnnnnnnnnnnnnnnnnnnnnnnnnnnnnnnnnnnnnnnnnnnnnnnnnnnnnnnnnnnnnnnnnnnnnnnnnnnnnnnnnnnnnnnnnnnnnnnnnnnnnnnnnnnnnnnnnnnnnnnnnnnnnnnnnnnnnnnnnnnnnnnnnnnnnnnnnnnnnnnnnnnnnnnnnnnnnnnnnnnnnnnnnnnnnnnnnnnnnnnnnnnnnnnnnnnnnnnnnnnnnnnnnnnnnnnnnnnnnnnnnnnnnnnnnnnnnnnnnnnnnnnnnnnnnnnnnnnnnnnnnnnnnnnnnnnnnnnnnnnnnnnnnnnnnnnnnnnnnnnnnnnnnnnnnnnnnnnnnnnnnnnnnnnnnnnnnnnnnnnnnnnnnnnnnnnnnnnnnnnnnnnnnnnnnnnnnnnnnnnnnnnnnnnnnnnnnnnnnnnnnnnnnnnnnnnnnnnnnnnnnnnnnnnnnnnnnnnnnnnnnnnnnnnnnnnnnnnnnnnnnnnnnnnnnnnnnnnnnnnnnnnnnnnnnnnnnnnnnnnnnnnnnnnnnnnnnnnnnnnnnnnnnnnnnnnnnnnnnnnnnnnnnnnnnnnnnnnnnnnnnnnnnnnnnnnnnnnnnnnnnnnnnnnnnnnnnnnnnnnnnnnnnnnnnnnnnnnnnnnnnnnnnnnnnnnnnnnnnnnnnnnnnnnnnnnnnnnnnnnnnnnnnnnnnnnnnnnnnnnnnnnnnnnnnnnnnnnnnnnnnnnnnnnnnnnnnnnnnnnnnnnnnnnnnnnnnnnnnnnnnnnnnnnnnnnnnnnnnnnnnnnnnnnnnnnnnnnnnnnnnnnnnnnnnnnnnnnnnnnnnnnnnnnnnnnnnnnnnnnnnnnnnnnnnnnnnnnnnnnnnnnnnnnnnnnnnnnnnnnnnnnnnnnnnnnnnnnnnnnnnnnnnnnnnnnnnnnnnnnnnnnnnnnnnnnnnnnnnnnnnnnnnnnnnnnnnnnnnnnnnnnnnnnnnnnnnnnnnnnnnnnnnnnnnnnnnnnnnnnnnnnnnnnnnnnnnnnnnnnnnnnnnnnnnnnnnnnnnnnnnnnnnnnnnnnnnnnnnnnnnnnnnnnnnnnnnnnnnnnnnnnnnnnnnnnnnnnnnnnnnnnnnnnnnnnnnnnnnnnnnnnnnnnnnnnnnnnnnnnnnnnnnnnnnnnnnnnnnnnnnnnnnnnnnnnnnnnnnnnnnnnnnnnnnnnnnnnnnnnnnnnnnnnnnnnnnnnnnnnnnnnnnnnnnnnnnnnnnnnnnnnnnnnnnnnnnnnnnnnnnnnnnnnnnnnnnnnnnnnnnnnnnnnnnnnnnnnnnnnnnnnnnnnnnnnnnnnnnnnnnnnnnnnnnnnnnnnnnnnnnnnnnnnnnnnnnnnnnnnnnnnnnnnnnnnnnnnnnnnnnnnnnnnnnnnnnnnnnnnnnnnnnnnnnnnnnnnnnnnnnnnnnnnnnnnnnnnnnnnnnnnnnnnnnnnnnnnnnnnnnnnnnnnnnnnnnnnnnnnnnnnnnnnnnnnnnnnnnnnnnnnnnnnnnnnnnnnnnnnnnnnnnnnnnnnnnnnnnnnnnnnnnnnnnnnnnnnnnnnnnnnnnnnnnnnnnnnnnnnnnnnnnnnnnnnnnnnnnnnnnnnnnnnnnnnnnnnnnnnnnnnnnnnnnnnnnnnnnnnnnnnnnnnnnnnnnnnnnnnnnnnnnnnnnnnnnnnnnnnnnnnnnnnnnnnnnnnnnnnnnnnnnnnnnnnnnnnnnnnnnnnnnnnnnnnnnnnnnnnnnnnnnnnnnnnnnnnnnnnnnnnnnnnnnnnnnnnnnnnnnnnnnnnnnnnnnnnnnnnnnnnnnnnnnnnnnnnnnnnnnnnnnnnnnnnnnnnnnnnnnnnnnnnnnnnnnnnnnnnnnnnnnnnnnnnnnnnnnnnnnnnnnnnnnnnnnnnnnnnnnnnnnnnnnnnnnnnnnnnnnnnnnnnnnnnnnnnnnnnnnnnnnnnnnnnnnnnnnnnnnnnnnnnnnnnnnnnnnnnnnnnnnnnnnnnnnnnnnnnnnnnnnnnnnnnnnnnnnnnnnnnnnnnnnnnnnnnnnnnnnnnnnnnnnnnnnnnnnnnnnnnnnnnnnnnnnnnnnnnnnnnnnnnnnnnnnnnnnnnnnnnnnnnnnnnnnnnnnnnnnnnnnnnnnnnnnnnnnnnnnnnnnnnnnnnnnnnnnnnnnnnnnnnnnnnnnnnnnnnnnnnnnnnnnnnnnnnnnnnnnnnnnnnnnnnnnnnnnnnnnnnnnnnnnnnnnnnnnnnnnnnnnnnnnnnnnnnnnnnnnnnnnnnnnnnnnnnnnnnnnnnnnnnnnnnnnnnnnnnnnnnnnnnnnnnnnnnnnnnnnnnnnnnnnnnnnnnnnnnnnnnnnnnnnnnnnnnnnnnnnnnnnnnnnnnnnnnnnnnnnnnnnnnnnnnnnnnnnnnnnnnnnnnnnnnnnnnnnnnnnnnnnnnnnnnnnnnnnnnnnnnnnnnnnnnnnnnnnnnnnnnnnnnnnnnnnnnnnnnnnnnnnnnnnnnnnnnnnnnnnnnnnnnnnnnnnnnnnnnnnnnnnnnnnnnnnnnnnnnnnnnnnnnnnnnnnnnnnnnnnnnnnnnnnnnnnnnnnnnnnnnnnnnnnnnnnnnnnnnnnnnnnnnnnnnnnnnnnnnnnnnnnnnnnnnnnnnnnnnnnnnnnnnnnnnnnnnnnnnnnnnnnnnnnnnnnnnnnnnnnnnnnnnnnnnnnnnnnnnnnnnnnnnnnnnnnnnnnnnnnnnnnnnnnnnnnnnnnnnnnnnnnnnnnnnnnnnnnnnnnnnnnnnnnnnnnnnnnnnnnnnnnnnnnnnnnnnnnnnnnnnnnnnnnnnnnnnnnnnnnnnnnnnnnnnnnnnnnnnnnnnnnnnnnnnnnnnnnnnnnnnnnnnnnnnnnnnnnnnnnnnnnnnnnnnnnnnnnnnnnnnnnnnnnnnnnnnnnnnnnnnnnnnnnnnnnnnnnnnnnnnnnnnnnnnnnnnnnnnnnnnnnnnnnnnnnnnnnnnnnnnnnnnnnnnnnnnnnnnnnnnnnnnnnnnnnnnnnnnnnnnnnnnnnnnnnnnnnnnnnnnnnnnnnnnnnnnnnnnnnnnnnnnnnnnnnnnnnnnnnnnnnnnnnnnnnnnnnnnnnnnnnnnnnnnnnnnnnnnnnnnnnnnnnnnnnnnnnnnnnnnnnnnnnnnnnnnnnnnnnnnnnnnnnnnnnnnnnnnnnnnnnnnnnnnnnnnnnnnnnnnnnnnnnnnnnnnnnnnnnnnnnnnnnnnnnnnnnnnnnnnnnnnnnnnnnnnnnnnnnnnnnnnnnnnnnnnnnnnnnnnnnnnnnnnnnnnnnnnnnnnnnnnnnnnnnnnnnnnnnnnnnnnnnnnnnnnnnnnnnnnnnnnnnnnnnnnnnnnnnnnnnnnnnnnnnnnnnnnnnnnnnnnnnnnnnnnnnnnnnnnnnnnnnnnnnnnnnnnnnnnnnnnnnnnnnnnnnnnnnnnnnnnnnnnnnnnnnnnnnnnnnnnnnnnnnnnnnnnnnnnnnnnnnnnnnnnnnnnnnnnnnnnnnnnnnnnnnnnnnnnnnnnnnnnnnnnnnnnnnnnnnnnnnnnnnnnnnnnnnnnnnnnnnnnnnnnnnnnnnnnnnnnnnnnnnnnnnnnnnnnnnnnnnnnnnnnnnnnnnnnnnnnnnnnnnnnnnnnnnnnnnnnnnnnnnnnnnnnnnnnnnnnnnnnnnnnnnnnnnnnnnnnnnnnnnnnnnnnnnnnnnnnnnnnnnnnnnnnnnnnnnnnnnnnnnnnnnnnnnnnnnnnnnnnnnnnnnnnnnnnnnnnnnnnnnnnnnnnnnnnnnnnnnnnnnnnnnnnnnnnnnnnnnnnnnnnnnnnnnnnnnnnnnnnnnnnnnnnnnnnnnnnnnnnnnnnnnnnnnnnnnnnnnnnnnnnnnnnnnnnnnnnnnnnnnnnnnnnnnnnnnnnnnnnnnnnnnnnnnnnnnnnnnnnnnnnnnnnnnnnnnnnnnnnnnnnnnnnnnnnnnnnnnnnnnnnnnnnnnnnnnnnnnnnnnnnnnnnnnnnnnnnnnnnnnnnnnnnnnnnnnnnnnnnnnnnnnnnnnnnnnnnnnnnnnnnnnnnnnnnnnnnnnnnnnnnnnnnnnnnnnnnnnnnnnnnnnnnnnnnnnnnnnnnnnnnnnnnnnnnnnnnnnnnnnnnnnnnnnnnnnnnnnnnnnnnnnnnnnnnnnnnnnnnnnnnnnnnnnnnnnnnnnnnnnnnnnnnnnnnnnnnnnnnnnnnnnnnnnnnnnnnnnnnnnnnnnnnnnnnnnnnnnnnnnnnnnnnnnnnnnnnnnnnnnnnnnnnnnnnnnnnnnnnnnnnnnnnnnnnnnnnnnnnnnnnnnnnnnnnnnnnnnnnnnnnnnnnnnnnnnnnnnnnnnnnnnnnnnnnnnnnnnnnnnnnnnnnnnnnnnnnnnnnnnnnnnnnnnnnnnnnnnnnnnnnnnnnnnnnnnnnnnnnnnnnnnnnnnnnnnnnnnnnnnnnnnnnnnnnnnnnnnnnnnnnnnnnnnnnnnnnnnnnnnnnnnnnnnnnnnnnnnnnnnnnnnnnnnnnnnnnnnnnnnnnnnnnnnnnnnnnnnnnnnnnnnnnnnnnnnnnnnnnnnnnnnnnnnnnnnnnnnnnnnnnnnnnnnnnnnnnnnnnnnnnnnnnnnnnnnnnnnnnnnnnnnnnnnnnnnnnnnnnnnnnnnnnnnnnnnnnnnnnnnnnnnnnnnnnnnnnnnnnnnnnnnnnnnnnnnnnnnnnnnnnnnnnnnnnnnnnnnnnnnnnnnnnnnnnnnnnnnnnnnnnnnnnnnnnnnnnnnnnnnnnnnnnnnnnnnnnnnnnnnnnnnnnnnnnnnnnnnnnnnnnnnnnnnnnnnnnnnnnnnnnnnnnnnnnnnnnnnnnnnnnnnnnnnnnnnnnnnnnnnnnnnnnnnnnnnnnnnnnnnnnnnnnnnnnnnnnnnnnnnnnnnnnnnnnnnnnnnnnnnnnnnnnnnnnnnnnnnnnnnnnnnnnnnnnnnnnnnnnnnnnnnnnnnnnnnnnnnnnnnnnnnnnnnnnnnnnnnnnnnnnnnnnnnnnnnnnnnnnnnnnnnnnnnnnnnnnnnnnnnnnnnnnnnnnnnnnnnnnnnnnnnnnnnnnnnnnnnnnnnnnnnnnnnnnnnnnnnnnnnnnnnnnnnnnnnnnnnnnnnnnnnnnnnnnnnnnnnnnnnnnnnnnnnnnnnnnnnnnnnnnnnnnnnnnnnnnnnnnnnnnnnnnnnnnnnnnnnnnnnnnnnnnnnnnnnnnnnnnnnnnnnnnnnnnnnnnnnnnnnnnnnnnnnnnnnnnnnnnnnnnnnnnnnnnnnnnnnnnnnnnnnnnnnnnnnnnnnnnnnnnnnnnnnnnnnnnnnnnnnnnnnnnnnnnnnnnnnnnnnnnnnnnnnnnnnnnnnnnnnnnnnnnnnnnnnnnnnnnnnnnnnnnnnnnnnnnnnnnnnnnnnnnnnnnnnnnnnnnnnnnnnnnnnnnnnnnnnnnnnnnnnnnnnnnnnnnnnnnnnnnnnnnnnnnnnnnnnnnnnnnnnnnnnnnnnnnnnnnnnnnnnnnnnnnnnnnnnnnnnnnnnnnnnnnnnnnnnnnnnnnnnnnnnnnnnnnnnnnnnnnnnnnnnnnnnnnnnnnnnnnnnnnnnnnnnnnnnnnnnnnnnnnnnnnnnnnnnnnnnnnnnnnnnnnnnnnnnnnnnnnnnnnnnnnnnnnnnnnnnnnnnnnnnnnnnnnnnnnnnnnnnnnnnnnnnnnnnnnnnnnnnnnnnnnnnnnnnnnnnnnnnnnnnnnnnnnnnnnnnnnnnnnnnnnnnnnnnnnnnnnnnnnnnnnnnnnnnnnnnnnnnnnnnnnnnnnnnnnnnnnnnnnnnnnnnnnnnnnnnnnnnnnnnnnnnnnnnnnnnnnnnnnnnnnnnnnnnnnnnnnnnnnnnnnnnnnnnnnnnnnnnnnnnnnnnnnnnnnnnnnnnnnnnnnnnnnnnnnnnnnnnnnnnnnnnnnnnnnnnnnnnnnnnnnnnnnnnnnnnnnnnnnnnnnnnnnnnnnnnnnnnnnnnnnnnnnnnnnnnnnnnnnnnnnnnnnnnnnnnnnnnnnnnnnnnnnnnnnnnnnnnnnnnnnnnnnnnnnnnnnnnnnnnnnnnnnnnnnnnnnnnnnnnnnnnnnnnnnnnnnnnnnnnnnnnnnnnnnnnnnnnnnnnnnnnnnnnnnnnnnnnnnnnnnnnnnnnnnnnnnnnnnnnnnnnnnnnnnnnnnnnnnnnnnnnnnnnnnnnnnnnnnnnnnnnnnnnnnnnnnnnnnnnnnnnnnnnnnnnnnnnnnnnnnnnnnnnnnnnnnnnnnnnnnnnnnnnnnnnnnnnnnnnnnnnnnnnnnnnnnnnnnnnnnnnnnnnnnnnnnnnnnnnnnnnnnnnnnnnnnnnnnnnnnnnnnnnnnnnnnnnnnnnnnnnnnnnnnnnnnnnnnnnnnnnnnnnnnnnnnnnnnnnnnnnnnnnnnnnnnnnnnnnnnnnnnnnnnnnnnnnnnnnnnnnnnnnnnnnnnnnnnnnnnnnnnnnnnnnnnnnnnnnnnnnnnnnnnnnnnnnnnnnnnnnnnnnnnnnnnnnnnnnnnnnnnnnnnnnnnnnnnnnnnnnnnnnnnnnnnnnnnnnnnnnnnnnnnnnnnnnnnnnnnnnnnnnnnnnnnnnnnnnnnnnnnnnnnnnnnnnnnnnnnnnnnnnnnnnnnnnnnnnnnnnnnnnnnnnnnnnnnnnnnnnnnnnnnnnnnnnnnnnnnnnnnnnnnnnnnnnnnnnnnnnnnnnnnnnnnnnnnnnnnnnnnnnnnnnnnnnnnnnnnnnnnnnnnnnnnnnnnnnnnnnnnnnnnnnnnnnnnnnnnnnnnnnnnnnnnnnnnnnnnnnnnnnnnnnnnnnnnnnnnnnnnnnnnnnnnnnnnnnnnnnnnnnnnnnnnnnnnnnnnnnnnnnnnnnnnnnnnnnnnnnnnnnnnnnnnnnnnnnnnnnnnnnnnnnnnnnnnnnnnnnnnnnnnnnnnnnnnnnnnnnnnnnnnnnnnnnnnnnnnnnnnnnnnnnnnnnnnnnnnnnnnnnnnnnnnnnnnnnnnnnnnnnnnnnnnnnnnnnnnnnnnnnnnnnnnnnnnnnnnnnnnnnnnnnnnnnnnnnnnnnnnnnnnnnnnnnnnnnnnnnnnnnnnnnnnnnnnnnnnnnnnnnnnnnnnnnnnnnnnnnnnnnnnnnnnnnnnnnnnnnnnnnnnnnnnnnnnnnnnnnnnnnnnnnnnnnnnnnnnnnnnnnnnnnnnnnnnnnnnnnnnnnnnnnnnnnnnnnnnnnnnnnnnnnnnnnnnnnnnnnnnnnnnnnnnnnnnnnnnnnnnnnnnnnnnnnnnnnnnnnnnnnnnnnnnnnnnnnnnnnnnnnnnnnnnnnnnnnnnnnnnnnnnnnnnnnnnnnnnnnnnnnnnnnnnnnnnnnnnnnnnnnnnnnnnnnnnnnnnnnnnnnnnnnnnnnnnnnnnnnnnnnnnnnnnnnnnnnnnnnnnnnnnnnnnnnnnnnnnnnnnnnnnnnnnnnnnnnnnnnnnnnnnnnnnnnnnnnnnnnnnnnnnnnnnnnnnnnnnnnnnnnnnnnnnnnnnnnnnnnnnnnnnnnnnnnnnnnnnnnnnnnnnnnnnnnnnnnnnnnnnnnnnnnnnnnnnnnnnnnnnnnnnnnnnnnnnnnnnnnnnnnnnnnnnnnnnnnnnnnnnnnnnnnnnnnnnnnnnnnnnnnnnnnnnnnnnnnnnnnnnnnnnnnnnnnnnnnnnnnnnnnnnnnnnnnnnnnnnnnnnnnnnnnnnnnnnnnnnnnnnnnnnnnnnnnnnnnnnnnnnnnnnnnnnnnnnnnnnnnnnnnnnnnnnnnnnnnnnnnnnnnnnnnnnnnnnnnnnnnnnnnnnnnnnnnnnnnnnnnnnnnnnnnnnnnnnnnnnnnnnnnnnnnnnnnnnnnnnnnnnnnnnnnnnnnnnnnnnnnnnnnnnnnnnnnnnnnnnnnnnnnnnnnnnnnnnnnnnnnnnnnnnnnnnnnnnnnnnnnnnnnnnnnnnnnnnnnnnnnnnnnnnnnnnnnnnnnnnnnnnnnnnnnnnnnnnnnnnnnnnnnnnnnnnnnnnnnnnnnnnnnnnnnnnnnnnnnnnnnnnnnnnnnnnnnnnnnnnnnnnnnnnnnnnnnnnnnnnnnnnnnnnnnnnnnnnnnnnnnnnnnnnnnnnnnnnnnnnnnnnnnnnnnnnnnnnnnnnnnnnnnnnnnnnnnnnnnnnnnnnnnnnnnnnnnnnnnnnnnnnnnnnnnnnnnnnnnnnnnnnnnnnnnnnnnnnnnnnnnnnnnnnnnnnnnnnnnnnnnnnnnnnnnnnnnnnnnnnnnnnnnnnnnnnnnnnnnnnnnnnnnnnnnnnnnnnnnnnnnnnnnnnnnnnnnnnnnnnnnnnnnnnnnnnnnnnnnnnnnnnnnnnnnnnnnnnnnnnnnnnnnnnnnnnnnnnnnnnnnnnnnnnnnnnnnnnnnnnnnnnnnnnnnnnnnnnnnnnnnnnnnnnnnnnnnnnnnnnnnnnnnnnnnnnnnnnnnnnnnnnnnnnnnnnnnnnnnnnnnnnnnnnnnnnnnnnnnnnnnnnnnnnnnnnnnnnnnnnnnnnnnnnnnnnnnnnnnnnnnnnnnnnnnnnnnnnnnnnnnnnnnnnnnnnnnnnnnnnnnnnnnnnnnnnnnnnnnnnnnnnnnnnnnnnnnnnnnnnnnnnnnnnnnnnnnnnnnnnnnnnnnnnnnnnnnnnnnnnnnnnnnnnnnnnnnnnnnnnnnnnnnnnnnnnnnnnnnnnnnnnnnnnnnnnnnnnnnnnnnnnnnnnnnnnnnnnnnnnnnnnnnnnnnnnnnnnnnnnnnnnnnnnnnnnnnnnnnnnnnnnnnnnnnnnnnnnnnnnnnnnnnnnnnnnnnnnnnnnnnnnnnnnnnnnnnnnnnnnnnnnnnnnnnnnnnnnnnnnnnnnnnnnnnnnnnnnnnnnnnnnnnnnnnnnnnnnnnnnnnnnnnnnnnnnnnnnnnnnnnnnnnnnnnnnnnnnnnnnnnnnnnnnnnnnnnnnnnnnnnnnnnnnnnnnnnnnnnnnnnnnnnnnnnnnnnnnnnnnnnnnnnnnnnnnnnnnnnnnnnnnnnnnnnnnnnnnnnnnnnnnnnnnnnnnnnnnnnnnnnnnnnnnnnnnnnnnnnnnnnnnnnnnnnnnnnnnnnnnnnnnnnnnnnnnnnnnnnnnnnnnnnnnnnnnnnnnnnnnnnnnnnnnnnnnnnnnnnnnnnnnnnnnnnnnnnnnnnnnnnnnnnnnnnnnnnnnnnnnnnnnnnnnnnnnnnnnnnnnnnnnnnnnnnnnnnnnnnnnnnnnnnnnnnnnnnnnnnnnnnnnnnnnnnnnnnnnnnnnnnnnnnnnnnnnnnnnnnnnnnnnnnnnnnnnnnnnnnnnnnnnnnnnnnnnnnnnnnnnnnnnnnnnnnnnnnnnnnnnnnnnnnnnnnnnnnnnnnnnnnnnnnnnnnnnnnnnnnnnnnnnnnnnnnnnnnnnnnnnnnnnnnnnnnnnnnnnnnnnnnnnnnnnnnnnnnnnnnnnnnnnnnnnnnnnnnnnnnnnnnnnnnnnnnnnnnnnnnnnnnnnnnnnnnnnnnnnnnnnnnnnnnnnnnnnnnnnnnnnnnnnnnnnnnnnnnnnnnnnnnnnnnnnnnnnnnnnnnnnnnnnnnnnnnnnnnnnnnnnnnnnnnnnnnnnnnnnnnnnnnnnnnnnnnnnnnnnnnnnnnnnnnnnnnnnnnnnnnnnnnnnnnnnnnnnnnnnnnnnnnnnnnnnnnnnnnnnnnnnnnnnnnnnnnnnnnnnnnnnnnnnnnnnnnnnnnnnnnnnnnnnnnnnnnnnnnnnnnnnnnnnnnnnnnnnnnnnnnnnnnnnnnnnnnnnnnnnnnnnnnnnnnnnnnnnnnnnnnnnnnnnnnnnnnnnnnnnnnnnnnnnnnnnnnnnnnnnnnnnnnnnnnnnnnnnnnnnnnnnnnnnnnnnnnnnnnnnnnnnnnnnnnnnnnnnnnnnnnnnnnnnnnnnnnnnnnnnnnnnnnnnnnnnnnnnnnnnnnnnnnnnnnnnnnnnnnnnnnnnnnnnnnnnnnnnnnnnnnnnnnnnnnnnnnnnnnnnnnnnnnnnnnnnnnnnnnnnnnnnnnnnnnnnnnnnnnnnnnnnnnnnnnnnnnnnnnnnnnnnnnnnnnnnnnnnnnnnnnnnnnnnnnnnnnnnnnnnnnnnnnnnnnnnnnnnnnnnnnnnnnnnnnnnnnnnnnnnnnnnnnnnnnnnnnnnnnnnnnnnnnnnnnnnnnnnnnnnnnnnnnnnnnnnnnnnnnnnnnnnnnnnnnnnnnnnnnnnnnnnnnnnnnnnnnnnnnnnnnnnnnnnnnnnnnnnnnnnnnnnnnnnnnnnnnnnnnnnnnnnnnnnnnnnnnnnnnnnnnnnnnnnnnnnnnnnnnnnnnnnnnnnnnnnnnnnnnnnnnnnnnnnnnnnnnnnnnnnnnnnnnnnnnnnnnnnnnnnnnnnnnnnnnnnnnnnnnnnnnnnnnnnnnnnnnnnnnnnnnnnnnnnnnnnnnnnnnnnnnnnnnnnnnnnnnnnnnnnnnnnnnnnnnnnnnnnnnnnnnnnnnnnnnnnnnnnnnnnnnnnnnnnnnnnnnnnnnnnnnnnnnnnnnnnnnnnnnnnnnnnnnnnnnnnnnnnnnnnnnnnnnnnnnnnnnnnnnnnnnnnnnnnnnnnnnnnnnnnnnnnnnnnnnnnnnnnnnnnnnnnnnnnnnnnnnnnnnnnnnnnnnnnnnnnnnnnnnnnnnnnnnnnnnnnnnnnnnnnnnnnnnnnnnnnnnnnnnnnnnnnnnnnnnnnnnnnnnnnnnnnnnnnnnnnnnnnnnnnnnnnnnnnnnnnnnnnnnnnnnnnnnnnnnnnnnnnnnnnnnnnnnnnnnnnnnnnnnnnnnnnnnnnnnnnnnnnnnnnnnnnnnnnnnnnnnnnnnnnnnnnnnnnnnnnnnnnnnnnnnnnnnnnnnnnnnnnnnnnnnnnnnnnnnnnnnnnnnnnnnnnnnnnnnnnnnnnnnnnnnnnnnnnnnnnnnnnnnnnnnnnnnnnnnnnnnnnnnnnnnnnnnnnnnnnnnnnnnnnnnnnnnnnnnnnnnnnnnnnnnnnnnnnnnnnnnnnnnnnnnnnnnnnnnnnnnnnnnnnnnnnnnnnnnnnnnnnnnnnnnnnnnnnnnnnnnnnnnnnnnnnnnnnnnnnnnnnnnnnnnnnnnnnnnnnnnnnnnnnnnnnnnnnnnnnnnnnnnnnnnnnnnnnnnnnnnnnnnnnnnnnnnnnnnnnnnnnnnnnnnnnnnnnnnnnnnnnnnnnnnnnnnnnnnnnnnnnnnnnnnnnnnnnnnnnnnnnnnnnnnnnnnnnnnnnnnnnnnnnnnnnnnnnnnnnnnnnnnnnnnnnnnnnnnnnnnnnnnnnnnnnnnnnnnnnnnnnnnnnnnnnnnnnnnnnnnnnnnnnnnnnnnnnnnnnnnnnnnnnnnnnnnnnnnnnnnnnnnnnnnnnnnnnnnnnnnnnnnnnnnnnnnnnnnnnnnnnnnnnnnnnnnnnnnnnnnnnnnnnnnnnnnnnnnnnnnnnnnnnnnnnnnnnnnnnnnnnnnnnnnnnnnnnnnnnnnnnnnnnnnnnnnnnnnnnnnnnnnnnnnnnnnnnnnnnnnnnnnnnnnnnnnnnnnnnnnnnnnnnnnnnnnnnnnnnnnnnnnnnnnnnnnnnnnnnnnnnnnnnnnnnnnnnnnnnnnnnnnnnnnnnnnnnnnnnnnnnnnnnnnnnnnnnnnnnnnnnnnnnnnnnnnnnnnnnnnnnnnnnnnnnnnnnnnnnnnnnnnnnnnnnnnnnnnnnnnnnnnnnnnnnnnnnnnnnnnnnnnnnnnnnnnnnnnnnnnnnnnnnnnnnnnnnnnnnnnnnnnnnnnnnnnnnnnnnnnnnnnnnnnnnnnnnnnnnnnnnnnnnnnnnnnnnnnnnnnnnnnnnnnnnnnnnnnnnnnnnnnnnnnnnnnnnnnnnnnnnnnnnnnnnnnnnnnnnnnnnnnnnnnnnnnnnnnnnnnnnnnnnnnnnnnnnnnnnnnnnnnnnnnnnnnnnnnnnnnnnnnnnnnnnnnnnnnnnnnnnnnnnnnnnnnnnnnnnnnnnnnnnnnnnnnnnnnnnnnnnnnnnnnnnnnnnnnnnnnnnnnnnnnnnnnnnnnnnnnnnnnnnnnnnnnnnnnnnnnnnnnnnnnnnnnnnnnnnnnnnnnnnnnnnnnnnnnnnnnnnnnnnnnnnnnnnnnnnnnnnnnnnnnnnnnnnnnnnnnnnnnnnnnnnnnnnnnnnnnnnnnnnnnnnnnnnnnnnnnnnnnnnnnnnnnnnnnnnnnnnnnnnnnnnnnnnnnnnnnnnnnnnnnnnnnnnnnnnnnnnnnnnnnnnnnnnnnnnnnnnnnnnnnnnnnnnnnnnnnnnnnnnnnnnnnnnnnnnnnnnnnnnnnnnnnnnnnnnnnnnnnnnnnnnnnnnnnnnnnnnnnnnnnnnnnnnnnnnnnnnnnnnnnnnnnnnnnnnnnnnnnnnnnnnnnnnnnnnnnnnnnnnnnnnnnnnnnnnnnnnnnnnnnnnnnnnnnnnnnnnnnnnnnnnnnnnnnnnnnnnnnnnnnnnnnnnnnnnnnnnnnnnnnnnnnnnnnnnnnnnnnnnnnnnnnnnnnnnnnnnnnnnnnnnnnnnnnnnnnnnnnnnnnnnnnnnnnnnnnnnnnnnnnnnnnnnnnnnnnnnnnnnnnnnnnnnnnnnnnnnnnnnnnnnnnnnnnnnnnnnnnnnnnnnnnnnnnnnnnnnnnnnnnnnnnnnnnnnnnnnnnnnnnnnnnnnnnnnnnnnnnnnnnnnnnnnnnnnnnnnnnnnnnnnnnnnnnnnnnnnnnnnnnnnnnnnnnnnnnnnnnnnnnnnnnnnnnnnnnnnnnnnnnnnnnnnnnnnnnnnnnnnnnnnnnnnnnnnnnnnnnnnnnnnnnnnnnnnnnnnnnnnnnnnnnnnnnnnnnnnnnnnnnnnnnnnnnnnnnnnnnnnnnnnnnnnnnnnnnnnnnnnnnnnnnnnnnnnnnnnnnnnnnnnnnnnnnnnnnnnnnnnnnnnnnnnnnnnnnnnnnnnnnnnnnnnnnnnnnnnnnnnnnnnnnnnnnnnnnnnnnnnnnnnnnnnnnnnnnnnnnnnnnnnnnnnnnnnnnnnnnnnnnnnnnnnnnnnnnnnnnnnnnnnnnnnnnnnnnnnnnnnnnnnnnnnnnnnnnnnnnnnnnnnnnnnnnnnnnnnnnnnnnnnnnnnnnnnnnnnnnnnnnnnnnnnnnnnnnnnnnnnnnnnnnnnnnnnnnnnnnnnnnnnnnnnnnnnnnnnnnnnnnnnnnnnnnnnnnnnnnnnnnnnnnnnnnnnnnnnnnnnnnnnnnnnnnnnnnnnnnnnnnnnnnnnnnnnnnnnnnnnnnnnnnnnnnnnnnnnnnnnnnnnnnnnnnnnnnnnnnnnnnnnnnnnnnnnnnnnnnnnnnnnnnnnnnnnnnnnnnnnnnnnnnnnnnnnnnnnnnnnnnnnnnnnnnnnnnnnnnnnnnnnnnnnnnnnnnnnnnnnnnnnnnnnnnnnnnnnnnnnnnnnnnnnnnnnnnnnnnnnnnnnnnnnnnnnnnnnnnnnnnnnnnnnnnnnnnnnnnnnnnnnnnnnnnnnnnnnnnnnnnnnnnnnnnnnnnnnnnnnnnnnnnnnnnnnnnnnnnnnnnnnnnnnnnnnnnnnnnnnnnnnnnnnnnnnnnnnnnnnnnnnnnnnnnnnnnnnnnnnnnnnnnnnnnnnnnnnnnnnnnnnnnnnnnnnnnnnnnnnnnnnnnnnnnnnnnnnnnnnnnnnnnnnnnnnnnnnnnnnnnnnnnnnnnnnnnnnnnnnnnnnnnnnnnnnnnnnnnnnnnnnnnnnnnnnnnnnnnnnnnnnnnnnnnnnnnnnnnnnnnnnnnnnnnnnnnnnnnnnnnnnnnnnnnnnnnnnnnnnnnnnnnnnnnnnnnnnnnnnnnnnnnnnnnnnnnnnnnnnnnnnnnnnnnnnnnnnnnnnnnnnnnnnnnnnnnnnnnnnnnnnnnnnnnnnnnnnnnnnnnnnnnnnnnnnnnnnnnnnnnnnnnnnnnnnnnnnnnnnnnnnnnnnnnnnnnnnnnnnnnnnnnnnnnnnnnnnnnnnnnnnnnnnnnnnnnnnnnnnnnnnnnnnnnnnnnnnnnnnnnnnnnnnnnnnnnnnnnnnnnnnnnnnnnnnnnnnnnnnnnnnnnnnnnnnnnnnnnnnnnnnnnnnnnnnnnnnnnnnnnnnnnnnnnnnnnnnnnnnnnnnnnnnnnnnnnnnnnnnnnnnnnnnnnnnnnnnnnnnnnnnnnnnnnnnnnnnnnnnnnnnnnnnnnnnnnnnnnnnnnnnnnnnnnnnnnnnnnnnnnnnnnnnnnnnnnnnnnnnnnnnnnnnnnnnnnnnnnnnnnnnnnnnnnnnnnnnnnnnnnnnnnnnnnnnnnnnnnnnnnnnnnnnnnnnnnnnnnnnnnnnnnnnnnnnnnnnnnnnnnnnnnnnnnnnnnnnnnnnnnnnnnnnnnnnnnnnnnnnnnnnnnnnnnnnnnnnnnnnnnnnnnnnnnnnnnnnnnnnnnnnnnnnnnnnnnnnnnnnnnnnnnnnnnnnnnnnnnnnnnnnnnnnnnnnnnnnnnnnnnnnnnnnnnnnnnnnnnnnnnnnnnnnnnnnnnnnnnnnnnnnnnnnnnnnnnnnnnnnnnnnnnnnnnnnnnnnnnnnnnnnnnnnnnnnnnnnnnnnnnnnnnnnnnnnnnnnnnnnnnnnnnnnnnnnnnnnnnnnnnnnnnnnnnnnnnnnnnnnnnnnnnnnnnnnnnnnnnnnnnnnnnnnnnnnnnnnnnnnnnnnnnnnnnnnnnnnnnnnnnnnnnnnnnnnnnnnnnnnnnnnnnnnnnnnnnnnnnnnnnnnnnnnnnnnnnnnnnnnnnnnnnnnnnnnnnnnnnnnnnnnnnnnnnnnnnnnnnnnnnnnnnnnnnnnnnnnnnnnnnnnnnnnnnnnnnnnnnnnnnnnnnnnnnnnnnnnnnnnnnnnnnnnnnnnnnnnnnnnnnnnnnnnnnnnnnnnnnnnnnnnnnnnnnnnnnnnnnnnnnnnnnnnnnnnnnnnnnnnnnnnnnnnnnnnnnnnnnnnnnnnnnnnnnnnnnnnnnnnnnnnnnnnnnnnnnnnnnnnnnnnnnnnnnnnnnnnnnnnnnnnnnnnnnnnnnnnnnnnnnnnnnnnnnnnnnnnnnnnnnnnnnnnnnnnnnnnnnnnnnnnnnnnnnnnnnnnnnnnnnnnnnnnnnnnnnnnnnnnnnnnnnnnnnnnnnnnnnnnnnnnnnnnnnnnnnnnnnnnnnnnnnnnnnnnnnnnnnnnnnnnnnnnnnnnnnnnnnnnnnnnnnnnnnnnnnnnnnnnnnnnnnnnnnnnnnnnnnnnnnnnnnnnnnnnnnnnnnnnnnnnnnnnnnnnnnnnnnnnnnnnnnnnnnnnnnnnnnnnnnnnnnnnnnnnnnnnnnnnnnnnnnnnnnnnnnnnnnnnnnnnnnnnnnnnnnnnnnnnnnnnnnnnnnnnnnnnnnnnnnnnnnnnnnnnnnnnnnnnnnnnnnnnnnnnnnnnnnnnnnnnnnnnnnnnnnnnnnnnnnnnnnnnnnnnnnnnnnnnnnnnnnnnnnnnnnnnnnnnnnnnnnnnnnnnnnnnnnnnnnnnnnnnnnnnnnnnnnnnnnnnnnnnnnnnnnnnnnnnnnnnnnnnnnnnnnnnnnnnnnnnnnnnnnnnnnnnnnnnnnnnnnnnnnnnnnnnnnnnnnnnnnnnnnnnnnnnnnnnnnnnnnnnnnnnnnnnnnnnnnnnnnnnnnnnnnnnnnnnnnnnnnnnnnnnnnnnnnnnnnnnnnnnnnnnnnnnnnnnnnnnnnnnnnnnnnnnnnnnnnnnnnnnnnnnnnnnnnnnnnnnnnnnnnnnnnnnnnnnnnnnnnnnnnnnnnnnnnnnnnnnnnnnnnnnnnnnnnnnnnnnnnnnnnnnnnnnnnnnnnnnnnnnnnnnnnnnnnnnnnnnnnnnnnnnnnnnnnnnnnnnnnnnnnnnnnnnnnnnnnnnnnnnnnnnnnnnnnnnnnnnnnnnnnnnnnnnnnnnnnnnnnnnnnnnnnnnnnnnnnnnnnnnnnnnnnnnnnnnnnnnnnnnnnnnnnnnnnnnnnnnnnnnnnnnnnnnnnnnnnnnnnnnnnnnnnnnnnnnnnnnnnnnnnnnnnnnnnnnnnnnnnnnnnnnnnnnnnnnnnnnnnnnnnnnnnnnnnnnnnnnnnnnnnnnnnnnnnnnnnnnnnnnnnnnnnnnnnnnnnnnnnnnnnnnnnnnnnnnnnnnnnnnnnnnnnnnnnnnnnnnnnnnnnnnnnnnnnnnnnnnnnnnnnnnnnnnnnnnnnnnnnnnnnnnnnnnnnnnnnnnnnnnnnnnnnnnnnnnnnnnnnnnnnnnnnnnnnnnnnnnnnnnnnnnnnnnnnnnnnnnnnnnnnnnnnnnnnnnnnnnnnnnnnnnnnnnnnnnnnnnnnnnnnnnaagctttgattgggccgttactgtcttttgacctttcttgtttgcttgcccttttgtttctttcctcctttttccttccttcctgtctttcttcttccttccttcctttcttcctttttctttttaattttcctcctttctctttctcctttctttccttccttctttcctctttttttctttcctccctccctccctttctttcttccttcctttctttcttccctccttccctccccaccctccctcccttcccctcgtctcccttcccctcgtctcccttcccctcccctccctccctcccttcctcctttttctttccctttcctccttccttccttcctctcttcttttctccatccctttcttccttttaacatttgatcatgggtaccatttcatcaagattctgttacttaggtccaaggactagtgaccaaattgtttttcccaggagtaaacttttctacaagacatagagaaatgactgccagtgccatcaggcacaccatcctgtgtgataggtaacctaaaataatggtacagcggggagtaactggaagagtcacaactacacaaatctcttgcattttcctgatcattaaatgaattagggatttcctggtttgagatttgtggacaaggagaactacttctttgtacaagaggcttgtgccaggagaagacacgctgtggttacaatgttactgtctctagctatggtcatttcatgtctttaactgagtgtacctagagtgtaatacagtgcagcagtgatgggctgaaggcctaatgcaccagcacacatgcctggaagacctaacgttgagaatccgcatttttttcatcactcacatttattttgcatctccctgttttgattaccttcagagacccaagcacttgcttttgtatatttgagtctgggttttattttccttttagaaatagtccaaaatccttttagagcctagacctttgaataaagtgctaacttaacctgaggaatgctgtttttttgttcacaaataaggcttaattgtgaagtcgtgagaattgctttctgagctgacttataaatttacccacctctttttccccaaacccccaaaaaatcctccagaaggtgagcccagcttgttgtaaaagattttgaagcagaagtcctgggtttaagcttcagttctctgccttaccagaatcgggatgtgtggggcaggcctacctcctctttcttcatctgcaaaatacattgaatgaaatcatattttttcctaagtatatgacatgtaaagtggtatttcaaaaactcattaatctgcatgaccaggtcagaaaagacacaccttttgccttgtgtctagtgtgtgactgtcctcacatgtagatgacccaggccacatccgctgatgttgtcttcctttacttctttgtcccttccaatgactcctttatgaagtcaatcagcagtgtttctaagccaggttccttctcttcacacatccccaacccacagggcaagtcatccacattttgcctctctattttttgtgctttgggaaacacattttacaacttccaaactatttgcctaagttcatctgagcacatctagaattattccactcctctgcatcagtgctaaaagtacaatcatgtataagctgttatactcccgttattttgtacctcatgtgcaggtagattgcaagttccttgcaggcaggtactacatctacttgaattgcttcacgatcacataacacaatgcagtgttaaaagtagaaaagtaattgacatcttgactaacagaaacactaaattcagtgtattgtgatgatacctttttaagagataggctatagaaatagaaaatcatcttagttggaattgaaagtcaagaagcaacattttaagtaagagatgaaaatacttaaaagggaaaggagcagtgcttacacagatgaggggaaaaaataaaatgtatcatctaaaaatttaaatcaaatatattaggttggtgcaaaagtaactgcgatttttgccattaaaagtaatagcaaaaaccacggttacttttgcaccaacctaatagatgggaaaaataagaggaatgaatattttaagctttgctatataattaaaatattcttagaagtctggagtctgtgaaggtcacaccctctggtcttctcccagcccatagggtataaataatctgaattgacggcatccagggatctcagaaattattagtacatcccacagtgaattaccaccttactaaaatattcatgggtatatactatggatttgttttatcctatttagtcttaaaaactataaagaaatctgcaggcttattaacatattactcagaatcatattgtctccaaagcacaaactgaatcagttacaagatattggactagagatcatggcaaatcagaggtacataagacctagttccgttgtggagctaaacaaactgcagagacctaaagggaagccttgcaccacactctaggtttggagctcaggttttgagtggtgtcagcactccagaacacatgggatccccgggaggtggaaattgagccgtctttggagaatcagctaatgagacagatgcatgttaaatgtctgttgtggcccaggcactctgctaggcagaggggtgaaccagaagaatgagattcatggggccaaagaatttgccttctggtgtaagaaaagatggaggcagcttggcagaaagaaaaaaaaggtaaaagatagaaatgaaatacagaataatctatctcctcatcccacaagcaattctgcctggtttgtggctcacgcctgtaatcccagcactttgggaggccgaggcaggaggatcacttgaggtcaggagttcgagactagcctggaccacaaggtgaaacctcatctctactaaaaatgcaaaaaaatttagggccgggtgcagtggcagttctgcctggtttgaacatctggttcagttaaaatacttcatgaaaatatttagcttgatgcactgaaatccatcactgcttttgtgggatgcactgactgcagtctgactgttctcctagtggaaaggggagcaatagcttctgtctgcatgtgcatgaaacagatggaaatttagaagagattctagtgcagacaacttcatcccacccccgctgcccacagagctagccatgtgcacggtgtgtttgaacaatgttatgttgctgctgtgcacagagatccccagtctcataaaacatactggatggaaggctgtcgagagatcatcaggccccagtgcataagttcttcctaagcatccttaacaggtgatcacctcgcctattgagaaccctcaggaggcagcccacttacggaagcactgattgttacaaaagccctgaactaaatctgcttgtctctaaagccagccctgcagatgtctgcagtgtaactactttctcttctctcaagcagttcagcccttcaaatcattgacaacagctctacaaagccctctaaatagcccgttctcctggctaaagtgtgttggtttcctcagcatatgatgaaataaacaccatgatgcctttgccttgctttttcttgctggtctcactcttccctggcattcttcaatgtgcccaagtccttcctagaacattgcacccaaagggccttcctggtctttccagggaatgcagaatgaaaaagaaatcccatcccctgcctcgaaaggagctcttctgtgtgtaagtgtaccttccccctcagggcataatgggaaacagtttgccaaagctaactgtgtaatttcacatgactcactgccgttagtctgagaaagcatggcatattaaactcattttccatgcttcccaactttatttactattccatttctgaggggcagagagctgagcaggaataacaccttccttgctcctcctaatggggcacatgtgcacatataaaattgtgttcgatctttgcagccacgacccatgttaactgtcaactgagaactcatgagtcagtttctcaggaacagccctgaagacattatctcctgcatcttgtatttgtgcctttgatatttggagggaagggtaggatctggcaattatcgttatctcatttggttcagtgtatttcatttcagcctgttaagatcttttggaaatactgtatgtgctagttacagggacagtgataaataagacagcattcctgtccttgagatgctatttccacagctccatgagatgcctagttaaaaacagagccttttttggaaacagcctactaatctgttaaaataataatggaaaaagataaagttagcatacctgagctgcaagggctgcctcctggtctgatctctgataaggatcagatcctagagcctctgagatccctgtcctccctgtctgcacaagcactcgcagaaggagaaacagtttacggtggttcatcatgactttgaaccaagcttaaagtcaaagtcatactctttaaaccattggaaaccaagtttttgcgagttgcctaaagtgggcaaaaatcccacaatgcacctgagcacaagcaggaaaacatgccattgtctccccaggagccctccttgacttctactttactttatccattgacactagtcttataagtagctttgtctgtccaatttttaattgaatttcgtttttattttcgtgagtggaaatatcactttgaaagaaatcagtcctctcctgaaatccagaattcctggagctcagtttacatgtttgacgcgtgtcacatgattccacaagtcactcaagggcaggaggattaccatcgatacggaaagatttcttagaaagcttaagtgaaagggaaaccagggagaaagtgtgcttcgtgagaataggtatgcggacggctctttgtgacgctctgtgcaaccctcgtgtttgcattgaaccaagctgtgctgcagatggacacccatcccatttccccgactcataccagggaggcccactttgcaaggtacacagaggggaccacagagcagggggccatgcaggggaccaagggacattttagtgtaaccaaagtgtgaagtatgccctttatttcaaaagaataaagaaaatcacaggttttcccgctgatatgccagggacatttccaagagaattccttttttgagagaaatctcctttgatatcccatcagtcagccatactgcataattgttagatagtgaaagaaattcattttttaagtttgtcagaaaaataaattctttgaagtcttaaattgttgcctccggacatgacatatctggctcttccagaatccatgttagtcctagctgaggaagaaggagaaggagaggggcgtttgttgattattgattttgtaagatgccccacacgttggctattagcagaattctcacttctaaaaggaaaatgagtgtgagctatgttcaatgagaaacagttatttttgggacattctttgaggtaaaacacctccttaagatgctgcttccttattgctatgggaccaagattagagcaagaacatagtggttttcagaccctggacatcatccacagccgcagcagaggccctgcccacttgaacaatgagacaggccaccattttgtttcgagaatgagcaaagtgaaccaccatgccagatattgttaagtcagcaactcttctgaagatggacatagtaaaaaataaacaaacaaggcagcacttgagatggtcatggcagagcaatctcaacaagcgatttgttattttgcacagtgatgtacccactcattgaataaaatgcaccagaaccatgcactacagatgctaaggagagttgtccttcaacaaaggagataggccccactggccgtggggcagtttatgttatttggtccttgtcatgggcaggcatggccctttctatgcttcacagatgaggaaggtccctggcacaggtccagtctccagcatggcctagaggtggcaggtgctacttagcatcgccagcctcctgcttggtcatggggtcagccagtttataacacgaacggaggttaatgaactgatcttcccatcgcacaactggtatgaacccacatcttctgattataaatcttttgctctttaactcttagtcattaccactgtctagtgtaggcctgtgtgttcatggcctttgttgccaccaaaagatcaactattagctgaataacatactgagacatgttggtgttgtgttctaaatagcactagtaaactgttagggaaatctgactatatagctactatccagtctagtttttcttgcgaagtgtttgttgagtgtgtaatgaggagtaaggaaggtgaataagaaatggcctgagtctttataaaataagcaaggagagaaaacagttttgatgagaagcgcatggaatttttagaagataggacgtgtattatgtacctataagaatgggtaggattttagaagagatggatggggaaaaggaacagggagtgggaacaaaacgtggaccaaggaagagcaggtttagccatggaagcctcaccgccggctttggtttatcgtgggccaaggggacagaccctgtggggagggctggcagcagggaggtcttccagaagtctatcctgcaggcagtaacagccacccagtctataagctgagtgggcatgggggtgatggggaatgggtggggagttattggggtaacttaccccaaaatgatagctagctggaaccatttattctattgcattttatcaataaatcttataggaagtaccatcctagtgaaaaccctgtcacattgagggcattcatgcttatgttttaaaacatgttattgggtctatgaaaaataaggctgaaacctatgagcaccctccatgcaaagtttcagtcaagactttggaaacaagacagtgtcttactcactttataaattcattcagaaagccgtaggtttgaaaattccaaacttagatgtaagaagctctgagaaacacatgaaatcacccccacatcagtagagatgtctcagcagacatgggaagaggggcagcagggtgtagggaggtggggcagccccggggtgggccttgcaggctgggcttgaatcccatggccaccaccgtccgctgggaggcctggagccggctgcccactctctgaccagcacatgttgatgctgtatccttgaagggaccgtggtctgacatcctgtgatgcagacctgaatccagcacccacagggtctgcacattccctctttgaggtggagcccagctccagaggctggtccctgactctgtttctcaagaagcctgtacagatgttcccctcaccactgtttccagtcacctttggctttcacggtgcagatgctaagtttgattttcagagcccatctgggaatttagtgaactgaacaggtagcatttctgaacccacccataacccatgccctccccactgattttgaaagagagtttgctgcaggtgactttgcagctgggtagagaatcttggggcaggattccgaggcaggcagatgagtgaggataaattgggttctgacggcacgttacaccagtggactctaacgacgacctcacctcgtgcacagataattctgccttgtgcttaaccgttagaaatgtgtcactgaagtgtgaacatattatgctgttagatttcccatcatttctgttctttcattccctctcatttgcattggttactcataaatgtagatctttggtatgatttgtacaactgccgggtgtcaatctgtgaaagaaatagcagagcaagctgggctctggtagcgctttatccctgcgtgctggcttgcccgggttgactcagaggcagtctcacattcagctgcgctggggccaaggacccagggagccaagtgtgtttctgttttctgtatttagcaatttaagacctgcgtttaaatactagctatgcattctagcaaaagaggtttatattttaacacagtaactcttaattgtttaattcagttcgtgtgttacctctcggaataaaatagtggaagccaattaactatagacttcattagtttggatttaagatcaccaaaacatttaccacatctcaattgttcattacatgctctctcttttttaatgcagtttttataatatggggagtgggggtgtggatttaaccattatatttttatgatattgggagtagatttaaccattatgtaaattggattttttaattttaaaaagtcacttatcttgatgtaaaatcatgtcttagtaaccttgataaactaagttttgcatgattacaccttaaggttaaaacatatttcatttcatcatttcccagaaggggcactgaattcacccatttcctgtttttcatctcagaatgttctgtgtttcctccatatctactttcccggcagcaggaccctggaagcagtcacaccaacctcatttaccccacctgagatttgtgcgctttgaacatagttgcaatcaaatcaacaatatctttgctcagaaatggatatgtgaagtaaaatgtgctgccctgttcatgtatgaaatcattcagctagctggccagtgagcccttcattgcaacaaagatttttctagagcccctgcactatctggggctatgtcaggcctcacactcctgctcacacgtttggaggctaccttggccagtattaccttaatccagcatttaggggaaggagcatttcaagactaaattttctaaactgctcaagcctacctcattttatttcttgtgtattttaacacttttggatgaggactcttcctagaacctactaacaattcccccccgcccccatgccaagattctttaaagactttcttgaaaacgcttcagtcttttcttcttagctcaaaagtactatcctaaatactagctctggcattacagggagttaatttgtgggcacacacagtaaattataaaccccttaagcagagaagattgtattatcagtttattagttttcttattcattccttcagcacacatttctgttgcctccaatgcagcagagaaattgacttctacagtttccacaacagtccagatttcaactgtgtagtgctctttcagccagaaagtacacttgtgtttccctggccataggtcctgaacctcacttctgaaaagtcattgtgcatagagagctaatagctgtaccctaaatgatcctggctttgaattctcttatctgcttggatagtattatctgtctcttcctctgcattctaatttgctacttctaatctgctgggaattacaataagaaagaaccatttaatcatttttacaactgtgcctaaagagagtgtgtgtaagtgccgagagagtgtatgagggacttgcccatgagtaaatgcatgaattttaggtcaagggttttttgcttctcttttggttgattacctcagagatcagttttactttctttctcattcttgacctatcatcactagctgatatggatgatgtgtacaacttctgagtaagaataatgtcaatgggacgggatgggattggctggtgattctgttgatcttaaagtttatatattttaagtttagtgtttcagaatgagaccaaagcggtgacattttcaacctcttcggtctctcttcagttttttcattttaagtttttgttgtgcttctatcacttaaaggaagcctccaagttgaaatcaaatactaatgacatttttatctaatgtataaatgtgtttttattatttattaggaaatttattttacttggccctcagccatgacatatcatggcataatcactatcctaaatttgtatatcttatccttgcataaggtaagactttctatgaattacacatatttgtattttcctctcttacatattttaagaatttttttatactttgttttctgcaaatgaaatattgctcataagccaggtgatggctgtccacgcctcttttcccctgcttacccttgcttagatcttatggtagaatcttttcatagaagacacagaaagacatgaaagaaagagctggagaagcctgaggggctgcccagtgagtggtctgctaggatgctgtgccacagcccaggcacaggaggcagggagagcaatggggcccttcccttccaccaacattcagcagaatttgcagctccatgtttccaaagcttccagggcacttgcatttagagagagagagcaagcaagctgcctttcctcttcctcagttctgccagccacactcttgccatgatgagcagtttcagccaaaagctccttcccctgccctaacacctcctgcaaggcctgaggtctggaagccacctgcgcctgctggcccctcctttcttgtttctgcaatggatgttgtggccctgtgagggagaagagaaaaagaagttgccctcctccctctatcctcacctcctgccatgctgtcacccttataagagagaagggctaaccatccaggctaatcctccagtgatgcaggagaggacatcctggccggaagagtcagagcttccaggtgagctcaggtgggtcagcccccgaggctgtgaagagcccaggggccagtagatgccacttttgctccaggaagaatcttcaactgtgtcctttttattcaaggggctctcttttcagcgaatctctagatgtactagtcacaaacactcgcatttattaaaatgtatccatgatcccacaatccttttacatatttctctccaggagtatcacatttctgagggccctgtgcctgttttctgcaggaagttgctgttgtcccgggtccccctgcccccagcacctctgttacaagaagcagacccttcatgccacactgggacccagggaggccccaagccaggatgctgggatcttagtaaaggttggaatgatgtcagaacatagaggaggcagaattccccccatagcatcatcctggagggcgctgatttgtgtgctctgccaggttcatctgtgactcaggatttaaaagccccaggtgtggtgtcccttctgtgcctgcaaggtgcgtctttagcagttctccctggtgtggaaggatcagtggttcttgcagcctaggcaccctccacagcaagcccaacacaggtgctgtgagcagctggttcatgaacggtgatcctggggagaagaggaggatgaaaatggaaaaccagtgcaaaggtgtgtcatccagttggttactgctgtgggtgcccgggcttccatcccaccagagcccccactagccagggcagcctggcggaggtgagcatcattctgctttctggctgcacctgtgtggacagagcccgttccaaagcctcccaggcacagggcagacatcaagcaaggggcagagctggggcgagggctctgggtgcccccgttattgaacacaggcctgaagggagcctaagaggtggctggcaggagatactacaaggcagaaagacagggcagcagtctttgtactgtacgtttttgttttttaagagagaacaaaaagtcaaggttgagagatgagaaatactcttgccaaaaagagaacaccaaaatcctggagtcacgggtcttccattaccctctctagcatttctgcttgtcttttccctagtattggtgaagaatttttaaagtaaccaacccataccgttggttacaggccctgtggtcaccaggctgtctccccatgatggggatggagagtggttagtgcagaaacttagacctcccctccagcttgttgaatgccctgaagtttatctagaagggaagatactcaagcgtaggatttcagtgatgcatttggacagcatcagtactatgcttcagcgtcaaaaacgtcactttgggtaggaacaatacataatgcgtggcaatgccttttgtgacacctgttcaggagattcccataggaagcttctgaggcagagtcctcaggtgaggagggggacaggcctgggtcttgggggaaggtggagatgaccagcctcatgcctctctccccagtggcctcagtctccatcaggcaaatcttgagaagcctcctccattctgcaggcaaatgactgagatgtgtgagctctgcttcccaacaggcggaaattcacatggggaagggcacctgtgaatggccttctagaactatcaggaagttctggatttagtaccctgtgagagcagatggtcctgggtgcactcggatgatcctgcctagccagctggattgcagagtggtcatcattatcagtgagctattgaggggttgagagcagtcagtgtcatgtataaggatgggttggggtaccggccaacgcccgccttgaggcctggccgccggatgggaggcgagagcacaagagagtcctggctaggtgtgccccgctctgcagggccacaccatccactggaaaccctgtgcccactgggctgcgtgctaagaggctgtggccaatgctcttgtccaaattttactgaatctgcagtctctcttaattcactccaaagtttaatgtgttagcttgcgaataaataaataaataaataaataaataaataaatggaaagaaacagtcctcagaaagtcccagtcaaattttaattccaacagatattcagcagtttcctctaagaacaatgagagttctggggctagccagtgtttctcttggaaaataaggaagagggaaagcggtgcattcatttaaaaacctgccctagggaggcagcgttccctgtgaactccgaggccacagtgagcagagcaggctggaggcctcccggctgtcctgcccctcctgccacatgcctgtgaaaatgctagataaggactttttctcagcaacttccacgctccttcagtggggatgtctttgactcagagctctgccactggttatctccacgaacagaaaatgccacagatgggttaattcactgtgttgttctcattttccctcagtttcaggcttttctctccttgcctgttttcctcgcttaaaaaatgatgtgggggtccctaaacgcatctaccccgatagatttatgttttcttttccattagtccactttgcgtctcagccctaaaattaagtttttgattataatgtaaggaagttttaccatattttaactctggctttttaaatacaaaagaaaaataacagaatggccttctagaactatcaggaacttctggatctagtaccctgtggggacagatggtctggagccagcgcacttggatgatctctctcagccatctggaccatagagtgaacttgttactgtccctccaaggctgacaactatgagctcatactcttctagcagtttaatttagacccaagaaaggctgtgtgtgtgtgaatttgtgagagtgtgtgagtgtgtctttgtgcctgtgtttctgtgtgtgtctgtgtgtacatgtgtgtctgtggggtgtgtctgtgtgtgcacggctgtgtgtctgtgcgtgtgcatggctttgtctgtgtgtgtgcgcacgcactctgctaagctactcaatgcaattccttactcttacttccctttctgtcacttctccataattctttgtatttcggttgggctggtatctcgcggcggcttcctcttttcctgcattcctatatttcattatttgctcttgttcctcttctagggcttttacaatatagccaggaggatgtggaaacccagttacaagatgacacacaagcacagtgtcacaatcgctgtgcttgggccctacctcctggagaccagggtgggacggtgtctctggatatggagggaagggcggaagatcacggggtggcagaaggcccgactgtccggtcttctggaagctggggtctcgtggtcgctgggctggtggtgctctaaaacctagagtaaccgagagcaggatgactgcacccctgactgccgactcaccgggcttcggagggccatgggtgtgtgattccacttgtgatcctcctacttccccagcccaccctggtggtctcccacttctctctctctgcctgtggagtgttataaccgactccttcttctaggcatctccatcccaaccccagaccagttcccttaaaccacctcccaccacaggacccccacaagcagggacctctcacagttcctgttgcctggggacttcatctcagcttccaaggcctctggaaccaggccctgcatcctgggcatgactgtccccatgattctctgagccagccaccaccccaccacccccccaccgccaagtccactgctgaccctgctgtagccccccacctccacttgttgagattccctcttcctgcttctcattttgaatgtcacccttctgtgacttctcacaacccccctgccacccctccctccagttggcatggcttagtcttcctaagaacatgtgctgcttcccagtacccagggctgctgtgcaccgtggcacgtgagtttcggtgcatcttcctcctgctgtttataaattgcaacatccctggacagatcttggattttccctctataatttctctggagactccctcggggtttgcacacacatctgtggaatgcccaagttggagatggtcctccctgatgtgtagtgtgggctattcagagggcctcatttcataaactcattaacagctaggacgcgaagacttggagaagttagctcaggacacacggagtgggagggaggcaacgagttaagaaatgggctttggagtgcctcgaatttggcctccacttttcttttctactgtcttacctggtcttaggcaggtcgggtgaccatctggagtcggagtttctctcatttgtaaagcgggggtgatatttttctcacagggctgcttcaagggttaacaaagttaatgtctaggaaggacatagcatagcaccttcacctggttgcaagcccctggagtcacatggcaacagctgtggaaccaggtaaatgacttgacttacatgttacacgctcttagttgttcgatttgtaaatgggaagagtgtgtgacccaaattagtcgtttccagatatttcctggtaaatggttgttgaatcataaaactagaaagatgggaaagaaagggaggaaccccccttacttcgaagaagtgttgttgatgtgaaggacaggactttttgagacactctcatcctaagaaacagctgatatctactaggaaaaaacatgacatttgaagtttcttcctaagagatgtgaggttttgacagaagtgccaggaagccagaggtgtgtgagtagtgggccaatctcgcgtgaaggctgtgggacggggcaggagaggggcagccagcatttcctgagcgccagctaatggcggggacctggcacctttgctctgtgactctccagctgtatggtgacatgaggctggcgttttctttggtttcatacgtgaggaagctgaggcttggtgatgtcctgtgcatggctcggactccagagctactcagaggcagaggccgtctgtaaacaccttcaggtggttggaggcagggtgctgcagccaatgctgatcactcacaagccaaggctttattgtaagggctaaataaaataacatatgcctagcatttatacagcacggggctttttaggaaatagtgagacgaccatggagaggtggaggaagagagaagggaaagaagaaaaagaaaaaaaaagccttaaagagtttcttaagagaactatatattacaaagtccttggagttttttttccctggttagacataagtttacatgaaacgttaaacggcttaaagtagccacatctccttccttatgtcttctcacagccacttgtgagtttcttatcaagatacagaattatggccaagtgcggtagctcacacgtgtaatcccagcactttgagagactgaggtggaaggatcatgtgtgctcaggagtttcagaccaacctaggcaatatggtaaaaccctgtctctacaaaaaaatacaaaaattagctgggcatggtggcatattccaatagttccaggcactcgggaggctgagacaggaggattgcttgagcccaagaggtcaagactgcagtgagctgtgatcgagccactgcactacagcctgggccacagagcaagatcctgtctcaaaaaataaaataaaataaaataaattctgcaacaagtcacaattccttgctcagaaatctctacaggtgtgcttctttgttaagaaatggaggaaacatgaatttcatcctgacttctgagtcttgtagagaccagatctgactcctgcagccttctgcccacagagctggcaggcgggggaatgtgcgcagagtgaggaggagctgatctgacattccgaacagtggagactgctgcctatttggccgcaccactgtccttctgcatggaaaagtcacagtaaataatggactctctacctgtgagtcgattttactgagctgcctttttaaatatatgtgtagaaagggcgatctctgtgtgtcatttgcacatgtacatacacatgtacacacgtgcacacgtggtcactcatgtacacatgtgtgtgcaccagtgcaccagaccagatgcacccacccaattccacgctcctcagccccttgctttcctctgcagacagccagttcagctacagttatgccagattgcctgcactctgatctttaccatcaccagactctcagcttgagctcatgcctgagaaatccactttctgggaggaaggcagaagaaactgccaaggcaggactgaagacttgacctccacctgtagtggggtcaggtcaccagaggctggctgactccccaggatttctcagcagagtattacacaaataccccttccttaaagattagcaaccacttaaagacacaaagtgtgcaggactgtacccatggccgagagcggcgggattaagagggcaactgagttgttcttcccatccctcctcctctgtgctgagtcaccttctgcttggaattctgacagggacccgttgggcttctggaagggagggacagcagaggatccaccctctgtgtgtcctgggggagattacttatctctggcctccctgaagcagggcctgggcttctggaatctttgaggctgacaccctgccagccctggggatgagagggaatggccgtgtctgtctgcagagcctgaggaggagctgagcacagcctccagagttctcttcagttgatcgcttaggtggacaaaggccacagaaatggatttaaactcctcagccctttctttgcatgtttgttctcatttgaagtcagaagtgatatgtcctacacctcaagaacgtgtgaaatgcacatacaataaccccatttcaggaagccaagtccagcttaacagtcaaaacatttccttcagtctttagtccttcactttgccgaactcccttttacaccggcagcaacagtttaacctgttgcttctgtaagagtgtgctactgggaaaaccacatctaaaacacgtgtgcagttacatcagctagagcacatgctaaacagttgatcaaaggctcttgccttgtggcccacgctgcagacactctgacgactgccgagctccgcagccccatgtcgtcccttccgcactgcctgctgtgcctctcctctccatgtggcagggaacacagccagtcatcaccatgtggctctgcccggcgctgccccagcatgtcctgacagggcctagatatggaaaggtggctctccatgcacacaccccaagcccctcctgcccgccgtgtgacccacactcttatgggcagcccagttattttgtagcatttcccttccttatcattttggcccagtgatccagcacaaatctcccttattagaataaaatttggaatgacaaaattaaatttcatttttcacttatattgaggacctcacactcttcacccctgccacgatccctgacaagagccttcctatctaatcattgttcctccagccctcttagttttcttcagcctttcttgattgcctgaatgtccctttcccttctccttttaaagcatgaaccaagctttcttaccccgttctcattatcatttttgcattttcttctttgcatatgattctccttaaattataaaacttgggggtaatttctagaggtgccatcatagtgcttctgtctactcagtgtctttagaatcagcaaatatcatttttacaaaaaagtagtatttcttccaaaaaagagtaagcaagaaggttacaacactgggaaaatatccctaagcctgttcttcaacctgttgaatgttttcccctaaattgttatatggagatcctggacccggaagttggctgacatgaaacaggcctagcagggcagctgaggaaatgctccaacctcaggatccaggaagattgcacatggcaccaaaacaatcatttaaaagctaatcctggccaggcacagtggctcacgcctgtaatcccagcactttgggaggccgaggtgggctgatcacaaggtcaagagatcgagaccatcctgaccaacatggtgaaaccccatctctaccaaaagtacaaatattagctgggcatggtggtgcgcgcctgtagtcccagctacccgggaggctgaggcaggagaatcacttgaacccgggaggaggaggttgcagtgagccaagatcatgccactgcactccagcctggtgacagagcaagactccatctcaaaaaagaaaaaaaaagctaatcccataaaagaaccatcattttgaacctgctgtttcctttcttgtactctttagaagtacccatttctccctttctaagccataggtgtattaattggagctttttctatcttaattagttcactgtgaacaattaaaattgtgttaataaaacaaaaacaaaaataggactggtgcctagttgtactacatgaagagagaaagggccagacattggtttttcctaatcttctgtcaagttctccaaatcatctgctctggaaggtagctccaacagctgggatttgaagtaaagcatagtgactttggccatcactgacatgtcccatttgaagcaaccaaaactgtccctcgacctgacactcatccctgaaacaccatgagggtaagtgaggcgcttcggaaggtccactcaaccccattgccagatagagtaagtgtctgccaggggcatttggagctgaagggaagactgtacagactcacggtttgcaggcactgaaggcgttttcctgccttctttttcaccttcagtggacttgcaaagcactagccctattgtttttcccatctgggaaacatggtgaatgttggttggttgtagctaatcctatgggtcttgaggtctttgttgacaagaaggtagatgttatctttatctgcgtgtggctttctactaaaacatgagctacagggctctcttttttgttttaaagcatttttccataaggttcacccttactattgcttatctgaataatattacctgctgagaagtttattcattgctcaccagttgtagggagattttgacacaggactggaggatttttttctcatcgtaacagtgcagacccatggaaagcttggaagcagttgtgaccggataagagcaggttgaggatgataatcttagggcaatgagcaggttgattgagaggggtgcctgaaagcaaggtccccatgatgcaagcaaacaaactcacatgccagacggtggacaggaaacacaggcaggatgtggtgcaggctgggctgccttggctgggcaaaggcaggggcttcatggccatgctgggatgtgacgtggttggaaaacaataagaatggagacctctccaaagacctcagacataatttggccatgagaggcaagggtagaggcgagccccctgtgggttggaatgtatggaatccagatgaagcaccatcaacatgcatgggctacataggagagctgggtctgggggaaaagatgggatttgggtttgggtgtgcatgttccaggcatggagggaagaatgggcagaatgacgaggatcaagccctggtggagcccccagaccagggccctgggcatatttccacttgccttcttctgcaaacttttgtgtgcctgttgggtggaaggtactatgctggggccatccaggatccggagcagtgtaagacatcatggcctgcatggtgtgacccttgacatctgaaaagaacgagctggtggagtgggaaggagacaagtggcagcagagttgacatcatcaggactgactgcaggacaggcggtgaaacgagccactgaggagttacccagtgccctggggagcttagatgtgagacttacaccacccagcactccccagctctgtgtccctgggtcccactgaacttgattgtattttagttgcctcttttctaagaccggagcaacaataccttccttgagtgtgcatgtgcagtccatagatggcagccagtgttctcttcccatgagaagactctgagcctcctcactagagggtggtctaaaaacaaatggatccatccacagaaggtctgaaaggttttcatagaatcttgacttggtagcacttcaggatctaactcgtgctttccagaagtgtggcctgtggtgttctgtctggagtatttggtcctcccatccacctccaccttgctgtcctgtcctgtgactctcactagctcagtcaccgggtcaggaagccctgccatgaaatgctagatttggaggcattgccaaggtaccacaaaccatactcaaacaaggtcataatagactagtgatctcactgtggctaacaggttcatgtgatttaaagaatgacagcattttttctaaattttataaattttataaatttctcctaaatacaaatctgaatgtgtttacctttagacagattttcccagaaaattgtcagtgttctcgaatttgaaagtagatcagatctcctccctctagttttgaaaatctcaagtaggtttagcctctccccagagtgacaacggcacaagaagtttataattttatgcacagctaaatgcaaactgaaaagtgtggtttgtgggtatttcatttttcccataatgttcatcaatttggcaattcaaataggattcagaatccaaggtgttcgcagcattttatatgaaaatgtgcctgagagtttggggaatagaaattcttaccaaataagttaaatttgctcttgataagaatatattttgtaaaatgtagaaaactgagaaaaaaagtttgacacctgttttatctgcatccttttattaaacagtggcctgaatttactaaaggacagagaacagggttgagaggtaatcactgaataatagcttcgctaatcccacagtgactgcttcttatgacaagcaagagggtcaacttagaggcaggactgtcttcaggggcaaaagcaagtcagcacctacaaacctctccaagagagtgagaaaaagcaggttgtatggctcattttgcagcttgccagaagcaatgtgggaatattgtcagactgcacagacctggggccagctggctcctagagtgcgaggagctctcagtgactgctgtgcatactcacctgctctgtgactttgttcagtccctaccctggatgtgtggtgaagggtgccaggcttagctgctggaccagtgaggtccctgagggggcagggctaagaggtgtagcagtcgcacttgaccagtcattgattcactggttgggaatttgttcattgaggggacaccattactccccatgcctcacgtgcaggtgagtgtgtgtatatttgcattaacacacaaacacacttatgtgtgtccctgtatgtgcagctgcagtaccttacacatcttccagtgcctctcaagcatcataaaaacagcttccacaaaacctctactacccacctggcatccacagagctcccagtgattggctcccaaaagatactgaactttggcatggaacagagtgagtttccacatttgctgttgtacataattacctgtccagctagaatagtacacacttcttttactgagcccagaagtttatgtgcctgaacacggatggtacaggaacaagggtgagcgcttatcaattcagcattactctggagacatgaaacaaactaataggtacagctatattttgttttttaaacaattttgtgaaccacatatttgggacaaaaatcaacaagtaaatttgaattacactaggcaaaggactgattcttttgaaacgtgattgacattcaacgtctaactttccaaaagaagacatacatgtggcccacaatcatatgaaataaagttcatcatcattgatcattagagaaatgcaaatcaaaaccacaatgagataccatctcacaccagtcagaatggttattaataaaaagtcaaagaatgacagttgctggtgaggttgtagagaaaaaggaacgcttatacactgttgaggggattgtaaattagttcaaccatgtggaagacagtgtggcaattcctcaaagacctatataccatttgacccagcaatcccattactgcatatatacccaaaggaatatgagtcattctaccgtaagacacatgcacgcatttgtttgttgcagcactattcacgatagcaaaaacatggaatcaacctacatgcccatcaatgatagactggataaagaaaatgtggtacatataccccatggaatactatgcagccataagaaaaagaatgagatcatgccctttgcaggaacatggatggagctggaggccattatccttagcaaactaacccaggaacagaaaaccaagtgcagatgttctcacttttaagtgtgagctgaatgaggagaatacatgggcacatagaggggcctatcagagggtggagggtgggagaaggaagagtatcagaaaaaataacaggtagtagatttaataccggatgacaaaacaatctgtataacaaacccccatgacatgagtttacctatataacaaacccgcacatgtactcctgaacttaaaagttaaattaaaaaaaaattaatgtctaataatatattacagtattcttcatattcaatggcaatgtgtgaagtgggaagtgtcttgacagaattcggtgtttcaaggcttacactttgatgcccaagactgcacaaggctacattttctactggtgagacaaattccagacgcattgcattcagatctaatctcttagctccttaatcttcagggtactggtaaacatgaagacctccccagtgctgtagtcatcatgatatgtacagcaggtggctgagctctggatgtagactgcagggatatattaggaagttaattctcaaggcaagtcatcttcaagcaccatatcagcatgatcagcaatataagtagtatctcagtgctttgttgtttagtcagagttttgtactctatcacccattgtaatgttcctatttgcaaaaggtaatacataccctttaaaacatctttgctttttctcccattatcgagatgctagcagcttcataaagcagaataactaagggcaaacagattatataaagggttggagctcaatgaagacaacaagaacagcaaaggttattgtaaaactggctgcttgcaggccaacaagcacatccatatggaggcaatcagtttatgctacctctgtctgtttgatgggattcataatattgactttatccattagatttggactaccagggaataaaataagcagatggagagtaaggatttgctaggaaataattcagccagtcactttgaaagctgttcaagaaacagctttcaaagtgtctctcaaactatgtttgcccattatcccaataatttatttcccaataatttcatgggaaaagaaggaagttctgtggtcagataaatctggaaaacactggtttaagcaaagttcagtaggtctgcttccctgcaggtcacctcagagtctttactctgctaacctaggaactcatccaacaagtttaatttaacagctacactgtgtacgtcactttaacagtcactgagctgtgactcttgggggaaagattgtgcgtgtgtgtgtgtgtgtgtacacatgtgtgcacatgtgcagaatctaccaaatcttaagagaaaggaacatgctgggaaactgtcctgtgaaagagaatagaaacctgaagatttgaggcagtgatagcatttatgaaagcagcagataaggactaatcaccaaaaggggtagctcttttgttggttggggaaaacaggaatttttcccccacccaatgtgctgcattttctaattttctatgaacacttcctaagaaaaagctgaatgaagaacatttgcgatgcaatcagctcattaagaaacacgcacttttgtggagatacgtgctgtcccaggagatgctctgcgaggagccgagtgtttggactggagctgctgaatggtttctcacagttctagaatgtttggggctgcaccctctaagatgttgaacccatcagtaattgctccaaaccactttatgggatataatgctgtgagttgacacctgaggggattgtggtcctgttcatgagtaattacttttctgttgcctatagaagggccagcaatagcagatgagtagctgaacagtggttttgagtaataaaacgttcttttttaaaaaaaagtaatgctttctgttaaactctgactatactctctcctggtatcacaacccagctttctttttgccttctttattgcagttacatatggggctgatgactttagggatttccatgcaataattcccaaatctttctctcgtaagtatatgccttgcttctggaaaacaaaagcatgccttcatctcctatcatgtaaatatcgtacgtgcatgttccttcatcaacccccgagatacattaaatattcactgttctattcgttagacacctaccatatcatttttgggtatttataccataaagtgcaaaacgaaggtctaggcagttgtgcggtgtcctgggagcatggcagtggagtaacagtaagggttggagtcacagtagcactgatgggattgttacttcgcagatgctgctggacagctttgagattactcctgtaatcctttttattgagtgtgaggataaaatggccatattttctgtcaccaacaaagaactgaacatggtttcaagataatttttacaattttgtgggacaggagaaggagatatgctcttcatctgtggttctggagtattaatttcagaactgagaagagaaaattgcaggcctccaggccgttattctgtggtgcatcgctgctggagccaacgtactgttcctgcttggtgcccgcaggaccttctctgatctgagctgttaaaccaaaaacagatgtgaatttcatttttcttttttagatattgagctgataaatgataaatatatttgggtaacatcctcaaatgagtactttaaagaacagagagtgcttttgaaaatgtatagagagctgaatatttaaagccatacaagttgataatccccttaggacctgtattagtaaatcctctaatactataaagcaacatcagaaaacaggtcgcatttgttaacactgtgacaattataattataggctctaatttgaacagtgccagtaacagttaaagacaggtgtctgacatcctggttatcaaaaactatctggtgtctaaggaatttaacagtatcaaagtacatctttttgctcacaaactagattggctacttttccagcctatagaagttacagaaatctttcttttactgatattcctttgattccactttaaagcaatagcttgatacctactttttgagatgtatatgtatgtacttgtaaatgcttatatatgtgtatttgtttacacgtgagcttatatgaacatataaaacattatggtattggacagagaaatgatattgatttgaagaatcatattgttgaagtattttgagaagtcaaatgcacttgagagtaagctaatgcatcctaaaacatgtttctgtgaagtctgaggaaggtgtcagccagagcatatgttgaagcagacccttcagtgaagccttcagtctgtaagaatcgctgcatgtgaagatgtgttaatgttatgatagttacagtttttataaaagagatgatatacacttggatatgctttctgtctatatttatgcaaatgtgtccataaggtattggtgtctctctttctctcccactctccccagtgttggaattgtgactatcttctcacacaagcggctacttggtcttgatgccttcccccgcaaaacagcaaccaaactgttctgggccaatatcaccaccttgtggtcatgatgaagaattgccccctttgccctcaacacctcttttcttcttgaaaattaaaaacaacccctttcaccccctctactgtccttattccagtttgtgtccgtagttgctggaggaaagaaaatgcctattgctcttttttttattctctttatctgtttactcttctgcctttcttttctctccctgacttcattccatttaaaggccttaaattgcaaataacgaaaaaagtattttctaataatataccctagtgggacgaaaacaaccttctacattttaaatgatattaagttataataaatggttccatgaactttaaaacgcttaaaagttttataaatctcttttagaggcaacacaaaaatatctatatatatatcttctcttcacctcaaattttcatttaattaccgtgattcaagatatatcttaaatatttccatttcatttgatttttacttgctagtcaccagtgttgcaagaatatttctgtaccatttttcaagtaaaatattgagcatttcaagcttacatggcctaaactcacactagagtgactacttcggactatcttttcaatggaaaaatgcgttctgagtaccaaacatttactttttcagtaaatatgaagacacattctaaaaaggaaagggaaatgaagaggaagcttaattcattggtcaggtggggactaacagtgtacattatacctatgcattaaaaaatgtttaattatccatgagcacatacagtgcctggcacagattcaggcctcttggctcctcttggcatctgagttccttggattctccagattcttcaatccaaacttgtctatctaccaaagtccaccttccatacaggggtgtggggtctctcttagtactgttgggtgccaataacatagaagccctccaagataggtcaatgagattttaatttttcccaactttaaatagcatctgggaaggaaagcagcttttgactaggagtttgaaaacatccactcttcatatttattgtcacatttattgagtaataaaattgggctcttgtccattatctctcagtcaatgaaagagcccacggtgggcatgagccagagtgttccggagaaagagaggaccagtctccatttcatgttctatatttaatcagttcaattcagcaccttactgagtttgacatttttctaagtaatggggtggggggttacaaaatatttataactatctttcctatcttcagggagatgtaccatttcactgaagcaataccacagctaagcagttccagctccgagtaacagaggaaggagtgagcgatttaggaactcacagaagggcacggccaggcaactcgggccctggcaaatgttccatagagacagcatccatggggttgaaccaagcacaatgcctgcaaatcgggcaggcgggttcatggaattgattctagggcaggtatgatcagcaccatttaaggagtggcagttgttaagaaactgaagggatttctcatatggcattttcaacagaattcagcaggagccttgcatatcccttgggatgggttccggggtattatggagctgccaggaggtgctcagcttcagtaagtgccagtcattccttcccaacctcctccttcattagtggaagtatcagctggtgtcattgccttcttcaggaggatggatttcaaaatgaagggccaacaaaactcacattctcgcagagcctccgtcacaactgcatgtgttcactgccatcaacaggccaacacccacttgttcttttcttctaggtaaaggaaaaggtctgtgggacaaaggccctgaactcctcactccttgaatgggaggcatattggtggaggctgtcacacaactacaggtggcaggaacctgccatcagggttcccatcagcctccagggcttgcttctctgccctgtgtgtggacaccttccatcactggaaacccctctctcagaagaaccacttcttgccctcatctcccacttgcctctcctcggcaccttctccaccctcaggggccaagctgaggaagtgtgcatcctgtgccaccaaccttgctcgcaggaattagtttcagtccccagtgactgactcttccaaacctgcaccagcctatgctgcccttttgaaaggaggcgtgcgtacagcctggctggtacagaagattccagatttcagtgactacaggacgctgtcaccccttctgtttttcttttttctgtccacatctctgattgagcataccttcagggaaaaccccagaaacctttttcacacttacatgggaagccaagacactctcatcctgggcttgtgtttttaaaatctatattttaatttcacaggtccttacatttatgactaatagatttcagattttgagatacaatctgtagttgcaacttatgaagatagtttcaagccctgatttctgtcatctatgaaaacagtaagcaagttgcttgtattctcctcctagctggataagagacccccgttttcatggacagcctccttgggtggacagaagtctcctgatcttgtctatgtaaccagcacccactttgcatttttccgcaaagaaaagaggagcttaaccccatttacgggaaatccacgcactgcttgaatcttacgcgccccgtggtgacggtgttgcccactctgttcccttcccaccaaatcctgccagcacctggcagtcatccagtccttgtcttagacttcaccaacctttcccgtcataacatggcttagaagttgtccgaatagtgctagaagctttcagccctggaatgctcagcatctgccatctaacttccatttaaaacgttttgagcatttgctgatacaggttcctctgtcctttccccattattttcagttccttggccttgcccatagtgatctgtggatattgtctgcatactcttttttagaaacctagagcatcgcagtgtccttaattttcctcttcaaactctatatattcctgagctgatcatccctactgctgttcctacagaactgtgtgactaatcttctatatatgtccctacatctagccatctaggtggagatctaggtacctatctccctaaaattgtacttggtatccacattgacctcaggacagtatgtgataggctcttgtgccttttcgactaggagtttgaaaacatccactcttcatatttattgtcacatttgttgaataataaaattgggctcttgtccattatgtctcagtcagtgaaagagcccagggtgggcctgagccagagtgtttgtgtccctagttctcttttggttctgttacagctctcagtgacagtgtcattgaggctaacaaggacagagtactgctttcagccaccatttgtccaatgagtggctgatctccaggcctctggctttgagaacatctgtgatatctaaggcagcatccattgtgggctttcccccatgcttctgtttccttcctgtcacatagctttgcctcctcctgcaagcagcctgctgtagcagaaccggtgttcctgaagccagaaacccaaaggtcgtgtccaatgcttccctgctgttctgctccccacctgcaagcgcccacacactgatcaacagcacacgccatagagcatgccaaagaatcccagaaatactcattcttaatgatccagaagaacaagtgatagcttctggcaagttctaataggccatatgtgcccatgggaaagcaagagtcaattctctctagctggttgcctctgaatttatgaagtcaagccgcgtaggggaacatgccaagaggattatcccaatgcctgttctgcgtggtgtcctttttctagcctcggaagcactaggcctacaccttcgctatagccctcgtcttagcgcctgtatttgaaaaacttgccacaccaatcttaatttgctccattgtgttctaatctcattttaaaaaccacaaggtaaatgattaaaaataatcttagattaaggagtacacagatctttgcagcctcattgtgtttccagagcgggctagtgtagacactggtgaacaaggagggcctagagaattagctttctcccagaaagatgcacagcctctacctgagagtaccaattccagagaactcaatggtcattaagcaccattgcctcgacagccagccagcctcacttgcctgcctatctcctttattttccaagtatcttgtccctggcagtggggagaggttagcaggaggctgctcagatgctctcggtctctgatcttcaggatctgaaggggagagcatttgaagaatccccattgctggatttctcaggacaatcctgcataatgccaggatctgatggaggagacaggcagctctgttaatcctctggtgcatcctcacttctgtggtctccaagtccaccatgtcccagttaattcatttcattattcatctgtaagtcatttccctaaagagctaataagaaaacactggcagtacaatcagccctccatatccatgggttcagcctctggaaattcaacccactgtggcttgaaaatacagtattcaagagacatggaacctgtggatatagaaggcagatttttcgtatccataggttctatagggccattttagggacttgcacatctacagaccttcaggagtctcagaactgatgcactgcagataccaagagatgactgtaagtggttaggaatttggatgctggggccaggctgcctgcagttaccttccagctctgccacttgccagctatgtgaccttagcaagttgttcaacctctctgtgccttggcttcttcaactgtaaaataggataatgatagcacttcccttatggagtccttgtgaaggttaaatggcagagtacaattaatgtgctgtgtgcccagcgtgtggtattggggttaggtgaaagactgtactgggatcactgggggtgagcctccatgtgccatgccccaaccactatcctcagctaacttcttgtctgtcagtgttaggctggtgctataataatttccattttcatggatgaggaaatcaaggcacagagaagttacatgacttgcctaagatctcagtgcttttaaatagtgcagctaagattccagaccaggtatttttatttcagtgtctggactgtagatctctaaatcgagaggaactccctgaataaaataagcttggagtgctgttaactaagttggttatttaagacagttgttctcagtcctcagtgtacattagaatcttctggagggtatgttaaaacagactgctgggcccaccgagagttcctgagcctgcaactctgggttgagcctgagagtctgtgcttctagtaagttctcaggtgatgcttatgctgcttctcccaaattttgagaaccattgattgaaaatgttgatcaaaaattatgtggtctaggctgagcacagtggctcacaactgtaatctcaacactttgggaggccaagtcaggtggatcactgagctcaggagttcgagagcagcctggtcaacatgacaagacccatctctacaaaaaacaccaaaaaaaaatggctggatgtggtggtgcacacctgtagtcacaactactggggaggctgaggtgggaggatcacttgagcccgggagacagagcaagaccctgtctcaaaaaagaaacatttagtcttgattgtcatctatctcattgatcattttacttggcaaaatttacctacttactcttattagtctgtaaaaatggttattaaaatggtggctttcagtgtaactacaaattctcttagtcattatagtgttggattcaccaatgtatcatcagtcagtgtttctgaagtgtgtaaatgaaataactcctactttctttaggaagaaaaatattcaaatgacataattaccttgtgatgtgtgacttaaaggtaacagtaatgcagagtcaatagtggtcattgtattcaagacactaaaagttcacctcccaccccccccccccacccaccacccaacaaacacacaagcttctttccctttggaaaaaaaagctcttccagatacctacattcataaactatcccaattaacccttcagcaagtggaagaagtgtaagaaaggatacctcttctttagaacacagggtttgtttttatgttatttaagataaacaggaattcaaatggtcatgtaccaaagcaacacaaagaacttccggaaatctgaaagggaactgtggtcagaactctgagcatttttatgtttactgagttttgtcccaaagtttattaatgtttacatgccacaaggaaaggtagcatcacaataagagacgtttttcaggcttgataaccacttattaggtattttgccaaacaagttcacacatcctagagagctggattgtgtgacccagaacccaccctctagggcaaggtgcccatctgatgggtagggtgtaggagtaggcctcagaccactcctgacgtgaacctgcttaaagtgagggcccaattctaaagtgggaactatgtaaatacctttctagtgcattttcagataatcgccactgggcctatggatggagagggctggcagatctccctgtaaccccaggtgcatcccgaggcctgccaccgaagcccactcaaggctgaatgcacggcgagctcaggctgctctccccttggtatttgctaagaacttctgtttagtagctctccacacctatttgattgtctttttgctgctgtgttgttttgttgagttttttttttgcaatgacactgagtggcctcctgtattgtttctttcagccagtaatgttaaagtagagactcagagtgatgaagagaatgggcgtgcctgtgaaatgaatggggaagaatgtgcggaggatttacgaatgcttgatgcctcgggagagaaaatgaatggctcccacagggaccaaggcagctcggctttgtcgggagttggaggcattcgacttcctaacggaaaactaaagtgtgatatctgtgggatcatttgcatcgggcccaatgtgctcatggttcacaaaagaagccacactggtaaggcctggctcagtttttcctttagtggcctggagaaggtgcatggggtttgaaggaggaaagcatcctgtcttccttgtgttctgagcatgtttctaattgactggtagctcagttgttgcaagcgattggttccaagtggtaccgagtcatagagtccttgttctggtacagccttgtaaaggacttctcaacacgtaccaattccaccctataaataaaacaagggaaaagtgaacagcatcacatgagaggcttggcgagggctgctattatagtaacacatactaagtagtctcagctgagccctcagggtacgtgtgctgagtggtcaccctccacaaaacaaaaaatcctgatacaccaaaacttactcctcaaagtttccactgagaaaccatgagtaaaatgtgtgtttaaattgtatccaaactaacagggtttgatgtttagaaacaataatcaatgatggaatagcagcaaaatcgagttttcagaaagacctcagatgagctttcaaatggcttgccctctaacaggaaagactttgaatcagatgcttctattgccactggttatcagctcaaattcctaaagaacttcatcccaaataccctgtcttgctgaaaggtttactggaagtataagagaatgtcatgttctgtgtccagaaaggaaggaacacgggcaccctagtgtcagcgagttgtgctcaggctcacaggatgccccctcaccagaggcgtgggaacacggcgagccccagctggccgcgctctgccactgtttctaatagccggtcacgttgatggaagtgtcacagagttgtccaacagaactgtccagtcagaaaaccaccactcatggtgctggagtgtcttagaagtaaaatatgaataacacacacttatttaactataggcaggaggtttcttatgaattgaagagaaacttttctttgcgtgggaagctgttctaaagttgggtaaaacacaatagatccaccacctctagcagccactgatagctgaaacgtgaaacatagagaccctaagctatcactgcctctgagctggcattgttaggtcatcataaagctagcgtctcccactgcaaaacccaagaggaaaaaaatagttgaaaatcctattttaaaggcctagcagattctataagataccttgggaaaatgatgacgatgacttgaaatcagaccctcgtatgctgcttccgtgggggcgaacaaaaatatgttcatcaaaaattaagcagaaatgcagaaaattttgtgagccaaaaaagctgtgttatcaggaaatgcagatatttgtggggttgtaattttttatatttgaatcgggcggttttcaaaatgatctattccatttgtagtgtatctgaaaacctataaaaataagttgatatcaatagatatccatcttccataaaaattcaacttctaaaattaagcaaactttgctttttctaatggcccctttatcctcaaattacccactgaaatagacggatcacactcagccctaagtgaagcaagcgtgcatgagagtagtcccagcctcgcctttgtaatgaggtggaaattaacatgaaggtaggctaccctgtgatagacacttaacaggatactcggggacccatggtaatacatccctgataaggaatagacctcacaaatgaactacttgcctgttaattcatttaaagcctgactgtacagtgaaaattctcttaaataaatatttgataagtgaatcaaattctggcttactaaattgccaaaatataatgactgcctgccttgataaaaagaataattacatttaatgaataaacctgccaagtacagatatgccaggtggcacctgctgtttgctgctcacttctcccaacaaatagcagctaggtgccacctgcacaccaataagctgagtttttcacttacggaacaaataactttcagaagtcaattttatagtttctgccttgccctttgttaaaaaaatacacacacttgaagcaatgaactcatgaattgttttcatcatgcatttccacttgcctaaatataaagggtcccaggtagatacagaaatacctggtttggccaaacttggtttgaataactagacatgctagaaaaggttttcattttcctgggatctgagtggaatatgttagaaaaggcatgctttctgaattctctatgcttaaaacatttctagagcagtgcttctcaaacttgaaagagcatgtaaatcacctgagatctcgtgaacatacaactctgcttcagacctggggggaggcaggagagcaagcattcctaacaagctcccagcttgtggagcacagagccgcctcaggcagcagggcagtgcagctgagcagtgacagtgaacagggccattcagagggctctccacctggggcttaggtacgacgggaatccccactggacaggctaggacttgcactgtggccattgttcctcctcctgcccatggctgagtcagcttctcagtcccttccaggatacactgagaggattcaggggcggtctcgcctctgcccatatccccacgttggtgaagtaccactggcgccattttctaatcagctcatcggcaccagcacgtcacttcccctgttgtgcagctcagttttatatttctgactcgggtgtaatagtaacatcttccccaccaatgtctcagggttattgtgagaaccagagaggagagaggtaggaaggaagcaggaaatgcagggtgcaaatacaccacattattattctaaataatgggatttttaataacaaagaccaagaagattgtctgtgcctatctagttcccatctgtaagataaaaaggtgcagtccctgagcctcctaaaaacagcaccctaatggcactgctcctcccaggtatgattgcagtagacctacgtcagttcttgcagttcaaacacattttttcactttcttctgaaatgccctcaaattctatgacatagtatccatgaagacttccctttttacccagtgaagttactagagggggttcaaaccttcttacagagggttcctaaaatgggagatctgtggagtcattgggattaaaaattaaatttcaaattcatgacatcaatgtcctcatcccagttaaataaaagtaaatacaaccttgaagaaatttgacctactcagctgcaatagctgttgacctgcagaaggcaaatgatggaccccggccacgcaagaacacacatggcgtgggctgcgttcttgtgccccagctccatggacgtgtcttcttagctgtggacccctccaaaggaaactgcttgagtggagtgctctgtattgtcactcctgggaatgctctcttaacacccccatgccttgtgctatgtgttcataccagcataggcactcagaagcaaaaaaggtttccagtgaaatttgtttgcaggcaggtattaagacatcagacactgcaggatccaagtgaacccctgcccgcctgcctgcctgccctgctctgctctgcagaagggcatgtgtctgtagcaatctgccctttctgtctgcgatgggcagagaccctggctctgcctcctgttttccctgtagccctccagacctggggagagacatgggactccagcacctgcccagcacggaagggggtctttcccaggtgtaagtgtagggctgcattcactaatttagggtcataccacaaacactgttgtgtcaccaggatgttgtcacatgcttattgtgagcatttttgtgacatgagctttctcctgagaggccaccctgtccaaatgagagctgtagttggaggcacatccgtctcatgctgcctgggtctccctgcaccagctcactctacttttcctttttatccacttggagttaaatgcacacatttatgcacaagtgcacagaaggcccagaactgttcctaatagataattaaatgatctctctccagtggaaactctcctgggctacctggctgctagctgttttagcctcttcatccagtattgatttacatgcatcggtttgtaactcagacagtatagttagttagtttgtttcaccatcaccttccaacctgcttacgtttaaactccttctctctgcttagctaatacagatttctgtaaggatttggagaaataccagatacctcctggttagtatcaggacctctccattggcctataattgaacatcactgtaaattagtttcagcttttatagtaatgcatctaacccgccagcttaaaaaaaaagtgatgataatcatgaaattcaagtgtcaatatagacttttaaatctggtgtggatgttaatagtgccagatatgcttctgtgtaatcatttttgagaagtgctgtcttctttaccataatcacattaatcaatcgggaaatggttaaatagacattttaatacattgttttttcctgagaaaaaaagtgactccaggaaatatgttgttacaatatctcaacaccaggaattgtggtcacatagcattcttcttctaaataaagcatttgttttacaaaagagtttcatgtttacttaaacgtgacaaatgtatcactcttcgaagtgagagttaaatgaaatgttccctgatttagattccaagacctgtgactactcagtaggacaatagcatatttcttttactcagatacctgtttatccctttgtcagctccagaatggagacacaggtgctgccacacagaggagagggtcaggtgttttcttagtcacaaatgcagcagtctcacccctgaaagaattccttcataacaactaaattgcacctcttagaatacctgtacttaaaatataatttgtcttctatggatatagacaaataatagcttaaatgttttaggatttgtaaagaaagaaaaagctagaaatctcaatgcaactctgacttgtatgtcctgccataggaaggtttgggacttttctttggaagatgggaggcttccttcacagtttcttaacttctcattttattcaatctttctccatctctctctctctttctctcatcctcacgctctctgtctgtctctctcctgatttgtctgcttagggacagacaggtaatggagaagaaattgaaagggaaaatacagggaaaatgtaaatgaaaagaagttattataactgttataatgaagtgcctttcatttaaatataagaatgtaacgctgaaatgaacttgtgatcctgaaatgcatttttaatgagtttcctttttattttgctgcttcagtggcatattttaaagaccctttgaaaaaagccacattaaaaaaccccaccaaatgccacaacacgcaaaattggatattggtttattccaaaactgctgatcaggaagagtggctcttcatcacaaaatgttgcagtcactttatttaaatgagtttgaatttgcattgtgatgtgccattctgatttagggaaaaaaaattagattttcagatcaaattgacccagccagtgaagcgttaaggagctggcaggtttagtctgaaagcctcatgttctatcaaacctgcagccggtggaagtcaccaggcccccgtgggaaacaactttctcgtagcatcgtcctcatgtccccacgctgagtttagttctcaccagctctcctctctccgtcccaggagaacggcccttccagtgcaatcagtgcggggcctcattcacccagaagggcaacctgctccggcacatcaagctgcattccggggagaagcccttcaaatgccacctctgcaactacgcctgccgccggagggacgccctcactggccacctgaggacgcactccggtaggtcccctggatgcagtccggggctgtctgggtgtcccgggattcctccactctgcccgcctgggtcccggattgtgtccttgctggctaaccctgagtccctcccagctcgcagtcctgcatcgggtgtgagctgttgcttctttgacattgccccatcccccctccccatattctccttttcccactgcaccagggagattgggcgcaggacccccatgcacatacacacacagaagtctcaccttaggtagcatgtttcagaacaggcctcctcatcccgtttgtcaggctggtatggtttccctaaaggattttgcgggaaatgttttcaccaagtgtactgctaagacccaaaacgttttcaagtacaattctttctgttgttaagtcccgctttggagtgttttacacaggtgtaatggatagcttttttgcagagctggtagagaagggtgatttagggcgcacccacccagactgagccccgtgtggctctcacaccaaaaaccagccaaggccacagttacagaggccagtctggggctgttaccagattttagacagcagcctttctctttgaattagacagttaaagtacaacccacataatctggagtcttgacaagatcatcataggcataaacgctctatcattctcaaaacagtctcagcctgcaaagttcaaatccactaaagtttggttagatcctctgcctcctgagaaatggtcctgggtgtttcattatccagcagtcccataattctacagggcagaggaagagagggctcttggccggcctgtcatggatcatgtttgcctacagtgtggtctatacaacatgacatggcacaggtctccttcataccgtccagttggggatatttgctgtagcatactgcatgagacttcggaggcgaaaggttgatggcttttgtccttcccctcaaggagcttcctgccccagccagccaccagccagggcccttctccaagcagcagcctctctaagccggtgccctgggggatggcaatgcctcagaccagctactcctcacccaccctgggtagcaggataaggaggagcctccctcagggaggcagacgtgtgttctttgtgaaatatctgcagcggcccaggccatctcttcccaaatgtgatgcgtgtatttgatggttgagggttttagaggctgctcattgtgtccatctctttatcacacatttactgagcacccctgggtgcccattctgcacagaagacctcaggtgcacacaaggaaagcaccaatgtgttacaggaggcatgacagagtgtctgaggggacagtgggagcataaggaaggggacagtgggtcctggggtggaaagtcaggagagacttcccatagaagggaggggcttctgaagtacatgctggaaggcgagtgtctgaggtttgctttagagacattctaaactagtgtgtgagtcggcagtaatcccagagaggggtgcggcacccatgttggcaagaactcggtctcactcctggcaggtggtccctgcagtagttcacccagttggctggagacaaaaaggagaggagtcacaggggctggtgcatcacctcctctccatcctgacctccttcctggcggtgcacatggagaaggatccccacatgctcgccatcagaaaattgtcatgatttgggtgatttgacttcctaaaaacttccaagaaaggagctataccaagctgaggagttgcttgcccgagagggcgggcagatcagcaggggggccatggagtgggacacttgccttgttacagagggacagggagaacaggtggttcccctgagataggaagacagtagcatgacggtgagcatctttaaatgttcacatgggtgatgagcatgtatggtggtcccacctggagacaaaggtggtacctgggcctgataagcaaggcccatggaggcctcagctaagagaactgtgcagtctgtctgccatgctaaccagtggtctaggaagaagcttcacatctgttgtttctaaggagccatgtagacatagacacagttggcagcaatattgccttgggttagtgggaagcaccacttcccatgtcagtggaaaacacagacactcgttcttaggttgacaccaaccataggtcatcatcactcctagattactctgattgcaatggaatctctcatgcccatcagtccttaaaagcagagctgctctctttcctttcttgttgtggagttaggaacatgtagtggagtattttatgttattctggctccaggcctatgtatttcatttgaggcatgatggtttcctattctaagtaccactaagtattgagtagttataaaatggtggtagactttggactgtgtatttctattctggatccacggatgagcaagtggagaaaacccatcatggatgcagggctgctggggatctgtctgtccgaaaatgctatagagacacacactgctcttggggaaaaaaacagtgatgatttcttcaaaatgatttcactgaagtgaaataaggactttggccttgctctggcaaattcaaatgtggccacactctactccattgtggaatggtgactcccctgtcccatgaaaaaccaggatcaacatcacagctttctctagcaactggtggtggcctgaggtcttatgaactagcatgttagcagggatagagttagggaatttgtccgatgctgacagcaagagggtgctgggggagctggaggggtggagaagtgatctcccttcctgcctcatggcttcctttggaagttgcaagcttagaatttctttcccaaagaatattggactatgcttcaagagacacttgagttcagttgcttacagtgaacatacttcttatgttccagagttaaactcaatcatattttcagaaaaatagatattcagacatcatgtcatatttacaggaagctatttgatcatggaatttactgaagtgacagctttttcaggaaagggtatcgagtggttatctatatcctattaatttctaaaagcaatgctcaataaaatgtgcaattttaggcaatattctgtgtttcaacattatttccttatgttgggggtacatcactttatatagataaagaaagatccttttcattctctattaaatggtcgagaagtcaaattttggctttcatgttggtcttcttactgtagcttctgttcacctaagaaagagatttaaccaacataagctttggctaaaccattgtaccaaacatttctatttggatgctcttaacttttatacaatactttgaaatgtgttcaataaaacaacatgagaaagaagtagaagattctgctattaggttggaaattgatattccttacataagtgattaaagatactttattcagtttatcccttaaaatggtatctactgaagtccttaaacttaggcatgatattaattcctggctagtctttctttttcctaaaatatcactcaataaaatccaagaaggactaaaactcattatatagaactgcactgcccaatacagcagccactagccacatgcagtatttttaattataataagttaaaattaaacaaaattaaaacttcagccctcagtggcactagccacactttttgtgtccaacagctacatatggctggtggctgccatattggacagcactaatagagagcatttctatcatcataggaagttctgttgaacaaggctgatctggaagctacaccatcctaaagctctttggcaagaaagcagagcttttccataagctcagtttatgaacaatatattttgtattttctatgtatatgtatatgagaatacgtatacatagaaatatatgaaaatacatatacatataaatatacatatacataaaatagaaatacatatacatagaaaatacaaaatattttgtattacatatacatatgcatggaaatacaaaatattttgtattatataatgcaaatgtaagatatatttatattatgtaagaaaatacatttgtgcaataaaacgcttatttcattcaagcatatttgtccagcatggtttcttagagactgaagttacccagtttagcacctggaactgaattcactctggctgtgttagatgtagcaccagcgtcatgacagatccagcccacagcatagactgaggcctactctggaggcaaatctgcagacaatgtggccaacacatgggccttcctcacatctctgtccagtcgctggcatccacgttataacacagcagtggctcgttttctccagttaaaggctaggcttccgtgattgaagcaggagagaatttggtagtcagtaaagtagacaaactaagacaaaacaagagtcgcatgagttcttggtacaattaaagaaacccttggccaccaacgtttttaaattcaggaatttcaccaagtccgtaacagttttagctctcaagggtagaattttttttttaacttttttggtaataattgtattgcatgcattccccttacacagaaggctggcatttaattggggtcttgaactcaattgtgttttctgcagttggtaaacctcacaaatgtggatattgtggccgaagctataaacagcgaagctctttagaggaacataaagagcgctgccacaactacttggaaagcatgggccttccgggcacactgtacccaggtaagcgctgctgctcggaggccagcctggtgggctctccccccagcacggtggggaaggagggcgctctgcatgcagccttaggagcagagccttgggcctgcttcctgccggggctaggagggagggaagtttttggccaatagcatcagtttcaccagaagcacgttgtgcttcccagctttctaggtcctcatctgaccagagagagcttgattttaaaacccttcccacttccaatcgggagaaactcctaggatagcagtgaccttgaaagttttggggttgttttttggatgttggtgattttaaaacaacaacaaaaaaaacacctcaagtagtgatatttctttgtaaacaaaataaaatgtaaaatattgttttgaaacaattttttaacaaagttgatcaaataagaactttcaggctgtgattttaagcatcagttcagactgagggcagggtatccactcctgcatggagtgtgaggttgaagtttgttggaagcccctggtagttgataatattgaggttgttgaaggatgagaggaaaggtcgcttctttcttaggagctgtgatgctccactgtattgcataacgagatagcacttgattcagaccccagagcctgtagaataaatgatgtggagagagtattgaaaaaggctggatttatctgggggaatggcaatgttataaaaggttcttccctaattttttaagagataagcaatttataaagagatcaaataaaactaatctctttcaaaacagtattcatttagcactacccctggaaaaatcatcactagactgtgagtcgaaatttaacgaatggaggaaaatttattaagcctcattcacctttcggactttaacaaatggttcaaaagggaaaattcaccagagtaccctcagattattaatggcagatgagagcaggaaaaaagaatgttgagaatggctaaaaattgattccaattagtcttggcatggagaggcaacatctcacctggccagagccctgcagccagagtgctgtctcctctgccagtcagccagggatctggggcttacaggcgattcctccaggcctcaatcttctcacctgtgaaatgggaagataccattaaattgtcatttggcttctttcaaaatctcaggtctagaatggaaaggcattgaaggtgagtggaagagaagaaactggatgttaaaataataataatgtaacagttattaattcacatggccagaccccagggcagaagactaatggacgagaggatgattatgttcctttgaaataaaatgtcaacattcaaatattgtttttttctgtaaaaaataagtgaatgggtcttggaaggaagtgctcctaatgatgtagtttacatattaatgcttaataaaccattttatttactcaacaaatattcactgaggacttataatcaataataccaagccctattgaatacagtaatctaatatacacatagaattgaaaagacaaaatgaacaaaagaaacagacagtatatcatttctgtttcctccactgttttcattactaaagaaacaagctgcagtacacagccggctgagagctgcttccgggggagcaggagaagcagcactcatttcactgagacctgggtttgagttctctgtttttgaatgtgacccagagctcatcgcttaaatgcgactgataattcgtgcctggccaccctcatagcagcgctctgaaagaaacataaaggagtggatacacgtgtgagcaggagcctagacatgtgtcaggtacttacctaaacatggatgtttaggtcactgacatactgacaccatcaagctaattcttctctattggtctctatgtcagtaaggctacgtgccagtaatgtgtattaaatattaccctgtggtgagtatcaatttcaccctaaaatgttcatttattccctttggtggttaagttacttggactaccacagtgatgcctctatgtccccacactcaggaggtatgaaagcgtctctaggaaggagcagtggtctggtctcagtgtggcagcagacaaagccaggctcgcacttaattacattgaattatttctgtctggtatggcctcaaaaggtgcaaaatgatcataaatatctttcgacagtcacctttggtttttgcccttgccagcacctggcccttgtaggtgctgctggtttaaggaacttggagtattaaggggatccataaaaggactttgacagaagtcttcctgaactgtgcttagggccaggaaggcaggcaggggcttggtcatttcagctgtgctgtacccggatgagtggaaactgtgccttctgatgcatctctcctcctctgttcccctctaagaaccccttgtctgtgctcagatggatgagcaagtagtctcttctcccaccccaaaaacctccttagatggggtggattcagtaaaatcaaagcctcagttaggcaatataggaaaagatgaatttttgtgaatataattttctttagtaaaaggcttttggtcacctcttataatttctcaatgtctttatggaaaaaataagtttctcttgagcctttggtgcacaaacagagtcaccagcccttggaggtgcatgcatctaatgacagagcagcctgtgactcgcgagcatcaggctcacttgttccttgctgtgattgactctggggggtggaggcttttgggaggccctgcgccatggtgcagaggaagacccctgacctctgggagccctgggcaggctgtgggtgtggcttggcagagaaggatggacatgtcaggaagcatattagcttaatagatgaagtgtgtgaccagtgtaattgggttttatggatttatatttatcttgcatataaatcagggtgtggcctatatatgtttgcccatttaataaaaaacacatattccaaatgttaaaatataaaatataccagcaacaatagccaatttgaaatatatgttttcaaagtaacattcataatagcaatgaagacataaatacttagaaatgaagaaaaccagcaagccatagtgaggcaagaaagaaaacatgggagattggagaggtagagaggtctggatgccgtccatgggcctctgcccaaattagtgtatcatttcaacataaaactggcttgtaaattttactggaatctggtaaccatgtatcataaagtatctggatatatacatgagataattggcaactttttagaagaagaataatgtcaagtgatgtatgaaaatgtagctgaaatggatggaactctttgaagaatagacaaacaaatcaataatagagatggataccctactgaagaccccatgataaatcagcatgaaatatccgaggcaggaggaagcataaggcaggaacggtattggaagaattgatcaggcatttaagataatcagtttacattatcatctccttatacactaggataaattgccgggaaatgaaagagttatatttttataactccaaccacaataactgatgtaaatatagatccagctatgcaggatacaaagttgtatcttcaattatggaaagagatgacatagaacaattgagaatgactagaaatggcccacacatcagcatttacctccataatttctaaattttctacagcagtcaggggtgctttgattttcaggagtttgttgtatgctcagggataaggggctctgggtttttcctccacattgcccagatctgctgtaggctcttgggggccacatttttgtatctccgttcactgtgctggtccatgaagtcagatgttagatcacacagttctttgcgtctcagagggctgctgttagggactgactgaggtagcagatttgggagtattatgaaaagttaaaaggacttgtcaaagggacatcaatacttaatcccagtccagcctctggtgatggtggtggtgcctgtgcatttggacttaaagaggatgatgtgtggtgagcagctgttggaggaagaagcatttgcaggtggctggtcattggcattgctccggctgcctctgcctgtctggaagtgttgctgggaagattagaattaatctctaggaagggcctggctcttgtaggcacttaacaaatgtcagatttaacattggacgcgactgaaccctttaaacataagcctttctaaactggcctctctgtctttgactttagtcattaaagaagaaactaatcacagtgaaatggcagaagacctgtgcaagataggatcagagagatctctcgtgctggacagactagcaagtaacgtcgccaaacgtaagagctctatgcctcagaaatttcttggtaagagttaaatgtttgctgtctcttaaaaaaaaactatgtgggtgttttagatgcaagtagaaatgagttgagggtggaagaaagggaaaaaaatcttattttttcaaaaggaaaaattggtaagcttaacattccttaaatatcttagaattttttccaataagtatcttaaaaataacaaacctcccatcagtttttcctagatttgattttgcagcatctggggcctgccctgtgatctgcctgtggacatcgctcttaggggcggctgcaccagcgtgcacagggtggagagtttgggcctggctcgtccgggggacaccacactgcaggacactccaggcctggccggcttctcagagcttcagatcctcatttttcatatgaagctcctaatgctccccttatgggggactctgaagggttaatgggaggaatcatacagtgactgacccctgagaagtgtccagtgaagacagggcttagctaggattgctgttttgcctaatgctctgcgggattaaaaaaaaagaagaagaagaacaagaccattcgtctctctaggagcattgcccagagtaggtattagacacaccaacaccaccatccagccagacgctgcagggacagtgagccagggtccgagtggaaaggcgctaggcttgggaaccagctcagagtcaatacagagccaccgccactcaccaactctgtcagcttagtaaaatggctctgcccctagagccctggttccatcctttagtatctcacagggtgattgtgaatatcccatgactccaagattgagaaaacgtttagaatccctcggtgtgaaggttaactctgtccggaaagaggaccagtaaaagcttcatgaggctgagatgcactttggaagaggaatagagtttcagcacattctaggtgttggaggaatgggggaatctaggcagatgtttaaaatcaatgagaaaccagaatgctgaccatgagggttggagtgggggcctaaggacatgacggaggagcagggtgtgttcccagcttaactcaggtacccatggggaagcaggaaaagtgaaggtgtcctaggcagctctgccacaggatgaatggcttcagatgccaggtgagcgagggacccttcattcagtcagcaggaaagaagcactggcatattttttatgagaacaaaggctaggatagtaaagacagcaagtaccaaaaaatgactggaaaagggagactgtggaggcagtggcagcaggcatggaaagaagggcttgtgaaggggaaggggtggtgtcagaggaacatagggctgggggcagggattaggtgagggaaaccatgagtcacactgattctagagtagtgtgcccttgatgaaaaggataacaccaggttctaggaaaagatggggttctgtttttgacgtgttgattttcaaggacttctggtgtttgtgacacatggggaaattgtggtgggagagaggtggggccagaacaggggctggtgaggccaagggtcccagagggcacctgttgacctgcaggatgacatgaagggggaaggacagaggcaaggccaagtcctgggcaccagcctccctcttgcagcttcaaatagggctccattttgaccttttgattaattagaggtttgtcataggttgggggttgagaggagcaagggagagaaggattcagtgtacaaaaagaatgaaagccactggctgagccagtggggagttgtccacacacacatgagcctttggaccatgagaacgagggaggccttgccttcctgaacggagtaggagtgaggtcctgtgctgagcgtaagcagtgggattcccacagcactgggcacagagcccacgggctgcctcctgagcagccagcatctgcctggggtggacacagtgacagagagatgggtggtgactggggtatgggcagagataaggcagcaagtgtgtgcaaggggagtgaagggttactgaccttaagaagcagggatggcgtcctctgtcaggtgaggagcctggagaatgctttggtgaatgaacgtttgcagccccttttagcttttggagacttgaaaccaaaggagagattcatctgtgaaactctactggagccactccccaacccccacccttgtgagaccacaatgtgggcgttggcttgagatgcttctgtgttagtagaagaaataaacaacacagtgctctgatgaggcaaagcgaagatgaaaaaggagttcccaggggacatagtaggaacagtggacgagggtagcagaagaggagtttggagcaaaagactcacaagcagctgcataatctgttggtgcttggcagttcatttgtaaaaatgatgcctcttcctgccctaaaatacctaccttacccccgcttcaacttgatgagatttccatcagtcactcccaatgtgtcacagcttctgcagccctaaaattaaaaggtgagtgagtctctgaggcccctctccacttctcggatgctgagtttagccttcatgtgaatgtggaaagactaggaatacagctgttatcacacaagctggcccaatagtggttcagttgagagagccccatccttcagagtcagctccagctaggagtgactggtggccttgagcatggtgctgggcttagtgttgccatctgtggaatgggtgtgggtctgttgccctgcctcctcccagagctattctgaggctcagaaggggtgatggatgtgatggtgctcccaacactagaaagcatcttaagaatgtaagattttcatgatgactgttgctcagagtggctattatagttttgctttattgttctataacctatgattaaaatttttaccttaaactttgacgtgagtgtgaataagtatttgttttgccagcaacattcctcaccactggggccattaaagatctccccctctgagaccatcaaatacaggtcaacaggactgattaatctaattagaaaagggcttgtattaaatagcaatgataattgttgtttttagtctgtctggtgtttgacttgggaacgtttttaaaatagagaaaagcacaaagaggaaaacaacaattaccaatattcctgctacccattataattatctaggtatattttcttcttttgtaagaaaaagaaaccctgttatattgttaaaataacacaaagttaatataaagaattttaatgcaaagattaatgttttcaaatcaccacaaaacccaacatccagaaattaccaatattaaaagtagaaaagtatcattctaaatattttctgttgcatatgtatgtgagtggataggctgatgaattaggtggattgatggataggtaaatatgaaataaatactttcataaatattccaacttatcatacatgccttaaattcaagaggtgaaaaaagacccaaacaaaactagagaagcggcttattttaaatatcctctgacataaaggaatattatatttaaaggatcctctaagattaaaaatatgtactatgaaaaacattaagaaatttgaattttttttaatccatttgtttcaatttaagcagcatctactggctcactgctttgaaaaataaggacagtattccagttcacattcagtgttccagtgttcacattatcttattatttttacattgtccagctttgtaatattcacattctattctgtaatcataattcatagtagtttagttatttattactaactctatttaaatagattcaaggatcagaccctgcccttttcttcttatttatgtttattttgattaatctcttaattgattggactttacattcaagcaacttttttaaaaaaaagtttctatagatgttctatttctatcattgtattgtttttgaggatgttggcctgttgcctttgtatttgatgagcattttgacagagtctatggtcttgggccactctttctttttctcccttgagaactttttagattttgctgatggcattgcttgttgaatgttgctgtggaaacatcaagtctagtgtaactgtttcttcttcaaggtgatttgcattttattcctgaatgcctgagggttctttatttaaccttgaagttaaataccctaattaggatgtatcttggtctattcattcggaataaaaaattcctgccattttgtctagagagtcccttttttttctctttatttctgggaaattctcttttatataaatatgttttgttccatctattgtgatctctgttgagggataccagttgtccatatgttagataatttgtcttccatatctgttaacagttcttaaagttttttgtttatttctttgtctatttttacatttactcactgttctcttgtggttttcctctgtcagtaatttaatttttagtagttcctgttctattacttgctatttttaatccatgcattaattttataataatattattttgctccttattttgtctcctgagacccgaaatctcttttttcctcttactctgttgcttttgcattttattttgaatacttttaaaattgattccatgttatgaagcaattatgaggcatttcctctcttgttggaattaacgattttttcccctaggagggactctatggtctgtgttttacttcctttcttcccctgtatttctagaaaatattttcctagtaaccctgacatttcttttcatcttgcttattctagttggtctgatatagcttgattgacatttcagccttcttcccactatatttttttttcctgtgagagctattgggttttctaaatcctgaaagaatgccaaagatggggttggaggagtttggtgaggcaaagtgcagcctttgttaaaatacttttcctttgctctctctccctcatctgaaatttagttaaataccctaagccatcagcactgtacctagttggggaatgctttcatccccacaggagattctctggggctttgggccatcttccccttcagtgtagaccacagaggactttgcttctgtcccagggagcccgcaggggctcacttctccatgttcatctgattcttgtcagccaaggtttcaaatgcttttctgatcagaacagggaaaagatacctatctgaatcatgtctttatagatatgaggctatgagggaaaattctgaggttattcttgactcacacctaaagatttggaaatgagattagcagcaaagctttgccctacatctcatgtcagaattttctgtttctttctagtctttgagtgtatgtgtgttctcacacacgccataatgaaatgcatattatatataattatgtgtatatataatattctatgactatacatgacatgttcctttagctgattgctgttaagagaaatttataggtttttatttttcttgttttgttgggtattaaggaagagaaattctatggtaattttcatgtggcacagtaatctggcatatatgttgatttttttcctacacccatttgttgtgataccaagtttgaaaacaacagatttcagtggttgcttgggaaaccacagaaccatgacttggggagagacaggatgattaggtgggaaagcacccttttggtggggctgtaaagacttttatatttagcaaaattggctacaaagtccattcccctccttttcttgccttgatttggtagagggatagacttggatacaaactagaatggattcattcttctctggagttagtgtaacaagacatttagctgctcaacacaaaaacagaaacaaaaaaattgtgtggtttcagcagtgctatacaattactttttctgacctttaatggagagaaacaccacttctttggtccctaccatcagcttcatagggttttcatcctgttctgtttctgggagggcgtaactggccatgcacaagttttttttctctaatcagagtatgtgccacttctgaccaccagtagatgaaaacgaatggaaaccaggctattatatgatacatatccattacaaaataagacatgaaactcaaaggtactttatggtataatggggcatatattcctggacaattcttaatggtcacagattttataaaaggactattagtaaatgtatgaattacagagtaatttatccttctgttagtaagaaccagctgatgacctcagtgtcaggtgcatcgtggaaggtgttgggaccttcccttgccaccaccctcaccagccatcatcagccataacctgcacattggggaagttttgacttatccctcacttttgcccctcttcaagctgttctttccacagtgaatgagaaggccacttcttccttcaaacctttcagtggtttccattttcctttagacaaagtctctgcctagctggcctctgcctgcccctcctgcctacctctcgagcactgcccccacctagggctctggttccccaaccttcactcggtcctgccacacctcccagccccttctcccttcagaactttccttcttgttgtccccaacactgggacacaaaaccctccttatcaaccctccttatctggctgactcttacaagatcagaaacctgtgtaatgctctcatggcacgctccccttgtcttcgtggatttctcagatgggaaggaattatccatgcaatcacacataaacttctacctaccctcccctagtagctgtctgctgctaaggatggggaccattctcacttactcactgttctgtccctctgcccagtccagatgtgttgaaggatggaaatatacagagtagtggtaaaatataaaccgttcagacattccaaggatgggctcatgtgctttgactcattaatgtaccactgctgaaaacagaacacagccgcagtcttgccagtaagagtgcagttactgtaattaatgaatttgctaattaagccatgatttcatactgaacttatgaccaacatattgagaaggtgtgtcttcaagaaaatttattttttgtattaagatatttactccaaagctaattgaagaagccaaatctaggctctggtttcaccattgccagggaaatgagctcatggactcctatgaactgatgatgttagatcagaagtttctcaaggccagggcccaatcactgctgaggcgtcaacagtagttccttgtacatcaataattctcattacttttaaaaaataacagatgaatagcaactattttccctgtagctcccttgctgtgcctcctaccctccaccacatgtttctggggagccctgcttcgggcctgccaactacagagaattacttttgagtatcccttccactctcatctcaagacagagttcatctacctttgggttatttgtcaaaaatgtgtcattttattacaaaaaatatacaatcatcatgtattttgattaaattttacactagattattaaaattattaaatacaattattaaaattaataatttaacatatcacatattttaaatatattgtatataatgaataataatataattattgtctattttaattcaataaatgtatagtaagttagccagttgtaaattactgagaacactctactgaaaaagcatcatttcaaatacactatttaaaatattaaatgaaatacaataacataattaaactaatctttggttcccctatttatgtattcatttatccaacaaaatctccttaagtgcttataatgggtaggtcctggctcggtgtcccctagacagacgcatgggccttcccccagcccgtcagtatggtgcaggtgtgatgtgtccgcaggtgtgtgtgtatgtgtgcaggtgtggggtccgcaggcgtgctgggcccccaggccgtgttccccttcccctccccggttgtagatttcagctgttgctgccagacctgaccggttccggaggtggccgcgccccactcactgctacgagaaggagaacgaaatgatgaagtcccacgtgatggaccaagccatcaacaacgccatcaactacctgggggccgagtccctgcgcccgctggtgcagacgcccccgggcggttccgaggtggtcccggtcatcagcccgatgtaccagctgcacaagccgctcgcggagggcaccccgcgctccaaccactcggcccaggacagcgccgtggagaacctgctgctgctctccaaggccaagttggtgccctcggagcgcgaggcgtccccgagcaacagctgccaagactccacggacaccgagagcaacaacgaggagcagcgcagcggtctcatctacctgaccaaccacatcgccccgcacgcgcgcaacgggctgtcgctcaaggaggagcaccgcgcctacgacctgctgcgcgccgcctccgagaactcgcaggacgcgctccgcgtggtcagcaccagcggggagcagatgaaggtgtacaagtgcgaacactgccgggtgctcttcctggatcacgtcatgtacaccatccacatgggctgccacggcttccgtgatccttttgagtgcaacatgtgcggctaccacagccaggaccggtacgagttctcgtcgcacataacgcgaggggagcaccgcttccacatgagctaaagccctcccgcgcccccaccccagaccccgagccaccccaggaaaagcacaaggactgccgccttctcgctcccgccagcagcatagactggactggaccagacaatgttgtgtttggatttgtaactgttttttgttttttgtttgagttggttgattggggtttgatttgcttttgaaaagatttttatttttagaggcagggctgcattgggagcatccagaactgctaccttcctagatgtttccccagaccgctggctgagattccctcacctgtcgcttcctagaatccccttctccaaacgattagtctaaattttcagagagaaatagataaaacacgccacagcctgggaaggagcgtgctctaccctgtgctaagcacggggttcgcgcaccaggtgtctttttccagtccccagaagcagagagcacagcccctgctgtgtgggtctgcaggtgagcagacaggacaggtgtgccgccacccaagtgccaagacacagcagggccaacaacctgtgcccaggccagcttcgagctacatgcatctagggcggagaggctgcacttgtgagagaaaatactatttcaagtcatattctgcgtaggaaaatgaattggttggggaaagtcgtgtctgtcagactgccctgggtggagggagacgccgggctagagcctttgggatcgtcctggattcactggctttgcggaggctgctcagatggcctgagcctcccgaggcttgctgccccgtaggaggagactgtcttcccgtgggcatatctggggagccctgttccccgctttttcactcccatacctttaatggcccccaaaatctgtcactacaatttaaacaccagtcccgaaatttggatcttctttctttttgaatctctcaaacggcaacattcctcagaaaccaaagctttatttcaaatctcttccttccctggctggttccatctagtaccagaggcctcttttcctgaagaaatccaatcctagccctcattttaattatgtacatctgtttgtagccacaagcctgaatttctcagtgttggtaagtttctttacctaccctcactatatattattctcgttttaaaacccataaaggagtgatttagaacagtcattaattttcaactcaatgaaatatgtgaagcccagcatctctgttgctaacacacagagctcacctgtttgaaaccaagctttcaaacatgttgaagctctttactgtaaaggcaagccagcatgtgtgtccacacatacataggatggctggctctgcacctgtaggatattggaatgcacagggcaattgagggactgagccagaccttcggagagtaatgccaccagatcccctaggaaagaggaggcaaatggcactgcaggtgagaaccccgcccatccgtgctatgacatggaggcactgaagcccgaggaaggtgtgtggagattctaatcccaacaagcaagggtctccttcaagattaatgctatcaatcattaaggtcattactctcaaccacctaggcaatgaagaatataccatttcaaatatttacagtacttgtcttcaccaacactgtcccaaggtgaaatgaagcaacagagaggaaattgtacataagtacctcagcatttaatccaaacaggggttcttagtctcagcactatgacattttgggctgactacttatttgttaggcgggagctctcctgtgcattgtaggataattagcagtatccctggtggctacccaatagacgccagtagcaccccgaattgacaacccaaactctccagacatcaccaactgtcccctgcgaggagaaatcactcctgggggagaaccactgacccaaatgaattctaaaccaatcaaatgtctgggaagccctccaagaaaaaaaatagaaaagcacttgaagaatattcccaatattcccggtcagcagtatcaaggctgacttgtgttcatgtggagtcattataaattctataaatcaattattccccttcggtcttaaaaatatatttcctcataaacatttgagttttgttgaaaagatggagtttacaaagataccattcttgagtcatggatttctctgctcacagaagggtgtggcatttggaaacgggaataaacaaaattgctgcaccaatgcactgagtgaaggaagagagacagaggatcaagggctttagacagcactccttcaatatgcaatcacagagaaagatgcgccttatccaagttaatatctctaaggtgagagccttcttagagtcagtttgttgcaaatttcacctactctgttcttttccatccatccccctgagtcagttggttgaagggagttattttttcaagtggaattcaaacaaagctcaaaccagaactgtaaatagtgattgcaggaattcttttctaaactgctttgccctttcctctcactgccttttatagccaatataaatgtctctttgcacaccttttgttgtggttttatattgtaacaccatttttctttgaaactattgtatttaaagtaaggtttcatattatgtcagcaagtaattaacttatgtttaaaaggtggccatatcatgtaccaaaagttgctgaagtttctcttctagctggtaaagtaggagtttgcatgacttcacactttttttgcgtagtttcttctgttgtatgatggcgtgagtgtgtgtcttgggtaccgctgtgtactactgtgtgcctagattccatgcactctcgttgtgtttgaagtaaatattggagaccggagggtaacaggttggcctgttgattacagctagtaatcgctgtgtcttgttccgccccctccctgacaccccagcttcccaggatgtggaaagcctggatctcagctccttgccccatatcccttctgtaatttgtacctaaagagtgtgattatcctaattcaagagtcactaaaactcatcacattatcattgcatatcagcaaagggtaaagtcctagcaccaattgcttcacataccagcatgttccatttccaatttagaattagccacataataaaatcttagaatcttccttgagaaagagctgcctgagatgtagttttgttatatggttccccaccgaccatttttgtgcttttttcttgttttgttttgttttgactgcactgtgagttttgtagtgtcctcttcttgccaaaacaaacgcgagatgaactggacttatgtagacaaatcgtgatgccagtgtatccttcctttcttcagttccagcaataatgaatggtcaacttttttaaaatctagatctctctcattcatttcaatgtatttttactttaagatgaaccaaaattattagacttatttaagatgtacaggcatcagaaaaaagaagcacataatgcttttggtgcgatggcactcactgtgaacatgtgtaaccacatattaatatgcaatattgtttccaatactttctaatacagttttttataatgttgtgtgtggtgattgttcaggtcgaatctgttgtatccagtacagctttaggtcttcagctgcccttctggcgagtacatgcacaggattgtaaatgagaaatgcagtcatatttccagtctgcctctatgatgatgttaaattattgctgtttagctgtgaacaagggatgtaccactggaggaatagagtatccttttgtacacattttgaaatgcttcttctgtagtgatagaacaaataaatgcaacgaatactctgtctgccctatcccgtgaagtccacactggcgtaagagaaggcccagcagagcaggaatctgcctagactttctcccaatgagatcccaatatgagagggagaagagatgggcctcaggacagctgcaataccacttgggaacacatgtggtgtcttgatgtggccagcgcagcagttcagcacaacgtacctcccatctacaacagtgctggacgtgggaattctaagtcccagtcttgagggtgggtggagatggagggcaacaagagatacatttccagttctccactgcagcatgcttcagtcattctgtgagtggccgggcccagggccctcacaatttcactaccttgtcttttacatagtcataagaattatcctcaacatagccttttgacgctgtaaatcttgagtattcatttacccttttctgatctcctggaaacagctgcctgcctgcattgcacttctcttcccgaggagtggggtaaatttaaaagtcaagttatagtttggatgttagtatagaattttgaaattgggaattaaaaatcaggactggggactgggagaccaaaaatttctgatcccatttctgatggatgtgtcacaccttttctgtcaaaataaaatgtcttggaggttatgactccttggtgaa